European Patent Specification EP 3 494 222 B1, published December 3, 2025. Title: CONTROL OF COLEOPTERAN PESTS USING RNA MOLECULES. Applicant: Syngenta Participations, AG Donohue, Kevin V. Naudet, Yann Feldmann, Pascale Degrave, Lies Maillet, Isabelle. The sequence listing filed with the application follows.

SEQUENCE LISTING (403 sequences)

SEQ ID NO: 1 - DNA, 478 bp, Diabrotica virgifera
ggtttcatgacccctgagagaaagaagaaacttaggttactgttgagaaagaaagccgccgaagaattaaagaaagaacaagaacgcaaagcagccgaaaggaggcgtatcattgaagaaaggtgcggtaaacccaaacttgtcgatgacgcaaatgaaggcccattaaaacaagtatgtgagggatatcacagacgtattgtagacctagaaaataagaaatttgacctcgaaaaagaagtggaattcagagattttcagatctccgaattgaacagccaagtaaacgaccttagaggcaaattcgtcaaaccaaccttgaagaaggtatccaaatacgaaaacaaattcgccaaacttcaaaagaaggcagctgaatttaacttccgtaaccaactcaaagttgtcaagaagaaagaattcaccttagaagaagaagacaaagaaaagaaaccagactggtcaaagaagggagacg

SEQ ID NO: 2 - DNA, 529 bp, Diabrotica virgifera
agaagttgccgctttagtcgtagacaatggatccggtatgtgcaaagctggttttgctggggatgatgcacctcgtgctgtattcccttcaattgttggacgcccaagacatcagggtgtgatggtaggaatgggacaaaaagattcctatgtaggtgatgaagctcaaagtaaaagaggtatccttaccttaaaataccccatcgagcacggaatagtcacaaactgggatgatatggagaaaatttggcatcatacattctacaatgaactcagagtagccccagaagaacaccctgttctgttgacagaagctcctctcaaccccaaggccaacagggaaaagatgacacaaataatgtttgaaactttcaacaccccagccatgtatgttgccatccaggctgtactctccttgtatgcatctggtcgtacaactggtattgtgttggattctggtgatggtgtatcccacactgtcccaatctatgaaggttatgctcttcctcatgcaatccttcgtttggac

SEQ ID NO: 3 - DNA, 592 bp, Diabrotica virgifera
accggcctttgtatgtcttgggatatgtgcctaaagacgatagattatacctcgtagataaagagttgcgcgtagtaagctaccaattacttctttctgttcttgaatatcaaactgccgtcatgagaagagactttccaacagcagacagagtacttccgtccattcctaaggagcacagaacgagagtggcacatttcttagaaaagcaaggcttcaaacagcaagctttggccgtaagtacagatccagagcacagattcgagctggcagtagcattagaggatcttaatatagccaaaactctagctcaagaagcgaacagtccgcaaaagtggaatcaactagcagaattggcagctgctactaataatgtaagcgtagccaaggaatgtatgcaaaaagcgcaagattatggaggcttgttgcttcttgctacgagctccggtgatgaaaatttagtccgtactctaggagaaacgacacaagctgaaagcaaacataacttagcatttttgtcacacttgttagtaggtgatttaaacaaatgtctagacattcttattaataccggtagattgccagaagctgc

SEQ ID NO: 4 - DNA, 594 bp, Diabrotica virgifera
gaaagcagttggaagatggccgtactctctcagactacaacattcaaaaagagtctaccctccatttggtacttcgtcttagaggaggtatgcagatttttgttaaaactttaactggaaagaccatcacccttgaagtagaaccttctgataccatcgaaaatgtcaaagccaaaattcaagacaaagaaggtattccaccagatcaacaaagattaatctttgccggaaagcaattggaagatggtcgtacactctcagactacaacattcaaaaggaatctaccctccatttggtacttcgtcttagaggaggtatgcaaatctttgtaaaaacactcactggtaagaccatcaccctcgaggttgaaccatcagataccatcgagaatgtcaaagctaaaattcaagacaaagaaggtattccaccagatcaacagagattaatcttcgctggaaagcagttggaagatggccgtactctctcagactacaatattcagaaagagtctaccctccatttggtacttcgtcttagaggaggtatgcaaatctttgtaaaaactctcactggtaagaccatcaccctcgagg

SEQ ID NO: 5 - DNA, 547 bp, Diabrotica virgifera
taccccattgaacacggaattatcactaactgggacgatatggaaaagatctggcatcacaccttctacaatgaacttagagtagcccccgaagaacatcccattcttttgactgaagctccacttaacccaaaagccaacagagaaaagatgactcaaatcatgtttgaaactttcaatacccctgccatgtatgttgccattcaagctgtattgtctctgtacgcttccggtcgtaccactggtattgtacttgattctggagatggtgtatcccacacagtacccatctatgaaggttacgctctcccacacgccatcttgcgtttggacttggccggtagagacttgactgactaccttatgaagatcttaaccgaaagaggttactctttcaccaccacagctgaaagagaaatagttcgtgacatcaaggaaaaattgtgctatgtagctttggacttcgaacaggaaatggccacagcagccagctccacctccttagaaaagagttatgaacttcctgacggtcaagtcatcaccattg

SEQ ID NO: 6 - DNA, 592 bp, Diabrotica virgifera
aggaaaggaaggacccaagaccaaacaaccatcgagatacatccgttttatctacaatcgcgtcatattggaatgtccttctgtaagagctgctgcagtctccgccatggcacaattcggagcctcttgtcccgatttgttagaaaatatccaaatattactttcgaggtgtcagatggattcagacgatgaagttagggacagagctacatattatagtaatatacttaacaaaaatgataaaagtttatacaacaattacattttggattctttgcaggtttcaattccttcactagaaagatcgcttagagaatacattcaaaatccaactgacgaaccatttgacattaagtccgtacctgtagcagcagtgccaacagcagaagaacgagaagttaaaaacaaatctgaaggactgctagtctctcaaggtccagtccgacctcctccggtgtctagagaagaaaacttcgccgaaaaacttagtaacgttccgggtatacaacagttaggacctttgttcaaaacttccgacgtcgttgaactcactgaatctgaaacagagtattttgtccgctgtatcaagcac

SEQ ID NO: 7 - DNA, 500 bp, Diabrotica virgifera
tactaggcgaaagtgccgtcggtaagtcgagtttggtactgaggttcgtcaaaggacagttccacgaataccaggagagtaccataggagcagctttccttacacaaaccatatgcctcgacgatacaactgttaaatttgaaatttgggacacagcgggtcaagaaaggtaccacagtttagctcctatgtactataggggcgcacaggcagctatagtcgtctacgacataaccaatcaagacacattcggcagggcgaaaacgtgggtgaaggaacttcaaaggcaggccagtccgacgatcgtgatagctttggccggcaacaagcaagatttggccaacaaacgtatggtagaatacgaagaggcgcagacgtatgctgacgaaaacggcttactttttatggaaacttccgcaaagacggcaatgaacgtcaacgatatatttttagcaatagctaagaaactgcccaagaatgaacaaaccacaggtcaaggc

SEQ ID NO: 8 - DNA, 189 bp, Diabrotica virgifera
cgatgaggttgaaggaaggagaaaaattttgatggggcgaaaaagcattaccaggacatatcttcgtggaaatgctgttcctgcgtatgtgataataatccttgtaggaattggtcaaatcatcctgggagggatattgtacgttgcattgaggaagaagatcattgctgcacctgtaacggcatcata

SEQ ID NO: 9 - DNA, 393 bp, Diabrotica virgifera
tgaggtcgagccctcagatactatcgaaaatgtgaaagctaaaatccaggataaagaaggaattcccccagaccagcaacgtctcatcttcgctggaaaacaactcgaagatggtcgtaccttgtctgactataatattcaaaaagaatcaacccttcacttggtgttgagattgagaggaggtgctaagaaacgtaagaagaagaattactccacccccaagaaaatcaagcacaagaagaagaaggttaagttagctgtattgaaattttataaggttgacgaaaatggtaaaatccaccgattgagacgtgaatgccccgctgaacaatgtggagctggtgtcttcatggcagccatggaagacaggcattactgtggcaagtgcggtta

SEQ ID NO: 10 - DNA, 524 bp, Diabrotica virgifera
tctttgcctttggctacgattcgaggagggcattcaagaatggctccagaaattggattcagaacaattttacatcggagtatatgtacttatagtcgcttcactgatcgtcatgattgtgtcctttataggatgtattagtgccctgcaggagagtaccatggcccttttagtgtacatcggcacccaagtgctcagttttatattcggtttatccggttcggcggttcttctggataacagcgccagagattcccacttccaaccgaggatccgagagagtatgcgacgtcttatcatgaatgctcatcacgaccaatccagacaaacactagccatgattcaggaaaatgttggttgctgcggagctgatggcgcaacagactacctctctcttcagcagccccttccaagtcagtgcagagacaccgttactggaaacccattcttccacggatgtgtagatgaactcacctggttcttcgaagaaaaatgtggttggatagcaggtttagctatggcga

SEQ ID NO: 11 - DNA, 267 bp, Diabrotica virgifera
tcgtgctggtttacaatttcctgtaggtcgtattcatcgtttattgagaaaaggaaattatgccgaaagagttggtgctggagctcctgtatacttggcagctgttatggaatatttagctgctgaagttttggaattggcaggaaatgcagctagagataacaaaaagacccgtataattcctagacatttacaattggccataagaaatgacgaggaattgaacaaattactgtcaggagttaccatcgcccaaggtggagtatt

SEQ ID NO: 12 - DNA, 558 bp, Diabrotica virgifera
gtgcatgaagttggatggtgtagatctgcccccaccaattagcttcgacattgcggaagagcaaccgttaccaccttgccaacagacgttcttatgtaatggtgatggaggatccatagtgcgacagtttctcgagctgtatttcgtaatatatgattcagataataggcagtcccttcttcaggcatatcacgaaaaagccacattttcaatgacaatggcctacccgtacggctattccaaagacagtaaaggagtatcgtggttgaattggtatgccaccgataatagaaatttattacgagttcaagatccagacagaagaaacaagttgttaagacagggacaagttgctgtagtttcgttcttgcaagatatgccgcacacgaagcacgatattcacagttttacagtagatttgacagtttttacaccccagatgttatgtttgacagtggctggtatgtttaaagaattgaaaagtggccacaaagtacctcctttaagatatttcttcagaacccttgtaattgtacctgctggatcaggtttttgcat

SEQ ID NO: 13 - DNA, 582 bp, Diabrotica virgifera
gattcggagccctacaatgaaatgcaactaaaaatggatttagaaaagggtgaggttaaagtaaaaataagagcattagaaaaaataattcacatgattctggcaggagaaaggttgccgaatggatttctaatgaccatcataagaaacgttttacctttacaagatcatttggcaaaaaaactattattgattttctgggaaatagttccaaaaacaaatccagaaggtaaactactacaagagatgattttggtatgtgatgcctatagaaaagatctgcaacacccaaatgaatttttgagaggttctacacttcgcttcttgtgcaaactgaaggaaccagaattgttggaaccattaatgcccagtattagagcttgtttggatcataggcacagctatgtgaggaggaatgctgtactggcaatttttaccatttacaaaaattttgaagccctcattccagatgctcctgaactgatctccaattatttggatggtgagcaagacatgtcttgtaaaagaaatgcgtttttaatgcttcttcatgctgaccaagaaagggcgttgtcgtatttg

SEQ ID NO: 14 - DNA, 458 bp, Diabrotica virgifera
ttggcaaaaaggaaatgaggatattgatggtaggactcgatgcagctggtaaaaccacaattttatataaacttaaattaggagaaattgtaacaactattccaacaattggatttaatgtggagactgtagaatataagaacattagttttacagtatgggatgtaggtggtcaagataaaattaggccattgtggagacactatttccaaaacacacaaggcctaattttcgtagtagacagtaacgacagggaacgtatcactgaggctaaagatgaattaatgcgtatgttggccgaagatgaacttagagatgccgtacttctcattttcgccaacaaacaagatttgcccaatgcaatgaacgctgcagaaatcaccgacaaactcggtctccattcactacgcaaccgcaactggtacattcaagctacctgtgcaactagcggagatggt

SEQ ID NO: 15 - DNA, 592 bp, Diabrotica virgifera
ggtcgcgaaagaacagaaagattttttgaccgtatctgccgatggatgcgtacaagtaacaaaacctctcgaccgagatccgcctttcggtagcccaacacgacaagtcttcatctatgctcgtgataatgatggaggcacaaattcattgttggccactgcagaaattgaaattattttaatagatataaacgataatgctccctttttaaatgttacagaaattgtttattatgaaaaccaggatccaggttttataggtaacctaagtgccgatgattacgatggtcctgataatggacctccgtttgcttttcgattatcagacactgcttcagatagtattagatcgaaattttccattatcggaaaccagcttttcgctttagaaatgtttgatagagaagagcaaaaatattatgacattgccattgacattacagatagtggagtacctccactaacaggaactagtattcttagagttataatcggagatgtaaatgataatccagctacagacggaaacagcacgatctttgtgtataagtacgtcaatgggccagaaaatttcatggaaatcggacgtgta

SEQ ID NO: 16 - DNA, 214 bp, Diabrotica virgifera
gcatggggtatcatccagttgggtttcatgggtgtattctattacattggggctgtggctttagcagaagatattccagaggttgagtttaagggcgatttagacaaattttatagcgacgtcaacacgggtttcacacagaatgcttacaactgctggattgctgctctcctatacctgataacattagcagtatcagctcaccaattctggg

SEQ ID NO: 17 - DNA, 459 bp, Diabrotica virgifera
tagatgccgcaggtaaaaccacaatcttatacaaattgaagcttggtgaaatcgtaactacaataccaaccatcggcttcaatgtagaaaccgttgagtacaagaatatatctttcacggtatgggatgtaggtggccagacgagaatcagaaaactctggagacactatttcgccaacactgatggactcatttttgtggttgattccaacgaccgagaccgtatcgcggaagccgaagaagaattgcacaatatgttaggagaggacgatttaagagactgcattttgttaatattcgccaacaaacaagatttaccgaactcgatgtccactgctgaattgaccgataagcttaagttgcacactttgaagaataggaggtggtacatacaagccacatgtgctactcaagggaatggtttgtacgaaggactagattggttgtcgaatgaattgg

SEQ ID NO: 18 - DNA, 536 bp, Diabrotica virgifera
gctaccctagcgtccactgtaacactgatttttgccctctactactgcctcacgggaaaaggagagcaagttagtttagcatggttattgttgaatgtgtctccccacatgtgggcaggtctaggaattggccttgctgtatcattatcagttgtaggagctgctgcaggaattcacactacaggagtcagtatcgtaggagctggtgttaaagcccccagaatcaaaaccaaaaatttaatttctattattttctgtgaagctgtggctatctatgggttaattatggctatagtactctgtggaagttggaagaatttcgatgtagacctattcaacctcaaaactcataactttgctcaaaaccattatggatcacatgttatttttggatccggtttaactgttggatttgtaaatctattatgtggattttgtgttggagtagttggttctggtgcagccatttctgatgcagccaattcatcattattcgtcaaaattttgattattgagatttttggaagtgccattgg

SEQ ID NO: 19 - DNA, 547 bp, Diabrotica virgifera
accttatgggaaagcgtgtggacttttctgcacgtactgtcatcacaccagatcccaatttacgtatcgaccaagtaggagtgcctagaagtattgctcaaaacatgacgtttccagaaatcgtcacacctttcaattttgacaaaatgttggaattggtacagagaggtaattctcagtatccaggagctaagtatatcatcagagacaatggagagaggattgatttacgtttccacccaaaaccgtcagatttacatttgcagtgtggttataaggtagaaagacacatcagagacggcgatctagtaatcttcaaccgtcaaccaaccctccacaagatgagtatgatgggccacagagtcaaagtcttaccctggtcgacgttccgtatgaatctctcgtgcacctctccctacaacgccgattttgacggcgacgaaatgaacctccatgtgccccaaagtatggaaactcgagctgaagtcgaaaacctccacatcactcccaggcaaatcattactccgcaagctaaccaacccgtcat

SEQ ID NO: 20 - DNA, 564 bp, Diabrotica virgifera
cggatctctatttgggggatcaagtcgtattgaagatgcagtggaatgttacacaagagctgcaaacctttttaaaatggccaagagctgggatgctgccggtaaagccttttgtgaggctgctaatttgcattccagaactggtgctcgtcatgacgctgccactaattatatagatgctgcaaattgttacaaaaaagccgatgtatttgaggctgtaaactgctttataaaagctatagacatttataccgaaatgggtcgctttacaatggctgcaaaacaccatcagactattgcagaaatgtatgagactgatgctgtggacatcgaaagggctgttcaacactatgaacaggcggctgattacttcagaggagaagaaagcaatgcttccgccaataagtgtcttcttaaagtggctcaatatgcagcccaacttgaaaactatgaaaaagcagtgggaatttatcaagaagtggcttatgcagctctggaaagctctcttttaaaatacagtgcaaaggaatacttattcagagctgccctttgtcacctttgtgt

SEQ ID NO: 21 - DNA, 564 bp, Diabrotica virgifera
tgctgattggagattcaggagtaggaaaatcttgtcttctactgagatttgcagatgatacctacacagaaagctatattagtaccattggcgtagattttaaaatcaggacaatcgatttagatggaaagacaattaaattgcaaatttgggatacagcaggtcaggaaaggtttagaacgattacatcaagttattaccgaggagcacatggtattattgtagtgtacgattgcacagaccaagattcattcaataacgttaaacagtggctcgaagaaatcgaccgttatgcgtgtgacaatgtaaacaaattactggtagggaataaaagcgatttgacaactaagaaagttgtcgacttcactacagccaaggagtatgccgaccaattgggtataccatttttggaaacctcagctaagaatgcaaccaatgtagaacaggcctttatgactatggccgctgaaataaaaaatagagtaggacctccatcttctgcggtagaccaaggaaataaggttaggttcgatcaaagtcgcccagtcgaaacaaccaaatccg

SEQ ID NO: 22 - DNA, 502 bp, Diabrotica virgifera
gagctatagtggactgcgggttcgaacatccttcagaagttcaacatgaatgtattcctcaagctgtcattggcatggatattctgtgccaagctaaatccggtatgggaaaaacggctgtttttgtattagctacactccaagtaatagatcctacagaaaatgttgtatatgttctcgtcatgtgccataccagagagttagccttccagataagcaaagagtacgaacgtttcagtaaatatatgcccaatattaaagtaggggtcttctttggtggcttgcctatccagaaagatgaggaaacgttaaaaaataattgcccgcatatcgttgtgggtactccaggaagaattttagcattggtcagatcgaaaaaacttaatctcaaacatctaaagcattttattttggatgaatgtgataaaatgttggagttattagacatgagacgtgatgttcaagaaatatatcgtaacactccccacgaaaaacaagtcat

SEQ ID NO: 23 - DNA, 505 bp, Diabrotica virgifera
tggtagatttggctaacctcgtatattggtgtttaggtcttaatattccgtacgttagtttctatgattataaaggtaatttaaaaaagcatgaagagaagttgcaacaaattgtagaatccagaaaatcagagaatatcaacataatttggcacacccatgcagaacaaaggcataaaaatggatttttgggtccaaaaatccacgtaaaagtgttaacacacgcggacggaaagcaaagtatagtaaatgttactaaaaaattagctctaaataaagaaaaagacattagtaaagaaaaaattagtgaattactattaaggcagtatgaatttccagatccagaaatggctattatttgtggaaagaaactgaacatttataattatcctccttggcagttaagactcacagaattctttaaagtcaacaaagtcaacaacatcacattcccagtgtttgtggaaaaattggaaaagtacagcaaatgtgaacagagggtggg

SEQ ID NO: 24 - DNA, 410 bp, Diabrotica virgifera
aaccagggatctatttgcccgcaagtttaaaaaacgtggtgtaattccactttccacatatttgagagtctacaaagttggagatattgtagatatcaagggtaatggtgcagttcaaaagggtatgccccacaaagtgtaccatggtaagacaggacgtgttttcaatgttactgcacatgcattaggtgtaattgtaaacaaaagggttcgaggaagaatcatccccaaaagaatcaatctccgtattgaacatgtaaaccactccaagtgtcgtcaagacttcttgcaaagagtaaaatccaacgaaaagctacgtaaagaagctaaagaaaagaacattaaagtagaacttaggagacaacctgcccaacctaggccagcacatattgttagcggaaaggttccag

SEQ ID NO: 25 - DNA, 467 bp, Diabrotica virgifera
tgatggtaatagagtgctggctaaatactacgataaagatatatttcctacagcaaaagagcagaaagcttttgagaaaaatttgttcaataaaactcatagggcagacgcagaaattatcatgttggatggtttaacttgtgtgtatagaagtaatgtagatttattcttttatgttatgggcagttcacatgaaaatgagctaattttaatgagtgttttaaattgcttgtatgactcagtaagtcaaatattgaagaaaaatatgcaaaaacgagctgtcttggaatcactagatattgttatgctggctatggatgaaattgttgatggaggaataattatagattctgattcaagttcagtagtatctagaatagcattaaggactgatgatattccattaggagaacaaactgtagctcaggtattccaaacggccaaagaacagctgaaatggtcattgc

SEQ ID NO: 26 - DNA, 368 bp, Diabrotica virgifera
caccgaagaacaaattgctgaattcaaagaagctttctcactattcgataaagatggtgatggtacaattacgactaaagaattaggaacagtaatgagatctctaggacaaaatccaacagaggctgaattacaggatatgatcaatgaagtagatgccgatggtaacggcacgatcgatttcccagaatttttaacgatgatggcacgtaaaatgaaagataccgatagtgaggaagaaattcgtgaagcattccgagtgttcgacaaagacggcaatggtttcatctcagcagcagaattgcgccacgtcatgaccaacttgggtgaaaaattgacagacgaagaagtcgatgaaatgattcggg

SEQ ID NO: 27 - DNA, 430 bp, Diabrotica virgifera
ttcgcacaagatgactttggtggtgaaaatgttgatctatatgacgatgtaatatccgctcctcctggaaataatgacaacccaggtgattcaaatcatcatgctcctcctggtgctggtgaagatggtggaggtaattttgttgggtcaggaggagcacccaataatataaattcttctggaagaagacatcagctgtatgttggaaatctgacttggtggacaactgatcaagatatagaaaatgcagtgcatgatataggggtaaccgacttccatgaagttaagttttttgaacacagagcaaatggtcaatccaagggattctgtgtcatatctttgggatctgagggaagcatgagactctgcctggaactcctatctaaaaaagagatcaatggccaaaatccccttgttacccttcccacaa

SEQ ID NO: 28 - DNA, 505 bp, Diabrotica virgifera
taggaatggcattttcaggcttaatagctgatgcaaggcaaatcgttgagattgctagaaaagaagcatcaaattatagacatcaatatggttcaaatattcctcttaaatacctaaatgatagagtaagcatgtacatgcatgcatacactttatacagtgctgttagaccatttggttgcagtgtcatcttggccagttatgaagatagtgacccatctatgtatctgattgatccatctggagttagctatggatactttggatgtgctacaggtaaagcaaaacagtctgcaaagactgaaatagaaaaattgaagatggggaatctaacatgcaaagaacttgttaaagaagcagccaaaatcatttatttggtccatgatgagctgaaggataagaattttgaactggaactttcatgggtatgcaaagatacgaatggtttacataccaaagtgcctgaatcagtgtttgctgatgcagaaaaagctgccaaacaagc

SEQ ID NO: 29 - DNA, 548 bp, Diabrotica virgifera
tccatctagaggagcccaaatgatgatgaaatccaggctaaagggagcccaaaagggacatagtttattaaagaagaaagctgatgctttacaaatgagatttagaatgattttgaacaaaattattgagaccaaaactctcatgggtgaagtaatgaaagaagctgccttttctttagctgaagcaaagtttgcaactggtgacttcaatcaagttgttcttcaaaatgtcaccaaggctcaaataaaaataagaactaagaaagacaacgttgctggtgttactttaccagtgtttgaatgctaccaagatggtacagatacatatgagttggctggtttggctaggggaggtcaacaattgacaaaactcaagaagaattatcaaagtgctgttaaactgttggttgaattagcctctttgcaaacttcttttgtaactcttgatgatgtaatcaaaataacaaacagaagagtcaatgccattgaacatgttatcattccaagaatagagcgtactttggcttacatcatatccgaactggacg

SEQ ID NO: 30 - DNA, 521 bp, Diabrotica virgifera
gatctggaagcgctagttgcaaaagtagacgaaatgagaacccaaagagccatgctatgggctcaacttcgagaatctattcaccaagacgatattacaagttcccttgtaacgaaacaaccaaatcagtcgctggaacagctgttccagcaagaacttcaaaagcatcaaaatctgatttcgttgattgaacaaaacacctcggcacaagaaaacattaagagcgccttagtcgattcttacgcttacgctgtaaattcaagaaaatacatccaagatatactccaaaagagaaccacaaccataacgtcactgatagcatcgttcgactcttacgaagacttattggcaaaagctaacaaagggatagagttttactcaaaacttgaaacgaacgtatccaagttactgcaaagaataaggagtacctgcaaagttcaacaagaagagcgagatcagatgatgtcgactgcgcaagtgcctcaatgggagagtcatacgtcacttgccgctcctaaact

SEQ ID NO: 31 - DNA, 20 bp, Diabrotica virgifera
ggtttcatgacccctgagag

SEQ ID NO: 32 - DNA, 20 bp, Diabrotica virgifera
cgtctcccttctttgaccag

SEQ ID NO: 33 - DNA, 20 bp, Diabrotica virgifera
agaagttgccgctttagtcg

SEQ ID NO: 34 - DNA, 20 bp, Diabrotica virgifera
gtccaaacgaaggattgcat

SEQ ID NO: 35 - DNA, 20 bp, Diabrotica virgifera
accggcctttgtatgtcttg

SEQ ID NO: 36 - DNA, 20 bp, Diabrotica virgifera
gcagcttctggcaatctacc

SEQ ID NO: 37 - DNA, 20 bp, Diabrotica virgifera
gaaagcagttggaagatggc

SEQ ID NO: 38 - DNA, 20 bp, Diabrotica virgifera
cctcgagggtgatggtctta

SEQ ID NO: 39 - DNA, 20 bp, Diabrotica virgifera
taccccattgaacacggaat

SEQ ID NO: 40 - DNA, 20 bp, Diabrotica virgifera
caatggtgatgacttgaccg

SEQ ID NO: 41 - DNA, 20 bp, Diabrotica virgifera
aggaaaggaaggacccaaga

SEQ ID NO: 42 - DNA, 20 bp, Diabrotica virgifera
gtgcttgatacagcggacaa

SEQ ID NO: 43 - DNA, 20 bp, Diabrotica virgifera
tactaggcgaaagtgccgtc

SEQ ID NO: 44 - DNA, 20 bp, Diabrotica virgifera
gccttgacctgtggtttgtt

SEQ ID NO: 45 - DNA, 20 bp, Diabrotica virgifera
cgatgaggttgaaggaagga

SEQ ID NO: 46 - DNA, 20 bp, Diabrotica virgifera
tatgatgccgttacaggtgc

SEQ ID NO: 47 - DNA, 20 bp, Diabrotica virgifera
tgaggtcgagccctcagata

SEQ ID NO: 48 - DNA, 20 bp, Diabrotica virgifera
taaccgcacttgccacagta

SEQ ID NO: 49 - DNA, 20 bp, Diabrotica virgifera
tctttgcctttggctacgat

SEQ ID NO: 50 - DNA, 20 bp, Diabrotica virgifera
tcgccatagctaaacctgct

SEQ ID NO: 51 - DNA, 21 bp, Diabrotica virgifera
tcgtgctggtttacaatttcc

SEQ ID NO: 52 - DNA, 20 bp, Diabrotica virgifera
aatactccaccttgggcgat

SEQ ID NO: 53 - DNA, 20 bp, Diabrotica virgifera
gtgcatgaagttggatggtg

SEQ ID NO: 54 - DNA, 20 bp, Diabrotica virgifera
atgcaaaaacctgatccagc

SEQ ID NO: 55 - DNA, 20 bp, Diabrotica virgifera
gattcggagccctacaatga

SEQ ID NO: 56 - DNA, 20 bp, Diabrotica virgifera
caaatacgacaacgcccttt

SEQ ID NO: 57 - DNA, 20 bp, Diabrotica virgifera
ttggcaaaaaggaaatgagg

SEQ ID NO: 58 - DNA, 20 bp, Diabrotica virgifera
accatctccgctagttgcac

SEQ ID NO: 59 - DNA, 20 bp, Diabrotica virgifera
ggtcgcgaaagaacagaaag

SEQ ID NO: 60 - DNA, 20 bp, Diabrotica virgifera
tacacgtccgatttccatga

SEQ ID NO: 61 - DNA, 20 bp, Diabrotica virgifera
gcatggggtatcatccagtt

SEQ ID NO: 62 - DNA, 20 bp, Diabrotica virgifera
cccagaattggtgagctgat

SEQ ID NO: 63 - DNA, 20 bp, Diabrotica virgifera
tagatgccgcaggtaaaacc

SEQ ID NO: 64 - DNA, 20 bp, Diabrotica virgifera
ccaattcattcgacaaccaa

SEQ ID NO: 65 - DNA, 20 bp, Diabrotica virgifera
gctaccctagcgtccactgt

SEQ ID NO: 66 - DNA, 20 bp, Diabrotica virgifera
ccaatggcacttccaaaaat

SEQ ID NO: 67 - DNA, 20 bp, Diabrotica virgifera
accttatgggaaagcgtgtg

SEQ ID NO: 68 - DNA, 20 bp, Diabrotica virgifera
atgacgggttggttagcttg

SEQ ID NO: 69 - DNA, 20 bp, Diabrotica virgifera
cggatctctatttgggggat

SEQ ID NO: 70 - DNA, 20 bp, Diabrotica virgifera
acacaaaggtgacaaagggc

SEQ ID NO: 71 - DNA, 21 bp, Diabrotica virgifera
tgctgattggagattcaggag

SEQ ID NO: 72 - DNA, 20 bp, Diabrotica virgifera
cggatttggttgtttcgact

SEQ ID NO: 73 - DNA, 20 bp, Diabrotica virgifera
gagctatagtggactgcggg

SEQ ID NO: 74 - DNA, 20 bp, Diabrotica virgifera
atgacttgtttttcgtgggg

SEQ ID NO: 75 - DNA, 21 bp, Diabrotica virgifera
tggtagatttggctaacctcg

SEQ ID NO: 76 - DNA, 20 bp, Diabrotica virgifera
cccaccctctgttcacattt

SEQ ID NO: 77 - DNA, 20 bp, Diabrotica virgifera
aaccagggatctatttgccc

SEQ ID NO: 78 - DNA, 20 bp, Diabrotica virgifera
ctggaacctttccgctaaca

SEQ ID NO: 79 - DNA, 22 bp, Diabrotica virgifera
tgatggtaatagagtgctggct

SEQ ID NO: 80 - DNA, 21 bp, Diabrotica virgifera
gcaatgaccatttcagctgtt

SEQ ID NO: 81 - DNA, 20 bp, Diabrotica virgifera
caccgaagaacaaattgctg

SEQ ID NO: 82 - DNA, 20 bp, Diabrotica virgifera
cccgaatcatttcatcgact

SEQ ID NO: 83 - DNA, 20 bp, Diabrotica virgifera
ttcgcacaagatgactttgg

SEQ ID NO: 84 - DNA, 20 bp, Diabrotica virgifera
ttgtgggaagggtaacaagg

SEQ ID NO: 85 - DNA, 20 bp, Diabrotica virgifera
taggaatggcattttcaggc

SEQ ID NO: 86 - DNA, 20 bp, Diabrotica virgifera
gcttgtttggcagctttttc

SEQ ID NO: 87 - DNA, 20 bp, Diabrotica virgifera
tccatctagaggagcccaaa

SEQ ID NO: 88 - DNA, 20 bp, Diabrotica virgifera
cgtccagttcggatatgatg

SEQ ID NO: 89 - DNA, 20 bp, Diabrotica virgifera
gatctggaagcgctagttgc

SEQ ID NO: 90 - DNA, 20 bp, Diabrotica virgifera
agtttaggagcggcaagtga

SEQ ID NO: 91 - DNA, 633 bp, Diabrotica virgifera
atggcggacgatgagagaaagaaactggaggaggaaaagaagaggaaacaggccgaaattgaacgcaaaagggccgaggtcagggctcgtatggaagaggcctcaaaagccaagaaggccaagaaaggtttcatgacccctgagagaaagaagaaacttaggttactgttgagaaagaaagccgccgaagaattaaagaaagaacaagaacgcaaagcagccgaaaggaggcgtatcattgaagaaaggtgcggtaaacccaaacttgtcgatgacgcaaatgaaggcccattaaaacaagtatgtgagggatatcacagacgtattgtagacctagaaaataagaaatttgacctcgaaaaagaagtggaattcagagattttcagatctccgaattgaacagccaagtaaacgaccttagaggcaaattcgtcaaaccaaccttgaagaaggtatccaaatacgaaaacaaattcgccaaacttcaaaagaaggcagctgaatttaacttccgtaaccaactcaaagttgtcaagaagaaagaattcaccttagaagaagaagacaaagaaaagaaaccagactggtcaaagaagggagacgaaaagaaggtacaagaggctgaagcatga

SEQ ID NO: 92 - DNA, 603 bp, Diabrotica virgifera
atgtgtgaagaagaagttgccgctttagtcgtagacaatggatccggtatgtgcaaagctggttttgctggggatgatgcacctcgtgctgtattcccttcaattgttggacgcccaagacatcagggtgtgatggtaggaatgggacaaaaagattcctatgtaggtgatgaagctcaaagtaaaagaggtatccttaccttaaaataccccatcgagcacggaatagtcacaaactgggatgatatggagaaaatttggcatcatacattctacaatgaactcagagtagccccagaagaacaccctgttctgttgacagaagctcctctcaaccccaaggccaacagggaaaagatgacacaaataatgtttgaaactttcaacaccccagccatgtatgttgccatccaggctgtactctccttgtatgcatctggtcgtacaactggtattgtgttggattctggtgatggtgtatcccacactgtcccaatctatgaaggttatgctcttcctcatgcaatccttcgtttggacttagctggtagagacttgactgattacctcatgaaaattttgactgaacgtggctactctttc

SEQ ID NO: 93 - DNA, 2742 bp, Diabrotica virgifera
atgccacttcgattagatataaaaagaaagctaacagctcgctcagaccgggtaaaatgtgtggatcttcaccctacagaaccttggatgctgtgttctctttacagcggaaatataaacgtttggaacaccgaaaatcagcaactggttaagacttttgaagtatgtgatgtacctgttcggacagctaagtttttgcccaggaagaactggatagtcagtgggtctgatgatatgcagattcgagttttcaattacaataccttagatcgggtacattcttttgaggctcattcggattatgtgagatgtattgtcgtacaccctacacaaccttatatattaacaagtagtgatgatatgcttatcaagctttggaattgggaaaaagcatgggcttgtcagcaagttttcgaaggacacactcattatattatgcaaatcgccataaatccaaaagacaacaacacatttgccagtgcatccctagatagaacattgaaagtatggcaattgggagcgtccacagcgaatttcacactagaaggtcatgagaaaggcgttaactgtgtggactattatcacggtggagataaaccttatttaatctcaggcgctgatgatagattagtaaaaatctgggattatcaaaacaaaacttgtgttcaaactttggaaggacatgctcaaaatgtaaccgctgcatgtttccatccagaacttcctgtagctcttactggaagtgaagatggtactgtcagagtgtggcatgccaacacccataggttagaaagtagcttaaattatggctttgaaagagtatggactattttctgcctaaagggatccaataacgtggcattgggttatgatgaaggtagcattttggttaaagttggtagagaagaaccagctgttagtatggatgccagtggaggcaaaattatttgggccagacactctgaacttcaacaggcaaatctcaaggcgttagctgaaggtgcggaaataagagatggagaacgccttccagtttctgtaaaagatatgggtgcttgcgagatataccctcagacaattcaacacaatcccaatggccgttttgttgttgtctgtggggatggagaatacataatctacacagcaatggctttaagaaacaaagcgtttggtagcgcacaagaatttgtgtgggctcaagattccagcgaatatgccatcagagaatccggatctactatcagaatttttaagaatttcaaagagaagaagaattttaagtccgattttggagctgaaggtatatacggtggataccttttgggagtcaaatcggtttctggtttgactttctatgattgggaaactctcgatttagtcagaagaatcgagatacaaccaaaagcagtttactggtcagatagtggtaaattagtatgtttggccacagaagatagctactttattctttcttatgattctgatgaagttcaaaaagccagagataacaatcaggttgcggatgatggagtagaatcggctttcaatcttctaggtgaaataaacgaatcagtgcgaactggtctctgggtaggcgactgttttatctacacgaattctgttaatcgtatcaactacttcgttggaggtgaactggttacaattgctcatttggaccggcctttgtatgtcttgggatatgtgcctaaagacgatagattatacctcgtagataaagagttgcgcgtagtaagctaccaattacttctttctgttcttgaatatcaaactgccgtcatgagaagagactttccaacagcagacagagtacttccgtccattcctaaggagcacagaacgagagtggcacatttcttagaaaagcaaggcttcaaacagcaagctttggccgtaagtacagatccagagcacagattcgagctggcagtagcattagaggatcttaatatagccaaaactctagctcaagaagcgaacagtccgcaaaagtggaatcaactagcagaattggcagctgctactaataatgtaagcgtagccaaggaatgtatgcaaaaagcgcaagattatggaggcttgttgcttcttgctacgagctccggtgatgaaaatttagtccgtactctaggagaaacgacacaagctgaaagcaaacataacttagcatttttgtcacacttgttagtaggtgatttaaacaaatgtctagacattcttattaataccggtagattgccagaagctgcatttttcgccagatcttaccttcctgataagattacagaagtcgtggaactgtggaagactcagttatcttcagtcaatcaaaaagctggacagagccttgccgatcctaaaaactacgaaaatctgttccctggtttacaagaggcggtggtagctcagaaatttttggaacagcagaataaaggtttagcgcccgcaagagttgccaccaccattcctcctaatcacgacaggaatgttgtagccgaagttcaagcacaatcgaaacacgatgtaccatcatttagttcttcgtttatttcatcagaaatagaagcacaaacaaggagttctgctaaacctgaagaatcttcaaacattatacagctggaccaagatgacgacgatatcgatttagatttggacggtgtaaatatcgatgagaacattgacacgacggatatcaacatcgatgatgatttgctgagtgattga

SEQ ID NO: 94 - DNA, 1146 bp, Diabrotica virgifera
atgcagatctttgtaaaaacactcactggtaaaaccatcaccctcgaggttgaaccatcagataccatcgagaatgtcaaagctaaaattcaagacaaagaaggtattccaccagatcaacagagattaatctttgctggaaagcagttagaagatggccgtactctctcagactacaacattcagaaagaatctacactacacttagtgcttcgtcttagaggaggtatgcacatctttgtaaaaactctcactggtaagaccatcacccttgaggttgaaccatcagataccatcgagaatgtcaaagctaaaattcaagacaaagaaggtattccaccagatcaacagagattaatctttgctggaaagcagttggaagatggccgtactctctcagactacaacattcaaaaagagtctaccctccatttggtacttcgtcttagaggaggtatgcagatttttgttaaaactttaactggaaagaccatcacccttgaagtagaaccttctgataccatcgaaaatgtcaaagccaaaattcaagacaaagaaggtattccaccagatcaacaaagattaatctttgccggaaagcaattggaagatggtcgtacactctcagactacaacattcaaaaggaatctaccctccatttggtacttcgtcttagaggaggtatgcaaatctttgtaaaaacactcactggtaagaccatcaccctcgaggttgaaccatcagataccatcgagaatgtcaaagctaaaattcaagacaaagaaggtattccaccagatcaacagagattaatcttcgctggaaagcagttggaagatggccgtactctctcagactacaatattcagaaagagtctaccctccatttggtacttcgtcttagaggaggtatgcaaatctttgtaaaaactctcactggtaagaccatcaccctcgaggttgaaccatcagataccatcgagaatgtcaaagctaaaattcaagacaaagaaggtattccaccagatcaacaaagattaatctttgccggaaagcagttggaagatggccgtactctctcagactacaacattcaaaaagagtctacccttcacttggtacttcgtttaagaggaggaaattaa

SEQ ID NO: 95 - DNA, 1131 bp, Diabrotica virgifera
atgtgtgacgacgatgtagcggctcttgtcgtcgacaatggctccggaatgtgcaaagccggtttcgccggtgatgacgcccctcgtgctgtctttccatccatcgtaggtcgtcccagacaccaaggtgtcatggtgggtatgggtcaaaaagactcctacgtaggagacgaagcccaaagcaaaagaggtatcctcaccttaaaataccccattgaacacggaattatcactaactgggacgatatggaaaagatctggcatcacaccttctacaatgaacttagagtagcccccgaagaacatcccattcttttgactgaagctccacttaacccaaaagccaacagagaaaagatgactcaaatcatgtttgaaactttcaatacccctgccatgtatgttgccattcaagctgtattgtctctgtacgcttccggtcgtaccactggtattgtacttgattctggagatggtgtatcccacacagtacccatctatgaaggttacgctctcccacacgccatcttgcgtttggacttggccggtagagacttgactgactaccttatgaagatcttaaccgaaagaggttactctttcaccaccacagctgaaagagaaatagttcgtgacatcaaggaaaaattgtgctatgtagctttggacttcgaacaggaaatggccacagcagccagctccacctccttagaaaagagttatgaacttcctgacggtcaagtcatcaccattggtaatgaaaggttccgttgccctgaagctctcttccaaccttccttcttgggtatggaatcttgcggtatccacgaaactgtctacaactccatcatgaagtgcgatgtcgacatccgtaaagacttgtacgccaacactgtcctttctggaggtaccacaatgtaccctggtattgccgatcgtatgcaaaaggaaatcactgccttggctccatcaaccatcaaaatcaagatcatcgctcccccagaaagaaagtactccgtttggatcggtggctccatcttggcctccctctccaccttccaacagatgtggatctccaaacaagaatacgacgaatccggccctggaattgttcaccgcaaatgcttctaa

SEQ ID NO: 96 - DNA, 2640 bp, Diabrotica virgifera
atgggtacttttaaaagagatactcatgatgaggacgggggatcaagtgcttttcaaaatctggagaaaactactgttttgcaggaagctagagtttttaatgaaactagtgtaaatccaagaaaatgtacaccgatactaacaaaactgttgtacttattgaaccagggtgaaactttaagtgccaaagaggccacagatgttttctttgccatgaccaaactgttccaatcaaaagatgtaatattgagaaggatggtttatttgggaattaaagaactcagttctgttgctgatgatgtcattattgtaacatccagtcttacaaaagatatgactggtaaagaagacatgtacagagcagctgctataagagcattatgcagtattactgatgctactatgcttcaagctatagaacgttatatgaagcaagctattgtagatagaaacgcagctgtcagttcagcagcactaattagttcattacatatgagcaaattagctccagatgtagtaaaaagatgggtaaatgaagctcaggaagcagtaaatagtgataatgcaatggtacagtatcacgcattaggtcttctataccatattaggaagactgataagctagcagtgacaaaattgatttccaagctgaattcaatgggtttaaagagcccttatgctttgtgtatgttgataagaatcactgcaaaacttttagaagaagaggaccaagagtcactcctcaactccccatatacaataatatttacaatgggcttaaggaacaaatctgaaatggtggtgtatgaagctgcacatgccatggttaacctgaagttcacgagtagtaatgtgctagcacccgctataagtgttctacaactattttgtggatctcctaaagccacactcagatttgctgctgttagaactttaaatcaagtggccaccacccaccctgcgtcagtgacagcttgtaatttggatctagaaaatttgattactgatcctaataggtcaattgctacactggccattactactcttttgaaaacaggtgccgaatcttctgttgacagactaatgaaacaaatcgctacttttgtatctgaaatcagtgatgaatttaaagtggttgtcattcaggcaattaaggtattagctttgaaatttccaaggaaacatagcacgcttatgaatttcctatccgccatgttaagagatgagggaggtttagaatataaagcatccatagcagataccattataaccctaatcgaagataatcccgaagctaaagaatctggtttggcgcatctttgcgagttcattgaagactgtgaacatgtttctttggctgtgagaatcttgcatttgttaggaaaggaaggacccaagaccaaacaaccatcgagatacatccgttttatctacaatcgcgtcatattggaatgtccttctgtaagagctgctgcagtctccgccatggcacaattcggagcctcttgtcccgatttgttagaaaatatccaaatattactttcgaggtgtcagatggattcagacgatgaagttagggacagagctacatattatagtaatatacttaacaaaaatgataaaagtttatacaacaattacattttggattctttgcaggtttcaattccttcactagaaagatcgcttagagaatacattcaaaatccaactgacgaaccatttgacattaagtccgtacctgtagcagcagtgccaacagcagaagaacgagaagttaaaaacaaatctgaaggactgctagtctctcaaggtccagtccgacctcctccggtgtctagagaagaaaacttcgccgaaaaacttagtaacgttccgggtatacaacagttaggacctttgttcaaaacttccgacgtcgttgaactcactgaatctgaaacagagtattttgtccgctgtatcaagcactgtttcaaacatcacatcgtcctccaattcgattgtctgaataccttgccagaccagcttttagaaaacgttagagtggagatagacgccggtgaaaccttcgaaattttggcagaaataccttgtgaaaagttgcactataacgaaaccggtaccacatatgtagtagttaagttgcctgatgatgatctccccaactctgttggtacgtgtggagccgtgttgaagttcttagtgaaagattgtgatccatcaacgggaataccagattctgatgagggttacgatgatgaatatacactggaagacatcgaaataacattaggggaccaaattcaaaaagtaagcaaagtaaattgggctgcagcctgggaagaagctgcagctacttatgtagaaaaagaggatacatactccttgaccatcaatacgctaagtggcgctgttaagaatattattcagttcttgggattacagcctgcggaaaggactgacagagtaccggagggtaaatctacgcacacattacttcttgctggtgtattcaggggaggtattgacatactagtaagagcgaaactagctttgggcgaatgtgttacgatgcaactaacagtcaggtcgccagatcctgacgttgctgagcttataacttcaactgtaggttaa

SEQ ID NO: 97 - DNA, 651 bp, Diabrotica virgifera
atggcggcaaacagaactggacctgctcagagaccaaatggcgctacccaaggaaagatatgtcagttcaaactggtcctactaggcgaaagtgccgtcggtaagtcgagtttggtactgaggttcgtcaaaggacagttccacgaataccaggagagtaccataggagcagctttccttacacaaaccatatgcctcgacgatacaactgttaaatttgaaatttgggacacagcgggtcaagaaaggtaccacagtttagctcctatgtactataggggcgcacaggcagctatagtcgtctacgacataaccaatcaagacacattcggcagggcgaaaacgtgggtgaaggaacttcaaaggcaggccagtccgacgatcgtgatagctttggccggcaacaagcaagatttggccaacaaacgtatggtagaatacgaagaggcgcagacgtatgctgacgaaaacggcttactttttatggaaacttccgcaaagacggcaatgaacgtcaacgatatatttttagcaatagctaagaaactgcccaagaatgaacaaaccacaggtcaaggcggcagtgcccaaggcaggcggctagcggagggcgattcgggcgccaaggcacccggaaattgttgcaagtga

SEQ ID NO: 98 - DNA, 279 bp, Diabrotica virgifera
atgaagtttttaagatcgacagtgtgctacattgccatcttggcaattctctttaccctctgtgccgatgaggttgaaggaaggagaaaaattttgatggggcgaaaaagcattaccaggacatatcttcgtggaaatgctgttcctgcgtatgtgataataatccttgtaggaattggtcaaatcatcctgggagggatattgtacgttgcattgaggaagaagatcattgctgcacctgtaacggcatcatatgcagtggctagacaagaaccataa

SEQ ID NO: 99 - DNA, 474 bp, Diabrotica virgifera
atgcagatcttcgttaaaaccttaacgggtaagaccatcactcttgaggtcgagccctcagatactatcgaaaatgtgaaagctaaaatccaggataaagaaggaattcccccagaccagcaacgtctcatcttcgctggaaaacaactcgaagatggtcgtaccttgtctgactataatattcaaaaagaatcaacccttcacttggtgttgagattgagaggaggtgctaagaaacgtaagaagaagaattactccacccccaagaaaatcaagcacaagaagaagaaggttaagttagctgtattgaaattttataaggttgacgaaaatggtaaaatccaccgattgagacgtgaatgccccgctgaacaatgtggagctggtgtcttcatggcagccatggaagacaggcattactgtggcaagtgcggttacactcttgtcttctccaaaccaggagatgagaaatag

SEQ ID NO: 100 - DNA, 747 bp, Diabrotica virgifera
atgatgtccaaagcagacacacaggaagatgcctccttcgccaaattggaaaatcagattgctatcatcaaatacgtaatactctttaccaacgttttgcaatgggctctcggtgcagcaatcttcgctctttgcctttggctacgattcgaggagggcattcaagaatggctccagaaattggattcagaacaattttacatcggagtatatgtacttatagtcgcttcactgatcgtcatgattgtgtcctttataggatgtattagtgccctgcaggagagtaccatggcccttttagtgtacatcggcacccaagtgctcagttttatattcggtttatccggttcggcggttcttctggataacagcgccagagattcccacttccaaccgaggatccgagagagtatgcgacgtcttatcatgaatgctcatcacgaccaatccagacaaacactagccatgattcaggaaaatgttggttgctgcggagctgatggcgcaacagactacctctctcttcagcagccccttccaagtcagtgcagagacaccgttactggaaacccattcttccacggatgtgtagatgaactcacctggttcttcgaagaaaaatgtggttggatagcaggtttagctatggcgatatgcatgattaacgtccttagtattgttttatctacggtactcatccaggcattgaaaaaagaagaagaagcatccgattcatacaggagatag

SEQ ID NO: 101 - DNA, 375 bp, Diabrotica virgifera
atgtctggacgtggcaagggaggcaaagtaaagggaaaagcaaagtcccgatcaaatcgtgctggtttacaatttcctgtaggtcgtattcatcgtttattgagaaaaggaaattatgccgaaagagttggtgctggagctcctgtatacttggcagctgttatggaatatttagctgctgaagttttggaattggcaggaaatgcagctagagataacaaaaagacccgtataattcctagacatttacaattggccataagaaatgacgaggaattgaacaaattactgtcaggagttaccatcgcccaaggtggagtattgcctaatatacaagcagtactgttacctaaaaaaactgaaaagaaagcttaa

SEQ ID NO: 102 - DNA, 864 bp, Diabrotica virgifera
atgaagttggatggtgtagatctgcccccaccaattagcttcgacattgcggaagagcaaccgttaccaccttgccaacagacgttcttatgtaatggtgatggaggatccatagtgcgacagtttctcgagctgtatttcgtaatatatgattcagataataggcagtcccttcttcaggcatatcacgaaaaagccacattttcaatgacaatggcctacccgtacggctattccaaagacagtaaaggagtatcgtggttgaattggtatgccaccgataatagaaatttattacgagttcaagatccagacagaagaaacaagttgttaagacagggacaagttgctgtagtttcgttcttgcaagatatgccgcacacgaagcacgatattcacagttttacagtagatttgacagtttttacaccccagatgttatgtttgacagtggctggtatgtttaaagaattgaaaagtggccacaaagtacctcctttaagatatttcttcagaacccttgtaattgtacctgctggatcaggtttttgcatagcaaatgaagaacttcacatatccaatgcaactccggaccaagcaaaagatgctttcaagaccaccgttaatgtagctccggcaccagcccctgtgattacctctcctggacccagtataccacaacccgctgtgccagatgatgctacaaaacaagaaatggtaaaacagatgtccgcagtatccggaatgaatctcgagtggtcgctacagtgtctcgaagaaacacaatgggactaccagaaagccataatggtattccaaaatttaaacgcacaaggtgttgtaccacaagcagcatttattaaa

SEQ ID NO: 103 - DNA, 2868 bp, Diabrotica virgifera
atgactgcggtagaacaaccttgttacacactaataaacttgccaacagattcggagccctacaatgaaatgcaactaaaaatggatttagaaaagggtgaggttaaagtaaaaataagagcattagaaaaaataattcacatgattctggcaggagaaaggttgccgaatggatttctaatgaccatcataagaaacgttttacctttacaagatcatttggcaaaaaaactattattgattttctgggaaatagttccaaaaacaaatccagaaggtaaactactacaagagatgattttggtatgtgatgcctatagaaaagatctgcaacacccaaatgaatttttgagaggttctacacttcgcttcttgtgcaaactgaaggaaccagaattgttggaaccattaatgcccagtattagagcttgtttggatcataggcacagctatgtgaggaggaatgctgtactggcaatttttaccatttacaaaaattttgaagccctcattccagatgctcctgaactgatctccaattatttggatggtgagcaagacatgtcttgtaaaagaaatgcgtttttaatgcttcttcatgctgaccaagaaagggcgttgtcgtatttggcatcatgtttagatcaagtaaattcatttggagatattctacaactggtcatcgttgagttgatatataaggtgtgtcattccaatcctgcggaaagatctagatttattagatgtatatataacttgttgaactcaagcagtcctgctgtcaggtacgaagctgcaggaactttagtcaccctctccagtgccccgactgccgttaaagctgctgctagctgttacattgagttaattatcaaagaaagtgacaacaatgtaaaactcatcgttttggacaggctgatagcacttaaggagcttcctaatcacgaaagaattctgcaggatttagttatggacatactgagagtactctctgctcctgacttagaagtccgcaagaagactttaagtctagcccttgaattagtctcttcacggaacatagaagaaatggtattagtattaacaaaggaagtgagtaaaacggtagacagtgaacatgaggatacaggaaagtacaggcaattgttagtaaggactctacattcgtgttccattaagttcccagatatcgcacgtagtgttataccagtcttgattgaatttttatccgataataatgaactggctgccacagatgtattgctgttcttaagggaagccatacagaagtttaaagaattgcaaccgttaattattgagaaactcatcgaaactttcaaagacattaaattggtcaaagtccatagagcagcaatttggattttgggagaatacgcgagtactgcttccgatatagaagttatcgttggagaaattaacagattgttgggtgaaggatccctcgttgaagctgagcagaagttaatagcaggagatacggaagagaatgctcctgcacctgctgcaggcgccaccactttagttacttccgatggaacatatgctacccaatcagctttcaacactgtcagccaaaccactaaagaagcacgacctcctctaagacaatacctcatggatggtgattttttcatcggagcctctttggcatctacattaaccaaactgtctttgcggtatgaggacctcacctctcctgctgctagcaatggattcaatgccaaaattatgcttattatggctggaattcttcacttgggaaaatcaggacttcccacaaaatcaataaccaacgacgataaagaccacattctgttctgtttacgagtcctatctgatcgttctccaatcattgttgaaattttcaaaaaattgtgccgctcggcactaaatgagatgcttctagctaaggaatcggtagaagcgatctcgcaaaagagcaaagaaaaaaacaagcgtacgattcaaactgacgacgctataagcttcctgcaattagagacagataaaagtggagagctaggagaaaacgtattcgagatgtcgctgtcacaagctttagtaggaggtcgaacgggaggtggcgaatcagtattaagttccaataaattagataaaatcacacaactgactggtttttccgatccagtttattccgaagcatacgttcacgtgaatcagtacgatatcgtgcttgatgtcttaatcgtaaaccaaactaacgatactttacaaaactgcacgctagagctggctactttaggcgatttgaagttggtagagaagccacaacctgtcgtattggcgcccaaagacttttgcaacattaaagctaacgtgaaagtggcctcaactgaaaacggaattatatttggcaacattgtgtatgatgtcataggagcggggtcagataggaatgttgtagttttgaatgatatacacatagatataatggactatatagtgcctgctagttgtacagatagcgagtttatgagaatgtgggcggaatttgaatgggaaaataaggtaaccgttaacacacccctcacggaactttcagaatacctcgaacatctactcaaaagcacaaatttgaaatgtttaacatcagaaaaagctctgagcgggcagtgtggttttatggcagccaatttatatgcaaaatccatttttggagaagacgctttggccaacttaagtatagagaaaccttttaataaacccgatgcgccagtaagcggtcatattagaataagggccaaaagtcagggcatggccttaagtttaggagacaaagtcaatatgacacagaagagcacacaacataaagtagtagctgcataa

SEQ ID NO: 104 - DNA, 549 bp, Diabrotica virgifera
atgggtaatgtgtttgcaaatttattcaaaggcctctttggcaaaaaggaaatgaggatattgatggtaggactcgatgcagctggtaaaaccacaattttatataaacttaaattaggagaaattgtaacaactattccaacaattggatttaatgtggagactgtagaatataagaacattagttttacagtatgggatgtaggtggtcaagataaaattaggccattgtggagacactatttccaaaacacacaaggcctaattttcgtagtagacagtaacgacagggaacgtatcactgaggctaaagatgaattaatgcgtatgttggccgaagatgaacttagagatgccgtacttctcattttcgccaacaaacaagatttgcccaatgcaatgaacgctgcagaaatcaccgacaaactcggtctccattcactacgcaaccgcaactggtacattcaagctacctgtgcaactagcggagatggtctctatgaaggtctggactggttgtccaatcaattaaagaacgccaatcgctag

SEQ ID NO: 105 - DNA, 4425 bp, Diabrotica virgifera
atgggacggttgcactgtttattttgtattttcctatgttttaccgtcatcaacacgcagacaacgaatatacatggattctcggaaaattccgtggatacatttctatcacctcatgggaaaagtgcaaaattcgtgcaccaaaatcacaaacccaaaattgaaaattgtcagaactacaaaccctcggtgaaagaagaacagccaggcggaacgtacgtaacaacggttaccgctatcgatgacgatcctagggagggaggaggaacaattagttacaaactaattcatagagaaggagaacatgttttatttgacatagacaacgttactggtgttttgacaactatccagccatttgatcgggatgaaccagtaaggcagaaggaactttatgtaaccgtacaagcttcagacaacggcaggccaccattagcagatgtctgtacatttacagttaccattaccgacattaatgataatgcgccacagcttgataaactgaaatacgatgcacaagtttctgaagatttaaaagtaggaagtgaagtgatgagagtttttgcttacgacattgatgatggggaaaattcaagattatcgtataacttttcaaacgaaaatgctcaattcacccagtatttcaggatagatcgagatactggcgttgtgtatttaaaggaagctttaacagacaaaaagaatactagatttaacagtgctgtttatgtagccgataatggcgttaacgatcaagaaggccaaaaagattcaaccgctaagatatctataacagtagtagggtctgataaacagcctcccagatttactcaaaaaatgcctgatggaatcttggagatccccgaagattttaaagacttttctaaacatattgtcacagtcgaagcaacgtccaacattgcggatccacaacttgcttttgaattggtgaagggaaagacatatcaaaccaataaagaccaaacgtttcttttggaggcagaaggaaataaagcgcacataaagctagtgcgtccactggattatgaaacagtaacggaatatactctaactattcgagtaaaaaacaaagatttaatggattcttccataaatataccaattaaagtattagatgttaatgatgaaattcctaatttccttgaatttcttaaaggtagtgtcgtggaaaatgacaagccaggtgcacaagcgattcaagtaagagcaatcgataaagacggaactgctgctaacaacattgtgagctatgaactcgttgacaatacagatttgtttgcaataaaccgatctacgggagtaattacgtcgagagtggagtttgatcgtgaaactgtacctctatatcacgtaaacgttaaagcttatgataactctccgtctgctttgtataacacgacattgcctaacattgtaattcagacattccaaatcagtatagaagatcaaaatgacaacaaacctgtatttactcatccaatttatcagttcagtaatattactgagcttgctgataaatcgagtattgttggtgaagtcaaagctttagataatgacacggcttcagttataagttatagtattacaaatggaaatattgacgatgcgtttatgattgaaaattctaccggcagaataagagttaatggaaaactggattacgagaaaatcgaacaatacaacttaaccgttcgcgcatttgatggggcatttgaagattttgcaattgttttaatttccatacttaatgaaaatgacgaacctccagtttttgacgactatatcagagaaattcaaattaaagaggaagaacctatgatatccggatgcgttgttagagtgactgctcatgatccagatattaaagacaggcatgctgatcaacacatagtatatgaggtcgcgaaagaacagaaagattttttgaccgtatctgccgatggatgcgtacaagtaacaaaacctctcgaccgagatccgcctttcggtagcccaacacgacaagtcttcatctatgctcgtgataatgatggaggcacaaattcattgttggccactgcagaaattgaaattattttaatagatataaacgataatgctccctttttaaatgttacagaaattgtttattatgaaaaccaggatccaggttttataggtaacctaagtgccgatgattacgatggtcctgataatggacctccgtttgcttttcgattatcagacactgcttcagatagtattagatcgaaattttccattatcggaaaccagcttttcgctttagaaatgtttgatagagaagagcaaaaatattatgacattgccattgacattacagatagtggagtacctccactaacaggaactagtattcttagagttataatcggagatgtaaatgataatccagctacagacggaaacagcacgatctttgtgtataagtacgtcaatgggccagaaaatttcatggaaatcggacgtgtatatgttacagacctagacgattgggatttaaatgacaaagtctttgttcaagaagataactttgatgaatttgtgttaaaccagcataacaacggtatgattctgatgaaaccaacaacggctgagggaacttatgaggttcattacagggtcactgaaacccatgaacccacaatacacgaacatacagttaatgcaatagtcacgattacagttaaagtacttccagaggaagcggttgtaaaatcaggatcaattcgattgagaggaacaactaaggaagaattcatagaaaattcattgaatggaaagagcaaaagagacatattacaccaagaactctccaaaatattaaatacatctttagcgaatgttgatgtatttactgttttaaattcaccccaccagaatagttcgtttgtggatgttcgattttctgctcatggatctccatattatgctccagagaaactcgaaaacaaagttacagatcatcaaatggagcttgaacaaaaattagatgtggaattctacatgatcaacgtaaacgagtgccttaacgaaacaacgtgtggagctgaaaactcatgtacgaacaaattaaacataacacgagaaccagctgtagtgtttactaacagaacatcctttgtcggtgtaaatgcatttattgatcctgtgtgtgccgctttaccaagagatgttatggaatgtttcaacggaggcgtccttatcgaaaacacagcgtgtaattgtcctgcaggatttgaaggaccacattgtgaaatcctagctataggatttacaggaactggttgggctatgtatccatcctttgacgctacaaacaggactgagattatactgcatattttatcacaaactgataatggtttgatattttacaatggacctttaaatataagacaaacttctttgtctaaagattatatatcattagaacttaaagacggatatccattacttcaaatttgcaccggctcaagcactcaagaaatttatctgaaagagcgcattcacaaattgagcgatggatcgttacacaaaataaaaataggatctggatttgacgatatatccctggaagtagacgactgtggaacaacgtgttcaatttggactaataaactacataaaggtgttatccgagcaaatggcccccttcaactgggaggtatgaaaaacagattcaccgatcaagaattcaaacgaatttgggaccatttgccaccgactgccacccgtttctctggttgtattagaaatttgacgtataatgaattttactacaacctcggtgcaccttctgatgcattccaagcgtatcccgactgtaactatgcagtgatgcaagctgtgactttcggtatcgactccaatttcttggttgctattctggtttgtgtagcaattttgataattcttcttctggcagtagttgtacatagacgtaaacacgacaactttaacgaaaaagaaatcgatgatactcgcgaaaacattatcaactacgaagatgaaggtggcggcgaatgtgacaccaactacgacctgtctgttttccatcagaacaacattgtggacgaaaaaccattgatgagagacaaccccgatgtacctgcagatataagtggctttttagataacaagaaagacaactgtgataaagaccccgataatttgccttatgacgacgttcgccattatgcctacgagggagacggaaatagcaccggatccttatcttctctcgcttcatgtacggacgaaggagatttaaagttcaactacttatcaagttttggacccagattcagaaagttagccgacatgtatggagaagatccaagcgatgaagactcacacgatggaaacgaagaatcctggtgctag

SEQ ID NO: 106 - DNA, 291 bp, Diabrotica virgifera
atgcctttctgtggtcccaaattgtccctctgcggcctgattatcagtgcatggggtatcatccagttgggtttcatgggtgtattctattacattggggctgtggctttagcagaagatattccagaggttgagtttaagggcgatttagacaaattttatagcgacgtcaacacgggtttcacacagaatgcttacaactgctggattgctgctctcctatacctgataacattagcagtatcagctcaccaattctgggccaacaacagatcatcattgaacgtctaa

SEQ ID NO: 107 - DNA, 540 bp, Diabrotica virgifera
atgggtcttaccatatcagcagtgtttaataggttgtttagtaaaaagcctatgagaattttaatggtaggattagatgccgcaggtaaaaccacaatcttatacaaattgaagcttggtgaaatcgtaactacaataccaaccatcggcttcaatgtagaaaccgttgagtacaagaatatatctttcacggtatgggatgtaggtggccagacgagaatcagaaaactctggagacactatttcgccaacactgatggactcatttttgtggttgattccaacgaccgagaccgtatcgcggaagccgaagaagaattgcacaatatgttaggagaggacgatttaagagactgcattttgttaatattcgccaacaaacaagatttaccgaactcgatgtccactgctgaattgaccgataagcttaagttgcacactttgaagaataggaggtggtacatacaagccacatgtgctactcaagggaatggtttgtacgaaggactagattggttgtcgaatgaattggccaagtga

SEQ ID NO: 108 - DNA, 618 bp, Diabrotica virgifera
atgcggtacactttgagttacatcggtgctaccctagcgtccactgtaacactgatttttgccctctactactgcctcacgggaaaaggagagcaagttagtttagcatggttattgttgaatgtgtctccccacatgtgggcaggtctaggaattggccttgctgtatcattatcagttgtaggagctgctgcaggaattcacactacaggagtcagtatcgtaggagctggtgttaaagcccccagaatcaaaaccaaaaatttaatttctattattttctgtgaagctgtggctatctatgggttaattatggctatagtactctgtggaagttggaagaatttcgatgtagacctattcaacctcaaaactcataactttgctcaaaaccattatggatcacatgttatttttggatccggtttaactgttggatttgtaaatctattatgtggattttgtgttggagtagttggttctggtgcagccatttctgatgcagccaattcatcattattcgtcaaaattttgattattgagatttttggaagtgccattggtctcttcggtctgattgttggagtatacttgacgtcaagaggctctatggtttaa

SEQ ID NO: 109 - DNA, 5694 bp, Diabrotica virgifera
atggctaccaacgatagtaaagctccgttgaggacagttaaaagagtgcaatttggaatacttagtccagatgaaattagacgaatgtcagtcacagaagggggcatccgcttcccagaaaccatggaagcaggccgccccaaactatgcggtcttatggaccccagacaaggtgtcatagacagaagctcaagatgccagacatgtgccggaaatatgacagaatgtcctggacatttcggacatatcgagctggcaaaaccagttttccacgtaggattcgtaacaaaaacaataaagatcttgagatgcgtttgcttcttttgcagtaaattattagtcagtccaaataatccgaaaattaaagaagttgtaatgaaatcaaagggacagccacgtaaaagattagctttcgtttatgatctgtgtaaaggtaaaaatatttgtgaaggtggagatgaaatggatgtgggtaaagaaagcgaagatcccaataaaaaagcaggccatggtggttgtggtcgatatcaaccaaatatcagacgtgccggtttagatttaacagcagaatggaaacacgtcaatgaagacacacaagaaaagaaaatcgcactatctgccgaacgtgtctgggaaatcctaaaacatatcacagatgaagaatgtttcattcttggtatggatcccaaatttgctagaccagattggatgatagtaacggtacttcctgttcctcccctagcagtacgacctgctgtagttatgcacggatctgcaaggaatcaggatgatatcactcacaaattggccgacattatcaaggcgaataacgaattacagaagaacgagtctgcaggtgcagccgctcatataatcacagaaaatattaagatgttgcaatttcacgtcgccactttagttgacaacgatatgccgggaatgccgagagcaatgcaaaaatctggaaaacccctaaaagctatcaaagctcggctgaaaggtaaagaaggaaggattcgaggtaaccttatgggaaagcgtgtggacttttctgcacgtactgtcatcacaccagatcccaatttacgtatcgaccaagtaggagtgcctagaagtattgctcaaaacatgacgtttccagaaatcgtcacacctttcaattttgacaaaatgttggaattggtacagagaggtaattctcagtatccaggagctaagtatatcatcagagacaatggagagaggattgatttacgtttccacccaaaaccgtcagatttacatttgcagtgtggttataaggtagaaagacacatcagagacggcgatctagtaatcttcaaccgtcaaccaaccctccacaagatgagtatgatgggccacagagtcaaagtcttaccctggtcgacgttccgtatgaatctctcgtgcacctctccctacaacgccgattttgacggcgacgaaatgaacctccatgtgccccaaagtatggaaactcgagctgaagtcgaaaacctccacatcactcccaggcaaatcattactccgcaagctaaccaacccgtcatgggtattgtacaagatacgttgacagctgttaggaagatgacaaaaagggatgtattcatcgagaaggaacaaatgatgaatatattgatgttcttgccaatttgggatggtaaaatgccccgtccagccatcctcaaacccaaaccgttgtggacaggaaaacagatattttccctgatcattcctggcaatgtaaatatgatacgtacccattctacgcatccagacgacgaggacgacggtccctataaatggatatcgccaggagatacgaaagttatggtagaacatggagaattggtcatgggtatattgtgtaagaaaagtcttggaacatcagcaggttccctgctgcatatttgtatgttggaattaggacacgaagtgtgtggtagattttatggtaacattcaaactgtaatcaacaactggttgttgttagaaggtcacagcatcggtattggagacaccattgccgatcctcagacttacacagaaattcagagagccatcaggaaagccaaagaagatgtaatagaagtcatccagaaagctcacaacatggaactggaaccgactcccggtaatacgttgcgtcagactttcgaaaatcaagtaaacagaattctaaacgacgctcgtgacaaaactggtggttccgctaagaaatctttgactgaatacaataacctaaaggctatggtcgtatcgggatccaagggatccaacattaatatttcccaggttattgcttgcgtgggtcaacagaacgtagaaggtaaacgtattccatttggcttcagaaaacgcacgttgccgcacttcatcaaggacgattacggtcctgaatccagaggtttcgtagaaaattcgtatcttgccggtctcactccttcggagttctatttccacgctatgggaggtcgtgaaggtcttatcgatactgctgtaaaaactgccgaaactggttacatccagcgtcgtctgatcaaggctatggagagtgtaatggtacactacgacggtaccgtaagaaattctgtaggacaacttatccagttgagatacggtgaggacggactctgtggagagatggtagagtttcaatatttagcaacggtcaaattaagtaacaaggcgtttgagagaaaattcagatttgatccgagtaatgaaaggtatttgagaagagttttcaatgaagaagttatcaagcaactgatgggttcaggggaagtcatttccgaacttgagagagaatgggaacaactccagaaagacagagaagccttaagacaaatcttccctagcggagaatccaaagtagtactcccctgtaatttacaacgtatgatctggaatgtacaaaaaattttccacataaacaaacgagccccgacagacctgtccccgttaagagttatccaaggcgttcgagaattactcaggaaatgcgtcatcgtagctggcgaggatcgtctgtccaaacaagccaacgaaaacgcaacgttactcttccagtgtctagtcagatcgaccctctgcaccaaatgcgtttctgaagaattcaggctcagcaccgaagccttcgagtggttgataggagaaatcgagacgaggttccaacaagcccaagccaatcctggagaaatggtgggcgctctggccgcgcagtcactgggagaacccgctactcagatgacactgaacactttccattttgctggtgtatcctccaagaacgtaaccctgggtgtacctagattaaaggaaattattaatatttccaagaaacccaaggctccatctctaaccgtgtttttaactggtgcggctgctagagatgcggaaaaagcgaagaatgtgttatgcagacttgaacacaccactcttcgtaaagtaaccgccaacaccgccatctattacgatcctgacccacaaaataccgtcattcctgaggatcaggagttcgttaacgtctactatgaaatgcccgatttcgatcctacccgtatatcgccgtggttgcttcgtatcgaactggacagaaagagaatgacagataagaaactaactatggaacaaattgctgaaaagatcaacgctgggttcggggacgatttgaattgtattttcaacgacgacaatgctgaaaagttggtgctgcgtatcagaatcatgaacagcgacgatggaaaattcggagaaggtgctgatgaggacgtagacaaaatggatgacgacatgtttttgagatgcatcgaagcgaacatgctgagcgatatgaccttgcaaggtatagaagcgatttccaaggtatacatgcacttgccacagactgactcgaaaaaaaggatcgtcatcactgaaacaggcgaatttaaggccatcgcagaatggctattggaaactgacggtaccagcatgatgaaagtactgtcagaaagagacgtcgatccggtcaggacgttttctaacgacatttgtgaaatattttcggtacttggtatcgaggctgtgcgtaagtctgtagagaaggaaatgaacgctgtcctttcgttctacggtctgtatgtaaactatcgccatcttgccttgctttgtgacgtaatgacagccaaaggtcacttaatggccatcacccgtcacggtatcaacagacaagacactggagctctgatgaggtgttccttcgaggaaactgtagatgtattgatggacgctgccagtcatgcggaggtcgacccaatgagaggagtatctgaaaacattatcctcggtcaactaccaagaatgggcacaggctgcttcgatcttttgctggacgccgaaaaatgtaaaatgggaattgccatacctcaagcgcacagcagcgatctaatggcttcaggaatgttctttggattagccgctacacccagcagtatgagtccaggtggtgctatgaccccatggaatcaagcagctacaccatacgttggcagtatctggtctccacagaatttaatgggcagtggaatgacaccaggtggtgccgctttctccccatcagctgcgtcagatgcatcaggaatgtcaccagcttatggcggttggtcaccaacaccacaatctcctgcaatgtcgccatatatggcttctccacatggacaatcgccttcctacagtccatcaagtccagcgttccaacctacttcaccatccatgacgccgacctctcctggatattctcccagttctcctggttattcacctaccagtctcaattacagtccaacgagtcccagttattcacccacttctcagagttactccccaacctcacctagttactcaccgacttctccaaattattcacctacttccccaagctacagtccaacatcccctaactattcaccaacatctcccaactattcacccacttcacctagttatccttcaacttcgccaggttacagccccacttcacgcagctactcacccacatctcctagttactcaggaacttcgccctcttattcaccaacttcgccaagttactcccctacttctcctagttattcgccgtcgtctcctaattactctcccacttctccaaattacagtcccacttctcctaattactcaccgtcctctcctaggtacacgcccggttctcctagtttttccccaagttcgaacagttactctcccacatctcctcaatattctccaacatctccaagttattcgccttcttcgcccaaatattcaccaacttcccccaattattcgccaacatctccatcattttctggaggaagtccacaatattcacccacatcaccgaaatactctccaacctcgcccaattacactctgtcgagtccgcagcacactccaacaggtagcagtcgatattcaccgtcaacttcgagttattctcctaattcgcccaattattcaccgacgtctccacaatactccatccacagtacaaaatattcccctgcaagtcctacattcacacccaccagtcctagtttctctcccgcttcacccgcatattcgcctcaacctatgtattcaccttcttctcctaattattctcccactagtcccagtcaagacactgactaa

SEQ ID NO: 110 - DNA, 876 bp, Diabrotica virgifera
atgtcgtcaaatattcaaaaggcccagcagttgatggcggatgcagaaaagaaagtaacatctcgaggtttcttcggatctctatttgggggatcaagtcgtattgaagatgcagtggaatgttacacaagagctgcaaacctttttaaaatggccaagagctgggatgctgccggtaaagccttttgtgaggctgctaatttgcattccagaactggtgctcgtcatgacgctgccactaattatatagatgctgcaaattgttacaaaaaagccgatgtatttgaggctgtaaactgctttataaaagctatagacatttataccgaaatgggtcgctttacaatggctgcaaaacaccatcagactattgcagaaatgtatgagactgatgctgtggacatcgaaagggctgttcaacactatgaacaggcggctgattacttcagaggagaagaaagcaatgcttccgccaataagtgtcttcttaaagtggctcaatatgcagcccaacttgaaaactatgaaaaagcagtgggaatttatcaagaagtggcttatgcagctctggaaagctctcttttaaaatacagtgcaaaggaatacttattcagagctgccctttgtcacctttgtgttgatgtactcaatgcacaacatgctatagaaagctatatttcaaggtatcccgcatttcaagattcccgtgaatacaaacttttgaaaaccctcatagaaaacatcgaagagcaaaacgtagatggatatacagaagccgtcaaagattacgattcaatttctcgtcttgatcagtggtatactacaattcttttacgtattaagaaacaagtaagcgaaagccctgacttacgttaa

SEQ ID NO: 111 - DNA, 609 bp, Diabrotica virgifera
atgaatcccgagtatgattatttattcaaacttctgctgattggagattcaggagtaggaaaatcttgtcttctactgagatttgcagatgatacctacacagaaagctatattagtaccattggcgtagattttaaaatcaggacaatcgatttagatggaaagacaattaaattgcaaatttgggatacagcaggtcaggaaaggtttagaacgattacatcaagttattaccgaggagcacatggtattattgtagtgtacgattgcacagaccaagattcattcaataacgttaaacagtggctcgaagaaatcgaccgttatgcgtgtgacaatgtaaacaaattactggtagggaataaaagcgatttgacaactaagaaagttgtcgacttcactacagccaaggagtatgccgaccaattgggtataccatttttggaaacctcagctaagaatgcaaccaatgtagaacaggcctttatgactatggccgctgaaataaaaaatagagtaggacctccatcttctgcggtagaccaaggaaataaggttaggttcgatcaaagtcgcccagtcgaaacaaccaaatccggttgctgctga

SEQ ID NO: 112 - DNA, 789 bp, Diabrotica virgifera
atggcagacgctgatgatctattagattatgaagatgaggaacagacagaacaaaccgcaactgaaacggcaactacagaggtacagaaaaagggtgtcaagggcacatatgtatcaatacacagttctgggtttagagattttctgttaaaaccagcaattctcagagctatagtggactgcgggttcgaacatccttcagaagttcaacatgaatgtattcctcaagctgtcattggcatggatattctgtgccaagctaaatccggtatgggaaaaacggctgtttttgtattagctacactccaagtaatagatcctacagaaaatgttgtatatgttctcgtcatgtgccataccagagagttagccttccagataagcaaagagtacgaacgtttcagtaaatatatgcccaatattaaagtaggggtcttctttggtggcttgcctatccagaaagatgaggaaacgttaaaaaataattgcccgcatatcgttgtgggtactccaggaagaattttagcattggtcagatcgaaaaaacttaatctcaaacatctaaagcattttattttggatgaatgtgataaaatgttggagttattagacatgagacgtgatgttcaagaaatatatcgtaacactccccacgaaaaacaagtcatgatgttcagtgccaccttaagtaaagaaattagaccagtttgcaagaaatttatgcaagatgtaattcaaaattcttataatacacaattttgtaatgacgcacccactcgcaatgtttga

SEQ ID NO: 113 - DNA, 738 bp, Diabrotica virgifera
atgccggtcattgatggttataaagtactttacattttattacacagtttatatacaatttttgaaaatatttggaggactcttttatttatttatcaaaattgtataagggttataaaccctgaatctacattcgatgatgctgaccagttaaagaaaagactgtctagactaacaaaaaagcctcaacatttaactatcattattggtgtggaagaatattcattggtagatttggctaacctcgtatattggtgtttaggtcttaatattccgtacgttagtttctatgattataaaggtaatttaaaaaagcatgaagagaagttgcaacaaattgtagaatccagaaaatcagagaatatcaacataatttggcacacccatgcagaacaaaggcataaaaatggatttttgggtccaaaaatccacgtaaaagtgttaacacacgcggacggaaagcaaagtatagtaaatgttactaaaaaattagctctaaataaagaaaaagacattagtaaagaaaaaattagtgaattactattaaggcagtatgaatttccagatccagaaatggctattatttgtggaaagaaactgaacatttataattatcctccttggcagttaagactcacagaattctttaaagtcaacaaagtcaacaacatcacattcccagtgtttgtggaaaaattggaaaagtacagcaaatgtgaacagagggtgggaaaataa

SEQ ID NO: 114 - DNA, 480 bp, Diabrotica virgifera
atgaccaactctaaaggttaccgccgaggaaccagggatctatttgcccgcaagtttaaaaaacgtggtgtaattccactttccacatatttgagagtctacaaagttggagatattgtagatatcaagggtaatggtgcagttcaaaagggtatgccccacaaagtgtaccatggtaagacaggacgtgttttcaatgttactgcacatgcattaggtgtaattgtaaacaaaagggttcgaggaagaatcatccccaaaagaatcaatctccgtattgaacatgtaaaccactccaagtgtcgtcaagacttcttgcaaagagtaaaatccaacgaaaagctacgtaaagaagctaaagaaaagaacattaaagtagaacttaggagacaacctgcccaacctaggccagcacatattgttagcggaaaggttccagcacaggtgcttgctcctatcccatatgaattcattgcttag

SEQ ID NO: 115 - DNA, 537 bp, Diabrotica virgifera
atggaaggaatactactggaaccaacattgtataccataaaaggtattgctatattggactatgatggtaatagagtgctggctaaatactacgataaagatatatttcctacagcaaaagagcagaaagcttttgagaaaaatttgttcaataaaactcatagggcagacgcagaaattatcatgttggatggtttaacttgtgtgtatagaagtaatgtagatttattcttttatgttatgggcagttcacatgaaaatgagctaattttaatgagtgttttaaattgcttgtatgactcagtaagtcaaatattgaagaaaaatatgcaaaaacgagctgtcttggaatcactagatattgttatgctggctatggatgaaattgttgatggaggaataattatagattctgattcaagttcagtagtatctagaatagcattaaggactgatgatattccattaggagaacaaactgtagctcaggtattccaaacggccaaagaacagctgaaatggtcattgctgaaataa

SEQ ID NO: 116 - DNA, 450 bp, Diabrotica virgifera
atggctgaccaactcaccgaagaacaaattgctgaattcaaagaagctttctcactattcgataaagatggtgatggtacaattacgactaaagaattaggaacagtaatgagatctctaggacaaaatccaacagaggctgaattacaggatatgatcaatgaagtagatgccgatggtaacggcacgatcgatttcccagaatttttaacgatgatggcacgtaaaatgaaagataccgatagtgaggaagaaattcgtgaagcattccgagtgttcgacaaagacggcaatggtttcatctcagcagcagaattgcgccacgtcatgaccaacttgggtgaaaaattgacagacgaagaagtcgatgaaatgattcgggaggccgatatcgatggtgatggtcaagtcaattacgaagagttcgtcaccatgatgacttcaaagtga

SEQ ID NO: 117 - DNA, 2013 bp, Diabrotica virgifera
atgatgcaagcaaacaatcgagtcccacctataaagttggaaaacgatatagatctttacgccgatgatatcgaggatttcgcacaagatgactttggtggtgaaaatgttgatctatatgacgatgtaatatccgctcctcctggaaataatgacaacccaggtgattcaaatcatcatgctcctcctggtgctggtgaagatggtggaggtaattttgttgggtcaggaggagcacccaataatataaattcttctggaagaagacatcagctgtatgttggaaatctgacttggtggacaactgatcaagatatagaaaatgcagtgcatgatataggggtaaccgacttccatgaagttaagttttttgaacacagagcaaatggtcaatccaagggattctgtgtcatatctttgggatctgagggaagcatgagactctgcctggaactcctatctaaaaaagagatcaatggccaaaatccccttgttacccttcccacaaaacaagctcttagtaactttgaaagtcagtctaaaacacgcccttctcctactaataattctaactcacgtcctccccatcctaataataatgttcattcaggtcctatgcagaattatggaggtagaatgcctatgaacccttccatgcgtcccatgcccccaggtatgcaaggtgctccaagaatgcagggtccacctggatttaatggaccaccaaacatgaatcagcaaccccccaggttccaaggtaatccacaatggaatggacctagacctaatggtcctgggcccaatatgggaatgagacccatggggccacctcatggacaacaagggcccccaagaccaccaatgcagggaccaccgcagcaaggtcctccaagaggaatgccgccacaaggtccaccgcagatgcgtccagaatggaatcgaccaccaatgcaacaagggtaccctcaaggcccgccgcatatgcaaggacctaacatgggtccaagaggtccaccccaaatgggaccacccggggcgcctcaacagcaaggaccagctccgcacgtaaatccagcattctttcaacaaggaggaggaccaccgcccccaatgcaacacatgcctggaccagggcccgtcatgcctcctcaaggacccccgcaaggtccaccacacggacccgttggacctccacacggcccaccattgggtccagcgaatgttccgcctcatggaccacctcacggatatggtccacctgcagcgatgccacagccgccatacggtggcccacctccagaccaccgcgctgagattcctcagttaacagagcaagagtttgaggatataatgtcccggaatagaacagtttccagttcggcgattgggcgggccgtatccgacgccgcagctggagaatttgcaagcgccattgagactttggttactgctatttcactcatcaaacaatccaaagtggctaacgacgatcgttgcaagatccttataagttcgctgcaagatactttgcgtggtgtcgaagacaaaagctacagctccagccgcagagaccggtcaagatccagggacagatcacatagaagaactagaagagaacgatcctcgtcacggtacagagacagaagcagagagagggagcgtgaacgcgatagagatcgtgatcgtgaacgtgacagatattatgatagatacagcgaaagagaaagagaccgagatcgttcaagaagcagagaaagaacagaaagggatagagaacgagattatagagaccgggaacccgaagagacagataaagaaaaatctaaagtatccagagtctcaagatcaagaaacaaatctccggaacctgtcgaacctagcagcgaggtaccgaaatcatcccgctattatgaggataggtatcgggaacgagagagagaaggtcgacgagagagcgatcgcgaaagagaaagagatagaagaggggaagacagccataggtctcgacactag

SEQ ID NO: 118 - DNA, 765 bp, Diabrotica virgifera
atgagttctattggaactgggtacgatttatcagcttcccaattctctcctgatggaagagtatttcaagttgaatatgcaatgaaagcagttgaaaatagtggcaccgtaataggcctccgaggtacagatggcattgtattggctgctgaaaagctcattatgtcaaaattgcatgaaccaagtacaaataaacgaattttcaacattgataaacacataggaatggcattttcaggcttaatagctgatgcaaggcaaatcgttgagattgctagaaaagaagcatcaaattatagacatcaatatggttcaaatattcctcttaaatacctaaatgatagagtaagcatgtacatgcatgcatacactttatacagtgctgttagaccatttggttgcagtgtcatcttggccagttatgaagatagtgacccatctatgtatctgattgatccatctggagttagctatggatactttggatgtgctacaggtaaagcaaaacagtctgcaaagactgaaatagaaaaattgaagatggggaatctaacatgcaaagaacttgttaaagaagcagccaaaatcatttatttggtccatgatgagctgaaggataagaattttgaactggaactttcatgggtatgcaaagatacgaatggtttacataccaaagtgcctgaatcagtgtttgctgatgcagaaaaagctgccaaacaagcaatggaagcagattcagaatcagatacagaagatatgtaa

SEQ ID NO: 119 - DNA, 744 bp, Diabrotica virgifera
atggcttcaaaagacagattgatgatttttccatctagaggagcccaaatgatgatgaaatccaggctaaagggagcccaaaagggacatagtttattaaagaagaaagctgatgctttacaaatgagatttagaatgattttgaacaaaattattgagaccaaaactctcatgggtgaagtaatgaaagaagctgccttttctttagctgaagcaaagtttgcaactggtgacttcaatcaagttgttcttcaaaatgtcaccaaggctcaaataaaaataagaactaagaaagacaacgttgctggtgttactttaccagtgtttgaatgctaccaagatggtacagatacatatgagttggctggtttggctaggggaggtcaacaattgacaaaactcaagaagaattatcaaagtgctgttaaactgttggttgaattagcctctttgcaaacttcttttgtaactcttgatgatgtaatcaaaataacaaacagaagagtcaatgccattgaacatgttatcattccaagaatagagcgtactttggcttacatcatatccgaactggacgagttagaaagagaggagttctatagattaaagaagatccaggacaaaaagaagatcagcagagcaaaggccgagaaacaaaaacaagctcttctccaagctgggctacttaaagagtcccaggcaaacatgcttttggatgagggcgatgaagatctacttttctag

SEQ ID NO: 120 - DNA, 4818 bp, Diabrotica virgifera
atggaggcggctcccaagttaccgatgctctcgttcgagttaaatacttgtacagagaacgtccactttggcccccagttaaaacagtatattgctgctttttatggtgaagatccagaatcctacattacagaaatcagcaatcttgaatccttaagatcagctgcagttcgaccatcaacggatgtaaatggtgtacaactgttgaaaaagtatttctgtcagcttcgttttctcaaatctaggtttcccatggaagagaatcaagatgctgcagttctattttcatggaaaaataatgaattagacataacttcaacatccagtgatatcagatatgaattaatggtaataatgtataacattggagccttacacacttttcttggagccaacgactcaagaaacaatccggatggtatgaaaatggcatgtactcattttcaatgtgctgcatgggcttttcaaaacgtaaaagaaaagtaccaccaattcatatcaaacatctcattggtagaactggttcatttttttcaacaagtctgtttagctcaggctcaggagtgtatattagagaagagcatgtttgacaataggaaacctaccatcattgcaaaagttgctatccaagtctacagttattacagacagtctttacgtgtcttggaatcagtaaatgaagcctactttagggataaaacctacaaggagtggatgaaatatcttcaattcaagctgacctactacaaatgcatctcgttcctattccaagggcaacaagctgaggaacaacagaaaatgggagaaagggttgcattctatcaagctgcatgtgaacagctggacgaggcaaagaaaattgctgctacattaaaaaaccaacaccaccagcaagaaataaatgagggactagcattcactactgatgtggttgaaggtaaaagaaaagcagctaaaaatgaaaatgagttcatctaccatgaatcagtgcctgataaagaccaattgccagaggttaagggtgcttcattagtcaaaggaataccattcagtataaatgatatagaagtttcaggaccagatattttctcccgattggtcccaatggaggcacacgaagcagcttccttgtacagcgagaagaaagctcagagattaagacagatcggggaacttattgaaaataaagatcaaacattggctgaatttatgtcgtcaatgcagctagatctattgaccaagatgcaccaggctactggaataccgcaggagttgattgatagagcagcggctctatctgctaaacctaacgccattcaagatcttataagtgctatgggaaagctatctaatatataccaagacgttgaagcaagtttgaatgagattgattctttattaaaggccgaagaacaaagtgaacaaaagtaccaagaaacgattggtaaaagaccaccgagcattttagctacagatttaactagggaagcggcaaaatacagggaggctcatactaaagcgaacgactcaaaccaaactttacacagggcgatgatggctcacgtggctaatctgaaaatactccaacaaccgctaaagcagctgcaacatcagctgccctttgtcgagtttccaaatccaaatatcgacgaaaaatctttgaaagatctggaagcgctagttgcaaaagtagacgaaatgagaacccaaagagccatgctatgggctcaacttcgagaatctattcaccaagacgatattacaagttcccttgtaacgaaacaaccaaatcagtcgctggaacagctgttccagcaagaacttcaaaagcatcaaaatctgatttcgttgattgaacaaaacacctcggcacaagaaaacattaagagcgccttagtcgattcttacgcttacgctgtaaattcaagaaaatacatccaagatatactccaaaagagaaccacaaccataacgtcactgatagcatcgttcgactcttacgaagacttattggcaaaagctaacaaagggatagagttttactcaaaacttgaaacgaacgtatccaagttactgcaaagaataaggagtacctgcaaagttcaacaagaagagcgagatcagatgatgtcgactgcgcaagtgcctcaatgggagagtcatacgtcacttgccgctcctaaactgaaagattacttggactccaggaagaagagtgctgcgtattcggagccgagtgttcaaccacaacagccaactttaagttactcagctgctatggatctgcctcctggtattaggccgactccagttggatcagaaataacggatgtaccgaaaaatattcaaggtgaaccacaaggttatattccatataattaccaacaaccttctgttcctgcctcacagaatattgatgaagagactattaaaaaaatgaacgcattgatgccaggtgctaagacgtcagtgcctagtcagtacggatacagcaactacattccaccaacataccctcaaagtgcgtaccaaccaggtaatcagtcttacggaaaagaaactccagatattaactcaccgtacgaccctaccaaggcgttcacggctactactaacgcttatcgttcggtgcagagctcctcaactcaaggatacgtaccgtacgcagaatctaacgtttcgaatgttgacagagttggatatcctagcaggtatcagtaccaacaagtacctgagatagctactactccagctgatcccaatattaatgcgtactacccacatgggtactcaccgagccagaatttaccgaatgctaatactcaacatattaccggccaactgaagtaccattcggtggagtacgcttcttctgtgccgaacaacatcaattataacagctctacctactcgtcgccgctttctaatatgtctagtaccaattcctcaaatcctagtaacttgaataattcttacgagtactactatgacccgaataccagtagtggtgcagtaccgaatgcttcaaagcctcaacagtcgagcgccagctctgcaaacccgagtaccgctatgaacaactacaattattactacaatacaagtaccagcggtagtgtagcagcggatacttcaaaaatacaacaacaacaacagtacccaggtactcagatgagtcaagcgcagtactatcccgccaatgccagttattactcaaccagtacttacaataccaacgtccaaggtggtaccaatccctcgtacgcaactggacaaacatataatcaagtgacaccagtgacctctcaaaatgtttctcaaaattacaactttaaccaagttggttctggagcaggacaccagcatcagtactactcgtccgctaacgccgcagtaccatcccaacaagctgtaaataacagttcattaccaaactacggatacgatcagtattacggcaacaactataattccagtcaaccgagtacctacagcgcaaaccaagcacctcctgcagcacaagctgctccaagtaatattcctgctgccaccaaatcctcctctaatgtggatctgctcagtggcttggacttcagcataagccaagctcctctagtgcctcaacaaaacattacgataaaaccccaagaaaaggaaacaaaaccaccggctgtttcttctgaaaccaaaaaccaagatccaacaccagtaaccacgcccaaacaacccactggaccagaagtaaagcgcttgtacgtcaaaatcctgccgagcaaacccttaaacaacgatgatgtgaagaaattgttcggccaagagctggacaggtatgagaagttcgtggagaccttgacccacaaaactttgagcggtccgaccactctggatattaaatggaaggagatccaagaccagcaggattgcgagccgcagaagaagatcatttccgtcgctagatgttatcctatgaagaataggttcccggatatcttgccttacgacttttccagggtggagttgtgcgatagtaaagatgattatatcaacgcttcatacattaaggatatctcgccatatgctccgtcatttattgttacacaagtgccgttgtcttcaactgttggtgatatgtggacgatgattagagaacaacaggtcgaactgatcctctgtttggtaaacgacaatgagatcggtgaagatatttactggcccaaagaaaaaggcagtagtcttaacatacttaacatggtcataacgttgcaaaacgttatagttaagtctcattggactgaaagactgatagcgataaacttacctgaaaaacgggagtcccgtgtgataatgcatctacaatttacatcgtggcctggcagcttgtttccaacaaatcctgaaccgttcgtcagctacaccttggaatccatcaacctataccaacaacagaagaccaacacccatccggtggtggtccattgttcatctggcataggaagaagcggcctgctctgtttactgacagctgctatgttcgatgctgccaacaatgctaactcgataccagatcttacagctttgagtatcaagttgtccaattgcaggaagaatattctcagagatcgagagcatttgaagtttggttacgaaagttttttggcgtatattaggcatatagtttgtgaagataaagccagaaagaaactgaacgagatccagcccaaggttaaggaggaaccactggaaccacctgtcatagttccagaaccaaatatagatcctttaagtactttagacccattttgggctagtaaaagataa

SEQ ID NO: 121 - RNA, 478 nt, Diabrotica virgifera
gguuucaugaccccugagagaaagaagaaacuuagguuacuguugagaaagaaagccgccgaagaauuaaagaaagaacaagaacgcaaagcagccgaaaggaggcguaucauugaagaaaggugcgguaaacccaaacuugucgaugacgcaaaugaaggcccauuaaaacaaguaugugagggauaucacagacguauuguagaccuagaaaauaagaaauuugaccucgaaaaagaaguggaauucagagauuuucagaucuccgaauugaacagccaaguaaacgaccuuagaggcaaauucgucaaaccaaccuugaagaagguauccaaauacgaaaacaaauucgccaaacuucaaaagaaggcagcugaauuuaacuuccguaaccaacucaaaguugucaagaagaaagaauucaccuuagaagaagaagacaaagaaaagaaaccagacuggucaaagaagggagacg

SEQ ID NO: 122 - RNA, 529 nt, Diabrotica virgifera
agaaguugccgcuuuagucguagacaauggauccgguaugugcaaagcugguuuugcuggggaugaugcaccucgugcuguauucccuucaauuguuggacgcccaagacaucagggugugaugguaggaaugggacaaaaagauuccuauguaggugaugaagcucaaaguaaaagagguauccuuaccuuaaaauaccccaucgagcacggaauagucacaaacugggaugauauggagaaaauuuggcaucauacauucuacaaugaacucagaguagccccagaagaacacccuguucuguugacagaagcuccucucaaccccaaggccaacagggaaaagaugacacaaauaauguuugaaacuuucaacaccccagccauguauguugccauccaggcuguacucuccuuguaugcaucuggucguacaacugguauuguguuggauucuggugaugguguaucccacacugucccaaucuaugaagguuaugcucuuccucaugcaauccuucguuuggac

SEQ ID NO: 123 - RNA, 592 nt, Diabrotica virgifera
accggccuuuguaugucuugggauaugugccuaaagacgauagauuauaccucguagauaaagaguugcgcguaguaagcuaccaauuacuucuuucuguucuugaauaucaaacugccgucaugagaagagacuuuccaacagcagacagaguacuuccguccauuccuaaggagcacagaacgagaguggcacauuucuuagaaaagcaaggcuucaaacagcaagcuuuggccguaaguacagauccagagcacagauucgagcuggcaguagcauuagaggaucuuaauauagccaaaacucuagcucaagaagcgaacaguccgcaaaaguggaaucaacuagcagaauuggcagcugcuacuaauaauguaagcguagccaaggaauguaugcaaaaagcgcaagauuauggaggcuuguugcuucuugcuacgagcuccggugaugaaaauuuaguccguacucuaggagaaacgacacaagcugaaagcaaacauaacuuagcauuuuugucacacuuguuaguaggugauuuaaacaaaugucuagacauucuuauuaauaccgguagauugccagaagcugc

SEQ ID NO: 124 - RNA, 594 nt, Diabrotica virgifera
gaaagcaguuggaagauggccguacucucucagacuacaacauucaaaaagagucuacccuccauuugguacuucgucuuagaggagguaugcagauuuuuguuaaaacuuuaacuggaaagaccaucacccuugaaguagaaccuucugauaccaucgaaaaugucaaagccaaaauucaagacaaagaagguauuccaccagaucaacaaagauuaaucuuugccggaaagcaauuggaagauggucguacacucucagacuacaacauucaaaaggaaucuacccuccauuugguacuucgucuuagaggagguaugcaaaucuuuguaaaaacacucacugguaagaccaucacccucgagguugaaccaucagauaccaucgagaaugucaaagcuaaaauucaagacaaagaagguauuccaccagaucaacagagauuaaucuucgcuggaaagcaguuggaagauggccguacucucucagacuacaauauucagaaagagucuacccuccauuugguacuucgucuuagaggagguaugcaaaucuuuguaaaaacucucacugguaagaccaucacccucgagg

SEQ ID NO: 125 - RNA, 547 nt, Diabrotica virgifera
uaccccauugaacacggaauuaucacuaacugggacgauauggaaaagaucuggcaucacaccuucuacaaugaacuuagaguagcccccgaagaacaucccauucuuuugacugaagcuccacuuaacccaaaagccaacagagaaaagaugacucaaaucauguuugaaacuuucaauaccccugccauguauguugccauucaagcuguauugucucuguacgcuuccggucguaccacugguauuguacuugauucuggagaugguguaucccacacaguacccaucuaugaagguuacgcucucccacacgccaucuugcguuuggacuuggccgguagagacuugacugacuaccuuaugaagaucuuaaccgaaagagguuacucuuucaccaccacagcugaaagagaaauaguucgugacaucaaggaaaaauugugcuauguagcuuuggacuucgaacaggaaauggccacagcagccagcuccaccuccuuagaaaagaguuaugaacuuccugacggucaagucaucaccauug

SEQ ID NO: 126 - RNA, 592 nt, Diabrotica virgifera
aggaaaggaaggacccaagaccaaacaaccaucgagauacauccguuuuaucuacaaucgcgucauauuggaauguccuucuguaagagcugcugcagucuccgccauggcacaauucggagccucuugucccgauuuguuagaaaauauccaaauauuacuuucgaggugucagauggauucagacgaugaaguuagggacagagcuacauauuauaguaauauacuuaacaaaaaugauaaaaguuuauacaacaauuacauuuuggauucuuugcagguuucaauuccuucacuagaaagaucgcuuagagaauacauucaaaauccaacugacgaaccauuugacauuaaguccguaccuguagcagcagugccaacagcagaagaacgagaaguuaaaaacaaaucugaaggacugcuagucucucaagguccaguccgaccuccuccggugucuagagaagaaaacuucgccgaaaaacuuaguaacguuccggguauacaacaguuaggaccuuuguucaaaacuuccgacgucguugaacucacugaaucugaaacagaguauuuuguccgcuguaucaagcac

SEQ ID NO: 127 - RNA, 500 nt, Diabrotica virgifera
uacuaggcgaaagugccgucgguaagucgaguuugguacugagguucgucaaaggacaguuccacgaauaccaggagaguaccauaggagcagcuuuccuuacacaaaccauaugccucgacgauacaacuguuaaauuugaaauuugggacacagcgggucaagaaagguaccacaguuuagcuccuauguacuauaggggcgcacaggcagcuauagucgucuacgacauaaccaaucaagacacauucggcagggcgaaaacgugggugaaggaacuucaaaggcaggccaguccgacgaucgugauagcuuuggccggcaacaagcaagauuuggccaacaaacguaugguagaauacgaagaggcgcagacguaugcugacgaaaacggcuuacuuuuuauggaaacuuccgcaaagacggcaaugaacgucaacgauauauuuuuagcaauagcuaagaaacugcccaagaaugaacaaaccacaggucaaggc

SEQ ID NO: 128 - RNA, 189 nt, Diabrotica virgifera
cgaugagguugaaggaaggagaaaaauuuugauggggcgaaaaagcauuaccaggacauaucuucguggaaaugcuguuccugcguaugugauaauaauccuuguaggaauuggucaaaucauccugggagggauauuguacguugcauugaggaagaagaucauugcugcaccuguaacggcaucaua

SEQ ID NO: 129 - RNA, 393 nt, Diabrotica virgifera
ugaggucgagcccucagauacuaucgaaaaugugaaagcuaaaauccaggauaaagaaggaauucccccagaccagcaacgucucaucuucgcuggaaaacaacucgaagauggucguaccuugucugacuauaauauucaaaaagaaucaacccuucacuugguguugagauugagaggaggugcuaagaaacguaagaagaagaauuacuccacccccaagaaaaucaagcacaagaagaagaagguuaaguuagcuguauugaaauuuuauaagguugacgaaaaugguaaaauccaccgauugagacgugaaugccccgcugaacaauguggagcuggugucuucauggcagccauggaagacaggcauuacuguggcaagugcgguua

SEQ ID NO: 130 - RNA, 524 nt, Diabrotica virgifera
ucuuugccuuuggcuacgauucgaggagggcauucaagaauggcuccagaaauuggauucagaacaauuuuacaucggaguauauguacuuauagucgcuucacugaucgucaugauuguguccuuuauaggauguauuagugcccugcaggagaguaccauggcccuuuuaguguacaucggcacccaagugcucaguuuuauauucgguuuauccgguucggcgguucuucuggauaacagcgccagagauucccacuuccaaccgaggauccgagagaguaugcgacgucuuaucaugaaugcucaucacgaccaauccagacaaacacuagccaugauucaggaaaauguugguugcugcggagcugauggcgcaacagacuaccucucucuucagcagccccuuccaagucagugcagagacaccguuacuggaaacccauucuuccacggauguguagaugaacucaccugguucuucgaagaaaaaugugguuggauagcagguuuagcuauggcga

SEQ ID NO: 131 - RNA, 267 nt, Diabrotica virgifera
ucgugcugguuuacaauuuccuguaggucguauucaucguuuauugagaaaaggaaauuaugccgaaagaguuggugcuggagcuccuguauacuuggcagcuguuauggaauauuuagcugcugaaguuuuggaauuggcaggaaaugcagcuagagauaacaaaaagacccguauaauuccuagacauuuacaauuggccauaagaaaugacgaggaauugaacaaauuacugucaggaguuaccaucgcccaagguggaguauu

SEQ ID NO: 132 - RNA, 558 nt, Diabrotica virgifera
gugcaugaaguuggaugguguagaucugcccccaccaauuagcuucgacauugcggaagagcaaccguuaccaccuugccaacagacguucuuauguaauggugauggaggauccauagugcgacaguuucucgagcuguauuucguaauauaugauucagauaauaggcagucccuucuucaggcauaucacgaaaaagccacauuuucaaugacaauggccuacccguacggcuauuccaaagacaguaaaggaguaucgugguugaauugguaugccaccgauaauagaaauuuauuacgaguucaagauccagacagaagaaacaaguuguuaagacagggacaaguugcuguaguuucguucuugcaagauaugccgcacacgaagcacgauauucacaguuuuacaguagauuugacaguuuuuacaccccagauguuauguuugacaguggcugguauguuuaaagaauugaaaaguggccacaaaguaccuccuuuaagauauuucuucagaacccuuguaauuguaccugcuggaucagguuuuugcau

SEQ ID NO: 133 - RNA, 582 nt, Diabrotica virgifera
gauucggagcccuacaaugaaaugcaacuaaaaauggauuuagaaaagggugagguuaaaguaaaaauaagagcauuagaaaaaauaauucacaugauucuggcaggagaaagguugccgaauggauuucuaaugaccaucauaagaaacguuuuaccuuuacaagaucauuuggcaaaaaaacuauuauugauuuucugggaaauaguuccaaaaacaaauccagaagguaaacuacuacaagagaugauuuugguaugugaugccuauagaaaagaucugcaacacccaaaugaauuuuugagagguucuacacuucgcuucuugugcaaacugaaggaaccagaauuguuggaaccauuaaugcccaguauuagagcuuguuuggaucauaggcacagcuaugugaggaggaaugcuguacuggcaauuuuuaccauuuacaaaaauuuugaagcccucauuccagaugcuccugaacugaucuccaauuauuuggauggugagcaagacaugucuuguaaaagaaaugcguuuuuaaugcuucuucaugcugaccaagaaagggcguugucguauuug

SEQ ID NO: 134 - RNA, 458 nt, Diabrotica virgifera
uuggcaaaaaggaaaugaggauauugaugguaggacucgaugcagcugguaaaaccacaauuuuauauaaacuuaaauuaggagaaauuguaacaacuauuccaacaauuggauuuaauguggagacuguagaauauaagaacauuaguuuuacaguaugggauguagguggucaagauaaaauuaggccauuguggagacacuauuuccaaaacacacaaggccuaauuuucguaguagacaguaacgacagggaacguaucacugaggcuaaagaugaauuaaugcguauguuggccgaagaugaacuuagagaugccguacuucucauuuucgccaacaaacaagauuugcccaaugcaaugaacgcugcagaaaucaccgacaaacucggucuccauucacuacgcaaccgcaacugguacauucaagcuaccugugcaacuagcggagauggu

SEQ ID NO: 135 - RNA, 592 nt, Diabrotica virgifera
ggucgcgaaagaacagaaagauuuuuugaccguaucugccgauggaugcguacaaguaacaaaaccucucgaccgagauccgccuuucgguagcccaacacgacaagucuucaucuaugcucgugauaaugauggaggcacaaauucauuguuggccacugcagaaauugaaauuauuuuaauagauauaaacgauaaugcucccuuuuuaaauguuacagaaauuguuuauuaugaaaaccaggauccagguuuuauagguaaccuaagugccgaugauuacgaugguccugauaauggaccuccguuugcuuuucgauuaucagacacugcuucagauaguauuagaucgaaauuuuccauuaucggaaaccagcuuuucgcuuuagaaauguuugauagagaagagcaaaaauauuaugacauugccauugacauuacagauaguggaguaccuccacuaacaggaacuaguauucuuagaguuauaaucggagauguaaaugauaauccagcuacagacggaaacagcacgaucuuuguguauaaguacgucaaugggccagaaaauuucauggaaaucggacgugua

SEQ ID NO: 136 - RNA, 214 nt, Diabrotica virgifera
gcaugggguaucauccaguuggguuucauggguguauucuauuacauuggggcuguggcuuuagcagaagauauuccagagguugaguuuaagggcgauuuagacaaauuuuauagcgacgucaacacggguuucacacagaaugcuuacaacugcuggauugcugcucuccuauaccugauaacauuagcaguaucagcucaccaauucuggg

SEQ ID NO: 137 - RNA, 459 nt, Diabrotica virgifera
uagaugccgcagguaaaaccacaaucuuauacaaauugaagcuuggugaaaucguaacuacaauaccaaccaucggcuucaauguagaaaccguugaguacaagaauauaucuuucacgguaugggauguagguggccagacgagaaucagaaaacucuggagacacuauuucgccaacacugauggacucauuuuugugguugauuccaacgaccgagaccguaucgcggaagccgaagaagaauugcacaauauguuaggagaggacgauuuaagagacugcauuuuguuaauauucgccaacaaacaagauuuaccgaacucgauguccacugcugaauugaccgauaagcuuaaguugcacacuuugaagaauaggaggugguacauacaagccacaugugcuacucaagggaaugguuuguacgaaggacuagauugguugucgaaugaauugg

SEQ ID NO: 138 - RNA, 536 nt, Diabrotica virgifera
gcuacccuagcguccacuguaacacugauuuuugcccucuacuacugccucacgggaaaaggagagcaaguuaguuuagcaugguuauuguugaaugugucuccccacaugugggcaggucuaggaauuggccuugcuguaucauuaucaguuguaggagcugcugcaggaauucacacuacaggagucaguaucguaggagcugguguuaaagcccccagaaucaaaaccaaaaauuuaauuucuauuauuuucugugaagcuguggcuaucuauggguuaauuauggcuauaguacucuguggaaguuggaagaauuucgauguagaccuauucaaccucaaaacucauaacuuugcucaaaaccauuauggaucacauguuauuuuuggauccgguuuaacuguuggauuuguaaaucuauuauguggauuuuguguuggaguaguugguucuggugcagccauuucugaugcagccaauucaucauuauucgucaaaauuuugauuauugagauuuuuggaagugccauugg

SEQ ID NO: 139 - RNA, 547 nt, Diabrotica virgifera
accuuaugggaaagcguguggacuuuucugcacguacugucaucacaccagaucccaauuuacguaucgaccaaguaggagugccuagaaguauugcucaaaacaugacguuuccagaaaucgucacaccuuucaauuuugacaaaauguuggaauugguacagagagguaauucucaguauccaggagcuaaguauaucaucagagacaauggagagaggauugauuuacguuuccacccaaaaccgucagauuuacauuugcagugugguuauaagguagaaagacacaucagagacggcgaucuaguaaucuucaaccgucaaccaacccuccacaagaugaguaugaugggccacagagucaaagucuuacccuggucgacguuccguaugaaucucucgugcaccucucccuacaacgccgauuuugacggcgacgaaaugaaccuccaugugccccaaaguauggaaacucgagcugaagucgaaaaccuccacaucacucccaggcaaaucauuacuccgcaagcuaaccaacccgucau

SEQ ID NO: 140 - RNA, 564 nt, Diabrotica virgifera
cggaucucuauuugggggaucaagucguauugaagaugcaguggaauguuacacaagagcugcaaaccuuuuuaaaauggccaagagcugggaugcugccgguaaagccuuuugugaggcugcuaauuugcauuccagaacuggugcucgucaugacgcugccacuaauuauauagaugcugcaaauuguuacaaaaaagccgauguauuugaggcuguaaacugcuuuauaaaagcuauagacauuuauaccgaaaugggucgcuuuacaauggcugcaaaacaccaucagacuauugcagaaauguaugagacugaugcuguggacaucgaaagggcuguucaacacuaugaacaggcggcugauuacuucagaggagaagaaagcaaugcuuccgccaauaagugucuucuuaaaguggcucaauaugcagcccaacuugaaaacuaugaaaaagcagugggaauuuaucaagaaguggcuuaugcagcucuggaaagcucucuuuuaaaauacagugcaaaggaauacuuauucagagcugcccuuugucaccuuugugu

SEQ ID NO: 141 - RNA, 564 nt, Diabrotica virgifera
ugcugauuggagauucaggaguaggaaaaucuugucuucuacugagauuugcagaugauaccuacacagaaagcuauauuaguaccauuggcguagauuuuaaaaucaggacaaucgauuuagauggaaagacaauuaaauugcaaauuugggauacagcaggucaggaaagguuuagaacgauuacaucaaguuauuaccgaggagcacaugguauuauuguaguguacgauugcacagaccaagauucauucaauaacguuaaacaguggcucgaagaaaucgaccguuaugcgugugacaauguaaacaaauuacugguagggaauaaaagcgauuugacaacuaagaaaguugucgacuucacuacagccaaggaguaugccgaccaauuggguauaccauuuuuggaaaccucagcuaagaaugcaaccaauguagaacaggccuuuaugacuauggccgcugaaauaaaaaauagaguaggaccuccaucuucugcgguagaccaaggaaauaagguuagguucgaucaaagucgcccagucgaaacaaccaaauccg

SEQ ID NO: 142 - RNA, 502 nt, Diabrotica virgifera
gagcuauaguggacugcggguucgaacauccuucagaaguucaacaugaauguauuccucaagcugucauuggcauggauauucugugccaagcuaaauccgguaugggaaaaacggcuguuuuuguauuagcuacacuccaaguaauagauccuacagaaaauguuguauauguucucgucaugugccauaccagagaguuagccuuccagauaagcaaagaguacgaacguuucaguaaauauaugcccaauauuaaaguaggggucuucuuugguggcuugccuauccagaaagaugaggaaacguuaaaaaauaauugcccgcauaucguuguggguacuccaggaagaauuuuagcauuggucagaucgaaaaaacuuaaucucaaacaucuaaagcauuuuauuuuggaugaaugugauaaaauguuggaguuauuagacaugagacgugauguucaagaaauauaucguaacacuccccacgaaaaacaagucau

SEQ ID NO: 143 - RNA, 505 nt, Diabrotica virgifera
ugguagauuuggcuaaccucguauauugguguuuaggucuuaauauuccguacguuaguuucuaugauuauaaagguaauuuaaaaaagcaugaagagaaguugcaacaaauuguagaauccagaaaaucagagaauaucaacauaauuuggcacacccaugcagaacaaaggcauaaaaauggauuuuuggguccaaaaauccacguaaaaguguuaacacacgcggacggaaagcaaaguauaguaaauguuacuaaaaaauuagcucuaaauaaagaaaaagacauuaguaaagaaaaaauuagugaauuacuauuaaggcaguaugaauuuccagauccagaaauggcuauuauuuguggaaagaaacugaacauuuauaauuauccuccuuggcaguuaagacucacagaauucuuuaaagucaacaaagucaacaacaucacauucccaguguuuguggaaaaauuggaaaaguacagcaaaugugaacagaggguggg

SEQ ID NO: 144 - RNA, 410 nt, Diabrotica virgifera
aaccagggaucuauuugcccgcaaguuuaaaaaacgugguguaauuccacuuuccacauauuugagagucuacaaaguuggagauauuguagauaucaaggguaauggugcaguucaaaaggguaugccccacaaaguguaccaugguaagacaggacguguuuucaauguuacugcacaugcauuagguguaauuguaaacaaaaggguucgaggaagaaucauccccaaaagaaucaaucuccguauugaacauguaaaccacuccaagugucgucaagacuucuugcaaagaguaaaauccaacgaaaagcuacguaaagaagcuaaagaaaagaacauuaaaguagaacuuaggagacaaccugcccaaccuaggccagcacauauuguuagcggaaagguuccag

SEQ ID NO: 145 - RNA, 467 nt, Diabrotica virgifera
ugaugguaauagagugcuggcuaaauacuacgauaaagauauauuuccuacagcaaaagagcagaaagcuuuugagaaaaauuuguucaauaaaacucauagggcagacgcagaaauuaucauguuggaugguuuaacuuguguguauagaaguaauguagauuuauucuuuuauguuaugggcaguucacaugaaaaugagcuaauuuuaaugaguguuuuaaauugcuuguaugacucaguaagucaaauauugaagaaaaauaugcaaaaacgagcugucuuggaaucacuagauauuguuaugcuggcuauggaugaaauuguugauggaggaauaauuauagauucugauucaaguucaguaguaucuagaauagcauuaaggacugaugauauuccauuaggagaacaaacuguagcucagguauuccaaacggccaaagaacagcugaaauggucauugc

SEQ ID NO: 146 - RNA, 368 nt, Diabrotica virgifera
caccgaagaacaaauugcugaauucaaagaagcuuucucacuauucgauaaagauggugaugguacaauuacgacuaaagaauuaggaacaguaaugagaucucuaggacaaaauccaacagaggcugaauuacaggauaugaucaaugaaguagaugccgaugguaacggcacgaucgauuucccagaauuuuuaacgaugauggcacguaaaaugaaagauaccgauagugaggaagaaauucgugaagcauuccgaguguucgacaaagacggcaaugguuucaucucagcagcagaauugcgccacgucaugaccaacuugggugaaaaauugacagacgaagaagucgaugaaaugauucggg

SEQ ID NO: 147 - RNA, 430 nt, Diabrotica virgifera
uucgcacaagaugacuuugguggugaaaauguugaucuauaugacgauguaauauccgcuccuccuggaaauaaugacaacccaggugauucaaaucaucaugcuccuccuggugcuggugaagaugguggagguaauuuuguugggucaggaggagcacccaauaauauaaauucuucuggaagaagacaucagcuguauguuggaaaucugacuugguggacaacugaucaagauauagaaaaugcagugcaugauauagggguaaccgacuuccaugaaguuaaguuuuuugaacacagagcaaauggucaauccaagggauucugugucauaucuuugggaucugagggaagcaugagacucugccuggaacuccuaucuaaaaaagagaucaauggccaaaauccccuuguuacccuucccacaa

SEQ ID NO: 148 - RNA, 505 nt, Diabrotica virgifera
uaggaauggcauuuucaggcuuaauagcugaugcaaggcaaaucguugagauugcuagaaaagaagcaucaaauuauagacaucaauaugguucaaauauuccucuuaaauaccuaaaugauagaguaagcauguacaugcaugcauacacuuuauacagugcuguuagaccauuugguugcagugucaucuuggccaguuaugaagauagugacccaucuauguaucugauugauccaucuggaguuagcuauggauacuuuggaugugcuacagguaaagcaaaacagucugcaaagacugaaauagaaaaauugaagauggggaaucuaacaugcaaagaacuuguuaaagaagcagccaaaaucauuuauuugguccaugaugagcugaaggauaagaauuuugaacuggaacuuucauggguaugcaaagauacgaaugguuuacauaccaaagugccugaaucaguguuugcugaugcagaaaaagcugccaaacaagc

SEQ ID NO: 149 - RNA, 548 nt, Diabrotica virgifera
uccaucuagaggagcccaaaugaugaugaaauccaggcuaaagggagcccaaaagggacauaguuuauuaaagaagaaagcugaugcuuuacaaaugagauuuagaaugauuuugaacaaaauuauugagaccaaaacucucaugggugaaguaaugaaagaagcugccuuuucuuuagcugaagcaaaguuugcaacuggugacuucaaucaaguuguucuucaaaaugucaccaaggcucaaauaaaaauaagaacuaagaaagacaacguugcugguguuacuuuaccaguguuugaaugcuaccaagaugguacagauacauaugaguuggcugguuuggcuaggggaggucaacaauugacaaaacucaagaagaauuaucaaagugcuguuaaacuguugguugaauuagccucuuugcaaacuucuuuuguaacucuugaugauguaaucaaaauaacaaacagaagagucaaugccauugaacauguuaucauuccaagaauagagcguacuuuggcuuacaucauauccgaacuggacg

SEQ ID NO: 150 - RNA, 521 nt, Diabrotica virgifera
gaucuggaagcgcuaguugcaaaaguagacgaaaugagaacccaaagagccaugcuaugggcucaacuucgagaaucuauucaccaagacgauauuacaaguucccuuguaacgaaacaaccaaaucagucgcuggaacagcuguuccagcaagaacuucaaaagcaucaaaaucugauuucguugauugaacaaaacaccucggcacaagaaaacauuaagagcgccuuagucgauucuuacgcuuacgcuguaaauucaagaaaauacauccaagauauacuccaaaagagaaccacaaccauaacgucacugauagcaucguucgacucuuacgaagacuuauuggcaaaagcuaacaaagggauagaguuuuacucaaaacuugaaacgaacguauccaaguuacugcaaagaauaaggaguaccugcaaaguucaacaagaagagcgagaucagaugaugucgacugcgcaagugccucaaugggagagucauacgucacuugccgcuccuaaacu

SEQ ID NO: 151 - RNA, 633 nt, Diabrotica virgifera
auggcggacgaugagagaaagaaacuggaggaggaaaagaagaggaaacaggccgaaauugaacgcaaaagggccgaggucagggcucguauggaagaggccucaaaagccaagaaggccaagaaagguuucaugaccccugagagaaagaagaaacuuagguuacuguugagaaagaaagccgccgaagaauuaaagaaagaacaagaacgcaaagcagccgaaaggaggcguaucauugaagaaaggugcgguaaacccaaacuugucgaugacgcaaaugaaggcccauuaaaacaaguaugugagggauaucacagacguauuguagaccuagaaaauaagaaauuugaccucgaaaaagaaguggaauucagagauuuucagaucuccgaauugaacagccaaguaaacgaccuuagaggcaaauucgucaaaccaaccuugaagaagguauccaaauacgaaaacaaauucgccaaacuucaaaagaaggcagcugaauuuaacuuccguaaccaacucaaaguugucaagaagaaagaauucaccuuagaagaagaagacaaagaaaagaaaccagacuggucaaagaagggagacgaaaagaagguacaagaggcugaagcauga

SEQ ID NO: 152 - RNA, 603 nt, Diabrotica virgifera
augugugaagaagaaguugccgcuuuagucguagacaauggauccgguaugugcaaagcugguuuugcuggggaugaugcaccucgugcuguauucccuucaauuguuggacgcccaagacaucagggugugaugguaggaaugggacaaaaagauuccuauguaggugaugaagcucaaaguaaaagagguauccuuaccuuaaaauaccccaucgagcacggaauagucacaaacugggaugauauggagaaaauuuggcaucauacauucuacaaugaacucagaguagccccagaagaacacccuguucuguugacagaagcuccucucaaccccaaggccaacagggaaaagaugacacaaauaauguuugaaacuuucaacaccccagccauguauguugccauccaggcuguacucuccuuguaugcaucuggucguacaacugguauuguguuggauucuggugaugguguaucccacacugucccaaucuaugaagguuaugcucuuccucaugcaauccuucguuuggacuuagcugguagagacuugacugauuaccucaugaaaauuuugacugaacguggcuacucuuuc

SEQ ID NO: 153 - RNA, 2742 nt, Diabrotica virgifera
augccacuucgauuagauauaaaaagaaagcuaacagcucgcucagaccggguaaaauguguggaucuucacccuacagaaccuuggaugcuguguucucuuuacagcggaaauauaaacguuuggaacaccgaaaaucagcaacugguuaagacuuuugaaguaugugauguaccuguucggacagcuaaguuuuugcccaggaagaacuggauagucagugggucugaugauaugcagauucgaguuuucaauuacaauaccuuagaucggguacauucuuuugaggcucauucggauuaugugagauguauugucguacacccuacacaaccuuauauauuaacaaguagugaugauaugcuuaucaagcuuuggaauugggaaaaagcaugggcuugucagcaaguuuucgaaggacacacucauuauauuaugcaaaucgccauaaauccaaaagacaacaacacauuugccagugcaucccuagauagaacauugaaaguauggcaauugggagcguccacagcgaauuucacacuagaaggucaugagaaaggcguuaacuguguggacuauuaucacgguggagauaaaccuuauuuaaucucaggcgcugaugauagauuaguaaaaaucugggauuaucaaaacaaaacuuguguucaaacuuuggaaggacaugcucaaaauguaaccgcugcauguuuccauccagaacuuccuguagcucuuacuggaagugaagaugguacugucagaguguggcaugccaacacccauagguuagaaaguagcuuaaauuauggcuuugaaagaguauggacuauuuucugccuaaagggauccaauaacguggcauuggguuaugaugaagguagcauuuugguuaaaguugguagagaagaaccagcuguuaguauggaugccaguggaggcaaaauuauuugggccagacacucugaacuucaacaggcaaaucucaaggcguuagcugaaggugcggaaauaagagauggagaacgccuuccaguuucuguaaaagauaugggugcuugcgagauauacccucagacaauucaacacaaucccaauggccguuuuguuguugucuguggggauggagaauacauaaucuacacagcaauggcuuuaagaaacaaagcguuugguagcgcacaagaauuugugugggcucaagauuccagcgaauaugccaucagagaauccggaucuacuaucagaauuuuuaagaauuucaaagagaagaagaauuuuaaguccgauuuuggagcugaagguauauacgguggauaccuuuugggagucaaaucgguuucugguuugacuuucuaugauugggaaacucucgauuuagucagaagaaucgagauacaaccaaaagcaguuuacuggucagauagugguaaauuaguauguuuggccacagaagauagcuacuuuauucuuucuuaugauucugaugaaguucaaaaagccagagauaacaaucagguugcggaugauggaguagaaucggcuuucaaucuucuaggugaaauaaacgaaucagugcgaacuggucucuggguaggcgacuguuuuaucuacacgaauucuguuaaucguaucaacuacuucguuggaggugaacugguuacaauugcucauuuggaccggccuuuguaugucuugggauaugugccuaaagacgauagauuauaccucguagauaaagaguugcgcguaguaagcuaccaauuacuucuuucuguucuugaauaucaaacugccgucaugagaagagacuuuccaacagcagacagaguacuuccguccauuccuaaggagcacagaacgagaguggcacauuucuuagaaaagcaaggcuucaaacagcaagcuuuggccguaaguacagauccagagcacagauucgagcuggcaguagcauuagaggaucuuaauauagccaaaacucuagcucaagaagcgaacaguccgcaaaaguggaaucaacuagcagaauuggcagcugcuacuaauaauguaagcguagccaaggaauguaugcaaaaagcgcaagauuauggaggcuuguugcuucuugcuacgagcuccggugaugaaaauuuaguccguacucuaggagaaacgacacaagcugaaagcaaacauaacuuagcauuuuugucacacuuguuaguaggugauuuaaacaaaugucuagacauucuuauuaauaccgguagauugccagaagcugcauuuuucgccagaucuuaccuuccugauaagauuacagaagucguggaacuguggaagacucaguuaucuucagucaaucaaaaagcuggacagagccuugccgauccuaaaaacuacgaaaaucuguucccugguuuacaagaggcggugguagcucagaaauuuuuggaacagcagaauaaagguuuagcgcccgcaagaguugccaccaccauuccuccuaaucacgacaggaauguuguagccgaaguucaagcacaaucgaaacacgauguaccaucauuuaguucuucguuuauuucaucagaaauagaagcacaaacaaggaguucugcuaaaccugaagaaucuucaaacauuauacagcuggaccaagaugacgacgauaucgauuuagauuuggacgguguaaauaucgaugagaacauugacacgacggauaucaacaucgaugaugauuugcugagugauuga

SEQ ID NO: 154 - RNA, 1146 nt, Diabrotica virgifera
augcagaucuuuguaaaaacacucacugguaaaaccaucacccucgagguugaaccaucagauaccaucgagaaugucaaagcuaaaauucaagacaaagaagguauuccaccagaucaacagagauuaaucuuugcuggaaagcaguuagaagauggccguacucucucagacuacaacauucagaaagaaucuacacuacacuuagugcuucgucuuagaggagguaugcacaucuuuguaaaaacucucacugguaagaccaucacccuugagguugaaccaucagauaccaucgagaaugucaaagcuaaaauucaagacaaagaagguauuccaccagaucaacagagauuaaucuuugcuggaaagcaguuggaagauggccguacucucucagacuacaacauucaaaaagagucuacccuccauuugguacuucgucuuagaggagguaugcagauuuuuguuaaaacuuuaacuggaaagaccaucacccuugaaguagaaccuucugauaccaucgaaaaugucaaagccaaaauucaagacaaagaagguauuccaccagaucaacaaagauuaaucuuugccggaaagcaauuggaagauggucguacacucucagacuacaacauucaaaaggaaucuacccuccauuugguacuucgucuuagaggagguaugcaaaucuuuguaaaaacacucacugguaagaccaucacccucgagguugaaccaucagauaccaucgagaaugucaaagcuaaaauucaagacaaagaagguauuccaccagaucaacagagauuaaucuucgcuggaaagcaguuggaagauggccguacucucucagacuacaauauucagaaagagucuacccuccauuugguacuucgucuuagaggagguaugcaaaucuuuguaaaaacucucacugguaagaccaucacccucgagguugaaccaucagauaccaucgagaaugucaaagcuaaaauucaagacaaagaagguauuccaccagaucaacaaagauuaaucuuugccggaaagcaguuggaagauggccguacucucucagacuacaacauucaaaaagagucuacccuucacuugguacuucguuuaagaggaggaaauuaa

SEQ ID NO: 155 - RNA, 1131 nt, Diabrotica virgifera
augugugacgacgauguagcggcucuugucgucgacaauggcuccggaaugugcaaagccgguuucgccggugaugacgccccucgugcugucuuuccauccaucguaggucgucccagacaccaaggugucaugguggguaugggucaaaaagacuccuacguaggagacgaagcccaaagcaaaagagguauccucaccuuaaaauaccccauugaacacggaauuaucacuaacugggacgauauggaaaagaucuggcaucacaccuucuacaaugaacuuagaguagcccccgaagaacaucccauucuuuugacugaagcuccacuuaacccaaaagccaacagagaaaagaugacucaaaucauguuugaaacuuucaauaccccugccauguauguugccauucaagcuguauugucucuguacgcuuccggucguaccacugguauuguacuugauucuggagaugguguaucccacacaguacccaucuaugaagguuacgcucucccacacgccaucuugcguuuggacuuggccgguagagacuugacugacuaccuuaugaagaucuuaaccgaaagagguuacucuuucaccaccacagcugaaagagaaauaguucgugacaucaaggaaaaauugugcuauguagcuuuggacuucgaacaggaaauggccacagcagccagcuccaccuccuuagaaaagaguuaugaacuuccugacggucaagucaucaccauugguaaugaaagguuccguugcccugaagcucucuuccaaccuuccuucuuggguauggaaucuugcgguauccacgaaacugucuacaacuccaucaugaagugcgaugucgacauccguaaagacuuguacgccaacacuguccuuucuggagguaccacaauguacccugguauugccgaucguaugcaaaaggaaaucacugccuuggcuccaucaaccaucaaaaucaagaucaucgcucccccagaaagaaaguacuccguuuggaucgguggcuccaucuuggccucccucuccaccuuccaacagauguggaucuccaaacaagaauacgacgaauccggcccuggaauuguucaccgcaaaugcuucuaa

SEQ ID NO: 156 - RNA, 2640 nt, Diabrotica virgifera
auggguacuuuuaaaagagauacucaugaugaggacgggggaucaagugcuuuucaaaaucuggagaaaacuacuguuuugcaggaagcuagaguuuuuaaugaaacuaguguaaauccaagaaaauguacaccgauacuaacaaaacuguuguacuuauugaaccagggugaaacuuuaagugccaaagaggccacagauguuuucuuugccaugaccaaacuguuccaaucaaaagauguaauauugagaaggaugguuuauuugggaauuaaagaacucaguucuguugcugaugaugucauuauuguaacauccagucuuacaaaagauaugacugguaaagaagacauguacagagcagcugcuauaagagcauuaugcaguauuacugaugcuacuaugcuucaagcuauagaacguuauaugaagcaagcuauuguagauagaaacgcagcugucaguucagcagcacuaauuaguucauuacauaugagcaaauuagcuccagauguaguaaaaagauggguaaaugaagcucaggaagcaguaaauagugauaaugcaaugguacaguaucacgcauuaggucuucuauaccauauuaggaagacugauaagcuagcagugacaaaauugauuuccaagcugaauucaauggguuuaaagagcccuuaugcuuuguguauguugauaagaaucacugcaaaacuuuuagaagaagaggaccaagagucacuccucaacuccccauauacaauaauauuuacaaugggcuuaaggaacaaaucugaaauggugguguaugaagcugcacaugccaugguuaaccugaaguucacgaguaguaaugugcuagcacccgcuauaaguguucuacaacuauuuuguggaucuccuaaagccacacucagauuugcugcuguuagaacuuuaaaucaaguggccaccacccacccugcgucagugacagcuuguaauuuggaucuagaaaauuugauuacugauccuaauaggucaauugcuacacuggccauuacuacucuuuugaaaacaggugccgaaucuucuguugacagacuaaugaaacaaaucgcuacuuuuguaucugaaaucagugaugaauuuaaagugguugucauucaggcaauuaagguauuagcuuugaaauuuccaaggaaacauagcacgcuuaugaauuuccuauccgccauguuaagagaugagggagguuuagaauauaaagcauccauagcagauaccauuauaacccuaaucgaagauaaucccgaagcuaaagaaucugguuuggcgcaucuuugcgaguucauugaagacugugaacauguuucuuuggcugugagaaucuugcauuuguuaggaaaggaaggacccaagaccaaacaaccaucgagauacauccguuuuaucuacaaucgcgucauauuggaauguccuucuguaagagcugcugcagucuccgccauggcacaauucggagccucuugucccgauuuguuagaaaauauccaaauauuacuuucgaggugucagauggauucagacgaugaaguuagggacagagcuacauauuauaguaauauacuuaacaaaaaugauaaaaguuuauacaacaauuacauuuuggauucuuugcagguuucaauuccuucacuagaaagaucgcuuagagaauacauucaaaauccaacugacgaaccauuugacauuaaguccguaccuguagcagcagugccaacagcagaagaacgagaaguuaaaaacaaaucugaaggacugcuagucucucaagguccaguccgaccuccuccggugucuagagaagaaaacuucgccgaaaaacuuaguaacguuccggguauacaacaguuaggaccuuuguucaaaacuuccgacgucguugaacucacugaaucugaaacagaguauuuuguccgcuguaucaagcacuguuucaaacaucacaucguccuccaauucgauugucugaauaccuugccagaccagcuuuuagaaaacguuagaguggagauagacgccggugaaaccuucgaaauuuuggcagaaauaccuugugaaaaguugcacuauaacgaaaccgguaccacauauguaguaguuaaguugccugaugaugaucuccccaacucuguugguacguguggagccguguugaaguucuuagugaaagauugugauccaucaacgggaauaccagauucugaugaggguuacgaugaugaauauacacuggaagacaucgaaauaacauuaggggaccaaauucaaaaaguaagcaaaguaaauugggcugcagccugggaagaagcugcagcuacuuauguagaaaaagaggauacauacuccuugaccaucaauacgcuaaguggcgcuguuaagaauauuauucaguucuugggauuacagccugcggaaaggacugacagaguaccggaggguaaaucuacgcacacauuacuucuugcugguguauucaggggagguauugacauacuaguaagagcgaaacuagcuuugggcgaauguguuacgaugcaacuaacagucaggucgccagauccugacguugcugagcuuauaacuucaacuguagguuaa

SEQ ID NO: 157 - RNA, 651 nt, Diabrotica virgifera
auggcggcaaacagaacuggaccugcucagagaccaaauggcgcuacccaaggaaagauaugucaguucaaacugguccuacuaggcgaaagugccgucgguaagucgaguuugguacugagguucgucaaaggacaguuccacgaauaccaggagaguaccauaggagcagcuuuccuuacacaaaccauaugccucgacgauacaacuguuaaauuugaaauuugggacacagcgggucaagaaagguaccacaguuuagcuccuauguacuauaggggcgcacaggcagcuauagucgucuacgacauaaccaaucaagacacauucggcagggcgaaaacgugggugaaggaacuucaaaggcaggccaguccgacgaucgugauagcuuuggccggcaacaagcaagauuuggccaacaaacguaugguagaauacgaagaggcgcagacguaugcugacgaaaacggcuuacuuuuuauggaaacuuccgcaaagacggcaaugaacgucaacgauauauuuuuagcaauagcuaagaaacugcccaagaaugaacaaaccacaggucaaggcggcagugcccaaggcaggcggcuagcggagggcgauucgggcgccaaggcacccggaaauuguugcaaguga

SEQ ID NO: 158 - RNA, 279 nt, Diabrotica virgifera
augaaguuuuuaagaucgacagugugcuacauugccaucuuggcaauucucuuuacccucugugccgaugagguugaaggaaggagaaaaauuuugauggggcgaaaaagcauuaccaggacauaucuucguggaaaugcuguuccugcguaugugauaauaauccuuguaggaauuggucaaaucauccugggagggauauuguacguugcauugaggaagaagaucauugcugcaccuguaacggcaucauaugcaguggcuagacaagaaccauaa

SEQ ID NO: 159 - RNA, 474 nt, Diabrotica virgifera
augcagaucuucguuaaaaccuuaacggguaagaccaucacucuugaggucgagcccucagauacuaucgaaaaugugaaagcuaaaauccaggauaaagaaggaauucccccagaccagcaacgucucaucuucgcuggaaaacaacucgaagauggucguaccuugucugacuauaauauucaaaaagaaucaacccuucacuugguguugagauugagaggaggugcuaagaaacguaagaagaagaauuacuccacccccaagaaaaucaagcacaagaagaagaagguuaaguuagcuguauugaaauuuuauaagguugacgaaaaugguaaaauccaccgauugagacgugaaugccccgcugaacaauguggagcuggugucuucauggcagccauggaagacaggcauuacuguggcaagugcgguuacacucuugucuucuccaaaccaggagaugagaaauag

SEQ ID NO: 160 - RNA, 747 nt, Diabrotica virgifera
augauguccaaagcagacacacaggaagaugccuccuucgccaaauuggaaaaucagauugcuaucaucaaauacguaauacucuuuaccaacguuuugcaaugggcucucggugcagcaaucuucgcucuuugccuuuggcuacgauucgaggagggcauucaagaauggcuccagaaauuggauucagaacaauuuuacaucggaguauauguacuuauagucgcuucacugaucgucaugauuguguccuuuauaggauguauuagugcccugcaggagaguaccauggcccuuuuaguguacaucggcacccaagugcucaguuuuauauucgguuuauccgguucggcgguucuucuggauaacagcgccagagauucccacuuccaaccgaggauccgagagaguaugcgacgucuuaucaugaaugcucaucacgaccaauccagacaaacacuagccaugauucaggaaaauguugguugcugcggagcugauggcgcaacagacuaccucucucuucagcagccccuuccaagucagugcagagacaccguuacuggaaacccauucuuccacggauguguagaugaacucaccugguucuucgaagaaaaaugugguuggauagcagguuuagcuauggcgauaugcaugauuaacguccuuaguauuguuuuaucuacgguacucauccaggcauugaaaaaagaagaagaagcauccgauucauacaggagauag

SEQ ID NO: 161 - RNA, 375 nt, Diabrotica virgifera
augucuggacguggcaagggaggcaaaguaaagggaaaagcaaagucccgaucaaaucgugcugguuuacaauuuccuguaggucguauucaucguuuauugagaaaaggaaauuaugccgaaagaguuggugcuggagcuccuguauacuuggcagcuguuauggaauauuuagcugcugaaguuuuggaauuggcaggaaaugcagcuagagauaacaaaaagacccguauaauuccuagacauuuacaauuggccauaagaaaugacgaggaauugaacaaauuacugucaggaguuaccaucgcccaagguggaguauugccuaauauacaagcaguacuguuaccuaaaaaaacugaaaagaaagcuuaa

SEQ ID NO: 162 - RNA, 864 nt, Diabrotica virgifera
augaaguuggaugguguagaucugcccccaccaauuagcuucgacauugcggaagagcaaccguuaccaccuugccaacagacguucuuauguaauggugauggaggauccauagugcgacaguuucucgagcuguauuucguaauauaugauucagauaauaggcagucccuucuucaggcauaucacgaaaaagccacauuuucaaugacaauggccuacccguacggcuauuccaaagacaguaaaggaguaucgugguugaauugguaugccaccgauaauagaaauuuauuacgaguucaagauccagacagaagaaacaaguuguuaagacagggacaaguugcuguaguuucguucuugcaagauaugccgcacacgaagcacgauauucacaguuuuacaguagauuugacaguuuuuacaccccagauguuauguuugacaguggcugguauguuuaaagaauugaaaaguggccacaaaguaccuccuuuaagauauuucuucagaacccuuguaauuguaccugcuggaucagguuuuugcauagcaaaugaagaacuucacauauccaaugcaacuccggaccaagcaaaagaugcuuucaagaccaccguuaauguagcuccggcaccagccccugugauuaccucuccuggacccaguauaccacaacccgcugugccagaugaugcuacaaaacaagaaaugguaaaacagauguccgcaguauccggaaugaaucucgaguggucgcuacagugucucgaagaaacacaaugggacuaccagaaagccauaaugguauuccaaaauuuaaacgcacaagguguuguaccacaagcagcauuuauuaaa

SEQ ID NO: 163 - RNA, 2868 nt, Diabrotica virgifera
augacugcgguagaacaaccuuguuacacacuaauaaacuugccaacagauucggagcccuacaaugaaaugcaacuaaaaauggauuuagaaaagggugagguuaaaguaaaaauaagagcauuagaaaaaauaauucacaugauucuggcaggagaaagguugccgaauggauuucuaaugaccaucauaagaaacguuuuaccuuuacaagaucauuuggcaaaaaaacuauuauugauuuucugggaaauaguuccaaaaacaaauccagaagguaaacuacuacaagagaugauuuugguaugugaugccuauagaaaagaucugcaacacccaaaugaauuuuugagagguucuacacuucgcuucuugugcaaacugaaggaaccagaauuguuggaaccauuaaugcccaguauuagagcuuguuuggaucauaggcacagcuaugugaggaggaaugcuguacuggcaauuuuuaccauuuacaaaaauuuugaagcccucauuccagaugcuccugaacugaucuccaauuauuuggauggugagcaagacaugucuuguaaaagaaaugcguuuuuaaugcuucuucaugcugaccaagaaagggcguugucguauuuggcaucauguuuagaucaaguaaauucauuuggagauauucuacaacuggucaucguugaguugauauauaaggugugucauuccaauccugcggaaagaucuagauuuauuagauguauauauaacuuguugaacucaagcaguccugcugucagguacgaagcugcaggaacuuuagucacccucuccagugccccgacugccguuaaagcugcugcuagcuguuacauugaguuaauuaucaaagaaagugacaacaauguaaaacucaucguuuuggacaggcugauagcacuuaaggagcuuccuaaucacgaaagaauucugcaggauuuaguuauggacauacugagaguacucucugcuccugacuuagaaguccgcaagaagacuuuaagucuagcccuugaauuagucucuucacggaacauagaagaaaugguauuaguauuaacaaaggaagugaguaaaacgguagacagugaacaugaggauacaggaaaguacaggcaauuguuaguaaggacucuacauucguguuccauuaaguucccagauaucgcacguaguguuauaccagucuugauugaauuuuuauccgauaauaaugaacuggcugccacagauguauugcuguucuuaagggaagccauacagaaguuuaaagaauugcaaccguuaauuauugagaaacucaucgaaacuuucaaagacauuaaauuggucaaaguccauagagcagcaauuuggauuuugggagaauacgcgaguacugcuuccgauauagaaguuaucguuggagaaauuaacagauuguugggugaaggaucccucguugaagcugagcagaaguuaauagcaggagauacggaagagaaugcuccugcaccugcugcaggcgccaccacuuuaguuacuuccgauggaacauaugcuacccaaucagcuuucaacacugucagccaaaccacuaaagaagcacgaccuccucuaagacaauaccucauggauggugauuuuuucaucggagccucuuuggcaucuacauuaaccaaacugucuuugcgguaugaggaccucaccucuccugcugcuagcaauggauucaaugccaaaauuaugcuuauuauggcuggaauucuucacuugggaaaaucaggacuucccacaaaaucaauaaccaacgacgauaaagaccacauucuguucuguuuacgaguccuaucugaucguucuccaaucauuguugaaauuuucaaaaaauugugccgcucggcacuaaaugagaugcuucuagcuaaggaaucgguagaagcgaucucgcaaaagagcaaagaaaaaaacaagcguacgauucaaacugacgacgcuauaagcuuccugcaauuagagacagauaaaaguggagagcuaggagaaaacguauucgagaugucgcugucacaagcuuuaguaggaggucgaacgggagguggcgaaucaguauuaaguuccaauaaauuagauaaaaucacacaacugacugguuuuuccgauccaguuuauuccgaagcauacguucacgugaaucaguacgauaucgugcuugaugucuuaaucguaaaccaaacuaacgauacuuuacaaaacugcacgcuagagcuggcuacuuuaggcgauuugaaguugguagagaagccacaaccugucguauuggcgcccaaagacuuuugcaacauuaaagcuaacgugaaaguggccucaacugaaaacggaauuauauuuggcaacauuguguaugaugucauaggagcggggucagauaggaauguuguaguuuugaaugauauacacauagauauaauggacuauauagugccugcuaguuguacagauagcgaguuuaugagaaugugggcggaauuugaaugggaaaauaagguaaccguuaacacaccccucacggaacuuucagaauaccucgaacaucuacucaaaagcacaaauuugaaauguuuaacaucagaaaaagcucugagcgggcagugugguuuuauggcagccaauuuauaugcaaaauccauuuuuggagaagacgcuuuggccaacuuaaguauagagaaaccuuuuaauaaacccgaugcgccaguaagcggucauauuagaauaagggccaaaagucagggcauggccuuaaguuuaggagacaaagucaauaugacacagaagagcacacaacauaaaguaguagcugcauaa

SEQ ID NO: 164 - RNA, 549 nt, Diabrotica virgifera
auggguaauguguuugcaaauuuauucaaaggccucuuuggcaaaaaggaaaugaggauauugaugguaggacucgaugcagcugguaaaaccacaauuuuauauaaacuuaaauuaggagaaauuguaacaacuauuccaacaauuggauuuaauguggagacuguagaauauaagaacauuaguuuuacaguaugggauguagguggucaagauaaaauuaggccauuguggagacacuauuuccaaaacacacaaggccuaauuuucguaguagacaguaacgacagggaacguaucacugaggcuaaagaugaauuaaugcguauguuggccgaagaugaacuuagagaugccguacuucucauuuucgccaacaaacaagauuugcccaaugcaaugaacgcugcagaaaucaccgacaaacucggucuccauucacuacgcaaccgcaacugguacauucaagcuaccugugcaacuagcggagauggucucuaugaaggucuggacugguuguccaaucaauuaaagaacgccaaucgcuag

SEQ ID NO: 165 - RNA, 4425 nt, Diabrotica virgifera
augggacgguugcacuguuuauuuuguauuuuccuauguuuuaccgucaucaacacgcagacaacgaauauacauggauucucggaaaauuccguggauacauuucuaucaccucaugggaaaagugcaaaauucgugcaccaaaaucacaaacccaaaauugaaaauugucagaacuacaaacccucggugaaagaagaacagccaggcggaacguacguaacaacgguuaccgcuaucgaugacgauccuagggagggaggaggaacaauuaguuacaaacuaauucauagagaaggagaacauguuuuauuugacauagacaacguuacugguguuuugacaacuauccagccauuugaucgggaugaaccaguaaggcagaaggaacuuuauguaaccguacaagcuucagacaacggcaggccaccauuagcagaugucuguacauuuacaguuaccauuaccgacauuaaugauaaugcgccacagcuugauaaacugaaauacgaugcacaaguuucugaagauuuaaaaguaggaagugaagugaugagaguuuuugcuuacgacauugaugauggggaaaauucaagauuaucguauaacuuuucaaacgaaaaugcucaauucacccaguauuucaggauagaucgagauacuggcguuguguauuuaaaggaagcuuuaacagacaaaaagaauacuagauuuaacagugcuguuuauguagccgauaauggcguuaacgaucaagaaggccaaaaagauucaaccgcuaagauaucuauaacaguaguagggucugauaaacagccucccagauuuacucaaaaaaugccugauggaaucuuggagauccccgaagauuuuaaagacuuuucuaaacauauugucacagucgaagcaacguccaacauugcggauccacaacuugcuuuugaauuggugaagggaaagacauaucaaaccaauaaagaccaaacguuucuuuuggaggcagaaggaaauaaagcgcacauaaagcuagugcguccacuggauuaugaaacaguaacggaauauacucuaacuauucgaguaaaaaacaaagauuuaauggauucuuccauaaauauaccaauuaaaguauuagauguuaaugaugaaauuccuaauuuccuugaauuucuuaaagguagugucguggaaaaugacaagccaggugcacaagcgauucaaguaagagcaaucgauaaagacggaacugcugcuaacaacauugugagcuaugaacucguugacaauacagauuuguuugcaauaaaccgaucuacgggaguaauuacgucgagaguggaguuugaucgugaaacuguaccucuauaucacguaaacguuaaagcuuaugauaacucuccgucugcuuuguauaacacgacauugccuaacauuguaauucagacauuccaaaucaguauagaagaucaaaaugacaacaaaccuguauuuacucauccaauuuaucaguucaguaauauuacugagcuugcugauaaaucgaguauuguuggugaagucaaagcuuuagauaaugacacggcuucaguuauaaguuauaguauuacaaauggaaauauugacgaugcguuuaugauugaaaauucuaccggcagaauaagaguuaauggaaaacuggauuacgagaaaaucgaacaauacaacuuaaccguucgcgcauuugauggggcauuugaagauuuugcaauuguuuuaauuuccauacuuaaugaaaaugacgaaccuccaguuuuugacgacuauaucagagaaauucaaauuaaagaggaagaaccuaugauauccggaugcguuguuagagugacugcucaugauccagauauuaaagacaggcaugcugaucaacacauaguauaugaggucgcgaaagaacagaaagauuuuuugaccguaucugccgauggaugcguacaaguaacaaaaccucucgaccgagauccgccuuucgguagcccaacacgacaagucuucaucuaugcucgugauaaugauggaggcacaaauucauuguuggccacugcagaaauugaaauuauuuuaauagauauaaacgauaaugcucccuuuuuaaauguuacagaaauuguuuauuaugaaaaccaggauccagguuuuauagguaaccuaagugccgaugauuacgaugguccugauaauggaccuccguuugcuuuucgauuaucagacacugcuucagauaguauuagaucgaaauuuuccauuaucggaaaccagcuuuucgcuuuagaaauguuugauagagaagagcaaaaauauuaugacauugccauugacauuacagauaguggaguaccuccacuaacaggaacuaguauucuuagaguuauaaucggagauguaaaugauaauccagcuacagacggaaacagcacgaucuuuguguauaaguacgucaaugggccagaaaauuucauggaaaucggacguguauauguuacagaccuagacgauugggauuuaaaugacaaagucuuuguucaagaagauaacuuugaugaauuuguguuaaaccagcauaacaacgguaugauucugaugaaaccaacaacggcugagggaacuuaugagguucauuacagggucacugaaacccaugaacccacaauacacgaacauacaguuaaugcaauagucacgauuacaguuaaaguacuuccagaggaagcgguuguaaaaucaggaucaauucgauugagaggaacaacuaaggaagaauucauagaaaauucauugaauggaaagagcaaaagagacauauuacaccaagaacucuccaaaauauuaaauacaucuuuagcgaauguugauguauuuacuguuuuaaauucaccccaccagaauaguucguuuguggauguucgauuuucugcucauggaucuccauauuaugcuccagagaaacucgaaaacaaaguuacagaucaucaaauggagcuugaacaaaaauuagauguggaauucuacaugaucaacguaaacgagugccuuaacgaaacaacguguggagcugaaaacucauguacgaacaaauuaaacauaacacgagaaccagcuguaguguuuacuaacagaacauccuuugucgguguaaaugcauuuauugauccugugugugccgcuuuaccaagagauguuauggaauguuucaacggaggcguccuuaucgaaaacacagcguguaauuguccugcaggauuugaaggaccacauugugaaauccuagcuauaggauuuacaggaacugguugggcuauguauccauccuuugacgcuacaaacaggacugagauuauacugcauauuuuaucacaaacugauaaugguuugauauuuuacaauggaccuuuaaauauaagacaaacuucuuugucuaaagauuauauaucauuagaacuuaaagacggauauccauuacuucaaauuugcaccggcucaagcacucaagaaauuuaucugaaagagcgcauucacaaauugagcgauggaucguuacacaaaauaaaaauaggaucuggauuugacgauauaucccuggaaguagacgacuguggaacaacguguucaauuuggacuaauaaacuacauaaagguguuauccgagcaaauggcccccuucaacugggagguaugaaaaacagauucaccgaucaagaauucaaacgaauuugggaccauuugccaccgacugccacccguuucucugguuguauuagaaauuugacguauaaugaauuuuacuacaaccucggugcaccuucugaugcauuccaagcguaucccgacuguaacuaugcagugaugcaagcugugacuuucgguaucgacuccaauuucuugguugcuauucugguuuguguagcaauuuugauaauucuucuucuggcaguaguuguacauagacguaaacacgacaacuuuaacgaaaaagaaaucgaugauacucgcgaaaacauuaucaacuacgaagaugaagguggcggcgaaugugacaccaacuacgaccugucuguuuuccaucagaacaacauuguggacgaaaaaccauugaugagagacaaccccgauguaccugcagauauaaguggcuuuuuagauaacaagaaagacaacugugauaaagaccccgauaauuugccuuaugacgacguucgccauuaugccuacgagggagacggaaauagcaccggauccuuaucuucucucgcuucauguacggacgaaggagauuuaaaguucaacuacuuaucaaguuuuggacccagauucagaaaguuagccgacauguauggagaagauccaagcgaugaagacucacacgauggaaacgaagaauccuggugcuag

SEQ ID NO: 166 - RNA, 291 nt, Diabrotica virgifera
augccuuucuguggucccaaauugucccucugcggccugauuaucagugcaugggguaucauccaguuggguuucauggguguauucuauuacauuggggcuguggcuuuagcagaagauauuccagagguugaguuuaagggcgauuuagacaaauuuuauagcgacgucaacacggguuucacacagaaugcuuacaacugcuggauugcugcucuccuauaccugauaacauuagcaguaucagcucaccaauucugggccaacaacagaucaucauugaacgucuaa

SEQ ID NO: 167 - RNA, 540 nt, Diabrotica virgifera
augggucuuaccauaucagcaguguuuaauagguuguuuaguaaaaagccuaugagaauuuuaaugguaggauuagaugccgcagguaaaaccacaaucuuauacaaauugaagcuuggugaaaucguaacuacaauaccaaccaucggcuucaauguagaaaccguugaguacaagaauauaucuuucacgguaugggauguagguggccagacgagaaucagaaaacucuggagacacuauuucgccaacacugauggacucauuuuugugguugauuccaacgaccgagaccguaucgcggaagccgaagaagaauugcacaauauguuaggagaggacgauuuaagagacugcauuuuguuaauauucgccaacaaacaagauuuaccgaacucgauguccacugcugaauugaccgauaagcuuaaguugcacacuuugaagaauaggaggugguacauacaagccacaugugcuacucaagggaaugguuuguacgaaggacuagauugguugucgaaugaauuggccaaguga

SEQ ID NO: 168 - RNA, 618 nt, Diabrotica virgifera
augcgguacacuuugaguuacaucggugcuacccuagcguccacuguaacacugauuuuugcccucuacuacugccucacgggaaaaggagagcaaguuaguuuagcaugguuauuguugaaugugucuccccacaugugggcaggucuaggaauuggccuugcuguaucauuaucaguuguaggagcugcugcaggaauucacacuacaggagucaguaucguaggagcugguguuaaagcccccagaaucaaaaccaaaaauuuaauuucuauuauuuucugugaagcuguggcuaucuauggguuaauuauggcuauaguacucuguggaaguuggaagaauuucgauguagaccuauucaaccucaaaacucauaacuuugcucaaaaccauuauggaucacauguuauuuuuggauccgguuuaacuguuggauuuguaaaucuauuauguggauuuuguguuggaguaguugguucuggugcagccauuucugaugcagccaauucaucauuauucgucaaaauuuugauuauugagauuuuuggaagugccauuggucucuucggucugauuguuggaguauacuugacgucaagaggcucuaugguuuaa

SEQ ID NO: 169 - RNA, 5694 nt, Diabrotica virgifera
auggcuaccaacgauaguaaagcuccguugaggacaguuaaaagagugcaauuuggaauacuuaguccagaugaaauuagacgaaugucagucacagaagggggcauccgcuucccagaaaccauggaagcaggccgccccaaacuaugcggucuuauggaccccagacaaggugucauagacagaagcucaagaugccagacaugugccggaaauaugacagaauguccuggacauuucggacauaucgagcuggcaaaaccaguuuuccacguaggauucguaacaaaaacaauaaagaucuugagaugcguuugcuucuuuugcaguaaauuauuagucaguccaaauaauccgaaaauuaaagaaguuguaaugaaaucaaagggacagccacguaaaagauuagcuuucguuuaugaucuguguaaagguaaaaauauuugugaagguggagaugaaauggauguggguaaagaaagcgaagaucccaauaaaaaagcaggccauggugguuguggucgauaucaaccaaauaucagacgugccgguuuagauuuaacagcagaauggaaacacgucaaugaagacacacaagaaaagaaaaucgcacuaucugccgaacgugucugggaaauccuaaaacauaucacagaugaagaauguuucauucuugguauggaucccaaauuugcuagaccagauuggaugauaguaacgguacuuccuguuccuccccuagcaguacgaccugcuguaguuaugcacggaucugcaaggaaucaggaugauaucacucacaaauuggccgacauuaucaaggcgaauaacgaauuacagaagaacgagucugcaggugcagccgcucauauaaucacagaaaauauuaagauguugcaauuucacgucgccacuuuaguugacaacgauaugccgggaaugccgagagcaaugcaaaaaucuggaaaaccccuaaaagcuaucaaagcucggcugaaagguaaagaaggaaggauucgagguaaccuuaugggaaagcguguggacuuuucugcacguacugucaucacaccagaucccaauuuacguaucgaccaaguaggagugccuagaaguauugcucaaaacaugacguuuccagaaaucgucacaccuuucaauuuugacaaaauguuggaauugguacagagagguaauucucaguauccaggagcuaaguauaucaucagagacaauggagagaggauugauuuacguuuccacccaaaaccgucagauuuacauuugcagugugguuauaagguagaaagacacaucagagacggcgaucuaguaaucuucaaccgucaaccaacccuccacaagaugaguaugaugggccacagagucaaagucuuacccuggucgacguuccguaugaaucucucgugcaccucucccuacaacgccgauuuugacggcgacgaaaugaaccuccaugugccccaaaguauggaaacucgagcugaagucgaaaaccuccacaucacucccaggcaaaucauuacuccgcaagcuaaccaacccgucauggguauuguacaagauacguugacagcuguuaggaagaugacaaaaagggauguauucaucgagaaggaacaaaugaugaauauauugauguucuugccaauuugggaugguaaaaugccccguccagccauccucaaacccaaaccguuguggacaggaaaacagauauuuucccugaucauuccuggcaauguaaauaugauacguacccauucuacgcauccagacgacgaggacgacggucccuauaaauggauaucgccaggagauacgaaaguuaugguagaacauggagaauuggucauggguauauuguguaagaaaagucuuggaacaucagcagguucccugcugcauauuuguauguuggaauuaggacacgaagugugugguagauuuuaugguaacauucaaacuguaaucaacaacugguuguuguuagaaggucacagcaucgguauuggagacaccauugccgauccucagacuuacacagaaauucagagagccaucaggaaagccaaagaagauguaauagaagucauccagaaagcucacaacauggaacuggaaccgacucccgguaauacguugcgucagacuuucgaaaaucaaguaaacagaauucuaaacgacgcucgugacaaaacuggugguuccgcuaagaaaucuuugacugaauacaauaaccuaaaggcuauggucguaucgggauccaagggauccaacauuaauauuucccagguuauugcuugcgugggucaacagaacguagaagguaaacguauuccauuuggcuucagaaaacgcacguugccgcacuucaucaaggacgauuacgguccugaauccagagguuucguagaaaauucguaucuugccggucucacuccuucggaguucuauuuccacgcuaugggaggucgugaaggucuuaucgauacugcuguaaaaacugccgaaacugguuacauccagcgucgucugaucaaggcuauggagaguguaaugguacacuacgacgguaccguaagaaauucuguaggacaacuuauccaguugagauacggugaggacggacucuguggagagaugguagaguuucaauauuuagcaacggucaaauuaaguaacaaggcguuugagagaaaauucagauuugauccgaguaaugaaagguauuugagaagaguuuucaaugaagaaguuaucaagcaacugauggguucaggggaagucauuuccgaacuugagagagaaugggaacaacuccagaaagacagagaagccuuaagacaaaucuucccuagcggagaauccaaaguaguacuccccuguaauuuacaacguaugaucuggaauguacaaaaaauuuuccacauaaacaaacgagccccgacagaccuguccccguuaagaguuauccaaggcguucgagaauuacucaggaaaugcgucaucguagcuggcgaggaucgucuguccaaacaagccaacgaaaacgcaacguuacucuuccagugucuagucagaucgacccucugcaccaaaugcguuucugaagaauucaggcucagcaccgaagccuucgagugguugauaggagaaaucgagacgagguuccaacaagcccaagccaauccuggagaaauggugggcgcucuggccgcgcagucacugggagaacccgcuacucagaugacacugaacacuuuccauuuugcugguguauccuccaagaacguaacccuggguguaccuagauuaaaggaaauuauuaauauuuccaagaaacccaaggcuccaucucuaaccguguuuuuaacuggugcggcugcuagagaugcggaaaaagcgaagaauguguuaugcagacuugaacacaccacucuucguaaaguaaccgccaacaccgccaucuauuacgauccugacccacaaaauaccgucauuccugaggaucaggaguucguuaacgucuacuaugaaaugcccgauuucgauccuacccguauaucgccgugguugcuucguaucgaacuggacagaaagagaaugacagauaagaaacuaacuauggaacaaauugcugaaaagaucaacgcuggguucggggacgauuugaauuguauuuucaacgacgacaaugcugaaaaguuggugcugcguaucagaaucaugaacagcgacgauggaaaauucggagaaggugcugaugaggacguagacaaaauggaugacgacauguuuuugagaugcaucgaagcgaacaugcugagcgauaugaccuugcaagguauagaagcgauuuccaagguauacaugcacuugccacagacugacucgaaaaaaaggaucgucaucacugaaacaggcgaauuuaaggccaucgcagaauggcuauuggaaacugacgguaccagcaugaugaaaguacugucagaaagagacgucgauccggucaggacguuuucuaacgacauuugugaaauauuuucgguacuugguaucgaggcugugcguaagucuguagagaaggaaaugaacgcuguccuuucguucuacggucuguauguaaacuaucgccaucuugccuugcuuugugacguaaugacagccaaaggucacuuaauggccaucacccgucacgguaucaacagacaagacacuggagcucugaugagguguuccuucgaggaaacuguagauguauugauggacgcugccagucaugcggaggucgacccaaugagaggaguaucugaaaacauuauccucggucaacuaccaagaaugggcacaggcugcuucgaucuuuugcuggacgccgaaaaauguaaaaugggaauugccauaccucaagcgcacagcagcgaucuaauggcuucaggaauguucuuuggauuagccgcuacacccagcaguaugaguccagguggugcuaugaccccauggaaucaagcagcuacaccauacguuggcaguaucuggucuccacagaauuuaaugggcaguggaaugacaccagguggugccgcuuucuccccaucagcugcgucagaugcaucaggaaugucaccagcuuauggcgguuggucaccaacaccacaaucuccugcaaugucgccauauauggcuucuccacauggacaaucgccuuccuacaguccaucaaguccagcguuccaaccuacuucaccauccaugacgccgaccucuccuggauauucucccaguucuccugguuauucaccuaccagucucaauuacaguccaacgagucccaguuauucacccacuucucagaguuacuccccaaccucaccuaguuacucaccgacuucuccaaauuauucaccuacuuccccaagcuacaguccaacauccccuaacuauucaccaacaucucccaacuauucacccacuucaccuaguuauccuucaacuucgccagguuacagccccacuucacgcagcuacucacccacaucuccuaguuacucaggaacuucgcccucuuauucaccaacuucgccaaguuacuccccuacuucuccuaguuauucgccgucgucuccuaauuacucucccacuucuccaaauuacagucccacuucuccuaauuacucaccguccucuccuagguacacgcccgguucuccuaguuuuuccccaaguucgaacaguuacucucccacaucuccucaauauucuccaacaucuccaaguuauucgccuucuucgcccaaauauucaccaacuucccccaauuauucgccaacaucuccaucauuuucuggaggaaguccacaauauucacccacaucaccgaaauacucuccaaccucgcccaauuacacucugucgaguccgcagcacacuccaacagguagcagucgauauucaccgucaacuucgaguuauucuccuaauucgcccaauuauucaccgacgucuccacaauacuccauccacaguacaaaauauuccccugcaaguccuacauucacacccaccaguccuaguuucucucccgcuucacccgcauauucgccucaaccuauguauucaccuucuucuccuaauuauucucccacuagucccagucaagacacugacuaa

SEQ ID NO: 170 - RNA, 876 nt, Diabrotica virgifera
augucgucaaauauucaaaaggcccagcaguugauggcggaugcagaaaagaaaguaacaucucgagguuucuucggaucucuauuugggggaucaagucguauugaagaugcaguggaauguuacacaagagcugcaaaccuuuuuaaaauggccaagagcugggaugcugccgguaaagccuuuugugaggcugcuaauuugcauuccagaacuggugcucgucaugacgcugccacuaauuauauagaugcugcaaauuguuacaaaaaagccgauguauuugaggcuguaaacugcuuuauaaaagcuauagacauuuauaccgaaaugggucgcuuuacaauggcugcaaaacaccaucagacuauugcagaaauguaugagacugaugcuguggacaucgaaagggcuguucaacacuaugaacaggcggcugauuacuucagaggagaagaaagcaaugcuuccgccaauaagugucuucuuaaaguggcucaauaugcagcccaacuugaaaacuaugaaaaagcagugggaauuuaucaagaaguggcuuaugcagcucuggaaagcucucuuuuaaaauacagugcaaaggaauacuuauucagagcugcccuuugucaccuuuguguugauguacucaaugcacaacaugcuauagaaagcuauauuucaagguaucccgcauuucaagauucccgugaauacaaacuuuugaaaacccucauagaaaacaucgaagagcaaaacguagauggauauacagaagccgucaaagauuacgauucaauuucucgucuugaucagugguauacuacaauucuuuuacguauuaagaaacaaguaagcgaaagcccugacuuacguuaa

SEQ ID NO: 171 - RNA, 609 nt, Diabrotica virgifera
augaaucccgaguaugauuauuuauucaaacuucugcugauuggagauucaggaguaggaaaaucuugucuucuacugagauuugcagaugauaccuacacagaaagcuauauuaguaccauuggcguagauuuuaaaaucaggacaaucgauuuagauggaaagacaauuaaauugcaaauuugggauacagcaggucaggaaagguuuagaacgauuacaucaaguuauuaccgaggagcacaugguauuauuguaguguacgauugcacagaccaagauucauucaauaacguuaaacaguggcucgaagaaaucgaccguuaugcgugugacaauguaaacaaauuacugguagggaauaaaagcgauuugacaacuaagaaaguugucgacuucacuacagccaaggaguaugccgaccaauuggguauaccauuuuuggaaaccucagcuaagaaugcaaccaauguagaacaggccuuuaugacuauggccgcugaaauaaaaaauagaguaggaccuccaucuucugcgguagaccaaggaaauaagguuagguucgaucaaagucgcccagucgaaacaaccaaauccgguugcugcuga

SEQ ID NO: 172 - RNA, 789 nt, Diabrotica virgifera
auggcagacgcugaugaucuauuagauuaugaagaugaggaacagacagaacaaaccgcaacugaaacggcaacuacagagguacagaaaaagggugucaagggcacauauguaucaauacacaguucuggguuuagagauuuucuguuaaaaccagcaauucucagagcuauaguggacugcggguucgaacauccuucagaaguucaacaugaauguauuccucaagcugucauuggcauggauauucugugccaagcuaaauccgguaugggaaaaacggcuguuuuuguauuagcuacacuccaaguaauagauccuacagaaaauguuguauauguucucgucaugugccauaccagagaguuagccuuccagauaagcaaagaguacgaacguuucaguaaauauaugcccaauauuaaaguaggggucuucuuugguggcuugccuauccagaaagaugaggaaacguuaaaaaauaauugcccgcauaucguuguggguacuccaggaagaauuuuagcauuggucagaucgaaaaaacuuaaucucaaacaucuaaagcauuuuauuuuggaugaaugugauaaaauguuggaguuauuagacaugagacgugauguucaagaaauauaucguaacacuccccacgaaaaacaagucaugauguucagugccaccuuaaguaaagaaauuagaccaguuugcaagaaauuuaugcaagauguaauucaaaauucuuauaauacacaauuuuguaaugacgcacccacucgcaauguuuga

SEQ ID NO: 173 - RNA, 738 nt, Diabrotica virgifera
augccggucauugaugguuauaaaguacuuuacauuuuauuacacaguuuauauacaauuuuugaaaauauuuggaggacucuuuuauuuauuuaucaaaauuguauaaggguuauaaacccugaaucuacauucgaugaugcugaccaguuaaagaaaagacugucuagacuaacaaaaaagccucaacauuuaacuaucauuauugguguggaagaauauucauugguagauuuggcuaaccucguauauugguguuuaggucuuaauauuccguacguuaguuucuaugauuauaaagguaauuuaaaaaagcaugaagagaaguugcaacaaauuguagaauccagaaaaucagagaauaucaacauaauuuggcacacccaugcagaacaaaggcauaaaaauggauuuuuggguccaaaaauccacguaaaaguguuaacacacgcggacggaaagcaaaguauaguaaauguuacuaaaaaauuagcucuaaauaaagaaaaagacauuaguaaagaaaaaauuagugaauuacuauuaaggcaguaugaauuuccagauccagaaauggcuauuauuuguggaaagaaacugaacauuuauaauuauccuccuuggcaguuaagacucacagaauucuuuaaagucaacaaagucaacaacaucacauucccaguguuuguggaaaaauuggaaaaguacagcaaaugugaacagagggugggaaaauaa

SEQ ID NO: 174 - RNA, 480 nt, Diabrotica virgifera
augaccaacucuaaagguuaccgccgaggaaccagggaucuauuugcccgcaaguuuaaaaaacgugguguaauuccacuuuccacauauuugagagucuacaaaguuggagauauuguagauaucaaggguaauggugcaguucaaaaggguaugccccacaaaguguaccaugguaagacaggacguguuuucaauguuacugcacaugcauuagguguaauuguaaacaaaaggguucgaggaagaaucauccccaaaagaaucaaucuccguauugaacauguaaaccacuccaagugucgucaagacuucuugcaaagaguaaaauccaacgaaaagcuacguaaagaagcuaaagaaaagaacauuaaaguagaacuuaggagacaaccugcccaaccuaggccagcacauauuguuagcggaaagguuccagcacaggugcuugcuccuaucccauaugaauucauugcuuag

SEQ ID NO: 175 - RNA, 537 nt, Diabrotica virgifera
auggaaggaauacuacuggaaccaacauuguauaccauaaaagguauugcuauauuggacuaugaugguaauagagugcuggcuaaauacuacgauaaagauauauuuccuacagcaaaagagcagaaagcuuuugagaaaaauuuguucaauaaaacucauagggcagacgcagaaauuaucauguuggaugguuuaacuuguguguauagaaguaauguagauuuauucuuuuauguuaugggcaguucacaugaaaaugagcuaauuuuaaugaguguuuuaaauugcuuguaugacucaguaagucaaauauugaagaaaaauaugcaaaaacgagcugucuuggaaucacuagauauuguuaugcuggcuauggaugaaauuguugauggaggaauaauuauagauucugauucaaguucaguaguaucuagaauagcauuaaggacugaugauauuccauuaggagaacaaacuguagcucagguauuccaaacggccaaagaacagcugaaauggucauugcugaaauaa

SEQ ID NO: 176 - RNA, 450 nt, Diabrotica virgifera
auggcugaccaacucaccgaagaacaaauugcugaauucaaagaagcuuucucacuauucgauaaagauggugaugguacaauuacgacuaaagaauuaggaacaguaaugagaucucuaggacaaaauccaacagaggcugaauuacaggauaugaucaaugaaguagaugccgaugguaacggcacgaucgauuucccagaauuuuuaacgaugauggcacguaaaaugaaagauaccgauagugaggaagaaauucgugaagcauuccgaguguucgacaaagacggcaaugguuucaucucagcagcagaauugcgccacgucaugaccaacuugggugaaaaauugacagacgaagaagucgaugaaaugauucgggaggccgauaucgauggugauggucaagucaauuacgaagaguucgucaccaugaugacuucaaaguga

SEQ ID NO: 177 - RNA, 2013 nt, Diabrotica virgifera
augaugcaagcaaacaaucgagucccaccuauaaaguuggaaaacgauauagaucuuuacgccgaugauaucgaggauuucgcacaagaugacuuugguggugaaaauguugaucuauaugacgauguaauauccgcuccuccuggaaauaaugacaacccaggugauucaaaucaucaugcuccuccuggugcuggugaagaugguggagguaauuuuguugggucaggaggagcacccaauaauauaaauucuucuggaagaagacaucagcuguauguuggaaaucugacuugguggacaacugaucaagauauagaaaaugcagugcaugauauagggguaaccgacuuccaugaaguuaaguuuuuugaacacagagcaaauggucaauccaagggauucugugucauaucuuugggaucugagggaagcaugagacucugccuggaacuccuaucuaaaaaagagaucaauggccaaaauccccuuguuacccuucccacaaaacaagcucuuaguaacuuugaaagucagucuaaaacacgcccuucuccuacuaauaauucuaacucacguccuccccauccuaauaauaauguucauucagguccuaugcagaauuauggagguagaaugccuaugaacccuuccaugcgucccaugcccccagguaugcaaggugcuccaagaaugcaggguccaccuggauuuaauggaccaccaaacaugaaucagcaaccccccagguuccaagguaauccacaauggaauggaccuagaccuaaugguccugggcccaauaugggaaugagacccauggggccaccucauggacaacaagggcccccaagaccaccaaugcagggaccaccgcagcaagguccuccaagaggaaugccgccacaagguccaccgcagaugcguccagaauggaaucgaccaccaaugcaacaaggguacccucaaggcccgccgcauaugcaaggaccuaacauggguccaagagguccaccccaaaugggaccacccggggcgccucaacagcaaggaccagcuccgcacguaaauccagcauucuuucaacaaggaggaggaccaccgcccccaaugcaacacaugccuggaccagggcccgucaugccuccucaaggacccccgcaagguccaccacacggacccguuggaccuccacacggcccaccauuggguccagcgaauguuccgccucauggaccaccucacggauaugguccaccugcagcgaugccacagccgccauacgguggcccaccuccagaccaccgcgcugagauuccucaguuaacagagcaagaguuugaggauauaaugucccggaauagaacaguuuccaguucggcgauugggcgggccguauccgacgccgcagcuggagaauuugcaagcgccauugagacuuugguuacugcuauuucacucaucaaacaauccaaaguggcuaacgacgaucguugcaagauccuuauaaguucgcugcaagauacuuugcguggugucgaagacaaaagcuacagcuccagccgcagagaccggucaagauccagggacagaucacauagaagaacuagaagagaacgauccucgucacgguacagagacagaagcagagagagggagcgugaacgcgauagagaucgugaucgugaacgugacagauauuaugauagauacagcgaaagagaaagagaccgagaucguucaagaagcagagaaagaacagaaagggauagagaacgagauuauagagaccgggaacccgaagagacagauaaagaaaaaucuaaaguauccagagucucaagaucaagaaacaaaucuccggaaccugucgaaccuagcagcgagguaccgaaaucaucccgcuauuaugaggauagguaucgggaacgagagagagaaggucgacgagagagcgaucgcgaaagagaaagagauagaagaggggaagacagccauaggucucgacacuag

SEQ ID NO: 178 - RNA, 765 nt, Diabrotica virgifera
augaguucuauuggaacuggguacgauuuaucagcuucccaauucucuccugauggaagaguauuucaaguugaauaugcaaugaaagcaguugaaaauaguggcaccguaauaggccuccgagguacagauggcauuguauuggcugcugaaaagcucauuaugucaaaauugcaugaaccaaguacaaauaaacgaauuuucaacauugauaaacacauaggaauggcauuuucaggcuuaauagcugaugcaaggcaaaucguugagauugcuagaaaagaagcaucaaauuauagacaucaauaugguucaaauauuccucuuaaauaccuaaaugauagaguaagcauguacaugcaugcauacacuuuauacagugcuguuagaccauuugguugcagugucaucuuggccaguuaugaagauagugacccaucuauguaucugauugauccaucuggaguuagcuauggauacuuuggaugugcuacagguaaagcaaaacagucugcaaagacugaaauagaaaaauugaagauggggaaucuaacaugcaaagaacuuguuaaagaagcagccaaaaucauuuauuugguccaugaugagcugaaggauaagaauuuugaacuggaacuuucauggguaugcaaagauacgaaugguuuacauaccaaagugccugaaucaguguuugcugaugcagaaaaagcugccaaacaagcaauggaagcagauucagaaucagauacagaagauauguaa

SEQ ID NO: 179 - RNA, 744 nt, Diabrotica virgifera
auggcuucaaaagacagauugaugauuuuuccaucuagaggagcccaaaugaugaugaaauccaggcuaaagggagcccaaaagggacauaguuuauuaaagaagaaagcugaugcuuuacaaaugagauuuagaaugauuuugaacaaaauuauugagaccaaaacucucaugggugaaguaaugaaagaagcugccuuuucuuuagcugaagcaaaguuugcaacuggugacuucaaucaaguuguucuucaaaaugucaccaaggcucaaauaaaaauaagaacuaagaaagacaacguugcugguguuacuuuaccaguguuugaaugcuaccaagaugguacagauacauaugaguuggcugguuuggcuaggggaggucaacaauugacaaaacucaagaagaauuaucaaagugcuguuaaacuguugguugaauuagccucuuugcaaacuucuuuuguaacucuugaugauguaaucaaaauaacaaacagaagagucaaugccauugaacauguuaucauuccaagaauagagcguacuuuggcuuacaucauauccgaacuggacgaguuagaaagagaggaguucuauagauuaaagaagauccaggacaaaaagaagaucagcagagcaaaggccgagaaacaaaaacaagcucuucuccaagcugggcuacuuaaagagucccaggcaaacaugcuuuuggaugagggcgaugaagaucuacuuuucuag

SEQ ID NO: 180 - RNA, 4818 nt, Diabrotica virgifera
auggaggcggcucccaaguuaccgaugcucucguucgaguuaaauacuuguacagagaacguccacuuuggcccccaguuaaaacaguauauugcugcuuuuuauggugaagauccagaauccuacauuacagaaaucagcaaucuugaauccuuaagaucagcugcaguucgaccaucaacggauguaaaugguguacaacuguugaaaaaguauuucugucagcuucguuuucucaaaucuagguuucccauggaagagaaucaagaugcugcaguucuauuuucauggaaaaauaaugaauuagacauaacuucaacauccagugauaucagauaugaauuaaugguaauaauguauaacauuggagccuuacacacuuuucuuggagccaacgacucaagaaacaauccggaugguaugaaaauggcauguacucauuuucaaugugcugcaugggcuuuucaaaacguaaaagaaaaguaccaccaauucauaucaaacaucucauugguagaacugguucauuuuuuucaacaagucuguuuagcucaggcucaggaguguauauuagagaagagcauguuugacaauaggaaaccuaccaucauugcaaaaguugcuauccaagucuacaguuauuacagacagucuuuacgugucuuggaaucaguaaaugaagccuacuuuagggauaaaaccuacaaggaguggaugaaauaucuucaauucaagcugaccuacuacaaaugcaucucguuccuauuccaagggcaacaagcugaggaacaacagaaaaugggagaaaggguugcauucuaucaagcugcaugugaacagcuggacgaggcaaagaaaauugcugcuacauuaaaaaaccaacaccaccagcaagaaauaaaugagggacuagcauucacuacugaugugguugaagguaaaagaaaagcagcuaaaaaugaaaaugaguucaucuaccaugaaucagugccugauaaagaccaauugccagagguuaagggugcuucauuagucaaaggaauaccauucaguauaaaugauauagaaguuucaggaccagauauuuucucccgauuggucccaauggaggcacacgaagcagcuuccuuguacagcgagaagaaagcucagagauuaagacagaucggggaacuuauugaaaauaaagaucaaacauuggcugaauuuaugucgucaaugcagcuagaucuauugaccaagaugcaccaggcuacuggaauaccgcaggaguugauugauagagcagcggcucuaucugcuaaaccuaacgccauucaagaucuuauaagugcuaugggaaagcuaucuaauauauaccaagacguugaagcaaguuugaaugagauugauucuuuauuaaaggccgaagaacaaagugaacaaaaguaccaagaaacgauugguaaaagaccaccgagcauuuuagcuacagauuuaacuagggaagcggcaaaauacagggaggcucauacuaaagcgaacgacucaaaccaaacuuuacacagggcgaugauggcucacguggcuaaucugaaaauacuccaacaaccgcuaaagcagcugcaacaucagcugcccuuugucgaguuuccaaauccaaauaucgacgaaaaaucuuugaaagaucuggaagcgcuaguugcaaaaguagacgaaaugagaacccaaagagccaugcuaugggcucaacuucgagaaucuauucaccaagacgauauuacaaguucccuuguaacgaaacaaccaaaucagucgcuggaacagcuguuccagcaagaacuucaaaagcaucaaaaucugauuucguugauugaacaaaacaccucggcacaagaaaacauuaagagcgccuuagucgauucuuacgcuuacgcuguaaauucaagaaaauacauccaagauauacuccaaaagagaaccacaaccauaacgucacugauagcaucguucgacucuuacgaagacuuauuggcaaaagcuaacaaagggauagaguuuuacucaaaacuugaaacgaacguauccaaguuacugcaaagaauaaggaguaccugcaaaguucaacaagaagagcgagaucagaugaugucgacugcgcaagugccucaaugggagagucauacgucacuugccgcuccuaaacugaaagauuacuuggacuccaggaagaagagugcugcguauucggagccgaguguucaaccacaacagccaacuuuaaguuacucagcugcuauggaucugccuccugguauuaggccgacuccaguuggaucagaaauaacggauguaccgaaaaauauucaaggugaaccacaagguuauauuccauauaauuaccaacaaccuucuguuccugccucacagaauauugaugaagagacuauuaaaaaaaugaacgcauugaugccaggugcuaagacgucagugccuagucaguacggauacagcaacuacauuccaccaacauacccucaaagugcguaccaaccagguaaucagucuuacggaaaagaaacuccagauauuaacucaccguacgacccuaccaaggcguucacggcuacuacuaacgcuuaucguucggugcagagcuccucaacucaaggauacguaccguacgcagaaucuaacguuucgaauguugacagaguuggauauccuagcagguaucaguaccaacaaguaccugagauagcuacuacuccagcugaucccaauauuaaugcguacuacccacauggguacucaccgagccagaauuuaccgaaugcuaauacucaacauauuaccggccaacugaaguaccauucgguggaguacgcuucuucugugccgaacaacaucaauuauaacagcucuaccuacucgucgccgcuuucuaauaugucuaguaccaauuccucaaauccuaguaacuugaauaauucuuacgaguacuacuaugacccgaauaccaguaguggugcaguaccgaaugcuucaaagccucaacagucgagcgccagcucugcaaacccgaguaccgcuaugaacaacuacaauuauuacuacaauacaaguaccagcgguaguguagcagcggauacuucaaaaauacaacaacaacaacaguacccagguacucagaugagucaagcgcaguacuaucccgccaaugccaguuauuacucaaccaguacuuacaauaccaacguccaaggugguaccaaucccucguacgcaacuggacaaacauauaaucaagugacaccagugaccucucaaaauguuucucaaaauuacaacuuuaaccaaguugguucuggagcaggacaccagcaucaguacuacucguccgcuaacgccgcaguaccaucccaacaagcuguaaauaacaguucauuaccaaacuacggauacgaucaguauuacggcaacaacuauaauuccagucaaccgaguaccuacagcgcaaaccaagcaccuccugcagcacaagcugcuccaaguaauauuccugcugccaccaaauccuccucuaauguggaucugcucaguggcuuggacuucagcauaagccaagcuccucuagugccucaacaaaacauuacgauaaaaccccaagaaaaggaaacaaaaccaccggcuguuucuucugaaaccaaaaaccaagauccaacaccaguaaccacgcccaaacaacccacuggaccagaaguaaagcgcuuguacgucaaaauccugccgagcaaacccuuaaacaacgaugaugugaagaaauuguucggccaagagcuggacagguaugagaaguucguggagaccuugacccacaaaacuuugagcgguccgaccacucuggauauuaaauggaaggagauccaagaccagcaggauugcgagccgcagaagaagaucauuuccgucgcuagauguuauccuaugaagaauagguucccggauaucuugccuuacgacuuuuccaggguggaguugugcgauaguaaagaugauuauaucaacgcuucauacauuaaggauaucucgccauaugcuccgucauuuauuguuacacaagugccguugucuucaacuguuggugauauguggacgaugauuagagaacaacaggucgaacugauccucuguuugguaaacgacaaugagaucggugaagauauuuacuggcccaaagaaaaaggcaguagucuuaacauacuuaacauggucauaacguugcaaaacguuauaguuaagucucauuggacugaaagacugauagcgauaaacuuaccugaaaaacgggagucccgugugauaaugcaucuacaauuuacaucguggccuggcagcuuguuuccaacaaauccugaaccguucgucagcuacaccuuggaauccaucaaccuauaccaacaacagaagaccaacacccauccgguggugguccauuguucaucuggcauaggaagaagcggccugcucuguuuacugacagcugcuauguucgaugcugccaacaaugcuaacucgauaccagaucuuacagcuuugaguaucaaguuguccaauugcaggaagaauauucucagagaucgagagcauuugaaguuugguuacgaaaguuuuuuggcguauauuaggcauauaguuugugaagauaaagccagaaagaaacugaacgagauccagcccaagguuaaggaggaaccacuggaaccaccugucauaguuccagaaccaaauauagauccuuuaaguacuuuagacccauuuugggcuaguaaaagauaa

SEQ ID NO: 181 - RNA, 888 nt, Diabrotica virgifera
auggcggacgaugagagaaagaaacuggaggaggaaaagaagaggaaacaggccgaaauugaacgcaaaagggccgaggucagggcucguauggaagaggccucaaaagccaagaaggccaagaaagguuucaugaccccugagagaaagaagaaacuuagguuacuguugagaaagaaagccgccgaagaauuaaagaaagaacaagaacgcaaagcagccgaaaggaggcguaucauugaagaaaggugcgguaaacccaaacuugucgaugacgcaaaugaaggcccauuaaaacaaguaugugagggauaucacagacguauuguagaccuagaaaauaagaaauuugaccucgaaaaagaaguggaauucagagauuuucagaucuccgaauugaacagccaaguaaacgaccuuagaggcaaauucgucaaaccaaccuugaagaagguauccaaauacgaaaacaaauucgccaaacuucaaaagaaggcagcugaauuuaacuuccguaaccaacucaaaguugucaagaagaaagaauucaccuuagaagaagaagacaaagaaaagaaaccagacuggucaaagaagggagacgaaaagaagguacaagaggcugaagcaugauuuuucuccuuuguuaaagcccuuuugucaacaucaagggauaugucguuauuucgaugaucccaucgugauuucgauaucuuaaauauauuuauuuuauucauuacuuuccagacuaaaagagugucuguccgcauguauauuauuuguuuauguauaacuuauuaaaaaaugugaaguauuguaaaaaaaaaaaaaaaaaaaaaaaaaaaaaaaaaaaaaaaaaaaaaaaaaagaaaaaaaaaaaaaaaaaaa

SEQ ID NO: 182 - RNA, 791 nt, Diabrotica virgifera
ccgugaucucgagcgguuuuuaacagagagggaaaauguaaucauauauaugguugaauucuugaagguuagacuucauuccagucuugugauauuuagugcuuacuugguacagcaguuucagugcugugcuuuagaauaauuuauuuuuuaacauuuauauagaaaucaaauacuaaccaaucaacaugugugaagaagaaguugccgcuuuagucguagacaauggauccgguaugugcaaagcugguuuugcuggggaugaugcaccucgugcuguauucccuucaauuguuggacgcccaagacaucagggugugaugguaggaaugggacaaaaagauuccuauguaggugaugaagcucaaaguaaaagagguauccuuaccuuaaaauaccccaucgagcacggaauagucacaaacugggaugauauggagaaaauuuggcaucauacauucuacaaugaacucagaguagccccagaagaacacccuguucuguugacagaagcuccucucaaccccaaggccaacagggaaaagaugacacaaauaauguuugaaacuuucaacaccccagccauguauguugccauccaggcuguacucuccuuguaugcaucuggucguacaacugguauuguguuggauucuggugaugguguaucccacacugucccaaucuaugaagguuaugcucuuccucaugcaauccuucguuuggacuuagcugguagagacuugacugauuaccucaugaaaauuuugacugaacguggcuacucuuuc

SEQ ID NO: 183 - RNA, 2927 nt, Diabrotica virgifera
uaauuuuugacaguucgaaaauggugauguguuuauaauucgugucaauuuagugaaauagcauucaauuuuuuguauaagaucucuucaaaaugccacuucgauuagauauaaaaagaaagcuaacagcucgcucagaccggguaaaauguguggaucuucacccuacagaaccuuggaugcuguguucucuuuacagcggaaauauaaacguuuggaacaccgaaaaucagcaacugguuaagacuuuugaaguaugugauguaccuguucggacagcuaaguuuuugcccaggaagaacuggauagucagugggucugaugauaugcagauucgaguuuucaauuacaauaccuuagaucggguacauucuuuugaggcucauucggauuaugugagauguauugucguacacccuacacaaccuuauauauuaacaaguagugaugauaugcuuaucaagcuuuggaauugggaaaaagcaugggcuugucagcaaguuuucgaaggacacacucauuauauuaugcaaaucgccauaaauccaaaagacaacaacacauuugccagugcaucccuagauagaacauugaaaguauggcaauugggagcguccacagcgaauuucacacuagaaggucaugagaaaggcguuaacuguguggacuauuaucacgguggagauaaaccuuauuuaaucucaggcgcugaugauagauuaguaaaaaucugggauuaucaaaacaaaacuuguguucaaacuuuggaaggacaugcucaaaauguaaccgcugcauguuuccauccagaacuuccuguagcucuuacuggaagugaagaugguacugucagaguguggcaugccaacacccauagguuagaaaguagcuuaaauuauggcuuugaaagaguauggacuauuuucugccuaaagggauccaauaacguggcauuggguuaugaugaagguagcauuuugguuaaaguugguagagaagaaccagcuguuaguauggaugccaguggaggcaaaauuauuugggccagacacucugaacuucaacaggcaaaucucaaggcguuagcugaaggugcggaaauaagagauggagaacgccuuccaguuucuguaaaagauaugggugcuugcgagauauacccucagacaauucaacacaaucccaauggccguuuuguuguugucuguggggauggagaauacauaaucuacacagcaauggcuuuaagaaacaaagcguuugguagcgcacaagaauuugugugggcucaagauuccagcgaauaugccaucagagaauccggaucuacuaucagaauuuuuaagaauuucaaagagaagaagaauuuuaaguccgauuuuggagcugaagguauauacgguggauaccuuuugggagucaaaucgguuucugguuugacuuucuaugauugggaaacucucgauuuagucagaagaaucgagauacaaccaaaagcaguuuacuggucagauagugguaaauuaguauguuuggccacagaagauagcuacuuuauucuuucuuaugauucugaugaaguucaaaaagccagagauaacaaucagguugcggaugauggaguagaaucggcuuucaaucuucuaggugaaauaaacgaaucagugcgaacuggucucuggguaggcgacuguuuuaucuacacgaauucuguuaaucguaucaacuacuucguuggaggugaacugguuacaauugcucauuuggaccggccuuuguaugucuugggauaugugccuaaagacgauagauuauaccucguagauaaagaguugcgcguaguaagcuaccaauuacuucuuucuguucuugaauaucaaacugccgucaugagaagagacuuuccaacagcagacagaguacuuccguccauuccuaaggagcacagaacgagaguggcacauuucuuagaaaagcaaggcuucaaacagcaagcuuuggccguaaguacagauccagagcacagauucgagcuggcaguagcauuagaggaucuuaauauagccaaaacucuagcucaagaagcgaacaguccgcaaaaguggaaucaacuagcagaauuggcagcugcuacuaauaauguaagcguagccaaggaauguaugcaaaaagcgcaagauuauggaggcuuguugcuucuugcuacgagcuccggugaugaaaauuuaguccguacucuaggagaaacgacacaagcugaaagcaaacauaacuuagcauuuuugucacacuuguuaguaggugauuuaaacaaaugucuagacauucuuauuaauaccgguagauugccagaagcugcauuuuucgccagaucuuaccuuccugauaagauuacagaagucguggaacuguggaagacucaguuaucuucagucaaucaaaaagcuggacagagccuugccgauccuaaaaacuacgaaaaucuguucccugguuuacaagaggcggugguagcucagaaauuuuuggaacagcagaauaaagguuuagcgcccgcaagaguugccaccaccauuccuccuaaucacgacaggaauguuguagccgaaguucaagcacaaucgaaacacgauguaccaucauuuaguucuucguuuauuucaucagaaauagaagcacaaacaaggaguucugcuaaaccugaagaaucuucaaacauuauacagcuggaccaagaugacgacgauaucgauuuagauuuggacgguguaaauaucgaugagaacauugacacgacggauaucaacaucgaugaugauuugcugagugauugaaaauaacuuuuuuacuuuaguauuaaaucuguauauucauuccuauucuuaagaaaaucuauaugaauuuuaauguuuuaauaguuaagaaau

SEQ ID NO: 184 - RNA, 1620 nt, Diabrotica virgifera
uucauuucgccauuuugauuauuucaauuuuagaaaacguucaauaagcagggugcagggucaagaaguaaaguguucuagaaauacagauuaaauuguuuccuuuguguuauugaaaggcaaaaauaaaauaaugcagaucuuuguaaaaacacucacugguaaaaccaucacccucgagguugaaccaucagauaccaucgagaaugucaaagcuaaaauucaagacaaagaagguauuccaccagaucaacagagauuaaucuuuagaaagcguucgaguucgauaagcaagcaggucaagaaguaaaguguucuagaaauacagauuaaauuguuuccuuuguguuauugaaaggcaaaaaucaaauaaugcagaucuuuguaaaaacacucacugguaaaaccaucacccucgagguugaaccaucagauaccaucgagaaugucaaagcuaaaauucaagacaaagaagguauuccaccagaucaacagagauuaaucuuugcuggaaagcaguuagaagauggccguacucucucagacuacaacauucagaaagaaucuacacuacacuuagugcuucgucuuagaggagguaugcacaucuuuguaaaaacucucacugguaagaccaucacccuugagguugaaccaucagauaccaucgagaaugucaaagcuaaaauucaagacaaagaagguauuccaccagaucaacagagauuaaucuuugcuggaaagcaguuggaagauggccguacucucucagacuacaacauucaaaaagagucuacccuccauuugguacuucgucuuagaggagguaugcagauuuuuguuaaaacuuuaacuggaaagaccaucacccuugaaguagaaccuucugauaccaucgaaaaugucaaagccaaaauucaagacaaagaagguauuccaccagaucaacaaagauuaaucuuugccggaaagcaauuggaagauggucguacacucucagacuacaacauucaaaaggaaucuacccuccauuugguacuucgucuuagaggagguaugcaaaucuuuguaaaaacacucacugguaagaccaucacccucgagguugaaccaucagauaccaucgagaaugucaaagcuaaaauucaagacaaagaagguauuccaccagaucaacagagauuaaucuucgcuggaaagcaguuggaagauggccguacucucucagacuacaauauucagaaagagucuacccuccauuugguacuucgucuuagaggagguaugcaaaucuuuguaaaaacucucacugguaagaccaucacccucgagguugaaccaucagauaccaucgagaaugucaaagcuaaaauucaagacaaagaagguauuccaccagaucaacaaagauuaaucuuugccggaaagcaguuggaagauggccguacucucucagacuacaacauucaaaaagagucuacccuucacuugguacuucguuuaagaggaggaaauuaauaugguugaaauuaagcacauuuuuauauuuucaauaaauaaauuauaaauuauuaaaaaaaaaaaaaaaaaaaaaaaaaaaaaaaaaaaaaaaaaaaaaaa

SEQ ID NO: 185 - RNA, 2430 nt, Diabrotica virgifera
cucgaaacaaaugacugugaaugaaaagcccuauagcaacagcaacaacaaauauuugaauuuucgguaaauaacguuuaugaaaaauaauaauaauuuuaauuguuacauaagacacauaagaguacauaagauuguauuauggaagaacgagauuuaguuucuaauagacgcagaucauugcauaacuauggcgaagagaaaccuguuugucgaaaauuuccggauaaugaugaacaaaauuuccaauauccuccagauuauauccacaaaguaaauacagaaacggaaaaauggaaugcucaccucaguaacaucuuagucgaccaacagagguacaaagaaaaaauacgugaacuuaaaacuguaguguacaaugaaaacguuuugucacaugaucagcaggaauuuuuaaaaucuauagacuuuaauacauacuugagacaaacugaaauauuuuguaaaaaggugcauuuagccgcagaacuauacaguuucaauaaaagugaaaaauaucaagaguuacagaaaaccauugaacauguucaagaaaucauugauaguaaacugaagacauuuaaaggucgcuguaccaccaaaccaaaaaaccauaaaucaugugugacgacgauguagcggcucuugucgucgacaauggcuccggaaugugcaaagccgguuucgccggugaugacgccccucgugcugucuuuccauccaucguaggucgucccagacaccaaggugucaugguggguaugggucaaaaagacuccuacguaggagacgaagcccaaagcaaaagagguauccucaccuuaaaauaccccauugaacacggaauuaucacuaacugggacgauauggaaaagaucuggcaucacaccuucuacaaugaacuuagaguagcccccgaagaacaucccauucuuuugacugaagcuccacuuaacccaaaagccaacagagaaaagaugacucaaaucauguuugaaacuuucaauaccccugccauguauguugccauucaagcuguauugucucuguacgcuuccggucguaccacugguauuguacuugauucuggagaugguguaucccacacaguacccaucuaugaagguuacgcucucccacacgccaucuugcguuuggacuuggccgguagagacuugacugacuaccuuaugaagaucuuaaccgaaagagguuacucuuucaccaccacagcugaaagagaaauaguucgugacaucaaggaaaaauugugcuauguagcuuuggacuucgaacaggaaauggccacagcagccagcuccaccuccuuagaaaagaguuaugaacuuccugacggucaagucaucaccauugguaaugaaagguuccguugcccugaagcucucuuccaaccuuccuucuuggguauggaaucuugcgguauccacgaaacugucuacaacuccaucaugaagugcgaugucgacauccguaaagacuuguacgccaacacuguccuuucuggagguaccacaauguacccugguauugccgaucguaugcaaaaggaaaucacugccuuggcuccaucaaccaucaaaaucaagaucaucgcucccccagaaagaaaguacuccguuuggaucgguggcuccaucuuggccucccucuccaccuuccaacagauguggaucuccaaacaagaauacgacgaauccggcccuggaauuguucaccgcaaaugcuucuaaacuacuuuauauauuuaucguauacauauuaaguacaauacugagaguuggagcaugaauguauguuuuuauuuaugguuauauauaugaugacuuguugauauuguaacaauaaauucauuuuguauuacucugguaauauuuuauuuaugagaacaaccagauugaagucguaaagagccaauaacaaccugaagauaucaauugucaauugcuacugaguaauaguuugagguacuuagcuccagcuccuuuucacacgaaaguaagaaguaucugagcgagaauacauucuguauuguacuuuuuaaauaugcgacuuuuguaacaucaauuucauuguaaaauaucaucaucauuguuuuuauggaccuacgugacaguaggagacaccugacaagacuucuuuuccugcuguguauacgcaccuuuacaaacauccugcuggccuaauuguaguccuguaagggacauccuuuguugggcauggaguuuguuugugggaauuguauugacuacuauuauauaccuacuuuuauuauuaaggcauuugaaaucguaaacuaaaauugguuguuuauauuuuauaugaguauuuuuaguaguagauaagauuucaauugcaaaacuaccuauguauguauucauuagaaauaaauucuuauuccaaaauaaaguuuug

SEQ ID NO: 186 - RNA, 2822 nt, Diabrotica virgifera
guuuauuuuggucgucggcugaugugacguguaaagaaauuaaaucaaauuauuuuaaaguuuuuaaauuaaaauggguacuuuuaaaagagauacucaugaugaggacgggggaucaagugcuuuucaaaaucuggagaaaacuacuguuuugcaggaagcuagaguuuuuaaugaaacuaguguaaauccaagaaaauguacaccgauacuaacaaaacuguuguacuuauugaaccagggugaaacuuuaagugccaaagaggccacagauguuuucuuugccaugaccaaacuguuccaaucaaaagauguaauauugagaaggaugguuuauuugggaauuaaagaacucaguucuguugcugaugaugucauuauuguaacauccagucuuacaaaagauaugacugguaaagaagacauguacagagcagcugcuauaagagcauuaugcaguauuacugaugcuacuaugcuucaagcuauagaacguuauaugaagcaagcuauuguagauagaaacgcagcugucaguucagcagcacuaauuaguucauuacauaugagcaaauuagcuccagauguaguaaaaagauggguaaaugaagcucaggaagcaguaaauagugauaaugcaaugguacaguaucacgcauuaggucuucuauaccauauuaggaagacugauaagcuagcagugacaaaauugauuuccaagcugaauucaauggguuuaaagagcccuuaugcuuuguguauguugauaagaaucacugcaaaacuuuuagaagaagaggaccaagagucacuccucaacuccccauauacaauaauauuuacaaugggcuuaaggaacaaaucugaaauggugguguaugaagcugcacaugccaugguuaaccugaaguucacgaguaguaaugugcuagcacccgcuauaaguguucuacaacuauuuuguggaucuccuaaagccacacucagauuugcugcuguuagaacuuuaaaucaaguggccaccacccacccugcgucagugacagcuuguaauuuggaucuagaaaauuugauuacugauccuaauaggucaauugcuacacuggccauuacuacucuuuugaaaacaggugccgaaucuucuguugacagacuaaugaaacaaaucgcuacuuuuguaucugaaaucagugaugaauuuaaagugguugucauucaggcaauuaagguauuagcuuugaaauuuccaaggaaacauagcacgcuuaugaauuuccuauccgccauguuaagagaugagggagguuuagaauauaaagcauccauagcagauaccauuauaacccuaaucgaagauaaucccgaagcuaaagaaucugguuuggcgcaucuuugcgaguucauugaagacugugaacauguuucuuuggcugugagaaucuugcauuuguuaggaaaggaaggacccaagaccaaacaaccaucgagauacauccguuuuaucuacaaucgcgucauauuggaauguccuucuguaagagcugcugcagucuccgccauggcacaauucggagccucuugucccgauuuguuagaaaauauccaaauauuacuuucgaggugucagauggauucagacgaugaaguuagggacagagcuacauauuauaguaauauacuuaacaaaaaugauaaaaguuuauacaacaauuacauuuuggauucuuugcagguuucaauuccuucacuagaaagaucgcuuagagaauacauucaaaauccaacugacgaaccauuugacauuaaguccguaccuguagcagcagugccaacagcagaagaacgagaaguuaaaaacaaaucugaaggacugcuagucucucaagguccaguccgaccuccuccggugucuagagaagaaaacuucgccgaaaaacuuaguaacguuccggguauacaacaguuaggaccuuuguucaaaacuuccgacgucguugaacucacugaaucugaaacagaguauuuuguccgcuguaucaagcacuguuucaaacaucacaucguccuccaauucgauugucugaauaccuugccagaccagcuuuuagaaaacguuagaguggagauagacgccggugaaaccuucgaaauuuuggcagaaauaccuugugaaaaguugcacuauaacgaaaccgguaccacauauguaguaguuaaguugccugaugaugaucuccccaacucuguugguacguguggagccguguugaaguucuuagugaaagauugugauccaucaacgggaauaccagauucugaugaggguuacgaugaugaauauacacuggaagacaucgaaauaacauuaggggaccaaauucaaaaaguaagcaaaguaaauugggcugcagccugggaagaagcugcagcuacuuauguagaaaaagaggauacauacuccuugaccaucaauacgcuaaguggcgcuguuaagaauauuauucaguucuugggauuacagccugcggaaaggacugacagaguaccggaggguaaaucuacgcacacauuacuucuugcugguguauucaggggagguauugacauacuaguaagagcgaaacuagcuuugggcgaauguguuacgaugcaacuaacagucaggucgccagauccugacguugcugagcuuauaacuucaacuguagguuaaguuuaaaggcuacguuaaugauuauauuguauuacaauuuuuccauauguauaaauauuuugauuuauuuaaauuuuauuagaaauuaaacaauuuuaaguaaaaaaaa

SEQ ID NO: 187 - RNA, 3701 nt, Diabrotica virgifera
gucguuuaguagaagugucauuuuugucugcucucguuuucaucuuuuguguauaaaauuggugcuaagguagauaaacuauauucgaauaggcguuuuuaugucgcaagaaaguguuuuguauauuugugauacgugaucucguagagggaguccagaaauucauaauuuauaguuaaguaaaaaauggcggcaaacagaacuggaccugcucagagaccaaauggcgcuacccaaggaaagauaugucaguucaaacugguccuacuaggcgaaagugccgucgguaagucgaguuugguacugagguucgucaaaggacaguuccacgaauaccaggagaguaccauaggagcagcuuuccuuacacaaaccauaugccucgacgauacaacuguuaaauuugaaauuugggacacagcgggucaagaaagguaccacaguuuagcuccuauguacuauaggggcgcacaggcagcuauagucgucuacgacauaaccaaucaagacacauucggcagggcgaaaacgugggugaaggaacuucaaaggcaggccaguccgacgaucgugauagcuuuggccggcaacaagcaagauuuggccaacaaacguaugguagaauacgaagaggcgcagacguaugcugacgaaaacggcuuacuuuuuauggaaacuuccgcaaagacggcaaugaacgucaacgauauauuuuuagcaauagcuaagaaacugcccaagaaugaacaaaccacaggucaaggcggcagugcccaaggcaggcggcuagcggagggcgauucgggcgccaaggcacccggaaauuguugcaagugaugguauacgccugcaggucgaguguuguuauuaaaccgucacgagaaaggacuggcaagugcagcggcacucuagugauaucuauguguaauaaagguccuucuauuaacaaaaaaaaauuaauaaaaaaauauauuaaacuucauauacacugucacauauuccauuuagaugaugaaaaacaaaagagcagaagcauuuuggucucuaacggucauguugaguuggaaugucucguggggcauuuaaauuugugauaauuguaccuauauuuuguuuuuuuuauauauauaauuaauauaucugacaguguaaguuaagcguaaacuguuuauaucgaucguauuagcagcaccaauuaaaaaaauaaauaaaauugaagaucuuuuuuauuguuuuuguaauuuuaacucuuuggggaagguuacaaaagaauugauaacguuguguugaaaacauugcauuauaauaaaguaauuccacccacuuacgaauuauuuugaaaggagaaucaaaaaugugucaauugucaccugucaucuuaugaugacacucuaugagagugggggcaauugcagcgcgcgcauacuauucagucuagcuucauuaugucaauuaaaugucgauguuuaaaauuucaucgauuaguuugacaguucccaaaugaaaaaacaguuacuuccgcauaaaaauguauugcuucaaaacuuacuuucaguggcauuucaguggguuuuagccaucuuauggagaguggucuaacacacuuucuagguacagcugugguuuuuaaaaggaaauauaaugaaucgcuuuuguuuucgaaauuuacauugggaaucccuuaguguccuuauauuugcccuacagaguuucauuuaaacugaaauuggguaauuuacauagaccuaaagcuuucacgucuauauagccuaauuagaccacaaaauugacuugcuuuacgugaaauguaugaaccauucaaacauauuuauaugacaacaauauaauauaauacaauauaauauaaauaacugacaacauuuaaaauuagaauuuuuacccacaauuuuucucugccaugugucaucuaguacaagaaguauggcaauuuagcccuacuccucuuauuguacauuucuuguaauuccucauuuucuuuuucaauuacuucgaucuuuuaaacuuaauucaccaaguuuauuugcaauauuguucuugaagucuauaguuugaauuccuucaauauauuuguaauguuuuucuucagugucaauccuugcauuccaugaaagaacacgaaaaagaugcagcacuuuauuuguccauauuccugcuacauaguuauuuuucgauuaacacauucacugccagcguauaguaaacuggcacuuuacuauacgcuaaacaaaaauuuggccuugcagauuuuccuaaaacacguagcagcuacgccacugaauggacuuaggacccccuaucguuucgcugguugcaauaguccgguaacuagagaagcaauuauuauauaaaaguaaauuuaaauaauuguauuuugcuugcaguacugcauuuuaauaauuaguuuucuuuacuacauacaauuguuaccuuuuaauaacauaaucuaaaucuuacuuuuuuuuuuuuauuuuuuugggcuauggccuugacaauuauccaguaaccaggacuaauauaauuggccaauauaauuaaaagugcgaauaauaguacagagcguagaaauaggggucgcuuugccgaacuugcacggucccaauaguaaacuggcacuuuacuauacgcuaaacaaaaauuuggccuugcauauuuuccuaaaacacguagcagcuacgccacugaauggacuuaggacccccuaucguuucgcugguugcaauaguccgguaacuagagacaaaagugggucauuuugcacacuucauauaauucucguuuucuguacuucacgaguauuuuuuuugucggauauguauugaauaguaucggugacaacacacugcccugcgugacaccccuuucaaaaccuaugugggaacaauauguaucuuuagagaacuuuuuguacccuuccccuaaaaacuaaauauuuuuucacuuagugcaauuuuaauauuagucucaccuuauuucuagaauacggucggucuaaauguauaaucucaacuuucagcuuauacuucgaaaaccgagaaguauaaacuguaagaauauuuaacguuauauguauuuuauuaggauaaugauuguugaaaguauguuucccaacacguguaaguuacauuucguacucuuuccauuuuuauuacaaaaaaaaauguuuauuuagauaaacuguugcggaacauacuuucucgaugcaugacugaaaagaacguuaacauuuauacguauuuguuuuuauuuugugucugaugugacaacccagaucuuagcgaaagcguagaggacaaaagaugaguuuuuaaguuucccauugaacuuuuuccguccuuaaaucaaauacaacaacuauucacuuaaguuuucuaaacauuuuugcuaauaugggccccugcaccauucccgacuuaacagucuucauuuguuuuuauuagguuuguucguaguacgauccaaacgaucggcaaccguugccaaccauuagacgcaugcgcaguuaacagugagugaucguagacuacgaacacgcaugcgucugaugguuggcaacgguugcugaucguucuacgaacaaaccuauuauaaaccgccucuuuuguagguaaaguaaaccuuauaaucauuuuccgagucuacaauuucuguaggacaucaagcauuguaaaguuuaaugaaau

SEQ ID NO: 188 - RNA, 671 nt, Diabrotica virgifera
cugcgauauagguguguauuucagcuggaauuuguaaugaaaaaaacguagaaauauauacuacaaugaaguuuuuaagaucgacagugugcuacauugccaucuuggcaauucucuuuacccucugugccgaugagguugaaggaaggagaaaaauuuugauggggcgaaaaagcauuaccaggacauaucuucguggaaaugcuguuccugcguaugugauaauaauccuuguaggaauuggucaaaucauccugggagggauauuguacguugcauugaggaagaagaucauugcugcaccuguaacggcaucauaugcaguggcuagacaagaaccauaaauuuuauuugucuagaauauuauuuucuaaauaugcaucuuuuuuaaauuauugucuacguaaauaauaagucuagaaauauauaaaaauuguauaaaaucauguaccuauauuuuucaauuuuuauaaaaaacaacccgaaauuuaauauuuuacugaauuaacauuaucauuucuaucuacacucaccggcacaaaauuccgucacccaaaauuuuugauuaagcuugacaauuuauaacuauauuauuugugcuccgauuuucaacuucauguugugcaucaguuuguagguacauguauugauauuguuugguauuauuccgg

SEQ ID NO: 189 - RNA, 693 nt, Diabrotica virgifera
guagucgguauguauuugaauuuaucuuaauuuguuuaauauuaguaguuaaauauuaaacuauaguuagaaguuguuauauaguggaccaguaguugacuccccaaaaugcagaucuucguuaaaaccuuaacggguaagaccaucacucuugaggucgagcccucagauacuaucgaaaaugugaaagcuaaaauccaggauaaagaaggaauucccccagaccagcaacgucucaucuucgcuggaaaacaacucgaagauggucguaccuugucugacuauaauauucaaaaagaaucaacccuucacuugguguugagauugagaggaggugcuaagaaacguaagaagaagaauuacuccacccccaagaaaaucaagcacaagaagaagaagguuaaguuagcuguauugaaauuuuauaagguugacgaaaaugguaaaauccaccgauugagacgugaaugccccgcugaacaauguggagcuggugucuucauggcagccauggaagacaggcauuacuguggcaagugcgguuacacucuugucuucuccaaaccaggagaugagaaauagauauauguccuuguauauuguuuaagaaaaaaauagaaaaaccuuuguuuauuugaauaaaauauucgaggaagaaaaaaaaaaaaaaaaaaaaaaaaaaaaaaaaaaaaa

SEQ ID NO: 190 - RNA, 2684 nt, Diabrotica virgifera
gaauuuaauuucaaagauuuauguucaguaagcuuuguuucaaagugcgguacuaucgguuucauuuuauaucucuuuauaacggugucgcgaguuuucuugugaaaaaugauguccaaagcagacacacaggaagaugccuccuucgccaaauuggaaaaucagauugcuaucaucaaauacguaauacucuuuaccaacguuuugcaaugggcucucggugcagcaaucuucgcucuuugccuuuggcuacgauucgaggagggcauucaagaauggcuccagaaauuggauucagaacaauuuuacaucggaguauauguacuuauagucgcuucacugaucgucaugauuguguccuuuauaggauguauuagugcccugcaggagaguaccauggcccuuuuaguguacaucggcacccaagugcucaguuuuauauucgguuuauccgguucggcgguucuucuggauaacagcgccagagauucccacuuccaaccgaggauccgagagaguaugcgacgucuuaucaugaaugcucaucacgaccaauccagacaaacacuagccaugauucaggaaaauguugguugcugcggagcugauggcgcaacagacuaccucucucuucagcagccccuuccaagucagugcagagacaccguuacuggaaacccauucuuccacggauguguagaugaacucaccugguucuucgaagaaaaaugugguuggauagcagguuuagcuauggcgauaugcaugauuaacguccuuaguauuguuuuaucuacgguacucauccaggcauugaaaaaagaagaagaagcauccgauucauacaggagauagauuuagugagauagagauauaauguaguaauuagaauuuaauguaucuucaacuaaauuacuuuuucuuuagagauauaccugaaauuguaaagaacaggaaaauuaaauaagaaccaaaaacuaaagugaaccaacaauaauugaacauuccaaaauacacuuuuuuuguuaaguuaacuaaacgacauaaauuuuucauuuuuuaaguuuuuuauuguuuuuuuuaguauuauaauuuggauaagguguuuuuauauuaaguguguaauuauaaaguuuuuuuauaggacggaaccuaaauuauauagaaucauacaauaaacuauugucugcuuauugaauuuggaaaauaaacauuugguauauauuaaaaauaauaauauaugucuuaaugaggaacuaaugaaaacgucuauacauuuuugaauuuaauaccaacagauauuguaauuauuaauuuuaauuaaucaacuccaagucaacaucuggaaagcaauagaaauuaaaguaauuaacuaacuaguaacauucuagcaaccuguacaugugguuguauuacucuguuuugacauugacaaaacuagcuuugugaucaguuaucucuagcaguaauaaacucuagcuguauuuuguuuuauauauuuguccaaagaauugguuuauuuuaaagcaaauauaaugguuuaacccaggggugggcaaacuuuuuuugguaagggccauaaaauauuuuugaucuauuaccgagagccgcaauauuuguuaccuuaacauauucgaauuuuuaacuuuuuacuaauuuuguuuacguguguugggggggggggaugguuaaauuaaauaaacacaaauaaacauauucaguacgauucaaagauuauucaaaaaaauuuaaaaccaaauauugaaaaauaagccaacgguggcaaauuuuuacaggcagcucuaagaaaaaauggauuuugcaguagaucaaugcauaugaaacaaaaaauucaaaaauauguuauuagcuuaugaguuucucgagguaacgcuguugaguuuuuuaguuuuaacgauuuuugaguuuuugauaucacucaaaauaccagucaaaauaaggaaauuuuuguaaaaagugugaaaaucaacauauuuauuauuguuaaccaaaacauaucucgauagaguuacuucacgaagugaccaaagaaaaucuaugaaaaauuuuagguggagcugucaaguagguaguuuuugaguuacaauguccaccgccuuugaaaaaagcaguuuugagaaaaacgcauuugguuugacaacuuuuauuucccuuuguuuuuugucugucaaaucguaaagugauguacgccggaauauguuuuugaaucguagaguaauuuauaaaagagacgagaacagcuguuguacguuucucccuacgcucaggcuacugcaaagcgagucgaagguagggauauuaaacaugcuuuacuuccgguaauuuuacuccagucaagcugaaaauuuuagagaguagucuugaaguuuauuuauuuauuuauuuauguacuuucauuuaaaauauaaaaaaaaaucaaacauuuaaaacaaaaaaaauuuucaaaccguaacccuccccucuaaacagcauucgcauuuaauuaagcaugguauuucccucaaauauauguguaucuauauauuuauuuauuuuuauuuuaucucugaaccuauuucuuuuuccuuaauauuguucugaagcuauuugcuuguaacaucuuaugcaauuuacuguuuuguuugagaaugggccacaguuugaguuugaaauuaaauuuauuu

SEQ ID NO: 191 - RNA, 458 nt, Diabrotica virgifera
gcuugaucuucaagguagaacaacgcaaguagaaaucuaaaacaugucuggacguggcaagggaggcaaaguaaagggaaaagcaaagucccgaucaaaucgugcugguuuacaauuuccuguaggucguauucaucguuuauugagaaaaggaaauuaugccgaaagaguuggugcuggagcuccuguauacuuggcagcuguuauggaauauuuagcugcugaaguuuuggaauuggcaggaaaugcagcuagagauaacaaaaagacccguauaauuccuagacauuuacaauuggccauaagaaaugacgaggaauugaacaaauuacugucaggaguuaccaucgcccaagguggaguauugccuaauauacaagcaguacuguuaccuaaaaaaacugaaaagaaagcuuaagaguuaguauuccuuuuuauccaacccggcccuuuucagg

SEQ ID NO: 192 - RNA, 2478 nt, Diabrotica virgifera
acuagguaaauauaccuuguauauuugucuauuaacgguauuauuuauauuauuuuaaagugcgcaugcguguugugacaguuuauccaauuuucuuacaauuucagguacccucgaacgcaacuaauguucuuuuagauuguuagccagauuucacacaauacguggucacgucaggccgccguauucaguuuuugauuucaaacaaacugacugcugucugcauaaaaauccaaaaaaucuuuugccaauauuguugugacauuuuauuacguauacucguaaaggcguaauaaucaacuugaaauugcaauaaaacuaaaagcuaaauaacgauuuuucuaguaauaucugucauacgaauuugaauacuggaaauagaugaaauuaguaucguauuuuuucuuaaauuuugucacccaugaauuaaaagcuucagagucaaauuagauacauuaauuuguaaugcagaaauuuaacuguaacuuccugucauggaacuugauuuugauauuugaugguacuuucuuucuauuguuacugauaaaagauuaccaauuaaaaaauauaauguucauuguauucacaugauguauuacauuuguugguacucuuuugcgacaauuucgaccaauguacauuuagauuuugagcuuuacagcaauggaacugaaauuaacguucaagauaucaauacaaauaaaaagcucaaaaucucuggacgauaagaacacuuucaucacaugccaaugcuugcuuaacuuuuuuaaauuaaauuuuuuuguuaaaaucaaugcaguaaaaguuuuuuauguaagauaucucucccuaguguggagauaaacuaaggcauauagaauaugacaguaguuauauucuauacaaaaaaaauuaaguauccaugugguggggguaaauguaugagggucaacaggaucgauacugucuguguauuaaauaaucuaugcucuuagcgaauguucccagguuaguguuauguaaucgugggccucaucggccucaacacuuuuuuuugucuacagugaaguaagaaagcgguuuccaaagugcaugaaguuggaugguguagaucugcccccaccaauuagcuucgacauugcggaagagcaaccguuaccaccuugccaacagacguucuuauguaauggugauggaggauccauagugcgacaguuucucgagcuguauuucguaauauaugauucagauaauaggcagucccuucuucaggcauaucacgaaaaagccacauuuucaaugacaauggccuacccguacggcuauuccaaagacaguaaaggaguaucgugguugaauugguaugccaccgauaauagaaauuuauuacgaguucaagauccagacagaagaaacaaguuguuaagacagggacaaguugcuguaguuucguucuugcaagauaugccgcacacgaagcacgauauucacaguuuuacaguagauuugacaguuuuuacaccccagauguuauguuugacaguggcugguauguuuaaagaauugaaaaguggccacaaaguaccuccuuuaagauauuucuucagaacccuuguaauuguaccugcuggaucagguuuuugcauagcaaaugaagaacuucacauauccaaugcaacuccggaccaagcaaaagaugcuuucaagaccaccguuaauguagcuccggcaccagccccugugauuaccucuccuggacccaguauaccacaacccgcugugccagaugaugcuacaaaacaagaaaugguaaaacagauguccgcaguauccggaaugaaucucgaguggucgcuacagugucucgaagaaacacaaugggacuaccagaaagccauaaugguauuccaaaauuuaaacgcacaagguguuguaccacaagcagcauuuauuaaaugauacgaagauuauguuaacuuugguuaauuaauugacaguuaguuauaucuuggcaaauguaaauaguaucuuaaauuauagcuaauuuuuaguuuuauuauuguuuaagguaauguuaguuuaagaugucgaauuuuaaguuuguuacauacgaaaaucaaaucgaaaaaauguuaauagucccuuagaaauaccgguagcccuuaucuuagaagaaaggugguagauuuuaaauaaaaacuggguuacuucacaaaaaaaugucuauuuuaauuaguugaucucgauaacuuaauaugauuauauaaauacuggccuaaccuaacaaaucggacugaaacuuuuaauauuaccuaaacaagcaagauccauuuagacuaaaguuugaaguuuuggaauuguauugaaauuugaacauuacauaaacgguuaauuuuauaugagaacuucuuagacaauaauacuaauuaacuauuuucaaugggaaauaagccacaauuuuaccaaaaaaaugauuuuauuaacguuucgacgcccaag

SEQ ID NO: 193 - RNA, 3274 nt, Diabrotica virgifera
caaaacgucaacaaucugacacgucuguaauguuuagccugacuuuugaguaaaauuaccgaaaaacauaauuaaaauugauuuauuaagaguacauaauaacguacgaaaaugacugcgguagaacaaccuuguuacacacuaauaaacuugccaacagauucggagcccuacaaugaaaugcaacuaaaaauggauuuagaaaagggugagguuaaaguaaaaauaagagcauuagaaaaaauaauucacaugauucuggcaggagaaagguugccgaauggauuucuaaugaccaucauaagaaacguuuuaccuuuacaagaucauuuggcaaaaaaacuauuauugauuuucugggaaauaguuccaaaaacaaauccagaagguaaacuacuacaagagaugauuuugguaugugaugccuauagaaaagaucugcaacacccaaaugaauuuuugagagguucuacacuucgcuucuugugcaaacugaaggaaccagaauuguuggaaccauuaaugcccaguauuagagcuuguuuggaucauaggcacagcuaugugaggaggaaugcuguacuggcaauuuuuaccauuuacaaaaauuuugaagcccucauuccagaugcuccugaacugaucuccaauuauuuggauggugagcaagacaugucuuguaaaagaaaugcguuuuuaaugcuucuucaugcugaccaagaaagggcguugucguauuuggcaucauguuuagaucaaguaaauucauuuggagauauucuacaacuggucaucguugaguugauauauaaggugugucauuccaauccugcggaaagaucuagauuuauuagauguauauauaacuuguugaacucaagcaguccugcugucagguacgaagcugcaggaacuuuagucacccucuccagugccccgacugccguuaaagcugcugcuagcuguuacauugaguuaauuaucaaagaaagugacaacaauguaaaacucaucguuuuggacaggcugauagcacuuaaggagcuuccuaaucacgaaagaauucugcaggauuuaguuauggacauacugagaguacucucugcuccugacuuagaaguccgcaagaagacuuuaagucuagcccuugaauuagucucuucacggaacauagaagaaaugguauuaguauuaacaaaggaagugaguaaaacgguagacagugaacaugaggauacaggaaaguacaggcaauuguuaguaaggacucuacauucguguuccauuaaguucccagauaucgcacguaguguuauaccagucuugauugaauuuuuauccgauaauaaugaacuggcugccacagauguauugcuguucuuaagggaagccauacagaaguuuaaagaauugcaaccguuaauuauugagaaacucaucgaaacuuucaaagacauuaaauuggucaaaguccauagagcagcaauuuggauuuugggagaauacgcgaguacugcuuccgauauagaaguuaucguuggagaaauuaacagauuguugggugaaggaucccucguugaagcugagcagaaguuaauagcaggagauacggaagagaaugcuccugcaccugcugcaggcgccaccacuuuaguuacuuccgauggaacauaugcuacccaaucagcuuucaacacugucagccaaaccacuaaagaagcacgaccuccucuaagacaauaccucauggauggugauuuuuucaucggagccucuuuggcaucuacauuaaccaaacugucuuugcgguaugaggaccucaccucuccugcugcuagcaauggauucaaugccaaaauuaugcuuauuauggcuggaauucuucacuugggaaaaucaggacuucccacaaaaucaauaaccaacgacgauaaagaccacauucuguucuguuuacgaguccuaucugaucguucuccaaucauuguugaaauuuucaaaaaauugugccgcucggcacuaaaugagaugcuucuagcuaaggaaucgguagaagcgaucucgcaaaagagcaaagaaaaaaacaagcguacgauucaaacugacgacgcuauaagcuuccugcaauuagagacagauaaaaguggagagcuaggagaaaacguauucgagaugucgcugucacaagcuuuaguaggaggucgaacgggagguggcgaaucaguauuaaguuccaauaaauuagauaaaaucacacaacugacugguuuuuccgauccaguuuauuccgaagcauacguucacgugaaucaguacgauaucgugcuugaugucuuaaucguaaaccaaacuaacgauacuuuacaaaacugcacgcuagagcuggcuacuuuaggcgauuugaaguugguagagaagccacaaccugucguauuggcgcccaaagacuuuugcaacauuaaagcuaacgugaaaguggccucaacugaaaacggaauuauauuuggcaacauuguguaugaugucauaggagcggggucagauaggaauguuguaguuuugaaugauauacacauagauauaauggacuauauagugccugcuaguuguacagauagcgaguuuaugagaaugugggcggaauuugaaugggaaaauaagguaaccguuaacacaccccucacggaacuuucagaauaccucgaacaucuacucaaaagcacaaauuugaaauguuuaacaucagaaaaagcucugagcgggcagugugguuuuauggcagccaauuuauaugcaaaauccauuuuuggagaagacgcuuuggccaacuuaaguauagagaaaccuuuuaauaaacccgaugcgccaguaagcggucauauuagaauaagggccaaaagucagggcauggccuuaaguuuaggagacaaagucaauaugacacagaagagcacacaacauaaaguaguagcugcauaaauaaaaacguuuuuuucuguuucaacccuuuucuucauuuuaaaucauauucuguaauuuaauuaauuuaauaucauauuacugguuacacauuguuagauuauaaauaucuuuuaaagaauaaaauuuauuuagcuuuuacaaagagcggaaagcaaucuuuaucuucuucuaauaagaucaacaucaaguuuucuggaaaauauaauauauaauuuaaagauguuuagcauuuauuagugaaauacauggcuuacuauuuugaugacaaagucaguguaauauagaaaagcag

SEQ ID NO: 194 - RNA, 3652 nt, Diabrotica virgifera
gguagaugaugaugacccuaauaaugaaaacaacucaagucuucuuuuuaaaaacugcaaaaaagaacccuacggaguccaccucugaauuagguccaaaucuuugaacaaaacuccuugcuucgucugaaagagaaguuccgagccauccagguucuccuaaaguuaaaucugguuggacuaauuccaagaaauuaaaacuuuuuaaagcccaagcuacaaugccuucguucucagauaggguuauaguacauguacuguagaccaugauuccaccuggcuucaauaauuuugcugcauuuucaaacaguuuucuuuguaauggaacgaaugacuugaucucguuuucugacgaccuauuggccaguuguggucuuuucccaagaacacuacacggugcaucuaaaaguauuuugucgaacgauuggggugcgaaugguggaccgucuauaacauuuuuggaacuuaaaguaucugaaauuauugcaguagaaucagcuugaaaacuauacacuuuggcgccgaaauccucacagcguuuuugaaguugggcaaccuucuuuggaguuuugucuauggcuauuaauauucccuuauucugcauuagcucugcuauaugaguaguuuuauucccaggagaagcacacauaucaaguacuacaucaccagguuugggauuaagauuaugaacacauacaauagaugguauauuuuguaguaaaauaucuccgacugguaauaaacuuucgcuuaucgguacacauccugaaauuguuucuguuacuucuacagcaauaccacugggcgcaauauuaucaguugcaaacaacuggugccucugcaucuuaacuaucccauuuccaaugaauauuuugaagucgucuucauauauuuucugaagucccuuuuuacacuuuuuugcaacaucggcguaaauacuaacguuuucguuuaucugacaaccugaaaccauuccuaauacuccuggggcaaauauaugagcaccccgaagaauugcugcagcacaaucagugucuacuauaauuucuuuaucaaacuuuuuaaagccugcuggacaauuuaaacugucaauuauuaucacauugguaaaagagggauguauguaaacauuugguguaucauuacaauuuucugcaaaauagguuuuuaauaccuuuaaaacuuuggcaguauuuguuuuuauuguauuuacucuuaucgaaguuauuuuuggugcagaacauaaccauugcuguauuuuuaauaauucuucauuugaaaccgauguuuuuguuuuggugacacuaucgucaagaaauaaauucguuauuaauuuauuguugaacguugucuuaaacggggaauuaggguaaaccaucuuaaccuuuaagauaauuuaaaaucaacguaaaauaauucuguaaacaaaauuaaagucacaaaacgugcauacuugauagguuagaaguugaugacuaaaaacuaaaaggucacgugucaugcgccaaccaaugcgacacgcugguucccaagacguggcaugagcuacgauucucuuucaaguccgccauauugacauucgacaacuuuuuugggaggacaggugaauguuauagcguuuuucaaaguguaagguguuuauuuucaaaaaguuuauaaaauaagcaaucacuauggguaauguguuugcaaauuuauucaaaggccucuuuggcaaaaaggaaaugaggauauugaugguaggacucgaugcagcugguaaaaccacaauuuuauauaaacuuaaauuaggagaaauuguaacaacuauuccaacaauuggauuuaauguggagacuguagaauauaagaacauuaguuuuacaguaugggauguagguggucaagauaaaauuaggccauuguggagacacuauuuccaaaacacacaaggccuaauuuucguaguagacaguaacgacagggaacguaucacugaggcuaaagaugaauuaaugcguauguuggccgaagaugaacuuagagaugccguacuucucauuuucgccaacaaacaagauuugcccaaugcaaugaacgcugcagaaaucaccgacaaacucggucuccauucacuacgcaaccgcaacugguacauucaagcuaccugugcaacuagcggagauggucucuaugaaggucuggacugguuguccaaucaauuaaagaacgccaaucgcuagaacauaggaaaagagaggagugcgcaaaaaagugugcgagugcagaugguuuuuuucuuguacucuugucgugucuacuaccucgcgcgcgcgcgaaacguuucguauaccauauguugcaauuuuuguguccgauggggaaauucgucauguuucacuuuggggguuauaaaauuggcuguuggcgacaagugguguaugaggugaauccgaaaauaguuuuaggcaauauaucauaugaaucucagcuuucuuuagguugagaguuguuuuuguaguaaaagaaccuuaaacauccuucauuggcgauuuauuauuuuuuaacugcaugaaaaucuuaguuuuaauguuuuuauauaacacuuuuagauuguacuaacuuuuaacauuccacaaauuucucauaaaauugugauaucuuuucuaauaccucuuauaucaaugaacuuauuuuugcaggccaaaauauuuucuuagaaaguaauuuuguaucaucuauaaaaauuuaauuuugggaauucaauuaaagacuuuaacuggcaaauuuuaaaauguuacaagguucuagucacguauuuagucuggacuugcacuuuauagcacuugucgcagaaagcaucuaacccccaaacacguauggugauguccuauuugcagaaaaugcacuauaauauacgauaguaauuauuuauuguccucuuucuggugaaaacaggcuuuuuguaacauauauuuuuuauuguuuguaauagguuaaaauguacaguagacacuuauauuuaaaauaaauauuauuuuuuaucuaucaauccuuuuuguaacauaugguaaggcuguucguauuuaaaaaauaaaacaagaacauguuuuugaaaaguuuugggcacggcucaaguauuuuauuguuuaaauuuaagaugaaguacgaaugggcgcgcccgaauccgacaagauauuguauagccccguauucguugucaaaccaacgggucuugcucugguaguuaauuucggcguuagaguucaagaaggaaguagauuuuuuuauacuuauaguaaauauauuaugggauauuuaaagacuggccgauuggcuuaccagacuuacgucccgcagaucuuaaccggcgaugaguauucgagguuuguuucuggucagauucgggcacgucguacuguacauaaaauacuuuuguuuacuucucaaauuuguaacucaguuguggauacuuugaggcguaauuuuauuuugacaaacuguggauuuaagguuacauuauaagugauuuauuuaaagaaauauguuuuugauuuaucguggacauucccuguuugucagcuguauuaucaaauaaauuuauacuauuaaaaaaaaaaaaaaaaaaaaaaaaaaaaaaaaaaaaaaaaaaaaaaaaaaaaaaaaaaaaaaa

SEQ ID NO: 195 - RNA, 7631 nt, Diabrotica virgifera
cuucacuuuuacggguaaacgugcggaagguacguuccaaguucgaaccuagcgcuugauguucuguguacacucuguacaauuaaaauggcuuccaaguucuuugugaguuaacuuuguuaggugcauuuuaguaaauuucugaauuggguuguuaaauuuagaguguuagugcauaguaacuauuaaauaguggccuuaaaaagugcucuuaaugaggauuauaauaagaaaaacgaacuuuuaacaagaacaacgaguguccauucuaauguuauuacaaguagcuacuaaaaauauugcaaaaaaaacuuucgguaacuaaaaugggacgguugcacuguuuauuuuguauuuuccuauguuuuaccgucaucaacacgcagacaacgaauauacauggauucucggaaaauuccguggauacauuucuaucaccucaugggaaaagugcaaaauucgugcaccaaaaucacaaacccaaaauugaaaauugucagaacuacaaacccucggugaaagaagaacagccaggcggaacguacguaacaacgguuaccgcuaucgaugacgauccuagggagggaggaggaacaauuaguuacaaacuaauucauagagaaggagaacauguuuuauuugacauagacaacguuacugguguuuugacaacuauccagccauuugaucgggaugaaccaguaaggcagaaggaacuuuauguaaccguacaagcuucagacaacggcaggccaccauuagcagaugucuguacauuuacaguuaccauuaccgacauuaaugauaaugcgccacagcuugauaaacugaaauacgaugcacaaguuucugaagauuuaaaaguaggaagugaagugaugagaguuuuugcuuacgacauugaugauggggaaaauucaagauuaucguauaacuuuucaaacgaaaaugcucaauucacccaguauuucaggauagaucgagauacuggcguuguguauuuaaaggaagcuuuaacagacaaaaagaauacuagauuuaacagugcuguuuauguagccgauaauggcguuaacgaucaagaaggccaaaaagauucaaccgcuaagauaucuauaacaguaguagggucugauaaacagccucccagauuuacucaaaaaaugccugauggaaucuuggagauccccgaagauuuuaaagacuuuucuaaacauauugucacagucgaagcaacguccaacauugcggauccacaacuugcuuuugaauuggugaagggaaagacauaucaaaccaauaaagaccaaacguuucuuuuggaggcagaaggaaauaaagcgcacauaaagcuagugcguccacuggauuaugaaacaguaacggaauauacucuaacuauucgaguaaaaaacaaagauuuaauggauucuuccauaaauauaccaauuaaaguauuagauguuaaugaugaaauuccuaauuuccuugaauuucuuaaagguagugucguggaaaaugacaagccaggugcacaagcgauucaaguaagagcaaucgauaaagacggaacugcugcuaacaacauugugagcuaugaacucguugacaauacagauuuguuugcaauaaaccgaucuacgggaguaauuacgucgagaguggaguuugaucgugaaacuguaccucuauaucacguaaacguuaaagcuuaugauaacucuccgucugcuuuguauaacacgacauugccuaacauuguaauucagacauuccaaaucaguauagaagaucaaaaugacaacaaaccuguauuuacucauccaauuuaucaguucaguaauauuacugagcuugcugauaaaucgaguauuguuggugaagucaaagcuuuagauaaugacacggcuucaguuauaaguuauaguauuacaaauggaaauauugacgaugcguuuaugauugaaaauucuaccggcagaauaagaguuaauggaaaacuggauuacgagaaaaucgaacaauacaacuuaaccguucgcgcauuugauggggcauuugaagauuuugcaauuguuuuaauuuccauacuuaaugaaaaugacgaaccuccaguuuuugacgacuauaucagagaaauucaaauuaaagaggaagaaccuaugauauccggaugcguuguuagagugacugcucaugauccagauauuaaagacaggcaugcugaucaacacauaguauaugaggucgcgaaagaacagaaagauuuuuugaccguaucugccgauggaugcguacaaguaacaaaaccucucgaccgagauccgccuuucgguagcccaacacgacaagucuucaucuaugcucgugauaaugauggaggcacaaauucauuguuggccacugcagaaauugaaauuauuuuaauagauauaaacgauaaugcucccuuuuuaaauguuacagaaauuguuuauuaugaaaaccaggauccagguuuuauagguaaccuaagugccgaugauuacgaugguccugauaauggaccuccguuugcuuuucgauuaucagacacugcuucagauaguauuagaucgaaauuuuccauuaucggaaaccagcuuuucgcuuuagaaauguuugauagagaagagcaaaaauauuaugacauugccauugacauuacagauaguggaguaccuccacuaacaggaacuaguauucuuagaguuauaaucggagauguaaaugauaauccagcuacagacggaaacagcacgaucuuuguguauaaguacgucaaugggccagaaaauuucauggaaaucggacguguauauguuacagaccuagacgauugggauuuaaaugacaaagucuuuguucaagaagauaacuuugaugaauuuguguuaaaccagcauaacaacgguaugauucugaugaaaccaacaacggcugagggaacuuaugagguucauuacagggucacugaaacccaugaacccacaauacacgaacauacaguuaaugcaauagucacgauuacaguuaaaguacuuccagaggaagcgguuguaaaaucaggaucaauucgauugagaggaacaacuaaggaagaauucauagaaaauucauugaauggaaagagcaaaagagacauauuacaccaagaacucuccaaaauauuaaauacaucuuuagcgaauguugauguauuuacuguuuuaaauucaccccaccagaauaguucguuuguggauguucgauuuucugcucauggaucuccauauuaugcuccagagaaacucgaaaacaaaguuacagaucaucaaauggagcuugaacaaaaauuagauguggaauucuacaugaucaacguaaacgagugccuuaacgaaacaacguguggagcugaaaacucauguacgaacaaauuaaacauaacacgagaaccagcuguaguguuuacuaacagaacauccuuugucgguguaaaugcauuuauugauccugugugugccgcuuuaccaagagauguuauggaauguuucaacggaggcguccuuaucgaaaacacagcguguaauuguccugcaggauuugaaggaccacauugugaaauccuagcuauaggauuuacaggaacugguugggcuauguauccauccuuugacgcuacaaacaggacugagauuauacugcauauuuuaucacaaacugauaaugguuugauauuuuacaauggaccuuuaaauauaagacaaacuucuuugucuaaagauuauauaucauuagaacuuaaagacggauauccauuacuucaaauuugcaccggcucaagcacucaagaaauuuaucugaaagagcgcauucacaaauugagcgauggaucguuacacaaaauaaaaauaggaucuggauuugacgauauaucccuggaaguagacgacuguggaacaacguguucaauuuggacuaauaaacuacauaaagguguuauccgagcaaauggcccccuucaacugggagguaugaaaaacagauucaccgaucaagaauucaaacgaauuugggaccauuugccaccgacugccacccguuucucugguuguauuagaaauuugacguauaaugaauuuuacuacaaccucggugcaccuucugaugcauuccaagcguaucccgacuguaacuaugcagugaugcaagcugugacuuucgguaucgacuccaauuucuugguugcuauucugguuuguguagcaauuuugauaauucuucuucuggcaguaguuguacauagacguaaacacgacaacuuuaacgaaaaagaaaucgaugauacucgcgaaaacauuaucaacuacgaagaugaagguggcggcgaaugugacaccaacuacgaccugucuguuuuccaucagaacaacauuguggacgaaaaaccauugaugagagacaaccccgauguaccugcagauauaaguggcuuuuuagauaacaagaaagacaacugugauaaagaccccgauaauuugccuuaugacgacguucgccauuaugccuacgagggagacggaaauagcaccggauccuuaucuucucucgcuucauguacggacgaaggagauuuaaaguucaacuacuuaucaaguuuuggacccagauucagaaaguuagccgacauguauggagaagauccaagcgaugaagacucacacgauggaaacgaagaauccuggugcuagacuaaauuccaugacuccuuagaaagugacauuuuuguacuuaaauucuuuuauguuaaccaaagauugcgaaauuuuuuggaauggaacugaacaaacuuguacauauuuuugaaaaaggauguuucaacuguuugcaauacaagaauuguuacguaugcguuucaaaacauauauuuacauguaaccguucuuguauuguaaauauuuuuauacuaucuuuauacugacacuuagauaauguuaucuauuaaguggcaagcaguuugguuaagaauaacuuugagucuucuaucccaagguacugugauuugaacaaaguuagaauaagcaacuuccauaccaucaauccacuucauuuuauucaacauacugguuuuccgaaacuaaagaagcagccuaauacauagaguucaauaacuuuuauuaaacaauccguauuaggugcacauauucaucgcgcacaaguacauauuguggaacuguacacugacgaggaacaaauauucaauaagaaucuuuaaagcgaaaaauauugaaauacacgaucagauuuaacauauuauugucuagcucaaaagaaaauaauuuuuaucuugacaauagacauuuuucauauauaagcuaguagauuuauaucaaaaucuauaaaaaaaguggcuuaaaaguuucuuugauuuuugcgauucucuugaaugacuucaguauuuuuuacaaaauuauaagacuguuaaucguuuaagcuggcagcaugguaagauacguaugugaaaacuuguauauuuuacaaaauaacugaaaauuaguauguugcgaaaaacaaauggaaacaaauauacagugaaugucgaauaguauugucaaaauuaaagucauaauuuuuaaagauuguccaaacuagguuguugauguauguuaaucucugaaugccauccuuuagccaucauuguguauaucagcuguuuccuuuugcaguuugugugguacuccugaauguacggaauaaucacauaguuuucacgaucuuuuacuuuucuuuucugcagcuaauuacagggugguuguucccuuaucaauauugaaauucuuauauaaucaguuuuuccagacuuagaaaaguuaaaaaaacagcaucauaucccugcuauguuuauucuucguuguaaggacacucuaauuauuuccaauuagagaucucaagauguuauguuuacuagcagguauugaacgaaaacaauaauaaaagcaaaccgaguaaucaacaauaguuacaauaccuacaauuuacuaugccuucguagcuuauauuggagagaugaguggaauuucucaauaggcgcauauacacauaauaauaagacacauauucaaauugguuggugguuaaauagcucaaaaacgauacaaaggaaacauauagguaacaacaaaauacaagguaaaaauagagguacuuacaaucaggacgcuccaacgaagucacuauuuuacgucuuuacacucgaaucgucugaaugcaucucuuuccuuauguccucgggguagaaucuugcaccucaagugguugaaaguuccuuucuucgucacauguggauuucgcuaauaugcgaacaaggaacaacacaggcgucaaaaaggaauaugauuucgaacuauuuaaaacaaucaaaucaauuuaucggaauuccaacacaagauuuauaucagcauuucaguaguaaucucaccauauuccaaauuugucuuuuuguauccaucuuauuuugucuuuaucuuacuuuauauuguuuuguuuauuuuuuauuuaucuguauccuuaucuuuuucucuuugacuaucacagcaaauuuuuguaauuuggauuuacaauuaguuaugacuuuaaugaaaacaauacuuaccaucucuuuccuuaaaucgugcgauauaauuuaucaacaauguaguaucauaccacaacaaugucuaauaugaaacauacgagaggccuuaugcauaugccuuaacacguuuaggcacaaauaccaauaaaaaccuuacacgguucggcaauaaaaugagagaaccgcuauuuuauauacacgcauuuuuucuauuuuuauuaggauuuuguuaguuuuguuauuacuuaguauaaauuuaggauaguuauuuuguauuuuuauucucacguagggcucagucgacguagucguuugaauaacauuuuauuuaaaacugcagguuugagaauagccauucauuggugccguauuuaaaaaaagauuuuaaauguuucuuuacuggauauaucgaaauacaguuuuuucuuuacguaaggcaguuagauuauuaaaauagucuugugaaagcguauagcucagauguuuuuacaauauaguuucuaaauuagucuuaaaaggcaacuauucuuauugcaauauuucccaagcuaaauucacucgagacuuuggacucauaaauauacaaugacugaguucuacuugauuuccguuucauugacuauuuaauauuuauuuuuacaagucuugaugaaaauuuggaaauacaugauaucaaagcaauuuauaaucguaauuaggcuaauaguauccuaaggugauaguauuuccugauuuucaucaauuauauauauauauuaguaucacaaaauacagucuguagagacccgugucauagauaaccuaaccuuccauuguuacacaucuuguuaacaagucgauuugaaguggugccgguugugaagaugcguaucuugauguuccacggcuaaaaucgguucguucacaaaagcuuuuauauauuuuuuauuuacuuuucuucuuaaauguccggcuugaauuuucaagauccagugcugguacacaggagggcgcgacg

SEQ ID NO: 196 - RNA, 1028 nt, Diabrotica virgifera
gucagugcugugugcugucacugucacuacucuagugucacgauuuuuuagcccugaaauugucagauuaucacaugacauuuugagaaaacuaaauuaguaagugaacacgaauuuaguucaaaaugccuuucuguggucccaaauugucccucugcggccugauuaucagugcaugggguaucauccaguuggguuucauggguguauucuauuacauuggggcuguggcuuuagcagaagauauuccagagguugaguuuaagggcgauuuagacaaauuuuauagcgacgucaacacggguuucacacagaaugcuuacaacugcuggauugcugcucuccuauaccugauaacauuagcaguaucagcucaccaauucugggccaacaacagaucaucauugaacgucuaagaaucuuuuaauuugcuuuuguauauauuuauuuacauuccuucuccagcuguagauuuuaaauguauagacccucaaauacuucagaguaccaauuuuucuguuaaacuuagcggacucguacaccaaagcaauauccaaacgcaacaugaaacacucaacaucccauaaauaucagagguuauguaucccuugaacgcgcuuaaaacuaccuaggaguccucgaacuuuguucaccgacgcaaugcggauaaggaucauccaccgaaaaccagaugcgacacucagugcauauuaucuuuccacaguguauguuauaugcgauuucgauaggguauugcuuugguguacgaguccgcuuaggucagucaauguagcauguuguuguuuuuaaaguuuucauugguacuaaaacuuuuguucaccaacguaguauuauaaaaaucauaguaauauaaauaacgcugcaauguuaugaaucuuaccaaauuauuuuaugguucuguuguauuagugauuugaauuuaaaaauuguacacauuuacuaugaaauaaauugauuuauuguuaaaaaaaaaaaaaaaaaaaaaaaaaaaaaaaaaaaaaaaaaaa

SEQ ID NO: 197 - RNA, 3012 nt, Diabrotica virgifera
auuuaugguacacaucacuaaaguauuaaucaccacacuuuauaaauucaaauuuuuagaguuggaaucuacaaaguuagugauaauuagaaccauuguggcauucagaaacggucuaaacuuucaauguuagcaaccuuuuguauauagcuacaauaccgauauaacagugaacugaaaaacucuaguguagugauacaaagcauuuaccaugggucuuaccauaucagcaguguuuaauagguuguuuaguaaaaagccuaugagaauuuuaaugguaggauuagaugccgcagguaaaaccacaaucuuauacaaauugaagcuuggugaaaucguaacuacaauaccaaccaucggcuucaauguagaaaccguugaguacaagaauauaucuuucacgguaugggauguagguggccagacgagaaucagaaaacucuggagacacuauuucgccaacacugauggacucauuuuugugguugauuccaacgaccgagaccguaucgcggaagccgaagaagaauugcacaauauguuaggagaggacgauuuaagagacugcauuuuguuaauauucgccaacaaacaagauuuaccgaacucgauguccacugcugaauugaccgauaagcuuaaguugcacacuuugaagaauaggaggugguacauacaagccacaugugcuacucaagggaaugguuuguacgaaggacuagauugguugucgaaugaauuggccaagugaauagguagauguugugaagaguagcuuuuauauuuuuuauugauaauguaaaauccuguuuuauuugccucaguuugguagaauucauacaauauugcuucuauguugauaacuuuauauguuucuaucauuaaaauauggauaauuuuauccaaaaucuagcuaaaccacuauauaacgcguuggcuguguuacgagacaaauagaccucguauuauacuaacaguuggcucugucgacuauguuguaauacacuguggcauuacuggacauauaugccucguaaagcacucaaugcgggcuuauaaauaucucuaaaugcagccaaaguauuaaucuuagcuuuaacucuugauauuuuucaggauuuguguauaauuuauugaaaguuuaguuaaauauuacauuuuucuucgauuuuguucauuuaggcaaucucacauuauuuauauguaacauguuauugaaucauacccgccauagccaauuauauacccgccauagucuaauuucagagauuauuuuuuuguuuuauugacgugaguacauuuuuuaagaaauucguuucaacauuuuugucucuccucuauucauucauucauuaaagccggauuuacauauacaaguacuuggauccgagauaucaguagaacugcgaauuuuuacauuaaauaccagugauucaaaggaaauauucauuauaucugcaauagcuucauaugcauuauuuauuuuguugauaucacaauauuccuugaguuuacauuccacaaacauucaaaugaucaguaaaaacuaauaaacugucccaucuguucuccagacaaucuuaguuccacuuuuuuuuuuauuuguaaauuacaugugcucuuguauugcuacuugguuuguguucaacuuccauccaugcucguauccaaguaacaagaggcccugagaaggcguuuauacuucugacaugcacucugaguagaguaacucgaauucaaguacuuguaagggcgacuuuagaguuacaaucccuagggauuauaucuaaugccaugguguucaaaauccuaugcuuaggugagguggauuauuccuuugugucauguauaguuuccuguaugucuuugcugcuguugugacucuuuuucauuucuuccuguccuugcaccgaaauuucgagucuuguuuugaauuuaauaguauuuuguauuuugacaacgaaacccgauuugggcuucgaaacguuaauaaauucauuuuuuaguaaaauuguggcuuauuucccauaaaaaauacguaauuguuuugaauuauuugcucaaucuuaucaauuguuacauuuacauauuuuuuauuugggucgauuuucuuuguuuauucacaaaauuguuauaaccugucugagaaaucuuucaaauguuuuuuuacauuuccauuauucaauauuacacaauaucucuauugggaacgugcuuaguuuaucucuauuaggaagacuaguuuuaaaaacuaaaaauguuuucuucgauaguaaaauaaacaaccaguguuuaacaucuuugccacauuuaaagauauuuauaacacuacguugggugcgucaugaggcauauaugucccgaauacccccauuugccacuguguuacgacacaguugacguagccaagcguuaguguaguacgaggugucccguaacacagccaagauguuaacaauaaacauaaacaaaauacaauuuugugcuacuaucuaaauaagaugucaaugaguuauagaacaaagaauauuguaugaaucuauucgaccauaucauaaacugacuuuuucauguaguaaacaacguuucugcaacuccuucuucugugaauucacuuuuuguucuaccuagauuuaaauauuuauauaaauaaguuuccuauuauauacuacaguggaaccucgauaacucggauuaaucgggaccgcggccgauccggguuaucgaaaauccggguuagccggagaauauaguaaaaauuaauaaauaaccuccauuauaauuacaaaaacaugaaacacauaugcacaguacacaucuaaauuacguauaguuguauagaguguagaguuuuguucauuucuugguaaaaaacucagucauacuguagagauguaccgacaccauaauaugguaggucuggauccugcguacaaaaaaaaauugauaaauagcaagccgaaaauuuguuguuagcuugggggugucuagucggacagacauugauauaug

SEQ ID NO: 198 - RNA, 1212 nt, Diabrotica virgifera
caacacugcuaucugggcuguugcacuaaucauauggguugguuguuaguucacuuuuuucuacaguaccaugugucacuagcauaauacucaaaaaauuaauauuuaauuuugugaacuuaguuaacaucauuuugaaaaaugcgguacacuuugaguuacaucggugcuacccuagcguccacuguaacacugauuuuugcccucuacuacugccucacgggaaaaggagagcaaguuaguuuagcaugguuauuguugaaugugucuccccacaugugggcaggucuaggaauuggccuugcuguaucauuaucaguuguaggagcugcugcaggaauucacacuacaggagucaguaucguaggagcugguguuaaagcccccagaaucaaaaccaaaaauuuaauuucuauuauuuucugugaagcuguggcuaucuauggguuaauuauggcuauaguacucuguggaaguuggaagaauuucgauguagaccuauucaaccucaaaacucauaacuuugcucaaaaccauuauggaucacauguuauuuuuggauccgguuuaacuguuggauuuguaaaucuauuauguggauuuuguguuggaguaguugguucuggugcagccauuucugaugcagccaauucaucauuauucgucaaaauuuugauuauugagauuuuuggaagugccauuggucucuucggucugauuguuggaguauacuugacgucaagaggcucuaugguuuaaauguucaguaaaugaacaugaaaaauaaaaugaauaauuuguuaaaagugugugugaugaagauacaacuauuuucacuaguuuacgccccaaaauauuucauugugguuuuugaacaauauuuaaaauccauucuaaauuaaaauucuucaaauaauuguugaaaacagauucaagggucuuuaaucaguguauauaauaguauuaaauaaauauuccacuaauuuuguuaaucauuguuaaacauuguauaguuacaaaagaaauuuuuaauuuagaauaauaugcuuguacagcauguagucccacuaguauuaguauuuaaaaacuguauuaaaaauugucuuuucuaugucuaauaaaauuacagacgauuuuguuaaauuuuaauacagaucuaaaaaaaaaaaaaaaaaaaaaaaaaaaaaaaaaaaaaaaaaaaaaaaaaaaaaa

SEQ ID NO: 199 - RNA, 7646 nt, Diabrotica virgifera
cggauuucggagaguucgauucguugucgagccuucaaaauggcuaccaacgauaguaaagcuccguugaggacaguuaaaagagugcaauuuggaauacuuaguccagaugaaauuagacgaaugucagucacagaagggggcauccgcuucccagaaaccauggaagcaggccgccccaaacuaugcggucuuauggaccccagacaaggugucauagacagaagcucaagaugccagacaugugccggaaauaugacagaauguccuggacauuucggacauaucgagcuggcaaaaccaguuuuccacguaggauucguaacaaaaacaauaaagaucuugagaugcguuugcuucuuuugcaguaaauuauuagucaguccaaauaauccgaaaauuaaagaaguuguaaugaaaucaaagggacagccacguaaaagauuagcuuucguuuaugaucuguguaaagguaaaaauauuugugaagguggagaugaaauggauguggguaaagaaagcgaagaucccaauaaaaaagcaggccauggugguuguggucgauaucaaccaaauaucagacgugccgguuuagauuuaacagcagaauggaaacacgucaaugaagacacacaagaaaagaaaaucgcacuaucugccgaacgugucugggaaauccuaaaacauaucacagaugaagaauguuucauucuugguauggaucccaaauuugcuagaccagauuggaugauaguaacgguacuuccuguuccuccccuagcaguacgaccugcuguaguuaugcacggaucugcaaggaaucaggaugauaucacucacaaauuggccgacauuaucaaggcgaauaacgaauuacagaagaacgagucugcaggugcagccgcucauauaaucacagaaaauauuaagauguugcaauuucacgucgccacuuuaguugacaacgauaugccgggaaugccgagagcaaugcaaaaaucuggaaaaccccuaaaagcuaucaaagcucggcugaaagguaaagaaggaaggauucgagguaaccuuaugggaaagcguguggacuuuucugcacguacugucaucacaccagaucccaauuuacguaucgaccaaguaggagugccuagaaguauugcucaaaacaugacguuuccagaaaucgucacaccuuucaauuuugacaaaauguuggaauugguacagagagguaauucucaguauccaggagcuaaguauaucaucagagacaauggagagaggauugauuuacguuuccacccaaaaccgucagauuuacauuugcagugugguuauaagguagaaagacacaucagagacggcgaucuaguaaucuucaaccgucaaccaacccuccacaagaugaguaugaugggccacagagucaaagucuuacccuggucgacguuccguaugaaucucucgugcaccucucccuacaacgccgauuuugacggcgacgaaaugaaccuccaugugccccaaaguauggaaacucgagcugaagucgaaaaccuccacaucacucccaggcaaaucauuacuccgcaagcuaaccaacccgucauggguauuguacaagauacguugacagcuguuaggaagaugacaaaaagggauguauucaucgagaaggaacaaaugaugaauauauugauguucuugccaauuugggaugguaaaaugccccguccagccauccucaaacccaaaccguuguggacaggaaaacagauauuuucccugaucauuccuggcaauguaaauaugauacguacccauucuacgcauccagacgacgaggacgacggucccuauaaauggauaucgccaggagauacgaaaguuaugguagaacauggagaauuggucauggguauauuguguaagaaaagucuuggaacaucagcagguucccugcugcauauuuguauguuggaauuaggacacgaagugugugguagauuuuaugguaacauucaaacuguaaucaacaacugguuguuguuagaaggucacagcaucgguauuggagacaccauugccgauccucagacuuacacagaaauucagagagccaucaggaaagccaaagaagauguaauagaagucauccagaaagcucacaacauggaacuggaaccgacucccgguaauacguugcgucagacuuucgaaaaucaaguaaacagaauucuaaacgacgcucgugacaaaacuggugguuccgcuaagaaaucuuugacugaauacaauaaccuaaaggcuauggucguaucgggauccaagggauccaacauuaauauuucccagguuauugcuugcgugggucaacagaacguagaagguaaacguauuccauuuggcuucagaaaacgcacguugccgcacuucaucaaggacgauuacgguccugaauccagagguuucguagaaaauucguaucuugccggucucacuccuucggaguucuauuuccacgcuaugggaggucgugaaggucuuaucgauacugcuguaaaaacugccgaaacugguuacauccagcgucgucugaucaaggcuauggagaguguaaugguacacuacgacgguaccguaagaaauucuguaggacaacuuauccaguugagauacggugaggacggacucuguggagagaugguagaguuucaauauuuagcaacggucaaauuaaguaacaaggcguuugagagaaaauucagauuugauccgaguaaugaaagguauuugagaagaguuuucaaugaagaaguuaucaagcaacugauggguucaggggaagucauuuccgaacuugagagagaaugggaacaacuccagaaagacagagaagccuuaagacaaaucuucccuagcggagaauccaaaguaguacuccccuguaauuuacaacguaugaucuggaauguacaaaaaauuuuccacauaaacaaacgagccccgacagaccuguccccguuaagaguuauccaaggcguucgagaauuacucaggaaaugcgucaucguagcuggcgaggaucgucuguccaaacaagccaacgaaaacgcaacguuacucuuccagugucuagucagaucgacccucugcaccaaaugcguuucugaagaauucaggcucagcaccgaagccuucgagugguugauaggagaaaucgagacgagguuccaacaagcccaagccaauccuggagaaauggugggcgcucuggccgcgcagucacugggagaacccgcuacucagaugacacugaacacuuuccauuuugcugguguauccuccaagaacguaacccuggguguaccuagauuaaaggaaauuauuaauauuuccaagaaacccaaggcuccaucucuaaccguguuuuuaacuggugcggcugcuagagaugcggaaaaagcgaagaauguguuaugcagacuugaacacaccacucuucguaaaguaaccgccaacaccgccaucuauuacgauccugacccacaaaauaccgucauuccugaggaucaggaguucguuaacgucuacuaugaaaugcccgauuucgauccuacccguauaucgccgugguugcuucguaucgaacuggacagaaagagaaugacagauaagaaacuaacuauggaacaaauugcugaaaagaucaacgcuggguucggggacgauuugaauuguauuuucaacgacgacaaugcugaaaaguuggugcugcguaucagaaucaugaacagcgacgauggaaaauucggagaaggugcugaugaggacguagacaaaauggaugacgacauguuuuugagaugcaucgaagcgaacaugcugagcgauaugaccuugcaagguauagaagcgauuuccaagguauacaugcacuugccacagacugacucgaaaaaaaggaucgucaucacugaaacaggcgaauuuaaggccaucgcagaauggcuauuggaaacugacgguaccagcaugaugaaaguacugucagaaagagacgucgauccggucaggacguuuucuaacgacauuugugaaauauuuucgguacuugguaucgaggcugugcguaagucuguagagaaggaaaugaacgcuguccuuucguucuacggucuguauguaaacuaucgccaucuugccuugcuuugugacguaaugacagccaaaggucacuuaauggccaucacccgucacgguaucaacagacaagacacuggagcucugaugagguguuccuucgaggaaacuguagauguauugauggacgcugccagucaugcggaggucgacccaaugagaggaguaucugaaaacauuauccucggucaacuaccaagaaugggcacaggcugcuucgaucuuuugcuggacgccgaaaaauguaaaaugggaauugccauaccucaagcgcacagcagcgaucuaauggcuucaggaauguucuuuggauuagccgcuacacccagcaguaugaguccagguggugcuaugaccccauggaaucaagcagcuacaccauacguuggcaguaucuggucuccacagaauuuaaugggcaguggaaugacaccagguggugccgcuuucuccccaucagcugcgucagaugcaucaggaaugucaccagcuuauggcgguuggucaccaacaccacaaucuccugcaaugucgccauauauggcuucuccacauggacaaucgccuuccuacaguccaucaaguccagcguuccaaccuacuucaccauccaugacgccgaccucuccuggauauucucccaguucuccugguuauucaccuaccagucucaauuacaguccaacgagucccaguuauucacccacuucucagaguuacuccccaaccucaccuaguuacucaccgacuucuccaaauuauucaccuacuuccccaagcuacaguccaacauccccuaacuauucaccaacaucucccaacuauucacccacuucaccuaguuauccuucaacuucgccagguuacagccccacuucacgcagcuacucacccacaucuccuaguuacucaggaacuucgcccucuuauucaccaacuucgccaaguuacuccccuacuucuccuaguuauucgccgucgucuccuaauuacucucccacuucuccaaauuacagucccacuucuccuaauuacucaccguccucuccuagguacacgcccgguucuccuaguuuuuccccaaguucgaacaguuacucucccacaucuccucaauauucuccaacaucuccaaguuauucgccuucuucgcccaaauauucaccaacuucccccaauuauucgccaacaucuccaucauuuucuggaggaaguccacaauauucacccacaucaccgaaauacucuccaaccucgcccaauuacacucugucgaguccgcagcacacuccaacagguagcagucgauauucaccgucaacuucgaguuauucuccuaauucgcccaauuauucaccgacgucuccacaauacuccauccacaguacaaaauauuccccugcaaguccuacauucacacccaccaguccuaguuucucucccgcuucacccgcauauucgccucaaccuauguauucaccuucuucuccuaauuauucucccacuagucccagucaagacacugacuaaauauaaucauaagauuguagugguuaguuguauuuuauacauagauuuuaauucagaauuuaauauuauuuuuuacuauuuaccagggacauuuuuaaaguuguaaaaacacuuacauuuguuccaacggauuuuugcacaaacguaacgaaguuaaaucaaaacauuacaacugaaacauacgucgguauguacugucaaugugaucauuaggaaauggcuauuaucccggaggacguauuuuauaaaguuauuuuauugaaguguuugaucuuuuuucacuauugaggagauuuauggacucaacauuaaacagcuugaacaucauaccgacuacuacuaauauaaagauaaauauagaacgguaagaaauagauuaaaaaaaaauacaauaaguuaaacaguaaucuuaaaaauaaacaaauaaguuuccguuccgacagaacuauagccagauucuuguaguauaaugaaaauuuguagguuaaaaauauuacuugucacauuagcuuaaaaauaaauaauuaccggaaguaaucaaauaagagagcaacaguuagucguucuaacaauuagguuugaaaauaaaaauuauaaugaaauauacaaagacuaaaaguuuaaauaauaugaaaaccauuuuuaacccuccguuagucgcuaucggugucacacaccgacgacagaauuauucauucgggauuuacaaaauaacuguuuuuuucuauaccacuuucuguaccucuuccuaucaacuaaccucguguuaguauacauucuuaccuacuuggguacaguugugcgaguuuuauagcuauuuucggugcaagacuccguagcgacuaacggugugguuauuacuuuauuggcguaacuugcaguucagguaaagauuuagcaucuuauuauugcauuuuaucgguaaguuuuggucaaauuuuauuuauagauguccuuugaagccgaacgaaaacguuuguuggaauuaugggaaaugguuccuagcgaauauuuuuauauuacaaauaacaauauguuuauuguuauacuaggguuuuucauuuuauaucugucguuuuucaaugaagcauuuucaaaaauauuuuuuagucauuccuauacacaauauaaaauauuuguaugaauuuuauagcaauaacuuuuuuuuuuaaauugucggucucugacaccguagcgacucuugaugcuccguuuauccuagcgacuaacggggguuaaugugaauuuaucacaagcacaaagcacauagauaaaaccaaaccuauaaguuacuucuaauacaaaauaauuaaaugguuuugaagucauaaucucgccaguuuugugaagaauuauuaaggaccagacaggucuucaagucgugccguuuucugucugcuugucucugcaauaaaucuuaaacgaaaaguccuaaugauuuaaaacuuaauauuauguauauuuguacauaggauauuuacgauccaaggaagaacaaaggaauuuggugucaaugggucaaaguuuaccaaaaaaaguuacugauaauuccgauuagaaaggacguagagccuuuuaccaucaguuagagguuagagguucggcaaaggcuuuuguuacuuuacauaauucugucagguccuuugguacucauuauacaaaagcuuuuaauuuugcaccuuucacuuccuuccacuaauucgguaccacggacuaucgaaggaccaaauauaauuuuuuaacauaccuaaagcccuugccgaaugucuaaccgaagauucaauauuucacaucccaucuggaguucucuguaacuuugagaugauuuuuaaucuauugacgcgaaauucaauaguuuucuuggaccaaaaggacgcuguguaccaaguuucaugacuuuuccugaaagaguu

SEQ ID NO: 200 - RNA, 2600 nt, Diabrotica virgifera
guugacauugacaguggggacaccuauucuggcaauuggaauuaauuugucaauaucauuuuuugucgugaaauuguguguuguaggagaaaguaauauuauuaaaaaaugucgucaaauauucaaaaggcccagcaguugauggcggaugcagaaaagaaaguaacaucucgagguuucuucggaucucuauuugggggaucaagucguauugaagaugcaguggaauguuacacaagagcugcaaaccuuuuuaaaauggccaagagcugggaugcugccgguaaagccuuuugugaggcugcuaauuugcauuccagaacuggugcucgucaugacgcugccacuaauuauauagaugcugcaaauuguuacaaaaaagccgauguauuugaggcuguaaacugcuuuauaaaagcuauagacauuuauaccgaaaugggucgcuuuacaauggcugcaaaacaccaucagacuauugcagaaauguaugagacugaugcuguggacaucgaaagggcuguucaacacuaugaacaggcggcugauuacuucagaggagaagaaagcaaugcuuccgccaauaagugucuucuuaaaguggcucaauaugcagcccaacuugaaaacuaugaaaaagcagugggaauuuaucaagaaguggcuuaugcagcucuggaaagcucucuuuuaaaauacagugcaaaggaauacuuauucagagcugcccuuugucaccuuuguguugauguacucaaugcacaacaugcuauagaaagcuauauuucaagguaucccgcauuucaagauucccgugaauacaaacuuuugaaaacccucauagaaaacaucgaagagcaaaacguagauggauauacagaagccgucaaagauuacgauucaauuucucgucuugaucagugguauacuacaauucuuuuacguauuaagaaacaaguaagcgaaagcccugacuuacguuaagacguauuuagaaauuucuuauuaauauuucuuuaaguguuauuuaagagacccauaguuuauuuauuguuggauuauuauuugaguaugucgguauacaugaagugauuuaaccuucauauagcauuuuuaaauauggaagcgauacauuuaacauucauuuuuuacaaaaaaaauuaguauagcauuuugcaauuuaugguuucuaaggauaaaguuaucaaaugagcaaauucacuuaaguucuaacauguucgauaguauaauaagauuaacgauacuuuuaacgauauaucuguauaaauauucaaugaaaauacguaaguauuaagcaauuaccaacuaauauuauuauuugcucauuuagguucucauuuuucaauuuuugaaauuguuauucuugcuauuagaguaaaaagacuuaacaauaacaguugguacuacaauugcuuacuauauuagcaggcaaaucuugguuaucacaacaccaucuuauaucagacuuuagaaacagcuuguaaaauuauauauaaugagcacuguuauauugauucuuuuaaauauuuucucaucaucuaaaggugcgaacugacuugagcauuuuucuccgaacgaacugaaugagcagagcgugcuguagcaaauugcucuagucucuagucaguacguguucacgagcaaaauucugcugaacugaauuuucggaggagugucgguaaucguugaaagaucaaaagcuaucauuuguucuuuugugcucaauagcuacagacauuuaguguauuugguguguuccgauugauuuauaugagcccuuuucuguaguauguaauccaaucaucauaaucauucaacucggaucuauccacugcuggauguaggucucccucagucuguuccauguauuucuguuuugugcuguuugcauccaauuuuugucgagccguuuuaugucaucagaccaucuuguuggcggaugaccucuacuucgauauucuuguugucaugguauccaguguauuauucgcuguguccauuuguuauucgacauucuagcuauguguccagcccaguuccacuuuagggucauaauuauuucuauagcaucugucacuccuguucuucgucuuauuuccuuguuuguaauucgaucccuacgagaaauguguaauauugagcguuccauggcucuuuggguaacacaaauuuuauuucuuacuuuguugguuauuguuaaaguuucugcaccauauguaaguacuggcaacacacacugaucaaagacuuuccuuuugagacauacauauguguaauccaauacacgggcaauauuaucauaaaauauagaaaaugaugcauggauauuaauagcugaaguaggauguaccuccaaagaagcaaagaaaaagucauauuuauaugaaucuccugucgcuauuaaccacaaaguaacaguuaagcgaucucgaagagauauauauuauaccuuuucgaaauguuuugcaauuguaggaccuacuauaguccgucccaucuugacuuuacaguauggggagcaggggcggugcaguccuuaugagaguuuuuagcgcggugaugccgauuuuaccaaaaac

SEQ ID NO: 201 - RNA, 4648 nt, Diabrotica virgifera
uuggcaauacgucuaauacgucagucaaaugaaucaaguuguugggauugggauuuaacaaauacgucguucuaaauuucuaaaacugcauacaaaaaauccuuaaaaaacuagugaagauuacuaaagugcaauagauacaaaaacaauauuuuuacguauucaccauaauaauauaaacguagaaaaugaaucccgaguaugauuauuuauucaaacuucugcugauuggagauucaggaguaggaaaaucuugucuucuacugagauuugcagaugauaccuacacagaaagcuauauuaguaccauuggcguagauuuuaaaaucaggacaaucgauuuagauggaaagacaauuaaauugcaaauuugggauacagcaggucaggaaagguuuagaacgauuacaucaaguuauuaccgaggagcacaugguauuauuguaguguacgauugcacagaccaagauucauucaauaacguuaaacaguggcucgaagaaaucgaccguuaugcgugugacaauguaaacaaauuacugguagggaauaaaagcgauuugacaacuaagaaaguugucgacuucacuacagccaaggaguaugccgaccaauuggguauaccauuuuuggaaaccucagcuaagaaugcaaccaauguagaacaggccuuuaugacuauggccgcugaaauaaaaaauagaguaggaccuccaucuucugcgguagaccaaggaaauaagguuagguucgaucaaagucgcccagucgaaacaaccaaauccgguugcugcugaaaauauuuaguucucuuugguugaagguggucacucaugucaucucuuuuguacgguagcagcgcuacaguuacucuuauucuaguaauauccgucuguauguauaguuauuuuaaaguuuuugauuugauuuucacuuuagauuuuuuuuucaaaaauauagaaaacaccaauaucucuuagccuaaucuuaacucccuuagauaaauauguaauuaacaaaaauauuuauaaaaccauuuuuacuaaacuauuaguccacaguauaucguuccuuuucaaaaaugauuacaaaagucuuaaaaaugguuuuaauuguuucguuuaaacgagucuaccacuuuaugaaaaauuucagaaagauuauacguuaaaauaaaauaaauuauuuuugucggacaaaaaagaggggcaaacacccgcaagaugucacucuagcgcgguacaguuuuguuaauuuauuaguccacaguauaucguuccuuuucaaaaaugauuacaaaagucuuaaaaaugguuuuaauuguuucguuuaaacgagucuaccacuuuaugaaaaauuucagaaagauuauacguugaaauaaaaugaauuauuuuugucggacaaaaaagaggggcaaacacccgcaagaugucacucuagcgcgguacaguuuuguuaauuacaaaacucauaauuuucaauugaaaguauugauaauuacuaaauauuguggaucucuuguccgacagauuugcagccucguuucuuuagugggacagcggaaauauguuaauuaugguagguuaugguuugcgguuacaaaagucauaauuuuaauuuuuuaacguucaaacuguucaaaaaguaauuguccgacaaaaaaauuguucgacgcaaacuuauaacaaaaacagugacagucuacuuguguuugucgguauaaucgcaaauuaccuaccucuaguauagaugcuuagucuaguaauuagucuguuccgcucugcggaauugaguaaauggaauuaauuaaaaauaaguguaaacuaugaacaauaauauauuuauuugugucgauaaaaagacguguuuugcucgaaaggguguguuguugacgcaccgcaucuaucccgacgcccgcuggggugugacugccgacgggagguuguaaaucgacccgugguuauguaucgacugacgcuguggcugaaaaaaaccacaaacgcuaauauguuuguacuucuaacaucuggccagaaaagcgauaaauuacuacaucuguaguuuuaagaaacgucuucgaaugcauuuccaugcauugacauggaaucugauaagguaauuaauucauggggaauucaguuuguuaaacugaacacaccaaaaauaugguuagggauacauuucguuucguaaaacuucuuagcaucugguuuguauauuaaaugugaauuuauaugaccguuuugagaaaugauauuaaaaaauaaaauuagcaaaaauaguaauuaaagcgugucgccacaagucuauguuuacauucgguuucuauacauuuucugacguucuagacgucacuagacauaaaacuaaacagugcaacaaguaaaggguccagggcuauguuagcucaauuuaucuaguacuguggcgguugcaguaaaaaaaguuuugaaauuaauuugucggacuggcuaucugauacccaauuuuugucggacauugcucuauuuggauaaagaacccuccaaucuaucacuuucguguucgaaauuuuauaaucgcaaucugcauaauuguuaauuauuaacauauuuacguuguucgacuaaagaggggaggcugcgaauuugucugacaagagaucaacaaucuaguaauuaauuauuaauaaacuaaaaguggguaguucccuggguuggcuguauaccauguaguuaaaaaacucuaaacauguaguaaaaccacuucuauauaaaagguauauguacugaaauuuuaaaaaucccgauggauugaauaaacuagguucauucagaacguuuucggaccugucaguccaucaucagugaauucauauauacuugcgcuaacuagucccagaaccaaacaaugguuguacuuauaaaucaaucuacauuauaguguuauguauuuggaaaggcuaagcgccgauguucugauggacugauagguccgaaaacguucugaaugaaccuauuuuauuuaauucauugggauuuuuaaaauuguaguaaauauaccuuuuacacagaagugguuuuauuucauguuuuuuguccgacgaaaauaauuuauuuuauucuaacgcguaauuuuuugauuaaaauuaaaaauuauaguuuugcaaucucaaaacaaccgcgcuagagcuacagguuuaaaaggaagucaucaaaaccauuuuuaagacuuuuguaaucauuuuugaaaaacgacgauauacuguggacuacauauaugagaucauuagaacgagaaagauauacucaucgacuguuaauuuuguauuguuuuuaguauaccuuucucuguuuuauaaauccagaucaugauagauugacguuagaaauuauuguucgcuuuucaaacguguauuagcagaauuuuggcaaauuaaauauaaaaauucgagauccuuuauaaaaagguauauuuaaaauucccuaaguaaggguuauauuaaguaacagaacguuuucggauuaaaaaauccaccaucaguguuacaaaaaaaaaauagcaugccugaggcaccgaaauguuacggguaaaaacccuuuaaauguugacaguuguugucuuauacuaugauguugcuaauauuccuggauauuacccagggcaacacaggacucuucccacgugguugaaauuugagaauuucaaucacgaauuugacacuuccaaaauacguaaaguuuuccacaucuuuaaucugcauguugugaauaguaaauagagugucguuccuugcauugguucucauggacuugauuuuacuaauauuaauuuucaaaucuauuuuauuggcuucaguggaaagugaauuuugaaaaaaaaucugcuaaaaauaguuuaaaaaauauuuuuuuuuaguugugacacuauacagauaaaauaacgaaaaauuuacgaaauaauauuuaucaaaaguggcucuugcaguacagaauauaauaucauuauuauuaucuaguuaauagacucguacuuuuuaacgauguaacuuuaaaaacaauuaacaacguuaaaaaaauacugcaaaaaggaagauaaauaagugauaaaugugucacuuuucuugagcacuacgcagauuguuuggaauaaagcuaucacguauuauacuguguaaacuccacaaacgacacuuuauacacaucuuagaugaacaaaugccuggcacaagucgauaugugacacuguuuauguucggugcaccgucaguuuugguuaaucauuagugucagcuaacgaaaauacuuuaacuauaaacuugacacuuuuugagauaagauuuuguaguuuuauuaaacuguuggugcaauaaaaccguuuuuaaaauuuuuugaguugugacacuauuugagcggaggugcgacauguggaaaauauuuacaauuauuucauauaucacuuguucuauacaauaaaaaaacgucauuucuaacaugauuuuuagugauuucuguugguccaaaacaauuuauuauauuauccauauauacuuguuauuuuuuauguaaugauuuuucuuauucgcuacacauuaacgucauuuuuuguuuauaucaaauaaaaaguaauauuguaaguaauaugugauuguaaaucuuggucaaua

SEQ ID NO: 202 - RNA, 1577 nt, Diabrotica virgifera
agaaaacaagcgguuuauuugccgccauuuugacaagcuuacguaccuacauuuuuaauucguuguuuuauuuuuaguuuucaauaauacucuaaaaaauggcagacgcugaugaucuauuagauuaugaagaugaggaacagacagaacaaaccgcaacugaaacggcaacuacagagguacagaaaaagggugucaagggcacauauguaucaauacacaguucuggguuuagagauuuucuguuaaaaccagcaauucucagagcuauaguggacugcggguucgaacauccuucagaaguucaacaugaauguauuccucaagcugucauuggcauggauauucugugccaagcuaaauccgguaugggaaaaacggcuguuuuuguauuagcuacacuccaaguaauagauccuacagaaaauguuguauauguucucgucaugugccauaccagagaguuagccuuccagauaagcaaagaguacgaacguuucaguaaauauaugcccaauauuaaaguaggggucuucuuugguggcuugccuauccagaaagaugaggaaacguuaaaaaauaauugcccgcauaucguuguggguacuccaggaagaauuuuagcauuggucagaucgaaaaaacuuaaucucaaacaucuaaagcauuuuauuuuggaugaaugugauaaaauguuggaguuauuagacaugagacgugauguucaagaaauauaucguaacacuccccacgaaaaacaagucaugauguucagugccaccuuaaguaaagaaauuagaccaguuugcaagaaauuuaugcaagauguaauucaaaauucuuauaauacacaauuuuguaaugacgcacccacucgcaauguuugaaaaguucuaauucaaaauacgggccaaaguuuuauuaaaucgaaucauuuaaaagaugaggguguuggguuuaaaucauuagcgcauuguagcccaacgaguaggcaggggugggccgggccaagaagaggacacuauacaggauuuucuaaauuuccguaaaggguuccgcgaccacauuuucggccgagcuacaauguagaaaaauuuacacacccuccaaguccaauagaauuaaugggguuaauguuugaaguaccgauggaguucuuuguugauuuauuuagaagaguauuuuuggauaauuguucagagaucauuucaauggugaugcagcgaugaugggaugcgagauaucaacugacuguauguacgauggauucagucaagacuccugagccucguaacugcagacuauuucauuauuuuauuaacuaaaguaauaauugaguuuuuuaucgccucaauuauuauuucaaauaauuuauauaaagauuuagaaaacuaugauuuuguugaugguuauauuuaacugucggugaguauuuucauucacaaaaguguguguguuauugcguugccgcuccugaaauaucuagaggccaccuaucgauggaucaagaguaaacuaccuuuauaguucauaacauuuaaauuagaaugauauaauugcacauuaaaacauaauua

SEQ ID NO: 203 - RNA, 1039 nt, Diabrotica virgifera
gcaucuggucugcccgcauaagcuuguuggaacugccagugaguacacagugauguucacagggaagacagugaacggugagguguggaguaaugagaaucaugaguuucaucaggugcuaaugcaacuuccaacaaaaacagauuuuuuucguaaaaugugaacguguuagucagucaaaauagcaucaaaaugccggucauugaugguuauaaaguacuuuacauuuuauuacacaguuuauauacaauuuuugaaaauauuuggaggacucuuuuauuuauuuaucaaaauuguauaaggguuauaaacccugaaucuacauucgaugaugcugaccaguuaaagaaaagacugucuagacuaacaaaaaagccucaacauuuaacuaucauuauugguguggaagaauauucauugguagauuuggcuaaccucguauauugguguuuaggucuuaauauuccguacguuaguuucuaugauuauaaagguaauuuaaaaaagcaugaagagaaguugcaacaaauuguagaauccagaaaaucagagaauaucaacauaauuuggcacacccaugcagaacaaaggcauaaaaauggauuuuuggguccaaaaauccacguaaaaguguuaacacacgcggacggaaagcaaaguauaguaaauguuacuaaaaaauuagcucuaaauaaagaaaaagacauuaguaaagaaaaaauuagugaauuacuauuaaggcaguaugaauuuccagauccagaaauggcuauuauuuguggaaagaaacugaacauuuauaauuauccuccuuggcaguuaagacucacagaauucuuuaaagucaacaaagucaacaacaucacauucccaguguuuguggaaaaauuggaaaaguacagcaaaugugaacagagggugggaaaauaauuguuuuauaaaaaacuguuuuuguuuugguuaucuuuauuauuaagaaaaaaaaaaaaaaaaaaaaaaaaaaaaaaaaaaaaaaaaaaaaaaaagaacagaggguggg

SEQ ID NO: 204 - RNA, 697 nt, Diabrotica virgifera
cucgaauaaacgccacauccaaacaagaguugacguugacagcgacauuuccuccgccauuuccuuuuacuguguuucuuaggauuuggaagguacaaaaugaccaacucuaaagguuaccgccgaggaaccagggaucuauuugcccgcaaguuuaaaaaacgugguguaauuccacuuuccacauauuugagagucuacaaaguuggagauauuguagauaucaaggguaauggugcaguucaaaaggguaugccccacaaaguguaccaugguaagacaggacguguuuucaauguuacugcacaugcauuagguguaauuguaaacaaaaggguucgaggaagaaucauccccaaaagaaucaaucuccguauugaacauguaaaccacuccaagugucgucaagacuucuugcaaagaguaaaauccaacgaaaagcuacguaaagaagcuaaagaaaagaacauuaaaguagaacuuaggagacaaccugcccaaccuaggccagcacauauuguuagcggaaagguuccagcacaggugcuugcuccuaucccauaugaauucauugcuuagguuuguuuaucuuaaaauaaaauccuuuauauaauaaaaaaaaaaaaaaaaaaaaaaaaaaaaaaaaaaaaaaaaaaaaaaaaaaaaaaaaaaaaaaaaaaaaaaaaaaaaaaaaaaa

SEQ ID NO: 205 - RNA, 784 nt, Diabrotica virgifera
cugacuucaauuaaauggccucugucaaugucagaguaaaugucaaaguguaaaaaauaaaaaaaguaacaacacaacagauuuuauuaaguuguagacguguaauuuuuguaaauuuauucuaagccauuauuaauuaaaguaauacuaaaauggaaggaauacuacuggaaccaacauuguauaccauaaaagguauugcuauauuggacuaugaugguaauagagugcuggcuaaauacuacgauaaagauauauuuccuacagcaaaagagcagaaagcuuuugagaaaaauuuguucaauaaaacucauagggcagacgcagaaauuaucauguuggaugguuuaacuuguguguauagaaguaauguagauuuauucuuuuauguuaugggcaguucacaugaaaaugagcuaauuuuaaugaguguuuuaaauugcuuguaugacucaguaagucaaauauugaagaaaaauaugcaaaaacgagcugucuuggaaucacuagauauuguuaugcuggcuauggaugaaauuguugauggaggaauaauuauagauucugauucaaguucaguaguaucuagaauagcauuaaggacugaugauauuccauuaggagaacaaacuguagcucagguauuccaaacggccaaagaacagcugaaauggucauugcugaaauaaagugcguauuuuaaaacaagguaaucgguauuuauuucauguacaauuuaauuauuaaguguaaauaaauuuuuucuguuuaaagaugaaaaaaa

SEQ ID NO: 206 - RNA, 1850 nt, Diabrotica virgifera
guuugacgcauugcagguacaagccuaccaaucacaaacacacauuguacgaguagacguuguaaacaagccgcacccgauguucaaacuugacauaacauacgccacgucaacuagaucgcccaacacuacacaauuucccucacgaaaaaccaccgcauccaacacaguuuaaaauuguacagcgaaaauaccaucuucaauaguuuguaaagcugggaaaacaaauaggaaaauuuaaacguuucguguguuggcguaggaauauuucuaccgguuucugucauugccgcacuauugcgcuuuggugguuucgcagcagcaguuccccccucucuucucuuacgucgauccuaaacaaaacgagaaaagacaguuggcuggugcacuuugacgagaggcguuguuaguuacuucguugugucgacauuuuucuguuuaguguaccgauuaaucuucaaauauuacaauggcugaccaacucaccgaagaacaaauugcugaauucaaagaagcuuucucacuauucgauaaagauggugaugguacaauuacgacuaaagaauuaggaacaguaaugagaucucuaggacaaaauccaacagaggcugaauuacaggauaugaucaaugaaguagaugccgaugguaacggcacgaucgauuucccagaauuuuuaacgaugauggcacguaaaaugaaagauaccgauagugaggaagaaauucgugaagcauuccgaguguucgacaaagacggcaaugguuucaucucagcagcagaauugcgccacgucaugaccaacuugggugaaaaauugacagacgaagaagucgaugaaaugauucgggaggccgauaucgauggugauggucaagucaauuacgaagaguucgucaccaugaugacuucaaagugaggaaaccagaguugcauuuucagcuuuccauuguuucaucccggcucauugucuacauuuuucaacaccucgaacuuuuugcuuuguggccggguccacuaaagugaauaacuuaaccguuauuugauuuacaagacaaauuuaauuaauaaauauauuuauaaauuaauauaauuguguaaauuuuuguaauauauuuguuuuucuuucgcaggagucguuggcgagaucuagucgcuggcgauucuuguacuguaucaaauucugugcuacaugucuaguugaaguuuaaaaagaguuacaaagucacaaaguaugaaaacacguauauauaaugaagauaaaaaaaucguucuauuugauguuaguuuaggggauacagcauuagacacuuucaauuuuuuucauacuuugugauguaaauuacaucugaucugugcacuuacuauauaguauguauccccuuuuuugacauguucauucauuuuuccccuuucuuguacuguagguuuuacauuuuuagucuaggauuugaauuugcuggaaaguaagcacauuuuuauugucauccugugaugcguauggaaauguuaauauuuuuuggcucuuacuguaucacaggaaauggucuuuagaaauugaucgaaauuuuuuacaacaaaaauuuuauucuaauuucuuaagaccacucccuuucuuauuguaagauuucguuuuuauucaagccuguuaauuuuuuuauuuauucuuacuauuuaagauccaguaacgcauccguuacaaugugaaauuauuagauguuuaaauuugaaauaaaugugacuaaaauauuuuccugugacuuacugguacccaauauauuauuacuauaaaguuuuuauguuagaauuuuuuucuuuauuuaaaauaaaauauuugaauuaaaaaaaaa

SEQ ID NO: 207 - RNA, 3245 nt, Diabrotica virgifera
cagcgccauuuuaguauuuagcucugaagauugaguuuuuacuuccgugaaaaauuuuuacgaguuuuuauugucaucguuauaauauuuucgacaacugcaguucuguauauagucgguuugaaaaucuuaaagaaaauaaugaggguaugaauuuaaacgugcuccaauauuagcgcuuagcguguauuugccgguguauuguguucaacgucaccaucaaccaugaugcaagcaaacaaucgagucccaccuauaaaguuggaaaacgauauagaucuuuacgccgaugauaucgaggauuucgcacaagaugacuuugguggugaaaauguugaucuauaugacgauguaauauccgcuccuccuggaaauaaugacaacccaggugauucaaaucaucaugcuccuccuggugcuggugaagaugguggagguaauuuuguugggucaggaggagcacccaauaauauaaauucuucuggaagaagacaucagcuguauguuggaaaucugacuugguggacaacugaucaagauauagaaaaugcagugcaugauauagggguaaccgacuuccaugaaguuaaguuuuuugaacacagagcaaauggucaauccaagggauucugugucauaucuuugggaucugagggaagcaugagacucugccuggaacuccuaucuaaaaaagagaucaauggccaaaauccccuuguuacccuucccacaaaacaagcucuuaguaacuuugaaagucagucuaaaacacgcccuucuccuacuaauaauucuaacucacguccuccccauccuaauaauaauguucauucagguccuaugcagaauuauggagguagaaugccuaugaacccuuccaugcgucccaugcccccagguaugcaaggugcuccaagaaugcaggguccaccuggauuuaauggaccaccaaacaugaaucagcaaccccccagguuccaagguaauccacaauggaauggaccuagaccuaaugguccugggcccaauaugggaaugagacccauggggccaccucauggacaacaagggcccccaagaccaccaaugcagggaccaccgcagcaagguccuccaagaggaaugccgccacaagguccaccgcagaugcguccagaauggaaucgaccaccaaugcaacaaggguacccucaaggcccgccgcauaugcaaggaccuaacauggguccaagagguccaccccaaaugggaccacccggggcgccucaacagcaaggaccagcuccgcacguaaauccagcauucuuucaacaaggaggaggaccaccgcccccaaugcaacacaugccuggaccagggcccgucaugccuccucaaggacccccgcaagguccaccacacggacccguuggaccuccacacggcccaccauuggguccagcgaauguuccgccucauggaccaccucacggauaugguccaccugcagcgaugccacagccgccauacgguggcccaccuccagaccaccgcgcugagauuccucaguuaacagagcaagaguuugaggauauaaugucccggaauagaacaguuuccaguucggcgauugggcgggccguauccgacgccgcagcuggagaauuugcaagcgccauugagacuuugguuacugcuauuucacucaucaaacaauccaaaguggcuaacgacgaucguugcaagauccuuauaaguucgcugcaagauacuuugcguggugucgaagacaaaagcuacagcuccagccgcagagaccggucaagauccagggacagaucacauagaagaacuagaagagaacgauccucgucacgguacagagacagaagcagagagagggagcgugaacgcgauagagaucgugaucgugaacgugacagauauuaugauagauacagcgaaagagaaagagaccgagaucguucaagaagcagagaaagaacagaaagggauagagaacgagauuauagagaccgggaacccgaagagacagauaaagaaaaaucuaaaguauccagagucucaagaucaagaaacaaaucuccggaaccugucgaaccuagcagcgagguaccgaaaucaucccgcuauuaugaggauagguaucgggaacgagagagagaaggucgacgagagagcgaucgcgaaagagaaagagauagaagaggggaagacagccauaggucucgacacuagcauauaguuagcgguucacagaaacaacaacaaacaaguuauaguuggaguucaaacaaagauuaucguguuuaauuuagagauagguuauaauaugugauguuacuuuacauaaauuuaaacagguuccgaauguguaaguuaaaagagcaaaggaaacauucacuaacucauauuuugcuacuuguuucauuuugcaauggaacuucuggcuaucuuaaauguauucauaaaaaggauaaaaaacauuuaccuguuuauuguuguauuaaguaaaucauugacuauaauauugcgauaaauguuagauauuuuacuucaugggguuauacuuuugauguaaaaguuucacauauuuagcuuuaagcaaacgugacuuacuaugaauauaauaaauuauguaagaacaaaauuaaguaaugaauauaccacauaauucuucaacuaaugaguuacuauguacaguauauucuucuuacuauuucuucaguuuucuccuggaguagcaaaacuuguuuuuguaaaaugaauuuauuguuuaggcugugcuauauuaacacugggucgucuauuaaucuguuaaaaaacaguuuuugagagaauucuguucuuuauaaaaaauuacaggagggugaugaaaggcuuuauuguuacgugcauguugguaaaucgggaugcuucuaaaugauaaauaacuuuaggcaacuuguuguuucugugagcuguauuuuuucacauuuuuauguaaucauacauaaguaaaucauguaacguauaguugauaaguacaauauagauggaaaucaaguuuuguuuuuguguguaguauauggauuuaaaacauguaucuuuuaauaagaugauguuucaacauacaaugaauaauuuguguaauaaauugaauacuauucaacaugaauugucaaauucuuacaaaaaaucaugauaauuugaaggcaauugaccaugaacuacucacaaugcaucuaaaugugaguguauccucc

SEQ ID NO: 208 - RNA, 1023 nt, Diabrotica virgifera
gucgucagucgucaacaucaauuucaaguuucaagaaaaagcaaaucacuacgacuugccggauuuuguaguaguguuaauuuuguauuaaaaaaucaaaaugaguucuauuggaacuggguacgauuuaucagcuucccaauucucuccugauggaagaguauuucaaguugaauaugcaaugaaagcaguugaaaauaguggcaccguaauaggccuccgagguacagauggcauuguauuggcugcugaaaagcucauuaugucaaaauugcaugaaccaaguacaaauaaacgaauuuucaacauugauaaacacauaggaauggcauuuucaggcuuaauagcugaugcaaggcaaaucguugagauugcuagaaaagaagcaucaaauuauagacaucaauaugguucaaauauuccucuuaaauaccuaaaugauagaguaagcauguacaugcaugcauacacuuuauacagugcuguuagaccauuugguugcagugucaucuuggccaguuaugaagauagugacccaucuauguaucugauugauccaucuggaguuagcuauggauacuuuggaugugcuacagguaaagcaaaacagucugcaaagacugaaauagaaaaauugaagauggggaaucuaacaugcaaagaacuuguuaaagaagcagccaaaaucauuuauuugguccaugaugagcugaaggauaagaauuuugaacuggaacuuucauggguaugcaaagauacgaaugguuuacauaccaaagugccugaaucaguguuugcugaugcagaaaaagcugccaaacaagcaauggaagcagauucagaaucagauacagaagauauguaauaacuacauuuaguuuuuaauauuucgcugaugguggcuguucuuacaauauuucguguguuauguucauauauuauguaauacugugagaauuuccauuucaaggauagguuuauaacuuuuuuuucuaauaaauacauaacuuuaaaaaaaaaaaa

SEQ ID NO: 209 - RNA, 1439 nt, Diabrotica virgifera
aaagugucaggugcuguuggugucagcugacuuuuuacuuuuuguuccaguccuauauucaacacacuuuggauauuaaauauuuuauucuaaaucucaagaauggcuucaaaagacagauugaugauuuuuccaucuagaggagcccaaaugaugaugaaauccaggcuaaagggagcccaaaagggacauaguuuauuaaagaagaaagcugaugcuuuacaaaugagauuuagaaugauuuugaacaaaauuauugagaccaaaacucucaugggugaaguaaugaaagaagcugccuuuucuuuagcugaagcaaaguuugcaacuggugacuucaaucaaguuguucuucaaaaugucaccaaggcucaaauaaaaauaagaacuaagaaagacaacguugcugguguuacuuuaccaguguuugaaugcuaccaagaugguacagauacauaugaguuggcugguuuggcuaggggaggucaacaauugacaaaacucaagaagaauuaucaaagugcuguuaaacuguugguugaauuagccucuuugcaaacuucuuuuguaacucuugaugauguaaucaaaauaacaaacagaagagucaaugccauugaacauguuaucauuccaagaauagagcguacuuuggcuuacaucauauccgaacuggacgaguuagaaagagaggaguucuauagauuaaagaagauccaggacaaaaagaagaucagcagagcaaaggccgagaaacaaaaacaagcucuucuccaagcugggcuacuuaaagagucccaggcaaacaugcuuuuggaugagggcgaugaagaucuacuuuucuagaacaucaaacagccugaagugugguucuguacauaugaauaaauauauaacgcuaacuuguuuuuagacgguaacuguuuauuuuucgcauuaauuaauacauuuuuaagauauaucuuuauuuuuaacugguuuuuauucuuaugccuugcaauaguaaaagauauacgaacccggauauuuccuauauaaauaacuuccuacuuuuuauuaacuccaguuuuuaggauuuuaauacaauauucaacacaucgugcaauagaauuugaagugaauauuacuugcgaaaauuaaaaagguaccaaauauuuuucuuaauauugaacguauauuccagaauaguauuauaaaaguuuugauugaaauucuuguacgugacacuaugaacuuguagauuuuagagaaagcagcuuuucaauggaaaaugcuuuauugauauggacacuagauaauguaaauacuuguuaauauacuuugaacagauaaaauaguuuauucguuuuaaauucuuuaaaacucuaaauuguuuuucaucaaauguauacauggccuguaaauuguugguuagaaauaaaacucuguucaaaaaaaaa

SEQ ID NO: 210 - RNA, 5226 nt, Diabrotica virgifera
gcgauugcgucugcugaaugcacccauaguauuguggugacugugacaggugacagucggagucgacagugaaguacaaaucaaaaucauucccuauuugucaaacaaaaaugaaauuacguguauuauuauuuacccaaguaacuuuuuaauaauuuaagccgauuauugcacuguuaguacguauguacaccacaaauaaccaauauauucuuuguuucccaugauaacacaguucuaauuucacuguuagaugcauguuacauguuuuuaguggaaucauuacuggauaaaguccucucccauaauuaaauaaauacuuaaaaaauggaggcggcucccaaguuaccgaugcucucguucgaguuaaauacuuguacagagaacguccacuuuggcccccaguuaaaacaguauauugcugcuuuuuauggugaagauccagaauccuacauuacagaaaucagcaaucuugaauccuuaagaucagcugcaguucgaccaucaacggauguaaaugguguacaacuguugaaaaaguauuucugucagcuucguuuucucaaaucuagguuucccauggaagagaaucaagaugcugcaguucuauuuucauggaaaaauaaugaauuagacauaacuucaacauccagugauaucagauaugaauuaaugguaauaauguauaacauuggagccuuacacacuuuucuuggagccaacgacucaagaaacaauccggaugguaugaaaauggcauguacucauuuucaaugugcugcaugggcuuuucaaaacguaaaagaaaaguaccaccaauucauaucaaacaucucauugguagaacugguucauuuuuuucaacaagucuguuuagcucaggcucaggaguguauauuagagaagagcauguuugacaauaggaaaccuaccaucauugcaaaaguugcuauccaagucuacaguuauuacagacagucuuuacgugucuuggaaucaguaaaugaagccuacuuuagggauaaaaccuacaaggaguggaugaaauaucuucaauucaagcugaccuacuacaaaugcaucucguuccuauuccaagggcaacaagcugaggaacaacagaaaaugggagaaaggguugcauucuaucaagcugcaugugaacagcuggacgaggcaaagaaaauugcugcuacauuaaaaaaccaacaccaccagcaagaaauaaaugagggacuagcauucacuacugaugugguugaagguaaaagaaaagcagcuaaaaaugaaaaugaguucaucuaccaugaaucagugccugauaaagaccaauugccagagguuaagggugcuucauuagucaaaggaauaccauucaguauaaaugauauagaaguuucaggaccagauauuuucucccgauuggucccaauggaggcacacgaagcagcuuccuuguacagcgagaagaaagcucagagauuaagacagaucggggaacuuauugaaaauaaagaucaaacauuggcugaauuuaugucgucaaugcagcuagaucuauugaccaagaugcaccaggcuacuggaauaccgcaggaguugauugauagagcagcggcucuaucugcuaaaccuaacgccauucaagaucuuauaagugcuaugggaaagcuaucuaauauauaccaagacguugaagcaaguuugaaugagauugauucuuuauuaaaggccgaagaacaaagugaacaaaaguaccaagaaacgauugguaaaagaccaccgagcauuuuagcuacagauuuaacuagggaagcggcaaaauacagggaggcucauacuaaagcgaacgacucaaaccaaacuuuacacagggcgaugauggcucacguggcuaaucugaaaauacuccaacaaccgcuaaagcagcugcaacaucagcugcccuuugucgaguuuccaaauccaaauaucgacgaaaaaucuuugaaagaucuggaagcgcuaguugcaaaaguagacgaaaugagaacccaaagagccaugcuaugggcucaacuucgagaaucuauucaccaagacgauauuacaaguucccuuguaacgaaacaaccaaaucagucgcuggaacagcuguuccagcaagaacuucaaaagcaucaaaaucugauuucguugauugaacaaaacaccucggcacaagaaaacauuaagagcgccuuagucgauucuuacgcuuacgcuguaaauucaagaaaauacauccaagauauacuccaaaagagaaccacaaccauaacgucacugauagcaucguucgacucuuacgaagacuuauuggcaaaagcuaacaaagggauagaguuuuacucaaaacuugaaacgaacguauccaaguuacugcaaagaauaaggaguaccugcaaaguucaacaagaagagcgagaucagaugaugucgacugcgcaagugccucaaugggagagucauacgucacuugccgcuccuaaacugaaagauuacuuggacuccaggaagaagagugcugcguauucggagccgaguguucaaccacaacagccaacuuuaaguuacucagcugcuauggaucugccuccugguauuaggccgacuccaguuggaucagaaauaacggauguaccgaaaaauauucaaggugaaccacaagguuauauuccauauaauuaccaacaaccuucuguuccugccucacagaauauugaugaagagacuauuaaaaaaaugaacgcauugaugccaggugcuaagacgucagugccuagucaguacggauacagcaacuacauuccaccaacauacccucaaagugcguaccaaccagguaaucagucuuacggaaaagaaacuccagauauuaacucaccguacgacccuaccaaggcguucacggcuacuacuaacgcuuaucguucggugcagagcuccucaacucaaggauacguaccguacgcagaaucuaacguuucgaauguugacagaguuggauauccuagcagguaucaguaccaacaaguaccugagauagcuacuacuccagcugaucccaauauuaaugcguacuacccacauggguacucaccgagccagaauuuaccgaaugcuaauacucaacauauuaccggccaacugaaguaccauucgguggaguacgcuucuucugugccgaacaacaucaauuauaacagcucuaccuacucgucgccgcuuucuaauaugucuaguaccaauuccucaaauccuaguaacuugaauaauucuuacgaguacuacuaugacccgaauaccaguaguggugcaguaccgaaugcuucaaagccucaacagucgagcgccagcucugcaaacccgaguaccgcuaugaacaacuacaauuauuacuacaauacaaguaccagcgguaguguagcagcggauacuucaaaaauacaacaacaacaacaguacccagguacucagaugagucaagcgcaguacuaucccgccaaugccaguuauuacucaaccaguacuuacaauaccaacguccaaggugguaccaaucccucguacgcaacuggacaaacauauaaucaagugacaccagugaccucucaaaauguuucucaaaauuacaacuuuaaccaaguugguucuggagcaggacaccagcaucaguacuacucguccgcuaacgccgcaguaccaucccaacaagcuguaaauaacaguucauuaccaaacuacggauacgaucaguauuacggcaacaacuauaauuccagucaaccgaguaccuacagcgcaaaccaagcaccuccugcagcacaagcugcuccaaguaauauuccugcugccaccaaauccuccucuaauguggaucugcucaguggcuuggacuucagcauaagccaagcuccucuagugccucaacaaaacauuacgauaaaaccccaagaaaaggaaacaaaaccaccggcuguuucuucugaaaccaaaaaccaagauccaacaccaguaaccacgcccaaacaacccacuggaccagaaguaaagcgcuuguacgucaaaauccugccgagcaaacccuuaaacaacgaugaugugaagaaauuguucggccaagagcuggacagguaugagaaguucguggagaccuugacccacaaaacuuugagcgguccgaccacucuggauauuaaauggaaggagauccaagaccagcaggauugcgagccgcagaagaagaucauuuccgucgcuagauguuauccuaugaagaauagguucccggauaucuugccuuacgacuuuuccaggguggaguugugcgauaguaaagaugauuauaucaacgcuucauacauuaaggauaucucgccauaugcuccgucauuuauuguuacacaagugccguugucuucaacuguuggugauauguggacgaugauuagagaacaacaggucgaacugauccucuguuugguaaacgacaaugagaucggugaagauauuuacuggcccaaagaaaaaggcaguagucuuaacauacuuaacauggucauaacguugcaaaacguuauaguuaagucucauuggacugaaagacugauagcgauaaacuuaccugaaaaacgggagucccgugugauaaugcaucuacaauuuacaucguggccuggcagcuuguuuccaacaaauccugaaccguucgucagcuacaccuuggaauccaucaaccuauaccaacaacagaagaccaacacccauccgguggugguccauuguucaucuggcauaggaagaagcggccugcucuguuuacugacagcugcuauguucgaugcugccaacaaugcuaacucgauaccagaucuuacagcuuugaguaucaaguuguccaauugcaggaagaauauucucagagaucgagagcauuugaaguuugguuacgaaaguuuuuuggcguauauuaggcauauaguuugugaagauaaagccagaaagaaacugaacgagauccagcccaagguuaaggaggaaccacuggaaccaccugucauaguuccagaaccaaauauagauccuuuaaguacuuuagacccauuuugggcuaguaaaagauaagcuuuacauaguaaauauuuauacaaugauguauuauuauuuugaauguuaucuacaccuucauuaauauuaaauucccug

SEQ ID NO: 211 - RNA, 633 nt, Diabrotica virgifera
uaccgccugcuacucucuuucuuugaccuccuccuuuucuucuccuuuguccggcuuuaacuugcguuuucccggcuccagucccgagcauaccuucuccggaguuuucgguucuuccgguucuuuccaaaguacuggggacucucuuucuucuuugaauccaaugacaacucuuucuuucggcggcuucuuaauuucuuucuuguucuugcguuucgucggcuuuccuccgcauaguaacuucuuuccacgccauuuggguuugaacagcuacugcguuuacuuccggguaauuuuguucauacacucccuauagugucugcauaacaucuggaucuuuuauucuuuaaacuggagcuuuuucuucaccuuaagucucuaaaagucuagaggcuuaacuugucgguucauuugcuggaaucuccguuuaagcaguuugguuggaacuucuuccauagguuuaugcuuuuguuuaagcgguuugaaguuuucuuccgucgacuuaaauugaaggcauugguugaguuucaacaguucuucuuucuuaaguggaaucuucuucuucuguuucuuuucuuuggucugaccaguuucuucccucugcuuuucuuccauguucuccgacuucguacu

SEQ ID NO: 212 - RNA, 603 nt, Diabrotica virgifera
uacacacuucuucuucaacggcgaaaucagcaucuguuaccuaggccauacacguuucgaccaaaacgaccccuacuacguggagcacgacauaagggaaguuaacaaccugcggguucuguagucccacacuaccauccuuacccuguuuuucuaaggauacauccacuacuucgaguuucauuuucuccauaggaauggaauuuuaugggguagcucgugccuuaucaguguuugacccuacuauaccucuuuuaaaccguaguauguaagauguuacuugagucucaucggggucuucuugugggacaagacaacugucuucgaggagaguugggguuccgguugucccuuuucuacuguguuuauuacaaacuuugaaaguuguggggucgguacauacaacgguagguccgacaugagaggaacauacguagaccagcauguugaccauaacacaaccuaagaccacuaccacauagggugugacaggguuagauacuuccaauacgagaaggaguacguuaggaagcaaaccugaaucgaccaucucugaacugacuaauggaguacuuuuaaaacugacuugcaccgaugagaaag

SEQ ID NO: 213 - RNA, 2742 nt, Diabrotica virgifera
uacggugaagcuaaucuauauuuuucuuucgauugucgagcgagucuggcccauuuuacacaccuagaagugggaugucuuggaaccuacgacacaagagaaaugucgccuuuauauuugcaaaccuuguggcuuuuagucguugaccaauucugaaaacuucauacacuacauggacaagccugucgauucaaaaacggguccuucuugaccuaucagucacccagacuacuauacgucuaagcucaaaaguuaauguuauggaaucuagcccauguaagaaaacuccgaguaagccuaauacacucuacauaacagcaugugggauguguuggaauauauaauuguucaucacuacuauacgaauaguucgaaaccuuaacccuuuuucguacccgaacagucguucaaaagcuuccugugugaguaauauaauacguuuagcgguauuuagguuuucuguuguuguguaaacggucacguagggaucuaucuuguaacuuucauaccguuaacccucgcaggugucgcuuaaagugugaucuuccaguacucuuuccgcaauugacacaccugauaauagugccaccucuauuuggaauaaauuagaguccgcgacuacuaucuaaucauuuuuagacccuaauaguuuuguuuugaacacaaguuugaaaccuuccuguacgaguuuuacauuggcgacguacaaagguaggucuugaaggacaucgagaaugaccuucacuucuaccaugacagucucacaccguacgguuguggguauccaaucuuucaucgaauuuaauaccgaaacuuucucauaccugauaaaagacggauuucccuagguuauugcaccguaacccaauacuacuuccaucguaaaaccaauuucaaccaucucuucuuggucgacaaucauaccuacggucaccuccguuuuaauaaacccggucugugagacuugaaguuguccguuuagaguuccgcaaucgacuuccacgccuuuauucucuaccucuugcggaaggucaaagacauuuucuauacccacgaacgcucuauaugggagucuguuaaguuguguuaggguuaccggcaaaacaacaacagacaccccuaccucuuauguauuagaugugucguuaccgaaauucuuuguuucgcaaaccaucgcguguucuuaaacacacccgaguucuaaggucgcuuauacgguagucucuuaggccuagaugauagucuuaaaaauucuuaaaguuucucuucuucuuaaaauucaggcuaaaaccucgacuuccauauaugccaccuauggaaaacccucaguuuagccaaagaccaaacugaaagauacuaacccuuugagagcuaaaucagucuucuuagcucuauguugguuuucgucaaaugaccagucuaucaccauuuaaucauacaaaccggugucuucuaucgaugaaauaagaaagaauacuaagacuacuucaaguuuuucggucucuauuguuaguccaacgccuacuaccucaucuuagccgaaaguuagaagauccacuuuauuugcuuagucacgcuugaccagagacccauccgcugacaaaauagaugugcuuaagacaauuagcauaguugaugaagcaaccuccacuugaccaauguuaacgaguaaaccuggccggaaacauacagaacccuauacacggauuucugcuaucuaauauggagcaucuauuucucaacgcgcaucauucgaugguuaaugaagaaagacaagaacuuauaguuugacggcaguacucuucucugaaagguugucgucugucucaugaaggcagguaaggauuccucgugucuugcucucaccguguaaagaaucuuuucguuccgaaguuugucguucgaaaccggcauucaugucuaggucucgugucuaagcucgaccgucaucguaaucuccuagaauuauaucgguuuugagaucgaguucuucgcuugucaggcguuuucaccuuaguugaucgucuuaaccgucgacgaugauuauuacauucgcaucgguuccuuacauacguuuuucgcguucuaauaccuccgaacaacgaagaacgaugcucgaggccacuacuuuuaaaucaggcaugagauccucuuugcuguguucgacuuucguuuguauugaaucguaaaaacagugugaacaaucauccacuaaauuuguuuacagaucuguaagaauaauuauggccaucuaacggucuucgacguaaaaagcggucuagaauggaaggacuauucuaaugucuucagcaccuugacaccuucugagucaauagaagucaguuaguuuuucgaccugucucggaacggcuaggauuuuugaugcuuuuagacaagggaccaaauguucuccgccaccaucgagucuuuaaaaaccuugucgucuuauuuccaaaucgcgggcguucucaacgguggugguaaggaggauuagugcuguccuuacaacaucggcuucaaguucguguuagcuuugugcuacaugguaguaaaucaagaagcaaauaaaguagucuuuaucuucguguuuguuccucaagacgauuuggacuucuuagaaguuuguaauaugucgaccugguucuacugcugcuauagcuaaaucuaaaccugccacauuuauagcuacucuuguaacugugcugccuauaguuguagcuacuacuaaacgacucacuaacu

SEQ ID NO: 214 - RNA, 1173 nt, Diabrotica virgifera
cacaauaacuuuccguuuuuaguuuauuacgucuagaaacauuuuugugagugaccauuuugguagugggagcuccaacuugguagucuaugguagcucuuacaguuucgauuuuaaguucuguuucuuccauaagguggucuaguugucucuaauuagaaacgaccuuucgucaaucuucuaccggcaugagagagucugauguuguaagucuuucuuagaugugaugugaaucacgaagcagaaucuccuccauacguguagaaacauuuuugagagugaccauucugguagugggaacuccaacuugguagucuaugguagcucuuacaguuucgauuuuaaguucuguuucuuccauaagguggucuaguugucucuaauuagaaacgaccuuucgucaaccuucuaccggcaugagagagucugauguuguaaguuuuucucagaugggagguaaaccaugaagcagaaucuccuccauacgucuaaaaacaauuuugaaauugaccuuucugguagugggaacuucaucuuggaagacuaugguagcuuuuacaguuucgguuuuaaguucuguuucuuccauaagguggucuaguuguuucuaauuagaaacggccuuucguuaaccuucuaccagcaugugagagucugauguuguaaguuuuccuuagaugggagguaaaccaugaagcagaaucuccuccauacguuuagaaacauuuuugugagugaccauucugguagugggagcuccaacuugguagucuaugguagcucuuacaguuucgauuuuaaguucuguuucuuccauaagguggucuaguugucucuaauuagaagcgaccuuucgucaaccuucuaccggcaugagagagucugauguuauaagucuuucucagaugggagguaaaccaugaagcagaaucuccuccauacguuuagaaacauuuuugagagugaccauucugguagugggagcuccaacuugguagucuaugguagcucuuacaguuucgauuuuaaguucuguuucuuccauaagguggucuaguuguuucuaauuagaaacggccuuucgucaaccuucuaccggcaugagagagucugauguuguaaguuuuucucagaugggaagugaaccaugaagcaaauucuccuccuuuaauu

SEQ ID NO: 215 - RNA, 1131 nt, Diabrotica virgifera
uacacacugcugcuacaucgccgagaacagcagcuguuaccgaggccuuacacguuucggccaaagcggccacuacugcggggagcacgacagaaagguagguagcauccagcagggucugugguuccacaguaccacccauacccaguuuuucugaggaugcauccucugcuucggguuucguuuucuccauaggaguggaauuuuaugggguaacuugugccuuaauagugauugacccugcuauaccuuuucuagaccguaguguggaagauguuacuugaaucucaucgggggcuucuuguaggguaagaaaacugacuucgaggugaauuggguuuucgguugucucuuuucuacugaguuuaguacaaacuuugaaaguuauggggacgguacauacaacgguaaguucgacauaacagagacaugcgaaggccagcauggugaccauaacaugaacuaagaccucuaccacauagggugugucauggguagauacuuccaaugcgagagggugugcgguagaacgcaaaccugaaccggccaucucugaacugacugauggaauacuucuagaauuggcuuucuccaaugagaaagugguggugucgacuuucucuuuaucaagcacuguaguuccuuuuuaacacgauacaucgaaaccugaagcuuguccuuuaccggugucgucggucgagguggaggaaucuuuucucaauacuugaaggacugccaguucaguagugguaaccauuacuuuccaaggcaacgggacuucgagagaagguuggaaggaagaacccauaccuuagaacgccauaggugcuuugacagauguugagguaguacuucacgcuacagcuguaggcauuucugaacaugcgguugugacaggaaagaccuccaugguguuacaugggaccauaacggcuagcauacguuuuccuuuagugacggaaccgagguaguugguaguuuuaguucuaguagcgagggggucuuucuuucaugaggcaaaccuagccaccgagguagaaccggagggagagguggaagguugucuacaccuagagguuuguucuuaugcugcuuaggccgggaccuuaacaaguggcguuuacgaagauu

SEQ ID NO: 216 - RNA, 2640 nt, Diabrotica virgifera
uacccaugaaaauuuucucuaugaguacuacuccugcccccuaguucacgaaaaguuuuagaccucuuuugaugacaaaacguccuucgaucucaaaaauuacuuugaucacauuuagguucuuuuacauguggcuaugauuguuuugacaacaugaauaacuuggucccacuuugaaauucacgguuucuccggugucuacaaaagaaacgguacugguuugacaagguuaguuuucuacauuauaacucuuccuaccaaauaaacccuuaauuucuugagucaagacaacgacuacuacaguaauaacauuguaggucagaauguuuucuauacugaccauuucuucuguacaugucucgucgacgauauucucguaauacgucauaaugacuacgaugauacgaaguucgauaucuugcaauauacuucguucgauaacaucuaucuuugcgucgacagucaagucgucgugauuaaucaaguaauguauacucguuuaaucgaggucuacaucauuuuucuacccauuuacuucgaguccuucgucauuuaucacuauuacguuaccaugucauagugcguaauccagaagauaugguauaauccuucugacuauucgaucgucacuguuuuaacuaaagguucgacuuaaguuacccaaauuucucgggaauacgaaacacauacaacuauucuuagugacguuuugaaaaucuucuucuccugguucucagugaggaguugagggguauauguuauuauaaauguuacccgaauuccuuguuuagacuuuaccaccacauacuucgacguguacgguaccaauuggacuucaagugcucaucauuacacgaucgugggcgauauucacaagauguugauaaaacaccuagaggauuucggugugagucuaaacgacgacaaucuugaaauuuaguucaccgguggugggugggacgcagucacugucgaacauuaaaccuagaucuuuuaaacuaaugacuaggauuauccaguuaacgaugugaccgguaaugaugagaaaacuuuuguccacggcuuagaagacaacugucugauuacuuuguuuagcgaugaaaacauagacuuuagucacuacuuaaauuucaccaacaguaaguccguuaauuccauaaucgaaacuuuaaagguuccuuuguaucgugcgaauacuuaaaggauaggcgguacaauucucuacucccuccaaaucuuauauuucguagguaucgucuaugguaauauugggauuagcuucuauuagggcuucgauuucuuagaccaaaccgcguagaaacgcucaaguaacuucugacacuuguacaaagaaaccgacacucuuagaacguaaacaauccuuuccuuccuggguucugguuuguugguagcucuauguaggcaaaauagauguuagcgcaguauaaccuuacaggaagacauucucgacgacgucagaggcgguaccguguuaagccucggagaacagggcuaaacaaucuuuuauagguuuauaaugaaagcuccacagucuaccuaagucugcuacuucaaucccugucucgauguauaauaucauuauaugaauuguuuuuacuauuuucaaauauguuguuaauguaaaaccuaagaaacguccaaaguuaaggaagugaucuuucuagcgaaucucuuauguaaguuuuagguugacugcuugguaaacuguaauucaggcauggacaucgucgucacgguugucgucuucuugcucuucaauuuuuguuuagacuuccugacgaucagagaguuccaggucaggcuggaggaggccacagaucucuucuuuugaagcggcuuuuugaaucauugcaaggcccauauguugucaauccuggaaacaaguuuugaaggcugcagcaacuugagugacuuagacuuugucucauaaaacaggcgacauaguucgugacaaaguuuguaguguagcaggagguuaagcuaacagacuuauggaacggucuggucgaaaaucuuuugcaaucucaccucuaucugcggccacuuuggaagcuuuaaaaccgucuuuauggaacacuuuucaacgugauauugcuuuggccaugguguauacaucaucaauucaacggacuacuacuagagggguugagacaaccaugcacaccucggcacaacuucaagaaucacuuucuaacacuagguaguugcccuuauggucuaagacuacucccaaugcuacuacuuauaugugaccuucuguagcuuuauuguaauccccugguuuaaguuuuucauucguuucauuuaacccgacgucggacccuucuucgacgucgaugaauacaucuuuuucuccuauguaugaggaacugguaguuaugcgauucaccgcgacaauucuuauaauaagucaagaacccuaaugucggacgccuuuccugacugucucauggccucccauuuagaugcguguguaaugaagaacgaccacauaaguccccuccauaacuguaugaucauucucgcuuugaucgaaacccgcuuacacaaugcuacguugauugucaguccagcggucuaggacugcaacgacucgaauauugaaguugacauccaauu

SEQ ID NO: 217 - RNA, 651 nt, Diabrotica virgifera
uaccgccguuugucuugaccuggacgagucucugguuuaccgcgauggguuccuuucuauacagucaaguuugaccaggaugauccgcuuucacggcagccauucagcucaaaccaugacuccaagcaguuuccugucaaggugcuuaugguccucucaugguauccucgucgaaaggaauguguuugguauacggagcugcuauguugacaauuuaaacuuuaaacccugugucgcccaguucuuuccauggugucaaaucgaggauacaugauauccccgcguguccgucgauaucagcagaugcuguauugguuaguucuguguaagccgucccgcuuuugcacccacuuccuugaaguuuccguccggucaggcugcuagcacuaucgaaaccggccguuguucguucuaaaccgguuguuugcauaccaucuuaugcuucuccgcgucugcauacgacugcuuuugccgaaugaaaaauaccuuugaaggcguuucugccguuacuugcaguugcuauauaaaaaucguuaucgauucuuugacggguucuuacuuguuugguguccaguuccgccgucacggguuccguccgccgaucgccucccgcuaagcccgcgguuccgugggccuuuaacaacguucacu

SEQ ID NO: 218 - RNA, 279 nt, Diabrotica virgifera
uacuucaaaaauucuagcugucacacgauguaacgguagaaccguuaagagaaaugggagacacggcuacuccaacuuccuuccucuuuuuaaaacuaccccgcuuuuucguaaugguccuguauagaagcaccuuuacgacaaggacgcauacacuauuauuaggaacauccuuaaccaguuuaguaggacccucccuauaacaugcaacguaacuccuucuucuaguaacgacguggacauugccguaguauacgucaccgaucuguucuugguauu

SEQ ID NO: 219 - RNA, 474 nt, Diabrotica virgifera
uacgucuagaagcaauuuuggaauugcccauucugguagugagaacuccagcucgggagucuaugauagcuuuuacacuuucgauuuuagguccuauuucuuccuuaagggggucuggucguugcagaguagaagcgaccuuuuguugagcuucuaccagcauggaacagacugauauuauaaguuuuucuuaguugggaagugaaccacaacucuaacucuccuccacgauucuuugcauucuucuucuuaaugagguggggguucuuuuaguucguguucuucuucuuccaauucaaucgacauaacuuuaaaauauuccaacugcuuuuaccauuuuagguggcuaacucugcacuuacggggcgacuuguuacaccucgaccacagaaguaccgucgguaccuucuguccguaaugacaccguucacgccaaugugagaacagaagagguuugguccucuacucuuuauc

SEQ ID NO: 220 - RNA, 747 nt, Diabrotica virgifera
uacuacagguuucgucuguguguccuucuacggaggaagcgguuuaaccuuuuagucuaacgauaguaguuuaugcauuaugagaaaugguugcaaaacguuacccgagagccacgucguuagaagcgagaaacggaaaccgaugcuaagcuccucccguaaguucuuaccgaggucuuuaaccuaagucuuguuaaaauguagccucauauacaugaauaucagcgaagugacuagcaguacuaacacaggaaauauccuacauaaucacgggacguccucucaugguaccgggaaaaucacauguagccguggguucacgagucaaaauauaagccaaauaggccaagccgccaagaagaccuauugucgcggucucuaagggugaagguuggcuccuaggcucucucauacgcugcagaauaguacuuacgaguagugcugguuaggucuguuugugaucgguacuaaguccuuuuacaaccaacgacgccucgacuaccgcguugucugauggagagagaagucgucggggaagguucagucacgucucuguggcaaugaccuuuggguaagaaggugccuacacaucuacuugaguggaccaagaagcuucuuuuuacaccaaccuaucguccaaaucgauaccgcuauacguacuaauugcaggaaucauaacaaaauagaugccaugaguagguccguaacuuuuuucuucuucuucguaggcuaaguauguccucuauc

SEQ ID NO: 221 - RNA, 375 nt, Diabrotica virgifera
uacagaccugcaccguucccuccguuucauuucccuuuucguuucagggcuaguuuagcacgaccaaauguuaaaggacauccagcauaaguagcaaauaacucuuuuccuuuaauacggcuuucucaaccacgaccucgaggacauaugaaccgucgacaauaccuuauaaaucgacgacuucaaaaccuuaaccguccuuuacgucgaucucuauuguuuuucugggcauauuaaggaucuguaaauguuaaccgguauucuuuacugcuccuuaacuuguuuaaugacaguccucaaugguagcggguuccaccucauaacggauuauauguucgucaugacaauggauuuuuuugacuuuucuuucgaauu

SEQ ID NO: 222 - RNA, 864 nt, Diabrotica virgifera
uacuucaaccuaccacaucuagacgggggugguuaaucgaagcuguaacgccuucucguuggcaaugguggaacgguugucugcaagaauacauuaccacuaccuccuagguaucacgcugucaaagagcucgacauaaagcauuauauacuaagucuauuauccgucagggaagaaguccguauagugcuuuuucgguguaaaaguuacuguuaccggaugggcaugccgauaagguuucugucauuuccucauagcaccaacuuaaccauacgguggcuauuaucuuuaaauaaugcucaaguucuaggucugucuucuuuguucaacaauucugucccuguucaacgacaucaaagcaagaacguucuauacggcgugugcuucgugcuauaagugucaaaaugucaucuaaacugucaaaaauguggggucuacaauacaaacugucaccgaccauacaaauuucuuaacuuuucaccgguguuucauggaggaaauucuauaaagaagucuugggaacauuaacauggacgaccuaguccaaaaacguaucguuuacuucuugaaguguauagguuacguugaggccugguucguuuucuacgaaaguucugguggcaauuacaucgaggccguggucggggacacuaauggagaggaccugggucauaugguguugggcgacacggucuacuacgauguuuuguucuuuaccauuuugucuacaggcgucauaggccuuacuuagagcucaccagcgaugucacagagcuucuuuguguuacccugauggucuuucgguauuaccauaagguuuuaaauuugcguguuccacaacaugguguucgucguaaauaauuu

SEQ ID NO: 223 - RNA, 2868 nt, Diabrotica virgifera
uacugacgccaucuuguuggaacaaugugugauuauuugaacgguugucuaagccucgggauguuacuuuacguugauuuuuaccuaaaucuuuucccacuccaauuucauuuuuauucucguaaucuuuuuuauuaaguguacuaagaccguccucuuuccaacggcuuaccuaaagauuacugguaguauucuuugcaaaauggaaauguucuaguaaaccguuuuuuugauaauaacuaaaagacccuuuaucaagguuuuuguuuaggucuuccauuugaugauguucucuacuaaaaccauacacuacggauaucuuuucuagacguuguggguuuacuuaaaaacucuccaagaugugaagcgaagaacacguuugacuuccuuggucuuaacaaccuugguaauuacgggucauaaucucgaacaaaccuaguauccgugucgauacacuccuccuuacgacaugaccguuaaaaaugguaaauguuuuuaaaacuucgggaguaaggucuacgaggacuugacuagagguuaauaaaccuaccacucguucuguacagaacauuuucuuuacgcaaaaauuacgaagaaguacgacugguucuuucccgcaacagcauaaaccguaguacaaaucuaguucauuuaaguaaaccucuauaagauguugaccaguagcaacucaacuauauauuccacacaguaagguuaggacgccuuucuagaucuaaauaaucuacauauauauugaacaacuugaguucgucaggacgacaguccaugcuucgacguccuugaaaucagugggagaggucacggggcugacggcaauuucgacgacgaucgacaauguaacucaauuaauaguuucuuucacuguuguuacauuuugaguagcaaaaccuguccgacuaucgugaauuccucgaaggauuagugcuuucuuaagacguccuaaaucaauaccuguaugacucucaugagagacgaggacugaaucuucaggcguucuucugaaauucagaucgggaacuuaaucagagaagugccuuguaucuucuuuaccauaaucauaauuguuuccuucacucauuuugccaucugucacuuguacuccuauguccuuucauguccguuaacaaucauuccugagauguaagcacaagguaauucaagggucuauagcgugcaucacaauauggucagaacuaacuuaaaaauaggcuauuauuacuugaccgacggugucuacauaacgacaagaauucccuucgguaugucuucaaauuucuuaacguuggcaauuaauaacucuuugaguagcuuugaaaguuucuguaauuuaaccaguuucagguaucucgucguuaaaccuaaaacccucuuaugcgcucaugacgaaggcuauaucuucaauagcaaccucuuuaauugucuaacaacccacuuccuagggagcaacuucgacucgucuucaauuaucguccucuaugccuucucuuacgaggacguggacgacguccgcgguggugaaaucaaugaaggcuaccuuguauacgauggguuagucgaaaguugugacagucgguuuggugauuucuucgugcuggaggagauucuguuauggaguaccuaccacuaaaaaaguagccucggagaaaccguagauguaauugguuugacagaaacgccauacuccuggaguggagaggacgacgaucguuaccuaaguuacgguuuuaauacgaauaauaccgaccuuaagaagugaacccuuuuaguccugaaggguguuuuaguuauugguugcugcuauuucugguguaagacaagacaaaugcucaggauagacuagcaagagguuaguaacaacuuuaaaaguuuuuuaacacggcgagccgugauuuacucuacgaagaucgauuccuuagccaucuucgcuagagcguuuucucguuucuuuuuuuguucgcaugcuaaguuugacugcugcgauauucgaaggacguuaaucucugucuauuuucaccucucgauccucuuuugcauaagcucuacagcgacaguguucgaaaucauccuccagcuugcccuccaccgcuuagucauaauucaagguuauuuaaucuauuuuaguguguugacugaccaaaaaggcuaggucaaauaaggcuucguaugcaagugcacuuagucaugcuauagcacgaacuacagaauuagcauuugguuugauugcuaugaaauguuuugacgugcgaucucgaccgaugaaauccgcuaaacuucaaccaucucuucgguguuggacagcauaaccgcggguuucugaaaacguuguaauuucgauugcacuuucaccggaguugacuuuugccuuaauauaaaccguuguaacacauacuacaguauccucgccccagucuauccuuacaacaucaaaacuuacuauauguguaucuauauuaccugauauaucacggacgaucaacaugucuaucgcucaaauacucuuacacccgccuuaaacuuacccuuuuauuccauuggcaauuguguggggagugccuugaaagucuuauggagcuuguagaugaguuuucguguuuaaacuuuacaaauuguagucuuuuucgagacucgcccgucacaccaaaauaccgucgguuaaauauacguuuuagguaaaaaccucuucugcgaaaccgguugaauucauaucucuuuggaaaauuauuugggcuacgcggucauucgccaguauaaucuuauucccgguuuucagucccguaccggaauucaaauccucuguuucaguuauacugugucuucucguguguuguauuucaucaucgacguauu

SEQ ID NO: 224 - RNA, 549 nt, Diabrotica virgifera
uacccauuacacaaacguuuaaauaaguuuccggagaaaccguuuuuccuuuacuccuauaacuaccauccugagcuacgucgaccauuuugguguuaaaauauauuugaauuuaauccucuuuaacauuguugauaagguuguuaaccuaaauuacaccucugacaucuuauauucuuguaaucaaaaugucauacccuacauccaccaguucuauuuuaauccgguaacaccucugugauaaagguuuuguguguuccggauuaaaagcaucaucugucauugcugucccuugcauagugacuccgauuucuacuuaauuacgcauacaaccggcuucuacuugaaucucuacggcaugaagaguaaaagcgguuguuuguucuaaacggguuacguuacuugcgacgucuuuaguggcuguuugagccagagguaagugaugcguuggcguugaccauguaaguucgauggacacguugaucgccucuaccagagauacuuccagaccugaccaacagguuaguuaauuucuugcgguuagcgauc

SEQ ID NO: 225 - RNA, 4425 nt, Diabrotica virgifera
uacccugccaacgugacaaauaaaacauaaaaggauacaaaauggcaguaguugugcgucuguugcuuauauguaccuaagagccuuuuaaggcaccuauguaaagauaguggaguacccuuuucacguuuuaagcacgugguuuuaguguuuggguuuuaacuuuuaacagucuugauguuugggagccacuuucuucuugucgguccgccuugcaugcauuguugccaauggcgauagcuacugcuaggaucccucccuccuccuuguuaaucaauguuugauuaaguaucucuuccucuuguacaaaauaaacuguaucuguugcaaugaccacaaaacuguugauaggucgguaaacuagcccuacuuggucauuccgucuuccuugaaauacauuggcauguucgaagucuguugccguccggugguaaucgucuacagacauguaaaugucaaugguaauggcuguaauuacuauuacgcggugucgaacuauuugacuuuaugcuacguguucaaagacuucuaaauuuucauccuucacuucacuacucucaaaaacgaaugcuguaacuacuaccccuuuuaaguucuaauagcauauugaaaaguuugcuuuuacgaguuaagugggucauaaaguccuaucuagcucuaugaccgcaacacauaaauuuccuucgaaauugucuguuuuucuuaugaucuaaauugucacgacaaauacaucggcuauuaccgcaauugcuaguucuuccgguuuuucuaaguuggcgauucuauagauauugucaucaucccagacuauuugucggagggucuaaaugaguuuuuuacggacuaccuuagaaccucuaggggcuucuaaaauuucugaaaagauuuguauaacagugucagcuucguugcagguuguaacgccuagguguugaacgaaaacuuaaccacuucccuuucuguauaguuugguuauuucugguuugcaaagaaaaccuccgucuuccuuuauuucgcguguauuucgaucacgcaggugaccuaauacuuugucauugccuuauaugagauugauaagcucauuuuuuguuucuaaauuaccuaagaagguauuuauaugguuaauuucauaaucuacaauuacuacuuuaaggauuaaaggaacuuaaagaauuuccaucacagcaccuuuuacuguucgguccacguguucgcuaaguucauucucguuagcuauuucugccuugacgacgauuguuguaacacucgauacuugagcaacuguuaugucuaaacaaacguuauuuggcuagaugcccucauuaaugcagcucucaccucaaacuagcacuuugacauggagauauagugcauuugcaauuucgaauacuauugagaggcagacgaaacauauugugcuguaacggauuguaacauuaagucuguaagguuuagucauaucuucuaguuuuacuguuguuuggacauaaaugaguagguuaaauagucaagucauuauaaugacucgaacgacuauuuagcucauaacaaccacuucaguuucgaaaucuauuacugugccgaagucaauauucaauaucauaauguuuaccuuuauaacugcuacgcaaauacuaacuuuuaagauggccgucuuauucucaauuaccuuuugaccuaaugcucuuuuagcuuguuauguugaauuggcaagcgcguaaacuaccccguaaacuucuaaaacguuaacaaaauuaaagguaugaauuacuuuuacugcuuggaggucaaaaacugcugauauagucucuuuaaguuuaauuucuccuucuuggauacuauaggccuacgcaacaaucucacugacgaguacuaggucuauaauuucuguccguacgacuaguuguguaucauauacuccagcgcuuucuugucuuucuaaaaaacuggcauagacggcuaccuacgcauguucauuguuuuggagagcuggcucuaggcggaaagccaucggguugugcuguucagaaguagauacgagcacuauuacuaccuccguguuuaaguaacaaccggugacgucuuuaacuuuaauaaaauuaucuauauuugcuauuacgagggaaaaauuuacaaugucuuuaacaaauaauacuuuugguccuagguccaaaauauccauuggauucacggcuacuaaugcuaccaggacuauuaccuggaggcaaacgaaaagcuaauagucugugacgaagucuaucauaaucuagcuuuaaaagguaauagccuuuggucgaaaagcgaaaucuuuacaaacuaucucuucucguuuuuauaauacuguaacgguaacuguaaugucuaucaccucauggaggugauuguccuugaucauaagaaucucaauauuagccucuacauuuacuauuaggucgaugucugccuuugucgugcuagaaacacauauucaugcaguuacccggucuuuuaaaguaccuuuagccugcacauauacaaugucuggaucugcuaacccuaaauuuacuguuucagaaacaaguucuucuauugaaacuacuuaaacacaauuuggucguauuguugccauacuaagacuacuuugguuguugccgacucccuugaauacuccaaguaaugucccagugacuuuggguacuuggguguuaugugcuuguaugucaauuacguuaucagugcuaaugucaauuucaugaaggucuccuucgccaacauuuuaguccuaguuaagcuaacucuccuuguugauuccuucuuaaguaucuuuuaaguaacuuaccuuucucguuuucucuguauaaugugguucuugagagguuuuauaauuuauguagaaaucgcuuacaacuacauaaaugacaaaauuuaagugggguggucuuaucaagcaaacaccuacaagcuaaaagacgaguaccuagagguauaauacgaggucucuuugagcuuuuguuucaaugucuaguaguuuaccucgaacuuguuuuuaaucuacaccuuaagauguacuaguugcauuugcucacggaauugcuuuguugcacaccucgacuuuugaguacaugcuuguuuaauuuguauugugcucuuggucgacaucacaaaugauugucuuguaggaaacagccacauuuacguaaauaacuaggacacacacggcgaaaugguucucuacaauaccuuacaaaguugccuccgcaggaauagcuuuugugucgcacauuaacaggacguccuaaacuuccugguguaacacuuuaggaucgauauccuaaauguccuugaccaacccgauacauagguaggaaacugcgauguuuguccugacucuaauaugacguauaaaauaguguuugacuauuaccaaacuauaaaauguuaccuggaaauuuauauucuguuugaagaaacagauuucuaauauauaguaaucuugaauuucugccuauagguaaugaaguuuaaacguggccgaguucgugaguucuuuaaauagacuuucucgcguaaguguuuaacucgcuaccuagcaauguguuuuauuuuuauccuagaccuaaacugcuauauagggaccuucaucugcugacaccuuguugcacaaguuaaaccugauuauuugauguauuuccacaauaggcucguuuaccgggggaaguugacccuccauacuuuuugucuaaguggcuaguucuuaaguuugcuuaaacccugguaaacgguggcugacggugggcaaagagaccaacauaaucuuuaaacugcauauuacuuaaaaugauguuggagccacguggaagacuacguaagguucgcauagggcugacauugauacgucacuacguucgacacugaaagccauagcugagguuaaagaaccaacgauaagaccaaacacaucguuaaaacuauuaagaagaagaccgucaucaacauguaucugcauuugugcuguugaaauugcuuuuucuuuagcuacuaugagcgcuuuuguaauaguugaugcuucuacuuccaccgccgcuuacacugugguugaugcuggacagacaaaagguagucuuguuguaacaccugcuuuuugguaacuacucucuguuggggcuacauggacgucuauauucaccgaaaaaucuauuguucuuucuguugacacuauuucuggggcuauuaaacggaauacugcugcaagcgguaauacggaugcucccucugccuuuaucguggccuaggaauagaagagagcgaaguacaugccugcuuccucuaaauuucaaguugaugaauaguucaaaaccugggucuaagucuuucaaucggcuguacauaccucuucuagguucgcuacuucugagugugcuaccuuugcuucuuaggaccacgauc

SEQ ID NO: 226 - RNA, 291 nt, Diabrotica virgifera
uacggaaagacaccaggguuuaacagggagacgccggacuaauagucacguaccccauaguaggucaacccaaaguacccacauaagauaauguaaccccgacaccgaaaucgucuucuauaaggucuccaacucaaauucccgcuaaaucuguuuaaaauaucgcugcaguugugcccaaagugugucuuacgaauguugacgaccuaacgacgagaggauauggacuauuguaaucgucauagucgagugguuaagacccgguuguugucuaguaguaacuugcagauu

SEQ ID NO: 227 - RNA, 540 nt, Diabrotica virgifera
uacccagaaugguauagucgucacaaauuauccaacaaaucauuuuucggauacucuuaaaauuaccauccuaaucuacggcguccauuuugguguuagaauauguuuaacuucgaaccacuuuagcauugauguuaugguugguagccgaaguuacaucuuuggcaacucauguucuuauauagaaagugccauacccuacauccaccggucugcucuuagucuuuugagaccucugugauaaagcgguugugacuaccugaguaaaaacaccaacuaagguugcuggcucuggcauagcgccuucggcuucuucuuaacguguuauacaauccucuccugcuaaauucucugacguaaaacaauuauaagcgguuguuuguucuaaauggcuugagcuacaggugacgacuuaacuggcuauucgaauucaacgugugaaacuucuuauccuccaccauguauguucgguguacacgaugaguucccuuaccaaacaugcuuccugaucuaaccaacagcuuacuuaaccgguucacu

SEQ ID NO: 228 - RNA, 618 nt, Diabrotica virgifera
uacgccaugugaaacucaauguagccacgaugggaucgcaggugacauugugacuaaaaacgggagaugaugacggagugcccuuuuccucucguucaaucaaaucguaccaauaacaacuuacacagagggguguacacccguccagauccuuaaccggaacgacauaguaauagucaacauccucgacgacguccuuaagugugauguccucagucauagcauccucgaccacaauuucgggggucuuaguuuugguuuuuaaauuaaagauaauaaaagacacuucgacaccgauagauacccaauuaauaccgauaucaugagacaccuucaaccuucuuaaagcuacaucuggauaaguuggaguuuugaguauugaaacgaguuuugguaauaccuaguguacaauaaaaaccuaggccaaauugacaaccuaaacauuuagauaauacaccuaaaacacaaccucaucaaccaagaccacgucgguaaagacuacgucgguuaaguaguaauaagcaguuuuaaaacuaauaacucuaaaaaccuucacgguaaccagagaagccagacuaacaaccucauaugaacugcaguucuccgagauaccaaauu

SEQ ID NO: 229 - RNA, 5694 nt, Diabrotica virgifera
uaccgaugguugcuaucauuucgaggcaacuccugucaauuuucucacguuaaaccuuaugaaucaggucuacuuuaaucugcuuacagucagugucuucccccguaggcgaagggucuuugguaccuucguccggcgggguuugauacgccagaauaccuggggucuguuccacaguaucugucuucgaguucuacggucuguacacggccuuuauacugucuuacaggaccuguaaagccuguauagcucgaccguuuuggucaaaaggugcauccuaagcauuguuuuuguuauuucuagaacucuacgcaaacgaagaaaacgucauuuaauaaucagucagguuuauuaggcuuuuaauuucuucaacauuacuuuaguuucccugucggugcauuuucuaaucgaaagcaaauacuagacacauuuccauuuuuauaaacacuuccaccucuacuuuaccuacacccauuucuuucgcuucuaggguuauuuuuucguccgguaccaccaacaccagcuauaguugguuuauagucugcacggccaaaucuaaauugucgucuuaccuuugugcaguuacuucuguguguucuuuucuuuuagcgugauagacggcuugcacagacccuuuaggauuuuguauagugucuacuucuuacaaaguaagaaccauaccuaggguuuaaacgaucuggucuaaccuacuaucauugccaugaaggacaaggaggggaucgucaugcuggacgacaucaauacgugccuagacguuccuuaguccuacuauagugaguguuuaaccggcuguaauaguuccgcuuauugcuuaaugucuucuugcucagacguccacgucggcgaguauauuagugucuuuuauaauucuacaacguuaaagugcagcggugaaaucaacuguugcuauacggcccuuacggcucucguuacguuuuuagaccuuuuggggauuuucgauaguuucgagccgacuuuccauuucuuccuuccuaagcuccauuggaauacccuuucgcacaccugaaaagacgugcaugacaguaguguggucuaggguuaaaugcauagcugguucauccucacggaucuucauaacgaguuuuguacugcaaaggucuuuagcaguguggaaaguuaaaacuguuuuacaaccuuaaccaugucucuccauuaagagucauagguccucgauucauauaguagucucuguuaccucucuccuaacuaaaugcaaagguggguuuuggcagucuaaauguaaacgucacaccaauauuccaucuuucuguguagucucugccgcuagaucauuagaaguuggcaguugguugggagguguucuacucauacuacccggugucucaguuucagaaugggaccagcugcaaggcauacuuagagagcacguggagagggauguugcggcuaaaacugccgcugcuuuacuuggagguacacgggguuucauaccuuugagcucgacuucagcuuuuggagguguagugaggguccguuuaguaaugaggcguucgauugguugggcaguacccauaacauguucuaugcaacugucgacaauccuucuacuguuuuucccuacauaaguagcucuuccuuguuuacuacuuauauaacuacaagaacgguuaaacccuaccauuuuacggggcaggucgguaggaguuuggguuuggcaacaccuguccuuuugucuauaaaagggacuaguaaggaccguuacauuuauacuaugcauggguaagaugcguaggucugcugcuccugcugccagggauauuuaccuauagcgguccucuaugcuuucaauaccaucuuguaccucuuaaccaguacccauauaacacauucuuuucagaaccuuguagucguccaagggacgacguauaaacauacaaccuuaauccugugcuucacacaccaucuaaaauaccauuguaaguuugacauuaguuguugaccaacaacaaucuuccagugucguagccauaaccucugugguaacggcuaggagucugaaugugucuuuaagucucucgguaguccuuucgguuucuucuacauuaucuucaguaggucuuucgaguguuguaccuugaccuuggcugagggccauuaugcaacgcagucugaaagcuuuuaguucauuugucuuaagauuugcugcgagcacuguuuugaccaccaaggcgauucuuuagaaacugacuuauguuauuggauuuccgauaccagcauagcccuagguucccuagguuguaauuauaaaggguccaauaacgaacgcacccaguugucuugcaucuuccauuugcauaagguaaaccgaagucuuuugcgugcaacggcgugaaguaguuccugcuaaugccaggacuuaggucuccaaagcaucuuuuaagcauagaacggccagagugaggaagccucaagauaaaggugcgauacccuccagcacuuccagaauagcuaugacgacauuuuugacggcuuugaccaauguaggucgcagcagacuaguuccgauaccucucacauuaccaugugaugcugccauggcauucuuuaagacauccuguugaauaggucaacucuaugccacuccugccugagacaccucucuaccaucucaaaguuauaaaucguugccaguuuaauucauuguuccgcaaacucucuuuuaagucuaaacuaggcucauuacuuuccauaaacucuucucaaaaguuacuucuucaauaguucguugacuacccaaguccccuucaguaaaggcuugaacucucucuuacccuuguugaggucuuucugucucuucggaauucuguuuagaagggaucgccucuuagguuucaucaugaggggacauuaaauguugcauacuagaccuuacauguuuuuuaaaagguguauuuguuugcucggggcugucuggacaggggcaauucucaauagguuccgcaagcucuuaaugaguccuuuacgcaguagcaucgaccgcuccuagcagacagguuuguucgguugcuuuugcguugcaaugagaaggucacagaucagucuagcugggagacgugguuuacgcaaagacuucuuaaguccgagucguggcuucggaagcucaccaacuauccucuuuagcucugcuccaagguuguucggguucgguuaggaccucuuuaccacccgcgagaccggcgcgucagugacccucuugggcgaugagucuacugugacuugugaaagguaaaacgaccacauaggagguucuugcauugggacccacauggaucuaauuuccuuuaauaauuauaaagguucuuuggguuccgagguagagauuggcacaaaaauugaccacgccgacgaucucuacgccuuuuucgcuucuuacacaauacgucugaacuuguguggugagaagcauuucauuggcgguuguggcgguagauaaugcuaggacuggguguuuuauggcaguaaggacuccuaguccucaagcaauugcagaugauacuuuacgggcuaaagcuaggaugggcauauagcggcaccaacgaagcauagcuugaccugucuuucucuuacugucuauucuuugauugauaccuuguuuaacgacuuuucuaguugcgacccaagccccugcuaaacuuaacauaaaaguugcugcuguuacgacuuuucaaccacgacgcauagucuuaguacuugucgcugcuaccuuuuaagccucuuccacgacuacuccugcaucuguuuuaccuacugcuguacaaaaacucuacguagcuucgcuuguacgacucgcuauacuggaacguuccauaucuucgcuaaagguuccauauguacgugaacggugucugacugagcuuuuuuuccuagcaguagugacuuuguccgcuuaaauuccgguagcgucuuaccgauaaccuuugacugccauggucguacuacuuucaugacagucuuucucugcagcuaggccaguccugcaaaagauugcuguaaacacuuuauaaaagccaugaaccauagcuccgacacgcauucagacaucucuuccuuuacuugcgacaggaaagcaagaugccagacauacauuugauagcgguagaacggaacgaaacacugcauuacugucgguuuccagugaauuaccgguagugggcagugccauaguugucuguucugugaccucgagacuacuccacaaggaagcuccuuugacaucuacauaacuaccugcgacggucaguacgccuccagcuggguuacucuccucauagacuuuuguaauaggagccaguugaugguucuuacccguguccgacgaagcuagaaaacgaccugcggcuuuuuacauuuuacccuuaacgguauggaguucgcgugucgucgcuagauuaccgaaguccuuacaagaaaccuaaucggcgaugugggucgucauacucagguccaccacgauacugggguaccuuaguucgucgaugugguaugcaaccgucauagaccagaggugucuuaaauuacccgucaccuuacugugguccaccacggcgaaagagggguagucgacgcagucuacguaguccuuacaguggucgaauaccgccaaccagugguugugguguuagaggacguuacagcgguauauaccgaagagguguaccuguuagcggaaggaugucagguaguucaggucgcaagguuggaugaagugguagguacugcggcuggagaggaccuauaagagggucaagaggaccaauaaguggauggucagaguuaaugucagguugcucagggucaauaagugggugaagagucucaaugagggguuggaguggaucaaugaguggcugaagagguuuaauaaguggaugaagggguucgaugucagguuguaggggauugauaagugguuguagaggguugauaagugggugaaguggaucaauaggaaguugaagcgguccaaugucggggugaagugcgucgaugaguggguguagaggaucaaugaguccuugaagcgggagaauaagugguugaagcgguucaaugaggggaugaagaggaucaauaagcggcagcagaggauuaaugagagggugaagagguuuaaugucagggugaagaggauuaaugaguggcaggagaggauccaugugcgggccaagaggaucaaaaagggguucaagcuugucaaugagaggguguagaggaguuauaagagguuguagagguucaauaagcggaagaagcggguuuauaagugguugaaggggguuaauaagcgguuguagagguaguaaaagaccuccuucagguguuauaaguggguguaguggcuuuaugagagguuggagcggguuaaugugagacagcucaggcgucgugugagguuguccaucgucagcuauaaguggcaguugaagcucaauaagaggauuaagcggguuaauaaguggcugcagagguguuaugagguaggugucauguuuuauaaggggacguucaggauguaaguguggguggucaggaucaaagagagggcgaagugggcguauaagcggaguuggauacauaaguggaagaagaggauuaauaagagggugaucagggucaguucugugacugauu

SEQ ID NO: 230 - RNA, 876 nt, Diabrotica virgifera
uacagcaguuuauaaguuuuccgggucgucaacuaccgccuacgucuuuucuuucauuguagagcuccaaagaagccuagagauaaacccccuaguucagcauaacuucuacgucaccuuacaauguguucucgacguuuggaaaaauuuuaccgguucucgacccuacgacggccauuucggaaaacacuccgacgauuaaacguaaggucuugaccacgagcaguacugcgacggugauuaauauaucuacgacguuuaacaauguuuuuucggcuacauaaacuccgacauuugacgaaauauuuucgauaucuguaaauauggcuuuacccagcgaaauguuaccgacguuuugugguagucugauaacgucuuuacauacucugacuacgacaccuguagcuuucccgacaaguugugauacuuguccgccgacuaaugaagucuccucuucuuucguuacgaaggcgguuauucacagaagaauuucaccgaguuauacgucggguugaacuuuugauacuuuuucgucacccuuaaauaguucuucaccgaauacgucgagaccuuucgagagaaaauuuuaugucacguuuccuuaugaauaagucucgacgggaaacaguggaaacacaacuacaugaguuacguguuguacgauaucuuucgauauaaaguuccauagggcguaaaguucuaagggcacuuauguuugaaaacuuuugggaguaucuuuuguagcuucucguuuugcaucuaccuauaugucuucggcaguuucuaaugcuaaguuaaagagcagaacuagucaccauaugauguuaagaaaaugcauaauucuuuguucauucgcuuucgggacugaaugcaauu

SEQ ID NO: 231 - RNA, 609 nt, Diabrotica virgifera
uacuuagggcucauacuaauaaauaaguuugaagacgacuaaccucuaaguccucauccuuuuagaacagaagaugacucuaaacgucuacuauggaugugucuuucgauauaaucaugguaaccgcaucuaaaauuuuaguccuguuagcuaaaucuaccuuucuguuaauuuaacguuuaaacccuaugucguccaguccuuuccaaaucuugcuaauguaguucaauaauggcuccucguguaccauaauaacaucacaugcuaacgugucugguucuaaguaaguuauugcaauuugucaccgagcuucuuuagcuggcaauacgcacacuguuacauuuguuuaaugaccaucccuuauuuucgcuaaacuguugauucuuucaacagcugaagugaugucgguuccucauacggcugguuaacccauaugguaaaaaccuuuggagucgauucuuacguugguuacaucuuguccggaaauacugauaccggcgacuuuauuuuuuaucucauccuggagguagaagacgccaucugguuccuuuauuccaauccaagcuaguuucagcgggucagcuuuguugguuuaggccaacgacgacu

SEQ ID NO: 232 - RNA, 789 nt, Diabrotica virgifera
uaccgucugcgacuacuagauaaucuaauacuucuacuccuugucugucuuguuuggcguugacuuugccguugaugucuccaugucuuuuucccacaguucccguguauacauaguuaugugucaagacccaaaucucuaaaagacaauuuuggucguuaagagucucgauaucaccugacgcccaagcuuguaggaagucuucaaguuguacuuacauaaggaguucgacaguaaccguaccuauaagacacgguucgauuuaggccauacccuuuuugccgacaaaaacauaaucgaugugagguucauuaucuaggaugucuuuuacaacauauacaagagcaguacacgguauggucucucaaucggaaggucuauucguuucucaugcuugcaaagucauuuauauacggguuauaauuucauccccagaagaaaccaccgaacggauaggucuuucuacuccuuugcaauuuuuuauuaacgggcguauagcaacacccaugagguccuucuuaaaaucguaaccagucuagcuuuuuugaauuagaguuuguagauuucguaaaauaaaaccuacuuacacuauuuuacaaccucaauaaucuguacucugcacuacaaguucuuuauauagcauugugaggggugcuuuuuguucaguacuacaagucacgguggaauucauuucuuuaaucuggucaaacguucuuuaaauacguucuacauuaaguuuuaagaauauuauguguuaaaacauuacugcgugggugagcguuacaaacu

SEQ ID NO: 233 - RNA, 738 nt, Diabrotica virgifera
uacggccaguaacuaccaauauuucaugaaauguaaaauaaugugucaaauauauguuaaaaacuuuuauaaaccuccugagaaaauaaauaaauaguuuuaacauauucccaauauuugggacuuagauguaagcuacuacgacuggucaauuucuuuucugacagaucugauuguuuuuucggaguuguaaauugauaguaauaaccacaccuucuuauaaguaaccaucuaaaccgauuggagcauauaaccacaaauccagaauuauaaggcaugcaaucaaagauacuaauauuuccauuaaauuuuuucguacuucucuucaacguuguuuaacaucuuaggucuuuuagucucuuauaguuguauuaaaccguguggguacgucuuguuuccguauuuuuaccuaaaaacccagguuuuuaggugcauuuucacaauugugugcgccugccuuucguuucauaucauuuacaaugauuuuuuaaucgagauuuauuucuuuuucuguaaucauuucuuuuuuaaucacuuaaugauaauuccgucauacuuaaaggucuaggucuuuaccgauaauaaacaccuuucuuugacuuguaaauauuaauaggaggaaccgucaauucugagugucuuaagaaauuucaguuguuucaguuguuguaguguaagggucacaaacaccuuuuuaaccuuuucaugucguuuacacuugucucccacccuuuuauu

SEQ ID NO: 234 - RNA, 480 nt, Diabrotica virgifera
uacugguugagauuuccaauggcggcuccuuggucccuagauaaacgggcguucaaauuuuuugcaccacauuaaggugaaagguguauaaacucucagauguuucaaccucuauaacaucuauaguucccauuaccacgucaaguuuucccauacgggguguuucacaugguaccauucuguccugcacaaaaguuacaaugacguguacguaauccacauuaacauuuguuuucccaagcuccuucuuaguagggguuuucuuaguuagaggcauaacuuguacauuuggugagguucacagcaguucugaagaacguuucucauuuuagguugcuuuucgaugcauuucuucgauuucuuuucuuguaauuucaucuugaauccucuguuggacggguuggauccggucguguauaacaaucgccuuuccaaggucguguccacgaacgaggauaggguauacuuaaguaacgaauc

SEQ ID NO: 235 - RNA, 537 nt, Diabrotica virgifera
uaccuuccuuaugaugaccuugguuguaacauaugguauuuuccauaacgauauaaccugauacuaccauuaucucacgaccgauuuaugaugcuauuucuauauaaaggaugucguuuucucgucuuucgaaaacucuuuuuaaacaaguuauuuugaguaucccgucugcgucuuuaauaguacaaccuaccaaauugaacacacauaucuucauuacaucuaaauaagaaaauacaauacccgucaaguguacuuuuacucgauuaaaauuacucacaaaauuuaacgaacauacugagucauucaguuuauaacuucuuuuuauacguuuuugcucgacagaaccuuagugaucuauaacaauacgaccgauaccuacuuuaacaacuaccuccuuauuaauaucuaagacuaaguucaagucaucauagaucuuaucguaauuccugacuacuauaagguaauccucuuguuugacaucgaguccauaagguuugccgguuucuugucgacuuuaccaguaacgacuuuauu

SEQ ID NO: 236 - RNA, 450 nt, Diabrotica virgifera
uaccgacugguugaguggcuucuuguuuaacgacuuaaguuucuucgaaagagugauaagcuauuucuaccacuaccauguuaaugcugauuucuuaauccuugucauuacucuagagauccuguuuuagguugucuccgacuuaauguccuauacuaguuacuucaucuacggcuaccauugccgugcuagcuaaagggucuuaaaaauugcuacuaccgugcauuuuacuuucuauggcuaucacuccuucuuuaagcacuucguaaggcucacaagcuguuucugccguuaccaaaguagagucgucgucuuaacgcggugcaguacugguugaacccacuuuuuaacugucugcuucuucagcuacuuuacuaagcccuccggcuauagcuaccacuaccaguucaguuaaugcuucucaagcagugguacuacugaaguuucacu

SEQ ID NO: 237 - RNA, 2013 nt, Diabrotica virgifera
uacuacguucguuuguuagcucaggguggauauuucaaccuuuugcuauaucuagaaaugcggcuacuauagcuccuaaagcguguucuacugaaaccaccacuuuuacaacuagauauacugcuacauuauaggcgaggaggaccuuuauuacuguuggguccacuaaguuuaguaguacgaggaggaccacgaccacuucuaccaccuccauuaaaacaacccaguccuccucguggguuauuauauuuaagaagaccuucuucuguagucgacauacaaccuuuagacugaaccaccuguugacuaguucuauaucuuuuacgucacguacuauauccccauuggcugaagguacuucaauucaaaaaacuugugucucguuuaccaguuagguucccuaagacacaguauagaaacccuagacucccuucguacucugagacggaccuugaggauagauuuuuucucuaguuaccgguuuuaggggaacaaugggaaggguguuuuguucgagaaucauugaaacuuucagucagauuuugugcgggaagaggaugauuauuaagauugagugcaggagggguaggauuauuauuacaaguaaguccaggauacgucuuaauaccuccaucuuacggauacuugggaagguacgcaggguacggggguccauacguuccacgagguucuuacgucccagguggaccuaaauuaccuggugguuuguacuuagucguugggggguccaagguuccauuagguguuaccuuaccuggaucuggauuaccaggacccggguuauacccuuacucuggguaccccgguggaguaccuguuguucccggggguucuggugguuacgucccugguggcgucguuccaggagguucuccuuacggcgguguuccagguggcgucuacgcaggucuuaccuuagcuggugguuacguuguucccaugggaguuccgggcggcguauacguuccuggauuguacccagguucuccaggugggguuuacccuggugggccccgcggaguugucguuccuggucgaggcgugcauuuaggucguaagaaaguuguuccuccuccugguggcggggguuacguuguguacggaccuggucccgggcaguacggaggaguuccugggggcguuccagguggugugccugggcaaccuggaggugugccgggugguaacccaggucgcuuacaaggcggaguaccugguggagugccuauaccagguggacgucgcuacggugucggcgguaugccaccggguggaggucugguggcgcgacucuaaggagucaauugucucguucucaaacuccuauauuacagggccuuaucuugucaaaggucaagccgcuaacccgcccggcauaggcugcggcgucgaccucuuaaacguucgcgguaacucugaaaccaaugacgauaaagugaguaguuuguuagguuucaccgauugcugcuagcaacguucuaggaauauucaagcgacguucuaugaaacgcaccacagcuucuguuuucgaugucgaggucggcgucucuggccaguucuaggucccugucuaguguaucuucuugaucuucucuugcuaggagcagugccaugucucugucuucgucucucucccucgcacuugcgcuaucucuagcacuagcacuugcacugucuauaauacuaucuaugucgcuuucucuuucucuggcucuagcaaguucuucgucucuuucuugucuuucccuaucucuugcucuaauaucucuggcccuugggcuucucugucuauuucuuuuuagauuucauaggucucagaguucuaguucuuuguuuagaggccuuggacagcuuggaucgucgcuccauggcuuuaguagggcgauaauacuccuauccauagcccuugcucucucucuuccagcugcucucucgcuagcgcuuucucuuucucuaucuucuccccuucugucgguauccagagcugugauc

SEQ ID NO: 238 - RNA, 765 nt, Diabrotica virgifera
uacucaagauaaccuugacccaugcuaaauagucgaaggguuaagagaggacuaccuucucauaaaguucaacuuauacguuacuuucgucaacuuuuaucaccguggcauuauccggaggcuccaugucuaccguaacauaaccgacgacuuuucgaguaauacaguuuuaacguacuugguucauguuuauuugcuuaaaaguuguaacuauuuguguauccuuaccguaaaaguccgaauuaucgacuacguuccguuuagcaacucuaacgaucuuuucuucguaguuuaauaucuguaguuauaccaaguuuauaaggagaauuuauggauuuacuaucucauucguacauguacguacguaugugaaauaugucacgacaaucugguaaaccaacgucacaguagaaccggucaauacuucuaucacuggguagauacauagacuaacuagguagaccucaaucgauaccuaugaaaccuacacgauguccauuucguuuugucagacguuucugacuuuaucuuuuuaacuucuaccccuuagauuguacguuucuugaacaauuucuucgucgguuuuaguaaauaaaccagguacuacucgacuuccuauucuuaaaacuugaccuugaaaguacccauacguuucuaugcuuaccaaauguaugguuucacggacuuagucacaaacgacuacgucuuuuucgacgguuuguucguuaccuucgucuaagucuuagucuaugucuucuauacauu

SEQ ID NO: 239 - RNA, 744 nt, Diabrotica virgifera
uaccgaaguuuucugucuaacuacuaaaaagguagaucuccucggguuuacuacuacuuuagguccgauuucccucggguuuucccuguaucaaauaauuucuucuuucgacuacgaaauguuuacucuaaaucuuacuaaaacuuguuuuaauaacucugguuuugagaguacccacuucauuacuuucuucgacggaaaagaaaucgacuucguuucaaacguugaccacugaaguuaguucaacaagaaguuuuacagugguuccgaguuuauuuuuauucuugauucuuucuguugcaacgaccacaaugaaauggucacaaacuuacgaugguucuaccaugucuauguauacucaaccgaccaaaccgauccccuccaguuguuaacuguuuugaguucuucuuaauaguuucacgacaauuugacaaccaacuuaaucggagaaacguuugaagaaaacauugagaacuacuacauuaguuuuauuguuugucuucucaguuacgguaacuuguacaauaguaagguucuuaucucgcaugaaaccgaauguaguauaggcuugaccugcucaaucuuucucuccucaagauaucuaauuucuucuagguccuguuuuucuucuagucgucucguuuccggcucuuuguuuuuguucgagaagagguucgacccgaugaauuucucaggguccguuuguacgaaaaccuacucccgcuacuucuagaugaaaagauc

SEQ ID NO: 240 - RNA, 4818 nt, Diabrotica virgifera
uaccuccgccgaggguucaauggcuacgagagcaagcucaauuuaugaacaugucucuugcaggugaaaccgggggucaauuuugucauauaacgacgaaaaauaccacuucuaggucuuaggauguaaugucuuuagucguuagaacuuaggaauucuagucgacgucaagcugguaguugccuacauuuaccacauguugacaacuuuuucauaaagacagucgaagcaaaagaguuuagauccaaaggguaccuucucuuaguucuacgacgucaagauaaaaguaccuuuuuauuacuuaaucuguauugaaguuguaggucacuauagucuauacuuaauuaccauuauuacauauuguaaccucggaaugugugaaaagaaccucgguugcugaguucuuuguuaggccuaccauacuuuuaccguacaugaguaaaaguuacacgacguacccgaaaaguuuugcauuuucuuuucauggugguuaaguauaguuuguagaguaaccaucuugaccaaguaaaaaaaguuguucagacaaaucgaguccgaguccucacauauaaucucuucucguacaaacuguuauccuuuggaugguaguaacguuuucaacgauagguucagaugucaauaaugucugucagaaaugcacagaaccuuagucauuuacuucggaugaaaucccuauuuuggauguuccucaccuacuuuauagaaguuaaguucgacuggaugauguuuacguagagcaaggauaagguucccguuguucgacuccuuguugucuuuuacccucuuucccaacguaagauaguucgacguacacuugucgaccugcuccguuucuuuuaacgacgauguaauuuuuugguugugguggucguucuuuauuuacucccugaucguaagugaugacuacaccaacuuccauuuucuuuucgucgauuuuuacuuuuacucaaguagaugguacuuagucacggacuauuucugguuaacggucuccaauucccacgaaguaaucaguuuccuuaugguaagucauauuuacuauaucuucaaaguccuggucuauaaaagagggcuaaccaggguuaccuccgugugcuucgucgaaggaacaugucgcucuucuuucgagucucuaauucugucuagccccuugaauaacuuuuauuucuaguuuguaaccgacuuaaauacagcaguuacgucgaucuagauaacugguucuacgugguccgaugaccuuauggcguccucaacuaacuaucucgucgccgagauagacgauuuggauugcgguaaguucuagaauauucacgauacccuuucgauagauuauauaugguucugcaacuucguucaaacuuacucuaacuaagaaauaauuuccggcuucuuguuucacuuguuuucaugguucuuugcuaaccauuuucugguggcucguaaaaucgaugucuaaauugaucccuucgccguuuuaugucccuccgaguaugauuucgcuugcugaguuugguuugaaaugugucccgcuacuaccgagugcaccgauuagacuuuuaugagguuguuggcgauuucgucgacguuguagucgacgggaaacagcucaaagguuuagguuuauagcugcuuuuuagaaacuuucuagaccuucgcgaucaacguuuucaucugcuuuacucuuggguuucucgguacgauacccgaguugaagcucuuagauaagugguucugcuauaauguucaagggaacauugcuuuguugguuuagucagcgaccuugucgacaaggucguucuugaaguuuucguaguuuuagacuaaagcaacuaacuuguuuuguggagccguguucuuuuguaauucucgcggaaucagcuaagaaugcgaaugcgacauuuaaguucuuuuauguagguucuauaugagguuuucucuugguguugguauugcagugacuaucguagcaagcugagaaugcuucugaauaaccguuuucgauuguuucccuaucucaaaaugaguuuugaacuuugcuugcauagguucaaugacguuucuuauuccucauggacguuucaaguuguucuucucgcucuagucuacuacagcugacgcguucacggaguuacccucucaguaugcagugaacggcgaggauuugacuuucuaaugaaccugagguccuucuucucacgacgcauaagccucggcucacaaguugguguugucgguugaaauucaaugagucgacgauaccuagacggaggaccauaauccggcugaggucaaccuagucuuuauugccuacauggcuuuuuauaaguuccacuugguguuccaauauaagguauauuaaugguuguuggaagacaaggacggagugucuuauaacuacuucucugauaauuuuuuuacuugcguaacuacgguccacgauucugcagucacggaucagucaugccuaugucguugauguaaggugguuguaugggaguuucacgcaugguugguccauuagucagaaugccuuuucuuugaggucuauaauugaguggcaugcugggaugguuccgcaagugccgaugaugauugcgaauagcaagccacgucucgaggaguugaguuccuaugcauggcaugcgucuuagauugcaaagcuuacaacugucucaaccuauaggaucguccauagucaugguuguucauggacucuaucgaugaugaggucgacuaggguuauaauuacgcaugauggguguacccaugaguggcucggucuuaaauggcuuacgauuaugaguuguauaauggccgguugacuucaugguaagccaccucaugcgaagaagacacggcuuguuguaguuaauauugucgagauggaugagcagcggcgaaagauuauacagaucaugguuaaggaguuuaggaucauugaacuuauuaagaaugcucaugaugauacugggcuuauggucaucaccacgucauggcuuacgaaguuucggaguugucagcucgcggucgagacguuugggcucauggcgauacuuguugauguuaauaaugauguuauguucauggucgccaucacaucgucgccuaugaaguuuuuauguuguuguuguugucauggguccaugagucuacucaguucgcgucaugauagggcgguuacggucaauaaugaguuggucaugaauguuaugguugcagguuccaccaugguuagggagcaugcguugaccuguuuguauauuaguucacuguggucacuggagaguuuuacaaagaguuuuaauguugaaauugguucaaccaagaccucguccuguggucguagucaugaugagcaggcgauugcggcgucaugguaggguuguucgacauuuauugucaaguaaugguuugaugccuaugcuagucauaaugccguuguugauauuaaggucaguuggcucauggaugucgcguuugguucguggaggacgucguguucgacgagguucauuauaaggacgacggugguuuaggaggagauuacaccuagacgagucaccgaaccugaagucguauucgguucgaggagaucacggaguuguuuuguaaugcuauuuugggguucuuuuccuuuguuuugguggccgacaaagaagacuuugguuuuugguucuagguuguggucauuggugcggguuuguugggugaccuggucuucauuucgcgaacaugcaguuuuaggacggcucguuugggaauuuguugcuacuacacuucuuuaacaagccgguucucgaccuguccauacucuucaagcaccucuggaacuggguguuuugaaacucgccaggcuggugagaccuauaauuuaccuuccucuagguucuggucguccuaacgcucggcgucuucuucuaguaaaggcagcgaucuacaauaggauacuucuuauccaagggccuauagaacggaaugcugaaaaggucccaccucaacacgcuaucauuucuacuaauauaguugcgaaguauguaauuccuauagagcgguauacgaggcaguaaauaacaauguguucacggcaacagaaguugacaaccacuauacaccugcuacuaaucucuuguuguccagcuugacuaggagacaaaccauuugcuguuacucuagccacuucuauaaaugaccggguuucuuuuuccgucaucagaauuguaugaauuguaccaguauugcaacguuuugcaauaucaauucagaguaaccugacuuucugacuaucgcuauuugaauggacuuuuugcccucagggcacacuauuacguagauguuaaauguagcaccggaccgucgaacaaagguuguuuaggacuuggcaagcagucgauguggaaccuuagguaguuggauaugguuguugucuucugguuguggguaggccaccaccagguaacaaguagaccguauccuucuucgccggacgagacaaaugacugucgacgauacaagcuacgacgguuguuacgauugagcuauggucuagaaugucgaaacucauaguucaacagguuaacguccuucuuauaagagucucuagcucucguaaacuucaaaccaaugcuuucaaaaaaccgcauauaauccguauaucaaacacuucuauuucggucuuucuuugacuugcucuaggucggguuccaauuccuccuuggugaccuugguggacaguaucaaggucuugguuuauaucuaggaaauucaugaaaucuggguaaaacccgaucauuuucuauu

SEQ ID NO: 241 - protein, 166 aa, Diabrotica virgifera
MTPERKKKLRLLLRKKAAEELKKEQERKAAERRRIIEERCGKPKLVDDANEGPLKQVCEGYHRRIVDLENKKFDLEKEVEFRDFQISELNSQVNDLRGKFVKPTLKKVSKYENKFAKLQKKAAEFNFRNQLKVVKKKEFTLEEEDKEKKPDWSKKGDEKKVQEAEA

SEQ ID NO: 242 - protein, 201 aa, Diabrotica virgifera
MCEEEVAALVVDNGSGMCKAGFAGDDAPRAVFPSIVGRPRHQGVMVGMGQKDSYVGDEAQSKRGILTLKYPIEHGIVTNWDDMEKIWHHTFYNELRVAPEEHPVLLTEAPLNPKANREKMTQIMFETFNTPAMYVAIQAVLSLYASGRTTGIVLDSGDGVSHTVPIYEGYALPHAILRLDLAGRDLTDYLMKILTERGYSF

SEQ ID NO: 243 - protein, 913 aa, Diabrotica virgifera
MPLRLDIKRKLTARSDRVKCVDLHPTEPWMLCSLYSGNINVWNTENQQLVKTFEVCDVPVRTAKFLPRKNWIVSGSDDMQIRVFNYNTLDRVHSFEAHSDYVRCIVVHPTQPYILTSSDDMLIKLWNWEKAWACQQVFEGHTHYIMQIAINPKDNNTFASASLDRTLKVWQLGASTANFTLEGHEKGVNCVDYYHGGDKPYLISGADDRLVKIWDYQNKTCVQTLEGHAQNVTAACFHPELPVALTGSEDGTVRVWHANTHRLESSLNYGFERVWTIFCLKGSNNVALGYDEGSILVKVGREEPAVSMDASGGKIIWARHSELQQANLKALAEGAEIRDGERLPVSVKDMGACEIYPQTIQHNPNGRFVVVCGDGEYIIYTAMALRNKAFGSAQEFVWAQDSSEYAIRESGSTIRIFKNFKEKKNFKSDFGAEGIYGGYLLGVKSVSGLTFYDWETLDLVRRIEIQPKAVYWSDSGKLVCLATEDSYFILSYDSDEVQKARDNNQVADDGVESAFNLLGEINESVRTGLWVGDCFIYTNSVNRINYFVGGELVTIAHLDRPLYVLGYVPKDDRLYLVDKELRVVSYQLLLSVLEYQTAVMRRDFPTADRVLPSIPKEHRTRVAHFLEKQGFKQQALAVSTDPEHRFELAVALEDLNIAKTLAQEANSPQKWNQLAELAAATNNVSVAKECMQKAQDYGGLLLLATSSGDENLVRTLGETTQAESKHNLAFLSHLLVGDLNKCLDILINTGRLPEAAFFARSYLPDKITEVVELWKTQLSSVNQKAGQSLADPKNYENLFPGLQEAVVAQKFLEQQNKGLAPARVATTIPPNHDRNVVAEVQAQSKHDVPSFSSSFISSEIEAQTRSSAKPEESSNIIQLDQDDDDIDLDLDGVNIDENIDTTDINIDDDLLSD

SEQ ID NO: 244 - protein, 381 aa, Diabrotica virgifera
MQIFVKTLTGKTITLEVEPSDTIENVKAKIQDKEGIPPDQQRLIFAGKQLEDGRTLSDYNIQKESTLHLVLRLRGGMHIFVKTLTGKTITLEVEPSDTIENVKAKIQDKEGIPPDQQRLIFAGKQLEDGRTLSDYNIQKESTLHLVLRLRGGMQIFVKTLTGKTITLEVEPSDTIENVKAKIQDKEGIPPDQQRLIFAGKQLEDGRTLSDYNIQKESTLHLVLRLRGGMQIFVKTLTGKTITLEVEPSDTIENVKAKIQDKEGIPPDQQRLIFAGKQLEDGRTLSDYNIQKESTLHLVLRLRGGMQIFVKTLTGKTITLEVEPSDTIENVKAKIQDKEGIPPDQQRLIFAGKQLEDGRTLSDYNIQKESTLHLVLRLRGGN

SEQ ID NO: 245 - protein, 376 aa, Diabrotica virgifera
MCDDDVAALVVDNGSGMCKAGFAGDDAPRAVFPSIVGRPRHQGVMVGMGQKDSYVGDEAQSKRGILTLKYPIEHGIITNWDDMEKIWHHTFYNELRVAPEEHPILLTEAPLNPKANREKMTQIMFETFNTPAMYVAIQAVLSLYASGRTTGIVLDSGDGVSHTVPIYEGYALPHAILRLDLAGRDLTDYLMKILTERGYSFTTTAEREIVRDIKEKLCYVALDFEQEMATAASSTSLEKSYELPDGQVITIGNERFRCPEALFQPSFLGMESCGIHETVYNSIMKCDVDIRKDLYANTVLSGGTTMYPGIADRMQKEITALAPSTIKIKIIAPPERKYSVWIGGSILASLSTFQQMWISKQEYDESGPGIVHRKCF

SEQ ID NO: 246 - protein, 879 aa, Diabrotica virgifera
MGTFKRDTHDEDGGSSAFQNLEKTTVLQEARVFNETSVNPRKCTPILTKLLYLLNQGETLSAKEATDVFFAMTKLFQSKDVILRRMVYLGIKELSSVADDVIIVTSSLTKDMTGKEDMYRAAAIRALCSITDATMLQAIERYMKQAIVDRNAAVSSAALISSLHMSKLAPDVVKRWVNEAQEAVNSDNAMVQYHALGLLYHIRKTDKLAVTKLISKLNSMGLKSPYALCMLIRITAKLLEEEDQESLLNSPYTIIFTMGLRNKSEMVVYEAAHAMVNLKFTSSNVLAPAISVLQLFCGSPKATLRFAAVRTLNQVATTHPASVTACNLDLENLITDPNRSIATLAITTLLKTGAESSVDRLMKQIATFVSEISDEFKVVVIQAIKVLALKFPRKHSTLMNFLSAMLRDEGGLEYKASIADTIITLIEDNPEAKESGLAHLCEFIEDCEHVSLAVRILHLLGKEGPKTKQPSRYIRFIYNRVILECPSVRAAAVSAMAQFGASCPDLLENIQILLSRCQMDSDDEVRDRATYYSNILNKNDKSLYNNYILDSLQVSIPSLERSLREYIQNPTDEPFDIKSVPVAAVPTAEEREVKNKSEGLLVSQGPVRPPPVSREENFAEKLSNVPGIQQLGPLFKTSDVVELTESETEYFVRCIKHCFKHHIVLQFDCLNTLPDQLLENVRVEIDAGETFEILAEIPCEKLHYNETGTTYVVVKLPDDDLPNSVGTCGAVLKFLVKDCDPSTGIPDSDEGYDDEYTLEDIEITLGDQIQKVSKVNWAAAWEEAAATYVEKEDTYSLTINTLSGAVKNIIQFLGLQPAERTDRVPEGKSTHTLLLAGVFRGGIDILVRAKLALGECVTMQLTVRSPDPDVAELITSTVG

SEQ ID NO: 247 - protein, 216 aa, Diabrotica virgifera
MAANRTGPAQRPNGATQGKICQFKLVLLGESAVGKSSLVLRFVKGQFHEYQESTIGAAFLTQTICLDDTTVKFEIWDTAGQERYHSLAPMYYRGAQAAIVVYDITNQDTFGRAKTWVKELQRQASPTIVIALAGNKQDLANKRMVEYEEAQTYADENGLLFMETSAKTAMNVNDIFLAIAKKLPKNEQTTGQGGSAQGRRLAEGDSGAKAPGNCCK

SEQ ID NO: 248 - protein, 92 aa, Diabrotica virgifera
MKFLRSTVCYIAILAILFTLCADEVEGRRKILMGRKSITRTYLRGNAVPAYVIIILVGIGQIILGGILYVALRKKIIAAPVTASYAVARQEP

SEQ ID NO: 249 - protein, 157 aa, Diabrotica virgifera
MQIFVKTLTGKTITLEVEPSDTIENVKAKIQDKEGIPPDQQRLIFAGKQLEDGRTLSDYNIQKESTLHLVLRLRGGAKKRKKKNYSTPKKIKHKKKKVKLAVLKFYKVDENGKIHRLRRECPAEQCGAGVFMAAMEDRHYCGKCGYTLVFSKPGDEK

SEQ ID NO: 250 - protein, 248 aa, Diabrotica virgifera
MMSKADTQEDASFAKLENQIAIIKYVILFTNVLQWALGAAIFALCLWLRFEEGIQEWLQKLDSEQFYIGVYVLIVASLIVMIVSFIGCISALQESTMALLVYIGTQVLSFIFGLSGSAVLLDNSARDSHFQPRIRESMRRLIMNAHHDQSRQTLAMIQENVGCCGADGATDYLSLQQPLPSQCRDTVTGNPFFHGCVDELTWFFEEKCGWIAGLAMAICMINVLSIVLSTVLIQALKKEEEASDSYRR

SEQ ID NO: 251 - protein, 124 aa, Diabrotica virgifera
MSGRGKGGKVKGKAKSRSNRAGLQFPVGRIHRLLRKGNYAERVGAGAPVYLAAVMEYLAAEVLELAGNAARDNKKTRIIPRHLQLAIRNDEELNKLLSGVTIAQGGVLPNIQAVLLPKKTEKKA

SEQ ID NO: 252 - protein, 288 aa, Diabrotica virgifera
MKLDGVDLPPPISFDIAEEQPLPPCQQTFLCNGDGGSIVRQFLELYFVIYDSDNRQSLLQAYHEKATFSMTMAYPYGYSKDSKGVSWLNWYATDNRNLLRVQDPDRRNKLLRQGQVAVVSFLQDMPHTKHDIHSFTVDLTVFTPQMLCLTVAGMFKELKSGHKVPPLRYFFRTLVIVPAGSGFCIANEELHISNATPDQAKDAFKTTVNVAPAPAPVITSPGPSIPQPAVPDDATKQEMVKQMSAVSGMNLEWSLQCLEETQWDYQKAIMVFQNLNAQGVVPQAAFIK

SEQ ID NO: 253 - protein, 955 aa, Diabrotica virgifera
MTAVEQPCYTLINLPTDSEPYNEMQLKMDLEKGEVKVKIRALEKIIHMILAGERLPNGFLMTIIRNVLPLQDHLAKKLLLIFWEIVPKTNPEGKLLQEMILVCDAYRKDLQHPNEFLRGSTLRFLCKLKEPELLEPLMPSIRACLDHRHSYVRRNAVLAIFTIYKNFEALIPDAPELISNYLDGEQDMSCKRNAFLMLLHADQERALSYLASCLDQVNSFGDILQLVIVELIYKVCHSNPAERSRFIRCIYNLLNSSSPAVRYEAAGTLVTLSSAPTAVKAAASCYIELIIKESDNNVKLIVLDRLIALKELPNHERILQDLVMDILRVLSAPDLEVRKKTLSLALELVSSRNIEEMVLVLTKEVSKTVDSEHEDTGKYRQLLVRTLHSCSIKFPDIARSVIPVLIEFLSDNNELAATDVLLFLREAIQKFKELQPLIIEKLIETFKDIKLVKVHRAAIWILGEYASTASDIEVIVGEINRLLGEGSLVEAEQKLIAGDTEENAPAPAAGATTLVTSDGTYATQSAFNTVSQTTKEARPPLRQYLMDGDFFIGASLASTLTKLSLRYEDLTSPAASNGFNAKIMLIMAGILHLGKSGLPTKSITNDDKDHILFCLRVLSDRSPIIVEIFKKLCRSALNEMLLAKESVEAISQKSKEKNKRTIQTDDAISFLQLETDKSGELGENVFEMSLSQALVGGRTGGGESVLSSNKLDKITQLTGFSDPVYSEAYVHVNQYDIVLDVLIVNQTNDTLQNCTLELATLGDLKLVEKPQPVVLAPKDFCNIKANVKVASTENGIIFGNIVYDVIGAGSDRNVVVLNDIHIDIMDYIVPASCTDSEFMRMWAEFEWENKVTVNTPLTELSEYLEHLLKSTNLKCLTSEKALSGQCGFMAANLYAKSIFGEDALANLSIEKPFNKPDAPVSGHIRIRAKSQGMALSLGDKVNMTQKSTQHKVVAA

SEQ ID NO: 254 - protein, 447 aa, Diabrotica virgifera
MVYPNSPFKTTFNNKLITNLFLDDSVTKTKTSVSNEELLKIQQWLCSAPKITSIRVNTIKTNTAKVLKVLKTYFAENCNDTPNVYIHPSFTNVIIIDSLNCPAGFKKFDKEIIVDTDCAAAILRGAHIFAPGVLGMVSGCQINENVSIYADVAKKCKKGLQKIYEDDFKIFIGNGIVKMQRHQLFATDNIAPSGIAVEVTETISGCVPISESLLPVGDILLQNIPSIVCVHNLNPKPGDVVLDMCASPGNKTTHIAELMQNKGILIAIDKTPKKVAQLQKRCEDFGAKVYSFQADSTAIISDTLSSKNVIDGPPFAPQSFDKILLDAPCSVLGKRPQLANRSSENEIKSFVPLQRKLFENAAKLLKPGGIMVYSTCTITLSENEGIVAWALKSFNFLELVQPDLTLGEPGWLGTSLSDEARSFVQRFGPNSEVDSVGFFFAVFKKKT

SEQ ID NO: 255 - protein, 1474 aa, Diabrotica virgifera
MGRLHCLFCIFLCFTVINTQTTNIHGFSENSVDTFLSPHGKSAKFVHQNHKPKIENCQNYKPSVKEEQPGGTYVTTVTAIDDDPREGGGTISYKLIHREGEHVLFDIDNVTGVLTTIQPFDRDEPVRQKELYVTVQASDNGRPPLADVCTFTVTITDINDNAPQLDKLKYDAQVSEDLKVGSEVMRVFAYDIDDGENSRLSYNFSNENAQFTQYFRIDRDTGVVYLKEALTDKKNTRFNSAVYVADNGVNDQEGQKDSTAKISITVVGSDKQPPRFTQKMPDGILEIPEDFKDFSKHIVTVEATSNIADPQLAFELVKGKTYQTNKDQTFLLEAEGNKAHIKLVRPLDYETVTEYTLTIRVKNKDLMDSSINIPIKVLDVNDEIPNFLEFLKGSVVENDKPGAQAIQVRAIDKDGTAANNIVSYELVDNTDLFAINRSTGVITSRVEFDRETVPLYHVNVKAYDNSPSALYNTTLPNIVIQTFQISIEDQNDNKPVFTHPIYQFSNITELADKSSIVGEVKALDNDTASVISYSITNGNIDDAFMIENSTGRIRVNGKLDYEKIEQYNLTVRAFDGAFEDFAIVLISILNENDEPPVFDDYIREIQIKEEEPMISGCVVRVTAHDPDIKDRHADQHIVYEVAKEQKDFLTVSADGCVQVTKPLDRDPPFGSPTRQVFIYARDNDGGTNSLLATAEIEIILIDINDNAPFLNVTEIVYYENQDPGFIGNLSADDYDGPDNGPPFAFRLSDTASDSIRSKFSIIGNQLFALEMFDREEQKYYDIAIDITDSGVPPLTGTSILRVIIGDVNDNPATDGNSTIFVYKYVNGPENFMEIGRVYVTDLDDWDLNDKVFVQEDNFDEFVLNQHNNGMILMKPTTAEGTYEVHYRVTETHEPTIHEHTVNAIVTITVKVLPEEAVVKSGSIRLRGTTKEEFIENSLNGKSKRDILHQELSKILNTSLANVDVFTVLNSPHQNSSFVDVRFSAHGSPYYAPEKLENKVTDHQMELEQKLDVEFYMINVNECLNETTCGAENSCTNKLNITREPAVVFTNRTSFVGVNAFIDPVCAALPRDVMECFNGGVLIENTACNCPAGFEGPHCEILAIGFTGTGWAMYPSFDATNRTEIILHILSQTDNGLIFYNGPLNIRQTSLSKDYISLELKDGYPLLQICTGSSTQEIYLKERIHKLSDGSLHKIKIGSGFDDISLEVDDCGTTCSIWTNKLHKGVIRANGPLQLGGMKNRFTDQEFKRIWDHLPPTATRFSGCIRNLTYNEFYYNLGAPSDAFQAYPDCNYAVMQAVTFGIDSNFLVAILVCVAILIILLLAVVVHRRKHDNFNEKEIDDTRENIINYEDEGGGECDTNYDLSVFHQNNIVDEKPLMRDNPDVPADISGFLDNKKDNCDKDPDNLPYDDVRHYAYEGDGNSTGSLSSLASCTDEGDLKFNYLSSFGPRFRKLADMYGEDPSDEDSHDGNEESWC

SEQ ID NO: 256 - protein, 96 aa, Diabrotica virgifera
MPFCGPKLSLCGLIISAWGIIQLGFMGVFYYIGAVALAEDIPEVEFKGDLDKFYSDVNTGFTQNAYNCWIAALLYLITLAVSAHQFWANNRSSLNV

SEQ ID NO: 257 - protein, 179 aa, Diabrotica virgifera
MGLTISAVFNRLFSKKPMRILMVGLDAAGKTTILYKLKLGEIVTTIPTIGFNVETVEYKNISFTVWDVGGQTRIRKLWRHYFANTDGLIFVVDSNDRDRIAEAEEELHNMLGEDDLRDCILLIFANKQDLPNSMSTAELTDKLKLHTLKNRRWYIQATCATQGNGLYEGLDWLSNELAK

SEQ ID NO: 258 - protein, 205 aa, Diabrotica virgifera
MRYTLSYIGATLASTVTLIFALYYCLTGKGEQVSLAWLLLNVSPHMWAGLGIGLAVSLSVVGAAAGIHTTGVSIVGAGVKAPRIKTKNLISIIFCEAVAIYGLIMAIVLCGSWKNFDVDLFNLKTHNFAQNHYGSHVIFGSGLTVGFVNLLCGFCVGVVGSGAAISDAANSSLFVKILIIEIFGSAIGLFGLIVGVYLTSRGSMV

SEQ ID NO: 259 - protein, 1897 aa, Diabrotica virgifera
MATNDSKAPLRTVKRVQFGILSPDEIRRMSVTEGGIRFPETMEAGRPKLCGLMDPRQGVIDRSSRCQTCAGNMTECPGHFGHIELAKPVFHVGFVTKTIKILRCVCFFCSKLLVSPNNPKIKEVVMKSKGQPRKRLAFVYDLCKGKNICEGGDEMDVGKESEDPNKKAGHGGCGRYQPNIRRAGLDLTAEWKHVNEDTQEKKIALSAERVWEILKHITDEECFILGMDPKFARPDWMIVTVLPVPPLAVRPAVVMHGSARNQDDITHKLADIIKANNELQKNESAGAAAHIITENIKMLQFHVATLVDNDMPGMPRAMQKSGKPLKAIKARLKGKEGRIRGNLMGKRVDFSARTVITPDPNLRIDQVGVPRSIAQNMTFPEIVTPFNFDKMLELVQRGNSQYPGAKYIIRDNGERIDLRFHPKPSDLHLQCGYKVERHIRDGDLVIFNRQPTLHKMSMMGHRVKVLPWSTFRMNLSCTSPYNADFDGDEMNLHVPQSMETRAEVENLHITPRQIITPQANQPVMGIVQDTLTAVRKMTKRDVFIEKEQMMNILMFLPIWDGKMPRPAILKPKPLWTGKQIFSLIIPGNVNMIRTHSTHPDDEDDGPYKWISPGDTKVMVEHGELVMGILCKKSLGTSAGSLLHICMLELGHEVCGRFYGNIQTVINNWLLLEGHSIGIGDTIADPQTYTEIQRAIRKAKEDVIEVIQKAHNMELEPTPGNTLRQTFENQVNRILNDARDKTGGSAKKSLTEYNNLKAMVVSGSKGSNINISQVIACVGQQNVEGKRIPFGFRKRTLPHFIKDDYGPESRGFVENSYLAGLTPSEFYFHAMGGREGLIDTAVKTAETGYIQRRLIKAMESVMVHYDGTVRNSVGQLIQLRYGEDGLCGEMVEFQYLATVKLSNKAFERKFRFDPSNERYLRRVFNEEVIKQLMGSGEVISELEREWEQLQKDREALRQIFPSGESKVVLPCNLQRMIWNVQKIFHINKRAPTDLSPLRVIQGVRELLRKCVIVAGEDRLSKQANENATLLFQCLVRSTLCTKCVSEEFRLSTEAFEWLIGEIETRFQQAQANPGEMVGALAAQSLGEPATQMTLNTFHFAGVSSKNVTLGVPRLKEIINISKKPKAPSLTVFLTGAAARDAEKAKNVLCRLEHTTLRKVTANTAIYYDPDPQNTVIPEDQEFVNVYYEMPDFDPTRISPWLLRIELDRKRMTDKKLTMEQIAEKINAGFGDDLNCIFNDDNAEKLVLRIRIMNSDDGKFGEGADEDVDKMDDDMFLRCIEANMLSDMTLQGIEAISKVYMHLPQTDSKKRIVITETGEFKAIAEWLLETDGTSMMKVLSERDVDPVRTFSNDICEIFSVLGIEAVRKSVEKEMNAVLSFYGLYVNYRHLALLCDVMTAKGHLMAITRHGINRQDTGALMRCSFEETVDVLMDAASHAEVDPMRGVSENIILGQLPRMGTGCFDLLLDAEKCKMGIAIPQAHSSDLMASGMFFGLAATPSSMSPGGAMTPWNQAATPYVGSIWSPQNLMGSGMTPGGAAFSPSAASDASGMSPAYGGWSPTPQSPAMSPYMASPHGQSPSYSPSSPAFQPTSPSMTPTSPGYSPSSPGYSPTSLNYSPTSPSYSPTSQSYSPTSPSYSPTSPNYSPTSPSYSPTSPNYSPTSPNYSPTSPSYPSTSPGYSPTSRSYSPTSPSYSGTSPSYSPTSPSYSPTSPSYSPSSPNYSPTSPNYSPTSPNYSPSSPRYTPGSPSFSPSSNSYSPTSPQYSPTSPSYSPSSPKYSPTSPNYSPTSPSFSGGSPQYSPTSPKYSPTSPNYTLSSPQHTPTGSSRYSPSTSSYSPNSPNYSPTSPQYSIHSTKYSPASPTFTPTSPSFSPASPAYSPQPMYSPSSPNYSPTSPSQDTD

SEQ ID NO: 260 - protein, 291 aa, Diabrotica virgifera
MSSNIQKAQQLMADAEKKVTSRGFFGSLFGGSSRIEDAVECYTRAANLFKMAKSWDAAGKAFCEAANLHSRTGARHDAATNYIDAANCYKKADVFEAVNCFIKAIDIYTEMGRFTMAAKHHQTIAEMYETDAVDIERAVQHYEQAADYFRGEESNASANKCLLKVAQYAAQLENYEKAVGIYQEVAYAALESSLLKYSAKEYLFRAALCHLCVDVLNAQHAIESYISRYPAFQDSREYKLLKTLIENIEEQNVDGYTEAVKDYDSISRLDQWYTTILLRIKKQVSESPDLR

SEQ ID NO: 261 - protein, 202 aa, Diabrotica virgifera
MNPEYDYLFKLLLIGDSGVGKSCLLLRFADDTYTESYISTIGVDFKIRTIDLDGKTIKLQIWDTAGQERFRTITSSYYRGAHGIIVVYDCTDQDSFNNVKQWLEEIDRYACDNVNKLLVGNKSDLTTKKVVDFTTAKEYADQLGIPFLETSAKNATNVEQAFMTMAAEIKNRVGPPSSAVDQGNKVRFDQSRPVETTKSGCC

SEQ ID NO: 262 - protein, 262 aa, Diabrotica virgifera
MADADDLLDYEDEEQTEQTATETATTEVQKKGVKGTYVSIHSSGFRDFLLKPAILRAIVDCGFEHPSEVQHECIPQAVIGMDILCQAKSGMGKTAVFVLATLQVIDPTENVVYVLVMCHTRELAFQISKEYERFSKYMPNIKVGVFFGGLPIQKDEETLKNNCPHIVVGTPGRILALVRSKKLNLKHLKHFILDECDKMLELLDMRRDVQEIYRNTPHEKQVMMFSATLSKEIRPVCKKFMQDVIQNSYNTQFCNDAPTRNV

SEQ ID NO: 263 - protein, 245 aa, Diabrotica virgifera
MPVIDGYKVLYILLHSLYTIFENIWRTLLFIYQNCIRVINPESTFDDADQLKKRLSRLTKKPQHLTIIIGVEEYSLVDLANLVYWCLGLNIPYVSFYDYKGNLKKHEEKLQQIVESRKSENINIIWHTHAEQRHKNGFLGPKIHVKVLTHADGKQSIVNVTKKLALNKEKDISKEKISELLLRQYEFPDPEMAIICGKKLNIYNYPPWQLRLTEFFKVNKVNNITFPVFVEKLEKYSKCEQRVGK

SEQ ID NO: 264 - protein, 159 aa, Diabrotica virgifera
MTNSKGYRRGTRDLFARKFKKRGVIPLSTYLRVYKVGDIVDIKGNGAVQKGMPHKVYHGKTGRVFNVTAHALGVIVNKRVRGRIIPKRINLRIEHVNHSKCRQDFLQRVKSNEKLRKEAKEKNIKVELRRQPAQPRPAHIVSGKVPAQVLAPIPYEFIA

SEQ ID NO: 265 - protein, 178 aa, Diabrotica virgifera
MEGILLEPTLYTIKGIAILDYDGNRVLAKYYDKDIFPTAKEQKAFEKNLFNKTHRADAEIIMLDGLTCVYRSNVDLFFYVMGSSHENELILMSVLNCLYDSVSQILKKNMQKRAVLESLDIVMLAMDEIVDGGIIIDSDSSSVVSRIALRTDDIPLGEQTVAQVFQTAKEQLKWSLLK

SEQ ID NO: 266 - protein, 149 aa, Diabrotica virgifera
MADQLTEEQIAEFKEAFSLFDKDGDGTITTKELGTVMRSLGQNPTEAELQDMINEVDADGNGTIDFPEFLTMMARKMKDTDSEEEIREAFRVFDKDGNGFISAAELRHVMTNLGEKLTDEEVDEMIREADIDGDGQVNYEEFVTMMTSK

SEQ ID NO: 267 - protein, 670 aa, Diabrotica virgifera
MMQANNRVPPIKLENDIDLYADDIEDFAQDDFGGENVDLYDDVISAPPGNNDNPGDSNHHAPPGAGEDGGGNFVGSGGAPNNINSSGRRHQLYVGNLTWWTTDQDIENAVHDIGVTDFHEVKFFEHRANGQSKGFCVISLGSEGSMRLCLELLSKKEINGQNPLVTLPTKQALSNFESQSKTRPSPTNNSNSRPPHPNNNVHSGPMQNYGGRMPMNPSMRPMPPGMQGAPRMQGPPGFNGPPNMNQQPPRFQGNPQWNGPRPNGPGPNMGMRPMGPPHGQQGPPRPPMQGPPQQGPPRGMPPQGPPQMRPEWNRPPMQQGYPQGPPHMQGPNMGPRGPPQMGPPGAPQQQGPAPHVNPAFFQQGGGPPPPMQHMPGPGPVMPPQGPPQGPPHGPVGPPHGPPLGPANVPPHGPPHGYGPPAAMPQPPYGGPPPDHRAEIPQLTEQEFEDIMSRNRTVSSSAIGRAVSDAAAGEFASAIETLVTAISLIKQSKVANDDRCKILISSLQDTLRGVEDKSYSSSRRDRSRSRDRSHRRTRRERSSSRYRDRSRERERERDRDRDRERDRYYDRYSERERDRDRSRSRERTERDRERDYRDREPEETDKEKSKVSRVSRSRNKSPEPVEPSSEVPKSSRYYEDRYREREREGRRESDRERERDRRGEDSHRSRH

SEQ ID NO: 268 - protein, 254 aa, Diabrotica virgifera
MSSIGTGYDLSASQFSPDGRVFQVEYAMKAVENSGTVIGLRGTDGIVLAAEKLIMSKLHEPSTNKRIFNIDKHIGMAFSGLIADARQIVEIARKEASNYRHQYGSNIPLKYLNDRVSMYMHAYTLYSAVRPFGCSVILASYEDSDPSMYLIDPSGVSYGYFGCATGKAKQSAKTEIEKLKMGNLTCKELVKEAAKIIYLVHDELKDKNFELELSWVCKDTNGLHTKVPESVFADAEKAAKQAMEADSESDTEDM

SEQ ID NO: 269 - protein, 246 aa, Diabrotica virgifera
MASKDRLMIFPSRGAQMMMKSRLKGAQKGHSLLKKKADALQMRFRMILNKIIETKTLMGEVMKEAAFSLAEAKFATGDFNQVVLQNVTKAQIKIRTKKDNVAGVTLPVFECYQDGTDTYELAGLARGGQQLTKLKKNYQSAVKLLVELASLQTSFVTLDDVIKITNRRVNAIEHVIIPRIERTLAYIISELDELEREEFYRLKKIQDKKKISRAKAEKQKQALLQAGLLKESQANMLLDEGDEDLL

SEQ ID NO: 270 - protein, 1605 aa, Diabrotica virgifera
MEAAPKLPMLSFELNTCTENVHFGPQLKQYIAAFYGEDPESYITEISNLESLRSAAVRPSTDVNGVQLLKKYFCQLRFLKSRFPMEENQDAAVLFSWKNNELDITSTSSDIRYELMVIMYNIGALHTFLGANDSRNNPDGMKMACTHFQCAAWAFQNVKEKYHQFISNISLVELVHFFQQVCLAQAQECILEKSMFDNRKPTIIAKVAIQVYSYYRQSLRVLESVNEAYFRDKTYKEWMKYLQFKLTYYKCISFLFQGQQAEEQQKMGERVAFYQAACEQLDEAKKIAATLKNQHHQQEINEGLAFTTDVVEGKRKAAKNENEFIYHESVPDKDQLPEVKGASLVKGIPFSINDIEVSGPDIFSRLVPMEAHEAASLYSEKKAQRLRQIGELIENKDQTLAEFMSSMQLDLLTKMHQATGIPQELIDRAAALSAKPNAIQDLISAMGKLSNIYQDVEASLNEIDSLLKAEEQSEQKYQETIGKRPPSILATDLTREAAKYREAHTKANDSNQTLHRAMMAHVANLKILQQPLKQLQHQLPFVEFPNPNIDEKSLKDLEALVAKVDEMRTQRAMLWAQLRESIHQDDITSSLVTKQPNQSLEQLFQQELQKHQNLISLIEQNTSAQENIKSALVDSYAYAVNSRKYIQDILQKRTTTITSLIASFDSYEDLLAKANKGIEFYSKLETNVSKLLQRIRSTCKVQQEERDQMMSTAQVPQWESHTSLAAPKLKDYLDSRKKSAAYSEPSVQPQQPTLSYSAAMDLPPGIRPTPVGSEITDVPKNIQGEPQGYIPYNYQQPSVPASQNIDEETIKKMNALMPGAKTSVPSQYGYSNYIPPTYPQSAYQPGNQSYGKETPDINSPYDPTKAFTATTNAYRSVQSSSTQGYVPYAESNVSNVDRVGYPSRYQYQQVPEIATTPADPNINAYYPHGYSPSQNLPNANTQHITGQLKYHSVEYASSVPNNINYNSSTYSSPLSNMSSTNSSNPSNLNNSYEYYYDPNTSSGAVPNASKPQQSSASSANPSTAMNNYNYYYNTSTSGSVAADTSKIQQQQQYPGTQMSQAQYYPANASYYSTSTYNTNVQGGTNPSYATGQTYNQVTPVTSQNVSQNYNFNQVGSGAGHQHQYYSSANAAVPSQQAVNNSSLPNYGYDQYYGNNYNSSQPSTYSANQAPPAAQAAPSNIPAATKSSSNVDLLSGLDFSISQAPLVPQQNITIKPQEKETKPPAVSSETKNQDPTPVTTPKQPTGPEVKRLYVKILPSKPLNNDDVKKLFGQELDRYEKFVETLTHKTLSGPTTLDIKWKEIQDQQDCEPQKKIISVARCYPMKNRFPDILPYDFSRVELCDSKDDYINASYIKDISPYAPSFIVTQVPLSSTVGDMWTMIREQQVELILCLVNDNEIGEDIYWPKEKGSSLNILNMVITLQNVIVKSHWTERLIAINLPEKRESRVIMHLQFTSWPGSLFPTNPEPFVSYTLESINLYQQQKTNTHPVVVHCSSGIGRSGLLCLLTAAMFDAANNANSIPDLTALSIKLSNCRKNILRDREHLKFGYESFLAYIRHIVCEDKARKKLNEIQPKVKEEPLEPPVIVPEPNIDPLSTLDPFWASKR

SEQ ID NO: 271 - DNA, 513 bp, Diabrotica barberi
atgaaacctttcttggcccctgagagaaagaagaaacttaggttactgttgagaaagaaagccgctgaagaattaaagaaagaacaagaacgcaaagcagccgaaaggaggcgtattattgaagaaaggtgcggtaaacccaaacttgtcgacgacgcaaatgaaggctcattaaaacaagtatgtgagggatatcacagacgtattgtagacctagaaaataagaaatttgacctcgaaaaggaagtggaattcagagattttcagatctccgaattgaacagccaagtaaacgaccttagaggcaaattcgtcaaaccaaccttgaagaaggtatccaaatacgaaaacaaattcgccaaacttcaaaagaaggcagctgaatttaacttccgtaaccaactcaaagttgtcaagaagaaagaattcaccttagaagaagaagacaaagaaaagaaaccagactggtcaaagaagggagacgaaaagaaggtacaagaggctgaagcatga

SEQ ID NO: 272 - DNA, 279 bp, Diabrotica barberi
atgaagtttttaaaatcgacagtgtgctacattgccatcttggcaattctctttaccctctgtgccgatgaggttgaaggaaggagaaaaattttgatggggcgaaaaagcattaccaggacatatcttcgtggaaatgctgttcctgcgtatgtgataataatccttgtaggaattggtcaaatcatccttggagggatattgtacgtggcattgaagaagaagatcattgatgcacctgtaacgggatcatatgcagtggctagacaagaaccataa

SEQ ID NO: 273 - DNA, 651 bp, Diabrotica barberi
atggcggcaaacagaactggacctgctcagagaccaaatggcgctacccaaggaaagatatgtcagttcaaactggtcctactaggcgaaagtgccgtcggtaagtcgagtttggtactgaggttcgtcaaaggacagttccacgaataccaggagagtaccataggagcagctttccttacacaaaccatatgcctcgacgatacaactgttaaatttgaaatttgggacacagcgggtcaagaaaggtaccacagtttagctcctatgtactataggggcgcacaggcagctatagtcgtctacgacataaccaatcaagacacattcggcagggcgaaaacgtgggtgaaggaacttcaaaggcaggccagtccgacgatcgtgatagctttggccggcaacaagcaggatttggccaacaaacgtatggtagaatacgaagaggcgcaaacgtatgctgacgaaaacggcttactttttatggaaacttccgcaaagacggcaatgaacgtcaacgatatatttttagcaatagctaagaaactgcccaagaatgaacaaaccacaggtcaaggcggcagtgcccaaggcaggcggctagcggaaggcgattcgggcgccaaggcacccggaaattgttgcaagtga

SEQ ID NO: 274 - RNA, 513 nt, Diabrotica barberi
augaaaccuuucuuggccccugagagaaagaagaaacuuagguuacuguugagaaagaaagccgcugaagaauuaaagaaagaacaagaacgcaaagcagccgaaaggaggcguauuauugaagaaaggugcgguaaacccaaacuugucgacgacgcaaaugaaggcucauuaaaacaaguaugugagggauaucacagacguauuguagaccuagaaaauaagaaauuugaccucgaaaaggaaguggaauucagagauuuucagaucuccgaauugaacagccaaguaaacgaccuuagaggcaaauucgucaaaccaaccuugaagaagguauccaaauacgaaaacaaauucgccaaacuucaaaagaaggcagcugaauuuaacuuccguaaccaacucaaaguugucaagaagaaagaauucaccuuagaagaagaagacaaagaaaagaaaccagacuggucaaagaagggagacgaaaagaagguacaagaggcugaagcauga

SEQ ID NO: 275 - RNA, 279 nt, Diabrotica barberi
augaaguuuuuaaaaucgacagugugcuacauugccaucuuggcaauucucuuuacccucugugccgaugagguugaaggaaggagaaaaauuuugauggggcgaaaaagcauuaccaggacauaucuucguggaaaugcuguuccugcguaugugauaauaauccuuguaggaauuggucaaaucauccuuggagggauauuguacguggcauugaagaagaagaucauugaugcaccuguaacgggaucauaugcaguggcuagacaagaaccauaa

SEQ ID NO: 276 - RNA, 651 nt, Diabrotica barberi
auggcggcaaacagaacuggaccugcucagagaccaaauggcgcuacccaaggaaagauaugucaguucaaacugguccuacuaggcgaaagugccgucgguaagucgaguuugguacugagguucgucaaaggacaguuccacgaauaccaggagaguaccauaggagcagcuuuccuuacacaaaccauaugccucgacgauacaacuguuaaauuugaaauuugggacacagcgggucaagaaagguaccacaguuuagcuccuauguacuauaggggcgcacaggcagcuauagucgucuacgacauaaccaaucaagacacauucggcagggcgaaaacgugggugaaggaacuucaaaggcaggccaguccgacgaucgugauagcuuuggccggcaacaagcaggauuuggccaacaaacguaugguagaauacgaagaggcgcaaacguaugcugacgaaaacggcuuacuuuuuauggaaacuuccgcaaagacggcaaugaacgucaacgauauauuuuuagcaauagcuaagaaacugcccaagaaugaacaaaccacaggucaaggcggcagugcccaaggcaggcggcuagcggaaggcgauucgggcgccaaggcacccggaaauuguugcaaguga

SEQ ID NO: 277 - DNA, 744 bp, Diabrotica undecimpunctata
atggcggacgatgaggaaaagaagaggaaacaggccgaaattgaacgcaaaagggccgaggtcagggctcgtatggaagaggcctcaaaagccaagaaggccaagaaaggtttggcggacgatgagagaaagaaactggaggaggaaaagaagaggaaacaggccgaaattgaacgcaaaagggccgaggtcagggctcgtatggaagaggcctcaaaagccaagaaggccaagaaaggtttcatgacccctgagagaaagaagaaacttaggttactgttgagaaagaaagccgctgaagaattaaagaaagaacaagaacgcaaagcagctgaaaggaggcgtatcattgaagaaaggtgcggtaaacccaaacttgtcgatgatgcaaatgaagcctcattaaaacaagtatgtgagggatatcacagacgtattgtagacctagaaaataagaaatttgacctcgaaaaggaagtggaattcagagattttcagatctccgaattgaacagccaagtaaacgaccttagaggcaaattcgtcaaaccaaccttgaagaaggtatccaaatacgaaaacaaattcgccaaactccaaaagaaggcagctgaatttaacttccgtaaccaactcaaagttgtcaagaagaaagaattcaccttagaagaagaagacaaagaaaagaaaccagactggtcaaagaagggagacgaaaagaaggtacaagaggctgaagcatga

SEQ ID NO: 278 - DNA, 279 bp, Diabrotica undecimpunctata; identical to SEQ ID NO: 272

SEQ ID NO: 279 - DNA, 651 bp, Diabrotica undecimpunctata
atggcggcaaacagaactggacctgctcagagaccaaatggcgctacccaaggaaagatatgccagttcaaacttgtcctactaggcgaaagtgccgtcggtaagtcgagtttggtactgaggtttgtcaaaggacagttccacgaataccaggagagtaccataggagcagctttccttacacaaaccatatgcctcgacgatacaaccgttaaatttgaaatttgggacacagcgggtcaagaaaggtaccacagtttagctcctatgtactataggggcgcacaggcagctatagtcgtctacgacataaccaatcaagacacattcggcagggcgaaaacgtgggttaaggaacttcaaaggcaggcgagtccgacgatcgtgatagctttggccggcaacaagcaggatttggccaataaacgtatggtagaatacgaagaggcgcaaacgtatgctgacgaaaatggcttactttttatggaaacttccgcaaagacggcaatgaacgtcaacgatatatttttagcaatagctaagaaactgcccaagaatgaacaaacaacaggtcaaggaggcagtgcccaaggtaggcggctagcagaaggcgattcgggggccaaggcacctggaaactgttgcaagtga

SEQ ID NO: 280 - RNA, 744 nt, Diabrotica undecimpunctata
auggcggacgaugaggaaaagaagaggaaacaggccgaaauugaacgcaaaagggccgaggucagggcucguauggaagaggccucaaaagccaagaaggccaagaaagguuuggcggacgaugagagaaagaaacuggaggaggaaaagaagaggaaacaggccgaaauugaacgcaaaagggccgaggucagggcucguauggaagaggccucaaaagccaagaaggccaagaaagguuucaugaccccugagagaaagaagaaacuuagguuacuguugagaaagaaagccgcugaagaauuaaagaaagaacaagaacgcaaagcagcugaaaggaggcguaucauugaagaaaggugcgguaaacccaaacuugucgaugaugcaaaugaagccucauuaaaacaaguaugugagggauaucacagacguauuguagaccuagaaaauaagaaauuugaccucgaaaaggaaguggaauucagagauuuucagaucuccgaauugaacagccaaguaaacgaccuuagaggcaaauucgucaaaccaaccuugaagaagguauccaaauacgaaaacaaauucgccaaacuccaaaagaaggcagcugaauuuaacuuccguaaccaacucaaaguugucaagaagaaagaauucaccuuagaagaagaagacaaagaaaagaaaccagacuggucaaagaagggagacgaaaagaagguacaagaggcugaagcauga

SEQ ID NO: 281 - RNA, 279 nt, Diabrotica undecimpunctata; identical to SEQ ID NO: 275

SEQ ID NO: 282 - RNA, 651 nt, Diabrotica undecimpunctata
auggcggcaaacagaacuggaccugcucagagaccaaauggcgcuacccaaggaaagauaugccaguucaaacuuguccuacuaggcgaaagugccgucgguaagucgaguuugguacugagguuugucaaaggacaguuccacgaauaccaggagaguaccauaggagcagcuuuccuuacacaaaccauaugccucgacgauacaaccguuaaauuugaaauuugggacacagcgggucaagaaagguaccacaguuuagcuccuauguacuauaggggcgcacaggcagcuauagucgucuacgacauaaccaaucaagacacauucggcagggcgaaaacguggguuaaggaacuucaaaggcaggcgaguccgacgaucgugauagcuuuggccggcaacaagcaggauuuggccaauaaacguaugguagaauacgaagaggcgcaaacguaugcugacgaaaauggcuuacuuuuuauggaaacuuccgcaaagacggcaaugaacgucaacgauauauuuuuagcaauagcuaagaaacugcccaagaaugaacaaacaacaggucaaggaggcagugcccaagguaggcggcuagcagaaggcgauucgggggccaaggcaccuggaaacuguugcaaguga

SEQ ID NO: 283 - DNA, 478 bp, Diabrotica virgifera; identical to SEQ ID NO: 1

SEQ ID NO: 284 - DNA, 413 bp, Diabrotica virgifera
atggcggacgatgagagaaagaaactggaggaggaaaagaagaggaaacaggccgaaattgaacgcaaaagggccgaggtcagggctcgtatggaagaggcctcaaaagccaagaaggccaagaaaggtttcatgacccctgagagaaagaagaaacttaggttactgttgagaaagaaagccgccgaagaattaaagaaagaacaagaacgcaaagcagccgaaaggaggcgtatcattgaagaaaggtgcggtaaacccaaacttgtcgatgacgcaaatgaaggcccattaaaacaagtatgtgagggatatcacagacgtattgtagacctagaaaataagaaatttgacctcgaaaaagaagtggaattcagagattttcagatctccgaattgaacagccaagtaaa

SEQ ID NO: 285 - DNA, 100 bp, Diabrotica virgifera
agatctccgaattgaacagccaagtaaacgaccttagaggcaaattcgtcaaaccaaccttgaagaaggtatccaaatacgaaaacaaattcgccaaact

SEQ ID NO: 286 - DNA, 100 bp, Diabrotica virgifera
tcaaaagaaggcagctgaatttaacttccgtaaccaactcaaagttgtcaagaagaaagaattcaccttagaagaagaagacaaagaaaagaaaccagac

SEQ ID NO: 287 - DNA, 133 bp, Diabrotica virgifera
gaccttagaggcaaattcgtcaaaccaaccttgaagaaggtatccaaatacgaaaacaaattcgccaaacttcaaaagaaggcagctgaatttaacttccgtaaccaactcaaagttgtcaagaagaaagaat

SEQ ID NO: 288 - DNA, 500 bp, Diabrotica virgifera; identical to SEQ ID NO: 7

SEQ ID NO: 289 - DNA, 648 bp, Diabrotica virgifera
atggcggcaaacagaactggacctgctcagagaccaaatggcgctacccaaggaaagatatgtcagttcaaactggtcctactaggcgaaagtgccgtcggtaagtcgagtttggtactgaggttcgtcaaaggacagttccacgaataccaggagagtaccataggagcagctttccttacacaaaccatatgcctcgacgatacaactgttaaatttgaaatttgggacacagcgggtcaagaaaggtaccacagtttagctcctatgtactataggggcgcacaggcagctatagtcgtctacgacataaccaatcaagacacattcggcagggcgaaaacgtgggtgaaggaacttcaaaggcaggccagtccgacgatcgtgatagctttggccggcaacaagcaagatttggccaacaaacgtatggtagaatacgaagaggcgcagacgtatgctgacgaaaacggcttactttttatggaaacttccgcaaagacggcaatgaacgtcaacgatatatttttagcaatagctaagaaactgcccaagaatgaacaaaccacaggtcaaggcggcagtgcccaaggcaggcggctagcggagggcgattcgggcgccaaggcacccggaaattgttgcaag

SEQ ID NO: 290 - DNA, 188 bp, Diabrotica virgifera
atggcggcaaacagaactggacctgctcagagaccaaatggcgctacccaaggaaagatatgtcagttcaaactggtcctactaggcgaaagtgccgtcggtaagtcgagtttggtactgaggttcgtcaaaggacagttccacgaataccaggagagtaccataggagcagctttccttacacaaac

SEQ ID NO: 291 - DNA, 205 bp, Diabrotica virgifera
ggacagttccacgaataccaggagagtaccataggagcagctttccttacacaaaccatatgcctcgacgatacaactgttaaatttgaaatttgggacacagcgggtcaagaaaggtaccacagtttagctcctatgtactataggggcgcacaggcagctatagtcgtctacgacataaccaatcaagacacattcggcaggg

SEQ ID NO: 292 - DNA, 224 bp, Diabrotica virgifera
gcacaggcagctatagtcgtctacgacataaccaatcaagacacattcggcagggcgaaaacgtgggtgaaggaacttcaaaggcaggccagtccgacgatcgtgatagctttggccggcaacaagcaagatttggccaacaaacgtatggtagaatacgaagaggcgcagacgtatgctgacgaaaacggcttactttttatggaaacttccgcaaagacggc

SEQ ID NO: 293 - DNA, 196 bp, Diabrotica virgifera
gacgtatgctgacgaaaacggcttactttttatggaaacttccgcaaagacggcaatgaacgtcaacgatatatttttagcaatagctaagaaactgcccaagaatgaacaaaccacaggtcaaggcggcagtgcccaaggcaggcggctagcggagggcgattcgggcgccaaggcacccggaaattgttgcaag

SEQ ID NO: 294 - DNA, 189 bp, Diabrotica virgifera; identical to SEQ ID NO: 8

SEQ ID NO: 295 - DNA, 330 bp, Diabrotica virgifera
gtgtgtatttcagctggaatttgtaatgaaaaaaacgtagaaatatatactacaatgaagtttttaagatcgacagtgtgctacattgccatcttggcaattctctttaccctctgtgccgatgaggttgaaggaaggagaaaaattttgatggggcgaaaaagcattaccaggacatatcttcgtggaaatgctgttcctgcgtatgtgataataatccttgtaggaattggtcaaatcatcctgggagggatattgtacgttgcattgaggaagaagatcattgctgcacctgtaacggcatcatatgcagtggctagacaagaacca

SEQ ID NO: 296 - DNA, 197 bp, Diabrotica virgifera
gtgtgtatttcagctggaatttgtaatgaaaaaaacgtagaaatatatactacaatgaagtttttaagatcgacagtgtgctacattgccatcttggcaattctctttaccctctgtgccgatgaggttgaaggaaggagaaaaattttgatggggcgaaaaagcattaccaggacatatcttcgtggaaatgctgt

SEQ ID NO: 297 - DNA, 179 bp, Diabrotica virgifera
atggggcgaaaaagcattaccaggacatatcttcgtggaaatgctgttcctgcgtatgtgataataatccttgtaggaattggtcaaatcatcctgggagggatattgtacgttgcattgaggaagaagatcattgctgcacctgtaacggcatcatatgcagtggctagacaagaacc

SEQ ID NO: 298 - RNA, 478 nt, Diabrotica virgifera; identical to SEQ ID NO: 121

SEQ ID NO: 299 - RNA, 413 nt, Diabrotica virgifera
auggcggacgaugagagaaagaaacuggaggaggaaaagaagaggaaacaggccgaaauugaacgcaaaagggccgaggucagggcucguauggaagaggccucaaaagccaagaaggccaagaaagguuucaugaccccugagagaaagaagaaacuuagguuacuguugagaaagaaagccgccgaagaauuaaagaaagaacaagaacgcaaagcagccgaaaggaggcguaucauugaagaaaggugcgguaaacccaaacuugucgaugacgcaaaugaaggcccauuaaaacaaguaugugagggauaucacagacguauuguagaccuagaaaauaagaaauuugaccucgaaaaagaaguggaauucagagauuuucagaucuccgaauugaacagccaaguaaa

SEQ ID NO: 300 - RNA, 100 nt, Diabrotica virgifera
agaucuccgaauugaacagccaaguaaacgaccuuagaggcaaauucgucaaaccaaccuugaagaagguauccaaauacgaaaacaaauucgccaaacu

SEQ ID NO: 301 - RNA, 100 nt, Diabrotica virgifera
ucaaaagaaggcagcugaauuuaacuuccguaaccaacucaaaguugucaagaagaaagaauucaccuuagaagaagaagacaaagaaaagaaaccagac

SEQ ID NO: 302 - RNA, 133 nt, Diabrotica virgifera
gaccuuagaggcaaauucgucaaaccaaccuugaagaagguauccaaauacgaaaacaaauucgccaaacuucaaaagaaggcagcugaauuuaacuuccguaaccaacucaaaguugucaagaagaaagaau

SEQ ID NO: 303 - RNA, 500 nt, Diabrotica virgifera; identical to SEQ ID NO: 127

SEQ ID NO: 304 - RNA, 648 nt, Diabrotica virgifera
auggcggcaaacagaacuggaccugcucagagaccaaauggcgcuacccaaggaaagauaugucaguucaaacugguccuacuaggcgaaagugccgucgguaagucgaguuugguacugagguucgucaaaggacaguuccacgaauaccaggagaguaccauaggagcagcuuuccuuacacaaaccauaugccucgacgauacaacuguuaaauuugaaauuugggacacagcgggucaagaaagguaccacaguuuagcuccuauguacuauaggggcgcacaggcagcuauagucgucuacgacauaaccaaucaagacacauucggcagggcgaaaacgugggugaaggaacuucaaaggcaggccaguccgacgaucgugauagcuuuggccggcaacaagcaagauuuggccaacaaacguaugguagaauacgaagaggcgcagacguaugcugacgaaaacggcuuacuuuuuauggaaacuuccgcaaagacggcaaugaacgucaacgauauauuuuuagcaauagcuaagaaacugcccaagaaugaacaaaccacaggucaaggcggcagugcccaaggcaggcggcuagcggagggcgauucgggcgccaaggcacccggaaauuguugcaag

SEQ ID NO: 305 - RNA, 188 nt, Diabrotica virgifera
auggcggcaaacagaacuggaccugcucagagaccaaauggcgcuacccaaggaaagauaugucaguucaaacugguccuacuaggcgaaagugccgucgguaagucgaguuugguacugagguucgucaaaggacaguuccacgaauaccaggagaguaccauaggagcagcuuuccuuacacaaac

SEQ ID NO: 306 - RNA, 205 nt, Diabrotica virgifera
ggacaguuccacgaauaccaggagaguaccauaggagcagcuuuccuuacacaaaccauaugccucgacgauacaacuguuaaauuugaaauuugggacacagcgggucaagaaagguaccacaguuuagcuccuauguacuauaggggcgcacaggcagcuauagucgucuacgacauaaccaaucaagacacauucggcaggg

SEQ ID NO: 307 - RNA, 224 nt, Diabrotica virgifera
gcacaggcagcuauagucgucuacgacauaaccaaucaagacacauucggcagggcgaaaacgugggugaaggaacuucaaaggcaggccaguccgacgaucgugauagcuuuggccggcaacaagcaagauuuggccaacaaacguaugguagaauacgaagaggcgcagacguaugcugacgaaaacggcuuacuuuuuauggaaacuuccgcaaagacggc

SEQ ID NO: 308 - RNA, 196 nt, Diabrotica virgifera
gacguaugcugacgaaaacggcuuacuuuuuauggaaacuuccgcaaagacggcaaugaacgucaacgauauauuuuuagcaauagcuaagaaacugcccaagaaugaacaaaccacaggucaaggcggcagugcccaaggcaggcggcuagcggagggcgauucgggcgccaaggcacccggaaauuguugcaag

SEQ ID NO: 309 - RNA, 189 nt, Diabrotica virgifera; identical to SEQ ID NO: 128

SEQ ID NO: 310 - RNA, 330 nt, Diabrotica virgifera
guguguauuucagcuggaauuuguaaugaaaaaaacguagaaauauauacuacaaugaaguuuuuaagaucgacagugugcuacauugccaucuuggcaauucucuuuacccucugugccgaugagguugaaggaaggagaaaaauuuugauggggcgaaaaagcauuaccaggacauaucuucguggaaaugcuguuccugcguaugugauaauaauccuuguaggaauuggucaaaucauccugggagggauauuguacguugcauugaggaagaagaucauugcugcaccuguaacggcaucauaugcaguggcuagacaagaacca

SEQ ID NO: 311 - RNA, 197 nt, Diabrotica virgifera
guguguauuucagcuggaauuuguaaugaaaaaaacguagaaauauauacuacaaugaaguuuuuaagaucgacagugugcuacauugccaucuuggcaauucucuuuacccucugugccgaugagguugaaggaaggagaaaaauuuugauggggcgaaaaagcauuaccaggacauaucuucguggaaaugcugu

SEQ ID NO: 312 - RNA, 179 nt, Diabrotica virgifera
auggggcgaaaaagcauuaccaggacauaucuucguggaaaugcuguuccugcguaugugauaauaauccuuguaggaauuggucaaaucauccugggagggauauuguacguugcauugaggaagaagaucauugcugcaccuguaacggcaucauaugcaguggcuagacaagaacc

SEQ ID NO: 313 - DNA, 44 bp, Diabrotica virgifera
gaccttagaggcaaattcgtcaaaccaaccttgaagaaggtatc

SEQ ID NO: 314 - DNA, 45 bp, Diabrotica virgifera
caaatacgaaaacaaattcgccaaacttcaaaagaaggcagctga

SEQ ID NO: 315 - DNA, 44 bp, Diabrotica virgifera
atttaacttccgtaaccaactcaaagttgtcaagaagaaagaat

SEQ ID NO: 316 - DNA, 42 bp, Diabrotica virgifera
accaaccttgaagaaggtatccaaatacgaaaacaaattcgc

SEQ ID NO: 317 - DNA, 46 bp, Diabrotica virgifera
caaacttcaaaagaaggcagctgaatttaacttccgtaaccaactc

SEQ ID NO: 318 - DNA, 133 bp, Diabrotica virgifera
gaccttagaggcaaattcgtcaaaccaaccttgaagaaggtatcgacatggtgagcaagggcgaggagctgttcaccggggtggtgcccatcctggtcgagctggacggcgacgtaaacggccacaagttcag

SEQ ID NO: 319 - DNA, 134 bp, Diabrotica virgifera
caaatacgaaaacaaattcgccaaacttcaaaagaaggcagctgagacatggtgagcaagggcgaggagctgttcaccggggtggtgcccatcctggtcgagctggacggcgacgtaaacggccacaagttcag

SEQ ID NO: 320 - DNA, 133 bp, Diabrotica virgifera
atttaacttccgtaaccaactcaaagttgtcaagaagaaagaatgacatggtgagcaagggcgaggagctgttcaccggggtggtgcccatcctggtcgagctggacggcgacgtaaacggccacaagttcag

SEQ ID NO: 321 - DNA, 131 bp, Diabrotica virgifera
accaaccttgaagaaggtatccaaatacgaaaacaaattcgcgacatggtgagcaagggcgaggagctgttcaccggggtggtgcccatcctggtcgagctggacggcgacgtaaacggccacaagttcag

SEQ ID NO: 322 - DNA, 135 bp, Diabrotica virgifera
caaacttcaaaagaaggcagctgaatttaacttccgtaaccaactcgacatggtgagcaagggcgaggagctgttcaccggggtggtgcccatcctggtcgagctggacggcgacgtaaacggccacaagttcag

SEQ ID NO: 323 - DNA, 145 bp, Diabrotica virgifera
ggatccgacatggtgagcaagggcgaggagctgttcaccggggtggtgcccatcctggtcgaccaaccttgaagaaggtatcagctggacggcgacgtaaacggccacaagttcagcgtgtccggcgagggcgaggggcggccgc

SEQ ID NO: 324 - DNA, 145 bp, Diabrotica virgifera
ggatccgacatggtgagcaagggcgaggagctgttcaccggggtggtgcccatcctggtcgccaaccttgaagaaggtatccagctggacggcgacgtaaacggccacaagttcagcgtgtccggcgagggcgaggggcggccgc

SEQ ID NO: 325 - DNA, 145 bp, Diabrotica virgifera
ggatccgacatggtgagcaagggcgaggagctgttcaccggggtggtgcccatcctggtcgcaaccttgaagaaggtatccaagctggacggcgacgtaaacggccacaagttcagcgtgtccggcgagggcgaggggcggccgc

SEQ ID NO: 326 - DNA, 145 bp, Diabrotica virgifera
ggatccgacatggtgagcaagggcgaggagctgttcaccggggtggtgcccatcctggtcgaaccttgaagaaggtatccaaagctggacggcgacgtaaacggccacaagttcagcgtgtccggcgagggcgaggggcggccgc

SEQ ID NO: 327 - DNA, 145 bp, Diabrotica virgifera
ggatccgacatggtgagcaagggcgaggagctgttcaccggggtggtgcccatcctggtcgaccttgaagaaggtatccaatagctggacggcgacgtaaacggccacaagttcagcgtgtccggcgagggcgaggggcggccgc

SEQ ID NO: 328 - DNA, 145 bp, Diabrotica virgifera
ggatccgacatggtgagcaagggcgaggagctgttcaccggggtggtgcccatcctggtcgccttgaagaaggtatccaataagctggacggcgacgtaaacggccacaagttcagcgtgtccggcgagggcgaggggcggccgc

SEQ ID NO: 329 - DNA, 145 bp, Diabrotica virgifera
ggatccgacatggtgagcaagggcgaggagctgttcaccggggtggtgcccatcctggtcgcttgaagaaggtatccaatacagctggacggcgacgtaaacggccacaagttcagcgtgtccggcgagggcgaggggcggccgc

SEQ ID NO: 330 - DNA, 145 bp, Diabrotica virgifera
ggatccgacatggtgagcaagggcgaggagctgttcaccggggtggtgcccatcctggtcgttgaagaaggtatccaatacgagctggacggcgacgtaaacggccacaagttcagcgtgtccggcgagggcgaggggcggccgc

SEQ ID NO: 331 - DNA, 145 bp, Diabrotica virgifera
ggatccgacatggtgagcaagggcgaggagctgttcaccggggtggtgcccatcctggtcgtgaagaaggtatccaatacgaagctggacggcgacgtaaacggccacaagttcagcgtgtccggcgagggcgaggggcggccgc

SEQ ID NO: 332 - DNA, 145 bp, Diabrotica virgifera
ggatccgacatggtgagcaagggcgaggagctgttcaccggggtggtgcccatcctggtcggaagaaggtatccaatacgaaagctggacggcgacgtaaacggccacaagttcagcgtgtccggcgagggcgaggggcggccgc

SEQ ID NO: 333 - DNA, 145 bp, Diabrotica virgifera
ggatccgacatggtgagcaagggcgaggagctgttcaccggggtggtgcccatcctggtcgaagaaggtatccaatacgaaaagctggacggcgacgtaaacggccacaagttcagcgtgtccggcgagggcgaggggcggccgc

SEQ ID NO: 334 - DNA, 145 bp, Diabrotica virgifera
ggatccgacatggtgagcaagggcgaggagctgttcaccggggtggtgcccatcctggtcgagaaggtatccaatacgaaaaagctggacggcgacgtaaacggccacaagttcagcgtgtccggcgagggcgaggggcggccgc

SEQ ID NO: 335 - DNA, 145 bp, Diabrotica virgifera
ggatccgacatggtgagcaagggcgaggagctgttcaccggggtggtgcccatcctggtcggaaggtatccaatacgaaaacagctggacggcgacgtaaacggccacaagttcagcgtgtccggcgagggcgaggggcggccgc

SEQ ID NO: 336 - DNA, 145 bp, Diabrotica virgifera
ggatccgacatggtgagcaagggcgaggagctgttcaccggggtggtgcccatcctggtcgaaggtatccaatacgaaaacaagctggacggcgacgtaaacggccacaagttcagcgtgtccggcgagggcgaggggcggccgc

SEQ ID NO: 337 - DNA, 145 bp, Diabrotica virgifera
ggatccgacatggtgagcaagggcgaggagctgttcaccggggtggtgcccatcctggtcgaggtatccaatacgaaaacaaagctggacggcgacgtaaacggccacaagttcagcgtgtccggcgagggcgaggggcggccgc

SEQ ID NO: 338 - DNA, 145 bp, Diabrotica virgifera
ggatccgacatggtgagcaagggcgaggagctgttcaccggggtggtgcccatcctggtcgggtatccaatacgaaaacaaaagctggacggcgacgtaaacggccacaagttcagcgtgtccggcgagggcgaggggcggccgc

SEQ ID NO: 339 - DNA, 145 bp, Diabrotica virgifera
ggatccgacatggtgagcaagggcgaggagctgttcaccggggtggtgcccatcctggtcggtatccaatacgaaaacaaatagctggacggcgacgtaaacggccacaagttcagcgtgtccggcgagggcgaggggcggccgc

SEQ ID NO: 340 - DNA, 145 bp, Diabrotica virgifera
ggatccgacatggtgagcaagggcgaggagctgttcaccggggtggtgcccatcctggtcgtatccaatacgaaaacaaattagctggacggcgacgtaaacggccacaagttcagcgtgtccggcgagggcgaggggcggccgc

SEQ ID NO: 341 - DNA, 145 bp, Diabrotica virgifera
ggatccgacatggtgagcaagggcgaggagctgttcaccggggtggtgcccatcctggtcgatccaatacgaaaacaaattcagctggacggcgacgtaaacggccacaagttcagcgtgtccggcgagggcgaggggcggccgc

SEQ ID NO: 342 - DNA, 145 bp, Diabrotica virgifera
ggatccgacatggtgagcaagggcgaggagctgttcaccggggtggtgcccatcctggtcgtccaatacgaaaacaaattcgagctggacggcgacgtaaacggccacaagttcagcgtgtccggcgagggcgaggggcggccgc

SEQ ID NO: 343 - DNA, 145 bp, Diabrotica virgifera
ggatccgacatggtgagcaagggcgaggagctgttcaccggggtggtgcccatcctggtcgccaaatacgaaaacaaattcgagctggacggcgacgtaaacggccacaagttcagcgtgtccggcgagggcgaggggcggccgc

SEQ ID NO: 344 - DNA, 145 bp, Diabrotica virgifera
ggatccgacatggtgagcaagggcgaggagctgttcaccggggtggtgcccatcctggtcgcaaatacgaaaacaaattcgcagctggacggcgacgtaaacggccacaagttcagcgtgtccggcgagggcgaggggcggccgc

SEQ ID NO: 345 - RNA, 44 nt, Diabrotica virgifera
gaccuuagaggcaaauucgucaaaccaaccuugaagaagguauc

SEQ ID NO: 346 - RNA, 45 nt, Diabrotica virgifera
caaauacgaaaacaaauucgccaaacuucaaaagaaggcagcuga

SEQ ID NO: 347 - RNA, 44 nt, Diabrotica virgifera
auuuaacuuccguaaccaacucaaaguugucaagaagaaagaau

SEQ ID NO: 348 - RNA, 42 nt, Diabrotica virgifera
accaaccuugaagaagguauccaaauacgaaaacaaauucgc

SEQ ID NO: 349 - RNA, 46 nt, Diabrotica virgifera
caaacuucaaaagaaggcagcugaauuuaacuuccguaaccaacuc

SEQ ID NO: 350 - RNA, 21 nt, Diabrotica virgifera
accaaccuugaagaagguauc

SEQ ID NO: 351 - RNA, 21 nt, Diabrotica virgifera
ccaaccuugaagaagguaucc

SEQ ID NO: 352 - RNA, 21 nt, Diabrotica virgifera
caaccuugaagaagguaucca

SEQ ID NO: 353 - RNA, 21 nt, Diabrotica virgifera
aaccuugaagaagguauccaa

SEQ ID NO: 354 - RNA, 21 nt, Diabrotica virgifera
accuugaagaagguauccaau

SEQ ID NO: 355 - RNA, 21 nt, Diabrotica virgifera
ccuugaagaagguauccaaua

SEQ ID NO: 356 - RNA, 21 nt, Diabrotica virgifera
cuugaagaagguauccaauac

SEQ ID NO: 357 - RNA, 21 nt, Diabrotica virgifera
uugaagaagguauccaauacg

SEQ ID NO: 358 - RNA, 21 nt, Diabrotica virgifera
ugaagaagguauccaauacga

SEQ ID NO: 359 - RNA, 21 nt, Diabrotica virgifera
gaagaagguauccaauacgaa

SEQ ID NO: 360 - RNA, 21 nt, Diabrotica virgifera
aagaagguauccaauacgaaa

SEQ ID NO: 361 - RNA, 21 nt, Diabrotica virgifera
agaagguauccaauacgaaaa

SEQ ID NO: 362 - RNA, 21 nt, Diabrotica virgifera
gaagguauccaauacgaaaac

SEQ ID NO: 363 - RNA, 21 nt, Diabrotica virgifera
aagguauccaauacgaaaaca

SEQ ID NO: 364 - RNA, 21 nt, Diabrotica virgifera
agguauccaauacgaaaacaa

SEQ ID NO: 365 - RNA, 21 nt, Diabrotica virgifera
gguauccaauacgaaaacaaa

SEQ ID NO: 366 - RNA, 21 nt, Diabrotica virgifera
guauccaauacgaaaacaaau

SEQ ID NO: 367 - RNA, 21 nt, Diabrotica virgifera
uauccaauacgaaaacaaauu

SEQ ID NO: 368 - RNA, 21 nt, Diabrotica virgifera
auccaauacgaaaacaaauuc

SEQ ID NO: 369 - RNA, 21 nt, Diabrotica virgifera
uccaauacgaaaacaaauucg

SEQ ID NO: 370 - RNA, 21 nt, Diabrotica virgifera
ccaaauacgaaaacaaauucg

SEQ ID NO: 371 - RNA, 21 nt, Diabrotica virgifera
caaauacgaaaacaaauucgc

SEQ ID NO: 372 - DNA, 5055 bp, Diabrotica virgifera
atgacgcagcaactgttacctatcaagttccaagaacatttgcagcttaccaatgttggtatccatgctaccaacatcacgttcgccaatctcaccatggagagcgacaagtacatctgcgtgagagaaaaagttggagagacgtcccaagtagtcatcatagatatggccgatacggccaatcccatcagacgaccaatcaccgccgaaagtgctattatgaatccagcatccaaagtcatcgctcttaaaggtaaagcaggcgtagaaacacaaaaaacccttcaaatattcaacatagaaatgaagtcaaaaatgaaagcccacaccatgtctgaagacgtaattttctggaaatggatcagccccaatacgttagcgctagtcactgaaacttcagtgtatcattggtccatggaaggtgattcaattccacagaaaatgtttgacaggcattcttctcttaacggctgccaaatcatcaactaccgaacagatcccaaacaaaactggctgctactggtcggtattagcgctcagcaatctcgcgtcgttggtgctatgcaactgtactcagtagaaagaaaatgctcgcagccaatcgaaggtcacgccgcttctttcgcgaccttcaaaatggaaggaaaccctgaaccatcgactctcttctgttttgcagtgaggactttacaaggaggaaagttacatattatcgaggttggtcaaagtccagcaggcaaccaatcgtttcctaaaaagacagtggatgttttcttcccacccgaggcccaaaatgattttcctgtagctatgcaagtgtccgctaaatacgacgtcatttacctgattaccaaatacggctatattcatatgtatgacatcgagagcggcacctgtatctacatgaacagaatatctagtgacacaatattcgtaaccgcaccccacgaagctacgggaggaatcattggtgttaatagaaagggtcaagtcctatctgtctcggtagatgaggagagcattattcgatacatcaacaccgtcttacacaatgctgacttagcgctgcgtctagctacgagaaacaatctttcaggagccgaagaactgtttgttagtaaattccagatgttgttccagaacggacagtacgccgaagctgctaaagtggctgccaacgctccaaaaggaattttaagaaccccagctacaattcaaatgtttcaacaagtcccgactcaacctggacaaaacagtccccttttgcaatatttcggtatacttctagaccaagggcaactaaacagatacgaatctttggaattgtgtaaaccagttttgttgcaaggtcgcaaacagcttctagaaaaatggttaaaagaggaaaaattagaatgttccgaagaattaggagacctagtcaaacaggcagatcctactctggctttatctgtgtatcttagagctaatgtacctgcaaaagttatccaaagctttgccgaaactggccaattccaaaagatagtcctctacgccaaaaaagtgtcttatactcccgactatgtattcctgcttcgccaagtcatgcgcaccaatcccgaccaaggcgcagcatttgcagggatgttggtagcggacgacgaacctttggccgatatcaaccaaatcgtggacattttcatggagcaaaacatggtgcagcagtgtactgcgttcttgttggacgccttaaagaataacaggcctactgaggggcatctacaaactagactattagaaatgaacctgatgtccgcaccgcaagtagcagacgccattctcggcaacaacatgttcactcactacgaccggccccacgtagcccagctctgcgaaaaagctggtcttttacaaagagctctagaacactacactgatttgtatgacatcaaacgtgctgtggtacacacccacttgcttccagctgattggttggttaacttcttcggaactctcagcgtggaagacagtttggagtgcttgagggccatgctgaccgcgaatattcgacagaatttgcagatttgcgtgcagatcgctaccaagtaccacgaacaactcaccactaaggctttgatcgatttgtttgaaggatttaagagctatgagggtttgttctatttcctcggctccatcgtcaacttctcccaagaccaagaagtgcacttcaagtacatccaagccgcatgcaagactggccaaatcaaagaagtcgagcgtatctgtagggaatcaaactgctacaatcccgaaagagtcaagaatttcctgaaggaagccaaacttacagatcagttgccgttgattattgtctgtgacagatttgatttcgtccacgacttagtgttgtatctatatagaaattcgctgcagaaatatatcgagatttatgtccagaaggtcaatcccagccgtttaccggttgtggtaggaggtcttttagatgtcgactgttccgaagacataatcaaaaacctaattcttgtcgtcagaggccagttctccactgacgaattagtagaagaagtagaaaagaggaacagattgaaactgttgttgccctggttggagagcagagtacacgaaggatgtgtcgagccagctacgcacaatgctttggccaagatctacatcgattccaacaacaatgccgaaagattcttgaaggaaaatcaatggtacgattcccgagttgtgggacgttattgcgaaaagcgcgatccacatctggcttgcgttgcttacgaacgaggccaatgcgacagagaactgatagctgtatgtaacgaaaactctctatttaagtctgaagctcgttatttggtccgtagacgtgacggagaattatgggctgaggttttgaacgagagcaatccttacagacgtcagttgatagaccaagtagtgcaaacagctttaagtgaaacccaagaccccgaagatatctctgttaccgttaaagcattcatgacagctgatttaccaaatgagctcattgaattgttggaaaagattgtattggatagttctgtgttctccgagcatagaaaccttcaaaatttgcttatcctaacagcaatcaaagccgatgctacaagagttatggactacatcaaccgcttggataactacgatgcccctgatatcgcgaatatagccatcaacaaccatctctatgaagaagctttcgctattttcaagaaatttgatgtcaacacctcagctattcaagtattgatcgaacaagtcaacaatctggatcgtgcttatgaattcgcagaacgttgcaatgaaccggccgtatggagtcagctggccaaagcgcaactgaaccaaggcttagtcaaggaagcaatcgattcttacattaaagctgatgatccttcagcttataaggacgtcgttgagaccgcttcgaaaaataatagctgggaggacttagtgcggtatttgcagatggcaagaaagaaggccagagagagctacatcgaatctgaattgatttattcgtacgcgaagaccggaagattggctgatttggaagaattcatcagtggacccaaccatgctgatatccagaagattggtgataggtgctttgatgacaagatgtatgatgctgctaagctactctacaacaatgtatccaacttcgctcgtctcgctattactttagtgcatctaaaagaattccagggagctgttgacagtgctaggaaggctaatagtaccagaacatggaaggaagtgtgttttgcttgcgtcgatgccgaagaattcagattggctcagatgtgtggtatgcacatcgtggtacacgctgatgagttgcaagatttgattaattattatcaagatagaggatactttgaagaattaatcggcctattggaagcagcattgggcttggaaagggcacacatgggtatgttcaccgaattagcaattttgtattccaaatataagcccgccaaaatgcgcgaacatctggaactcttctggtctcgagtgaatatccccaaagttcttagggcagctgaacaagcacatttgtgggcagagctagtgtttttgtatgacaaatatgaagaatatgataacgctgtgttagccatgatggctcatcccaccgaagcttggcgcgaaggtcatttcaaggatattattacaaaagttgccaatatcgaactttattatagagctattcaattttacttggattacaaaccgctgttgttaaatgaccttttgttggtgttggcacccaggatggatcatactagggctgtttctttctttacaaaaacaggacacttacagttggttaaatcctatctccggtctgtgcaaaatttgaacaacaaagctatcaacgaggccctcaactctctacttatcgaagaagaagacttccagggtctgagaacgtccatcgacgccttcgataacttcgacaacatcggcttggctcagaaattggagaagcacgaactgacggagttcagacgcatcgccgcctacttgtacaaaggcaacaaccggtggaagcagagcgtagaactgtgcaaaaaggatagactatttagagacgctatggagtacacttctgaatctagaaatcaagaattggccgaagagttgctggcatggttcttggataggaaggcctatgattgtttttcggcatgtttgtatcactgctacgacttgttacggcccgacgttatccttgaactagcatggaaacacaacattatggacttcgcaatgcctttccttattcaagtaactagagaactgacgacaaaagtagaaaagctagaacaatcagatgcccaacgacaaagcgaggctgctgaagaaacgaacaagccaatgatgataccagaaccccaacttatgctaacggctggccctggcatgggtattccaccccaacagtatgtacctccccaaggctacgcgcagccaggctacgccccgcaaatggcttaccagggatacccaggcatgtaa

SEQ ID NO: 373 - RNA, 5055 nt, Diabrotica virgifera
augacgcagcaacuguuaccuaucaaguuccaagaacauuugcagcuuaccaauguugguauccaugcuaccaacaucacguucgccaaucucaccauggagagcgacaaguacaucugcgugagagaaaaaguuggagagacgucccaaguagucaucauagauauggccgauacggccaaucccaucagacgaccaaucaccgccgaaagugcuauuaugaauccagcauccaaagucaucgcucuuaaagguaaagcaggcguagaaacacaaaaaacccuucaaauauucaacauagaaaugaagucaaaaaugaaagcccacaccaugucugaagacguaauuuucuggaaauggaucagccccaauacguuagcgcuagucacugaaacuucaguguaucauugguccauggaaggugauucaauuccacagaaaauguuugacaggcauucuucucuuaacggcugccaaaucaucaacuaccgaacagaucccaaacaaaacuggcugcuacuggucgguauuagcgcucagcaaucucgcgucguuggugcuaugcaacuguacucaguagaaagaaaaugcucgcagccaaucgaaggucacgccgcuucuuucgcgaccuucaaaauggaaggaaacccugaaccaucgacucucuucuguuuugcagugaggacuuuacaaggaggaaaguuacauauuaucgagguuggucaaaguccagcaggcaaccaaucguuuccuaaaaagacaguggauguuuucuucccacccgaggcccaaaaugauuuuccuguagcuaugcaaguguccgcuaaauacgacgucauuuaccugauuaccaaauacggcuauauucauauguaugacaucgagagcggcaccuguaucuacaugaacagaauaucuagugacacaauauucguaaccgcaccccacgaagcuacgggaggaaucauugguguuaauagaaagggucaaguccuaucugucucgguagaugaggagagcauuauucgauacaucaacaccgucuuacacaaugcugacuuagcgcugcgucuagcuacgagaaacaaucuuucaggagccgaagaacuguuuguuaguaaauuccagauguuguuccagaacggacaguacgccgaagcugcuaaaguggcugccaacgcuccaaaaggaauuuuaagaaccccagcuacaauucaaauguuucaacaagucccgacucaaccuggacaaaacaguccccuuuugcaauauuucgguauacuucuagaccaagggcaacuaaacagauacgaaucuuuggaauuguguaaaccaguuuuguugcaaggucgcaaacagcuucuagaaaaaugguuaaaagaggaaaaauuagaauguuccgaagaauuaggagaccuagucaaacaggcagauccuacucuggcuuuaucuguguaucuuagagcuaauguaccugcaaaaguuauccaaagcuuugccgaaacuggccaauuccaaaagauaguccucuacgccaaaaaagugucuuauacucccgacuauguauuccugcuucgccaagucaugcgcaccaaucccgaccaaggcgcagcauuugcagggauguugguagcggacgacgaaccuuuggccgauaucaaccaaaucguggacauuuucauggagcaaaacauggugcagcaguguacugcguucuuguuggacgccuuaaagaauaacaggccuacugaggggcaucuacaaacuagacuauuagaaaugaaccugauguccgcaccgcaaguagcagacgccauucucggcaacaacauguucacucacuacgaccggccccacguagcccagcucugcgaaaaagcuggucuuuuacaaagagcucuagaacacuacacugauuuguaugacaucaaacgugcugugguacacacccacuugcuuccagcugauugguugguuaacuucuucggaacucucagcguggaagacaguuuggagugcuugagggccaugcugaccgcgaauauucgacagaauuugcagauuugcgugcagaucgcuaccaaguaccacgaacaacucaccacuaaggcuuugaucgauuuguuugaaggauuuaagagcuaugaggguuuguucuauuuccucggcuccaucgucaacuucucccaagaccaagaagugcacuucaaguacauccaagccgcaugcaagacuggccaaaucaaagaagucgagcguaucuguagggaaucaaacugcuacaaucccgaaagagucaagaauuuccugaaggaagccaaacuuacagaucaguugccguugauuauugucugugacagauuugauuucguccacgacuuaguguuguaucuauauagaaauucgcugcagaaauauaucgagauuuauguccagaaggucaaucccagccguuuaccgguugugguaggaggucuuuuagaugucgacuguuccgaagacauaaucaaaaaccuaauucuugucgucagaggccaguucuccacugacgaauuaguagaagaaguagaaaagaggaacagauugaaacuguuguugcccugguuggagagcagaguacacgaaggaugugucgagccagcuacgcacaaugcuuuggccaagaucuacaucgauuccaacaacaaugccgaaagauucuugaaggaaaaucaaugguacgauucccgaguugugggacguuauugcgaaaagcgcgauccacaucuggcuugcguugcuuacgaacgaggccaaugcgacagagaacugauagcuguauguaacgaaaacucucuauuuaagucugaagcucguuauuugguccguagacgugacggagaauuaugggcugagguuuugaacgagagcaauccuuacagacgucaguugauagaccaaguagugcaaacagcuuuaagugaaacccaagaccccgaagauaucucuguuaccguuaaagcauucaugacagcugauuuaccaaaugagcucauugaauuguuggaaaagauuguauuggauaguucuguguucuccgagcauagaaaccuucaaaauuugcuuauccuaacagcaaucaaagccgaugcuacaagaguuauggacuacaucaaccgcuuggauaacuacgaugccccugauaucgcgaauauagccaucaacaaccaucucuaugaagaagcuuucgcuauuuucaagaaauuugaugucaacaccucagcuauucaaguauugaucgaacaagucaacaaucuggaucgugcuuaugaauucgcagaacguugcaaugaaccggccguauggagucagcuggccaaagcgcaacugaaccaaggcuuagucaaggaagcaaucgauucuuacauuaaagcugaugauccuucagcuuauaaggacgucguugagaccgcuucgaaaaauaauagcugggaggacuuagugcgguauuugcagauggcaagaaagaaggccagagagagcuacaucgaaucugaauugauuuauucguacgcgaagaccggaagauuggcugauuuggaagaauucaucaguggacccaaccaugcugauauccagaagauuggugauaggugcuuugaugacaagauguaugaugcugcuaagcuacucuacaacaauguauccaacuucgcucgucucgcuauuacuuuagugcaucuaaaagaauuccagggagcuguugacagugcuaggaaggcuaauaguaccagaacauggaaggaaguguguuuugcuugcgucgaugccgaagaauucagauuggcucagaugugugguaugcacaucgugguacacgcugaugaguugcaagauuugauuaauuauuaucaagauagaggauacuuugaagaauuaaucggccuauuggaagcagcauugggcuuggaaagggcacacauggguauguucaccgaauuagcaauuuuguauuccaaauauaagcccgccaaaaugcgcgaacaucuggaacucuucuggucucgagugaauauccccaaaguucuuagggcagcugaacaagcacauuugugggcagagcuaguguuuuuguaugacaaauaugaagaauaugauaacgcuguguuagccaugauggcucaucccaccgaagcuuggcgcgaaggucauuucaaggauauuauuacaaaaguugccaauaucgaacuuuauuauagagcuauucaauuuuacuuggauuacaaaccgcuguuguuaaaugaccuuuuguugguguuggcacccaggauggaucauacuagggcuguuucuuucuuuacaaaaacaggacacuuacaguugguuaaauccuaucuccggucugugcaaaauuugaacaacaaagcuaucaacgaggcccucaacucucuacuuaucgaagaagaagacuuccagggucugagaacguccaucgacgccuucgauaacuucgacaacaucggcuuggcucagaaauuggagaagcacgaacugacggaguucagacgcaucgccgccuacuuguacaaaggcaacaaccgguggaagcagagcguagaacugugcaaaaaggauagacuauuuagagacgcuauggaguacacuucugaaucuagaaaucaagaauuggccgaagaguugcuggcaugguucuuggauaggaaggccuaugauuguuuuucggcauguuuguaucacugcuacgacuuguuacggcccgacguuauccuugaacuagcauggaaacacaacauuauggacuucgcaaugccuuuccuuauucaaguaacuagagaacugacgacaaaaguagaaaagcuagaacaaucagaugcccaacgacaaagcgaggcugcugaagaaacgaacaagccaaugaugauaccagaaccccaacuuaugcuaacggcuggcccuggcauggguauuccaccccaacaguauguaccuccccaaggcuacgcgcagccaggcuacgccccgcaaauggcuuaccagggauacccaggcauguaa

SEQ ID NO: 374 - RNA, 7132 nt, Diabrotica virgifera
ccggccuguacaaaagggcgacgccauauuagauguuugauucagcuagcugucaguuuagugaaaaaauugucauuuuccuuaaauuuccgaaaacguuucaauaaguaaaguggaaaguguuuaaauuuuauuuuguguuuuguugcaaagaaaaagcaacaugacgcagcaacuguuaccuaucaaguuccaagaacauuugcagcuuaccaauguugguauccaugcuaccaacaucacguucgccaaucucaccauggagagcgacaaguacaucugcgugagagaaaaaguuggagagacgucccaaguagucaucauagauauggccgauacggccaaucccaucagacgaccaaucaccgccgaaagugcuauuaugaauccagcauccaaagucaucgcucuuaaagguaaagcaggcguagaaacacaaaaaacccuucaaauauucaacauagaaaugaagucaaaaaugaaagcccacaccaugucugaagacguaauuuucuggaaauggaucagccccaauacguuagcgcuagucacugaaacuucaguguaucauugguccauggaaggugauucaauuccacagaaaauguuugacaggcauucuucucuuaacggcugccaaaucaucaacuaccgaacagaucccaaacaaaacuggcugcuacuggucgguauuagcgcucagcaaucucgcgucguuggugcuaugcaacuguacucaguagaaagaaaaugcucgcagccaaucgaaggucacgccgcuucuuucgcgaccuucaaaauggaaggaaacccugaaccaucgacucucuucuguuuugcagugaggacuuuacaaggaggaaaguuacauauuaucgagguuggucaaaguccagcaggcaaccaaucguuuccuaaaaagacaguggauguuuucuucccacccgaggcccaaaaugauuuuccuguagcuaugcaaguguccgcuaaauacgacgucauuuaccugauuaccaaauacggcuauauucauauguaugacaucgagagcggcaccuguaucuacaugaacagaauaucuagugacacaauauucguaaccgcaccccacgaagcuacgggaggaaucauugguguuaauagaaagggucaaguccuaucugucucgguagaugaggagagcauuauucgauacaucaacaccgucuuacacaaugcugacuuagcgcugcgucuagcuacgagaaacaaucuuucaggagccgaagaacuguuuguuaguaaauuccagauguuguuccagaacggacaguacgccgaagcugcuaaaguggcugccaacgcuccaaaaggaauuuuaagaaccccagcuacaauucaaauguuucaacaagucccgacucaaccuggacaaaacaguccccuuuugcaauauuucgguauacuucuagaccaagggcaacuaaacagauacgaaucuuuggaauuguguaaaccaguuuuguugcaaggucgcaaacagcuucuagaaaaaugguuaaaagaggaaaaauuagaauguuccgaagaauuaggagaccuagucaaacaggcagauccuacucuggcuuuaucuguguaucuuagagcuaauguaccugcaaaaguuauccaaagcuuugccgaaacuggccaauuccaaaagauaguccucuacgccaaaaaagugucuuauacucccgacuauguauuccugcuucgccaagucaugcgcaccaaucccgaccaaggcgcagcauuugcagggauguugguagcggacgacgaaccuuuggccgauaucaaccaaaucguggacauuuucauggagcaaaacauggugcagcaguguacugcguucuuguuggacgccuuaaagaauaacaggccuacugaggggcaucuacaaacuagacuauuagaaaugaaccugauguccgcaccgcaaguagcagacgccauucucggcaacaacauguucacucacuacgaccggccccacguagcccagcucugcgaaaaagcuggucuuuuacaaagagcucuagaacacuacacugauuuguaugacaucaaacgugcugugguacacacccacuugcuuccagcugauugguugguuaacuucuucggaacucucagcguggaagacaguuuggagugcuugagggccaugcugaccgcgaauauucgacagaauuugcagauuugcgugcagaucgcuaccaaguaccacgaacaacucaccacuaaggcuuugaucgauuuguuugaaggauuuaagagcuaugaggguuuguucuauuuccucggcuccaucgucaacuucucccaagaccaagaagugcacuucaaguacauccaagccgcaugcaagacuggccaaaucaaagaagucgagcguaucuguagggaaucaaacugcuacaaucccgaaagagucaagaauuuccugaaggaagccaaacuuacagaucaguugccguugauuauugucugugacagauuugauuucguccacgacuuaguguuguaucuauauagaaauucgcugcagaaauauaucgagauuuauguccagaaggucaaucccagccguuuaccgguugugguaggaggucuuuuagaugucgacuguuccgaagacauaaucaaaaaccuaauucuugucgucagaggccaguucuccacugacgaauuaguagaagaaguagaaaagaggaacagauugaaacuguuguugcccugguuggagagcagaguacacgaaggaugugucgagccagcuacgcacaaugcuuuggccaagaucuacaucgauuccaacaacaaugccgaaagauucuugaaggaaaaucaaugguacgauucccgaguugugggacguuauugcgaaaagcgcgauccacaucuggcuugcguugcuuacgaacgaggccaaugcgacagagaacugauagcuguauguaacgaaaacucucuauuuaagucugaagcucguuauuugguccguagacgugacggagaauuaugggcugagguuuugaacgagagcaauccuuacagacgucaguugauagaccaaguagugcaaacagcuuuaagugaaacccaagaccccgaagauaucucuguuaccguuaaagcauucaugacagcugauuuaccaaaugagcucauugaauuguuggaaaagauuguauuggauaguucuguguucuccgagcauagaaaccuucaaaauuugcuuauccuaacagcaaucaaagccgaugcuacaagaguuauggacuacaucaaccgcuuggauaacuacgaugccccugauaucgcgaauauagccaucaacaaccaucucuaugaagaagcuuucgcuauuuucaagaaauuugaugucaacaccucagcuauucaaguauugaucgaacaagucaacaaucuggaucgugcuuaugaauucgcagaacguugcaaugaaccggccguauggagucagcuggccaaagcgcaacugaaccaaggcuuagucaaggaagcaaucgauucuuacauuaaagcugaugauccuucagcuuauaaggacgucguugagaccgcuucgaaaaauaauagcugggaggacuuagugcgguauuugcagauggcaagaaagaaggccagagagagcuacaucgaaucugaauugauuuauucguacgcgaagaccggaagauuggcugauuuggaagaauucaucaguggacccaaccaugcugauauccagaagauuggugauaggugcuuugaugacaagauguaugaugcugcuaagcuacucuacaacaauguauccaacuucgcucgucucgcuauuacuuuagugcaucuaaaagaauuccagggagcuguugacagugcuaggaaggcuaauaguaccagaacauggaaggaaguguguuuugcuugcgucgaugccgaagaauucagauuggcucagaugugugguaugcacaucgugguacacgcugaugaguugcaagauuugauuaauuauuaucaagauagaggauacuuugaagaauuaaucggccuauuggaagcagcauugggcuuggaaagggcacacauggguauguucaccgaauuagcaauuuuguauuccaaauauaagcccgccaaaaugcgcgaacaucuggaacucuucuggucucgagugaauauccccaaaguucuuagggcagcugaacaagcacauuugugggcagagcuaguguuuuuguaugacaaauaugaagaauaugauaacgcuguguuagccaugauggcucaucccaccgaagcuuggcgcgaaggucauuucaaggauauuauuacaaaaguugccaauaucgaacuuuauuauagagcuauucaauuuuacuuggauuacaaaccgcuguuguuaaaugaccuuuuguugguguuggcacccaggauggaucauacuagggcuguuucuuucuuuacaaaaacaggacacuuacaguugguuaaauccuaucuccggucugugcaaaauuugaacaacaaagcuaucaacgaggcccucaacucucuacuuaucgaagaagaagacuuccagggucugagaacguccaucgacgccuucgauaacuucgacaacaucggcuuggcucagaaauuggagaagcacgaacugacggaguucagacgcaucgccgccuacuuguacaaaggcaacaaccgguggaagcagagcguagaacugugcaaaaaggauagacuauuuagagacgcuauggaguacacuucugaaucuagaaaucaagaauuggccgaagaguugcuggcaugguucuuggauaggaaggccuaugauuguuuuucggcauguuuguaucacugcuacgacuuguuacggcccgacguuauccuugaacuagcauggaaacacaacauuauggacuucgcaaugccuuuccuuauucaaguaacuagagaacugacgacaaaaguagaaaagcuagaacaaucagaugcccaacgacaaagcgaggcugcugaagaaacgaacaagccaaugaugauaccagaaccccaacuuaugcuaacggcuggcccuggcauggguauuccaccccaacaguauguaccuccccaaggcuacgcgcagccaggcuacgccccgcaaauggcuuaccagggauacccaggcauguaauauaaggccccuuuuacagccaacuguauaggaaaguggaauuaguuuucaaguuaaacugaggagcuagugcuaaggacaauagagaaguuauaacuaaaaaaauagcgguuccaauucguuucguguauuaugaacaacguuacuuucuaaaagaagaagaauauauugaggaguucguuuuaaaauuauguacaaguagaaguuuuaauacuugguuaacuaaaaacguuacauuuuuuugagauuacaaauaacugaauaauugaaaauauuacuuacaauuuuaugcgaacugcucgauaaauuucucaaaaauagcaaaacaaauaauagguuuauugaaguguuacagaaaauuuaggcauuuccuuuaaaucaaauaaauguuucauuauuugugugaaaaguuauuuauuaacauuauucaucuuuugcuaaaaaacaguugagauuauugcaaaauguuauugcauuuugaaaguaaagauguaaauguguuacaaaugaucuauuuguaguuuugucaucauuauguuuuguuuuuccguccauuguugaguauauuucuucauaaauaaaguaucagaugauguuuauauauaauacaauaauuuuuauucuuuaaucgcuucaauauuuguuauaaugucuucaauuucaacauauuguuuuuuuugucguauuggucuuuuuaguguuuccugccaccucuaaccaauuauuaggcgauuuuacaugaggauuaagccuacagaugucaaaauggcgucauaucuaucgaaugacaacugacaguugaagugucauauuuaaauuaugaucauacuguuccgucuuucuucgucuguaauucuaauucguucauaacgaucuaccuacucuuuucauuuuuuuuuguguaguuauuuaggcauuuuuaagucuacgacugucaaaauagugucaacugacaaguuggaagugucauacuuaaauuaucaccauuuuauccugacucccuuugucuucaauuuugauuucauaauaauuuuuauuucagugcccacuugaaccuuuuuuuauaauuuacauaucucauagucauuuuuaggcguuuaacuuacaacauuguuuccacacacauuuuccagcuucgauaucaguuauugauuuacaauaauuuaaauuugcuccuuuauacaaauguaacaacccaauuccaacccuuuuauuaauuuucuuuuuguuuugauaagauuuauuugcaacaaacaauucuagcgaaggaagaauuuccaacaaguuaaaaacaaacuuauuucaauugucaaaccuuuuaauuuucuuucgaaaucuugauauuucuuucgcuagaauaauugccccaaauugaauuucagguacuuuccuucgagucaagaucuggucauaaccccaaaaaagacaguugacgugucgugucaugacacugacguuugaacacuucaauugucaguugucauggaagaccguugguagagauaaaaugaccaaauuuucuguagcacauuauguaagcuuaaagcuuaaagaauaaaugcuuaaacaaauucuaguuaaauacaaucaaucuuguugaacuguuuguuguaguuuuaauucauucgcaucauuuucggacauuaggcuucguuuugacgggacacuugauuuacuuuuucaguuggagaauguauauauauuuuuauguacuagcaccccacuuuagaauguauauaaucuaaagaaauuauuuuguuuuccgagagaauuaucaaugcguucuuuuguuuguuuucuuuuuuuuaguccguuuaucauuccuuuauuuaaacauagauauauguauaugaagugacuauuuaacuuauauuauuauaugaauuauaugaaagugauucuucaauguuuaau

SEQ ID NO: 375 - RNA, 5055 nt, Diabrotica virgifera
uacugcgucguugacaauggauaguucaagguucuuguaaacgucgaaugguuacaaccauagguacgaugguuguagugcaagcgguuagagugguaccucucgcuguucauguagacgcacucucuuuuucaaccucucugcaggguucaucaguaguaucuauaccggcuaugccgguuaggguagucugcugguuaguggcggcuuucacgauaauacuuaggucguagguuucaguagcgagaauuuccauuucguccgcaucuuuguguuuuuugggaaguuuauaaguuguaucuuuacuucaguuuuuacuuucgggugugguacagacuucugcauuaaaagaccuuuaccuagucgggguuaugcaaucgcgaucagugacuuugaagucacauaguaaccagguaccuuccacuaaguuaaggugucuuuuacaaacuguccguaagaagagaauugccgacgguuuaguaguugauggcuugucuaggguuuguuuugaccgacgaugaccagccauaaucgcgagucguuagagcgcagcaaccacgauacguugacaugagucaucuuucuuuuacgagcgucgguuagcuuccagugcggcgaagaaagcgcuggaaguuuuaccuuccuuugggacuugguagcugagagaagacaaaacgucacuccugaaauguuccuccuuucaauguauaauagcuccaaccaguuucaggucguccguugguuagcaaaggauuuuucugucaccuacaaaagaagggugggcuccggguuuuacuaaaaggacaucgauacguucacaggcgauuuaugcugcaguaaauggacuaaugguuuaugccgauauaaguauacauacuguagcucucgccguggacauagauguacuugucuuauagaucacuguguuauaagcauuggcguggggugcuucgaugcccuccuuaguaaccacaauuaucuuucccaguucaggauagacagagccaucuacuccucucguaauaagcuauguaguuguggcagaauguguuacgacugaaucgcgacgcagaucgaugcucuuuguuagaaaguccucggcuucuugacaaacaaucauuuaaggucuacaacaaggucuugccugucaugcggcuucgacgauuucaccgacgguugcgagguuuuccuuaaaauucuuggggucgauguuaaguuuacaaaguuguucagggcugaguuggaccuguuuugucaggggaaaacguuauaaagccauaugaagaucugguucccguugauuugucuaugcuuagaaaccuuaacacauuuggucaaaacaacguuccagcguuugucgaagaucuuuuuaccaauuuucuccuuuuuaaucuuacaaggcuucuuaauccucuggaucaguuuguccgucuaggaugagaccgaaauagacacauagaaucucgauuacauggacguuuucaauagguuucgaaacggcuuugaccgguuaagguuuucuaucaggagaugcgguuuuuucacagaauaugagggcugauacauaaggacgaagcgguucaguacgcgugguuagggcugguuccgcgucguaaacgucccuacaaccaucgccugcugcuuggaaaccggcuauaguugguuuagcaccuguaaaaguaccucguuuuguaccacgucgucacaugacgcaagaacaaccugcggaauuucuuauuguccggaugacuccccguagauguuugaucugauaaucuuuacuuggacuacaggcguggcguucaucgucugcgguaagagccguuguuguacaagugagugaugcuggccggggugcaucgggucgagacgcuuuuucgaccagaaaauguuucucgagaucuugugaugugacuaaacauacuguaguuugcacgacaccaugugugggugaacgaaggucgacuaaccaaccaauugaagaagccuugagagucgcaccuucugucaaaccucacgaacucccgguacgacuggcgcuuauaagcugucuuaaacgucuaaacgcacgucuagcgaugguucauggugcuuguugaguggugauuccgaaacuagcuaaacaaacuuccuaaauucucgauacucccaaacaagauaaaggagccgagguagcaguugaagaggguucugguucuucacgugaaguucauguagguucggcguacguucugaccgguuuaguuucuucagcucgcauagacaucccuuaguuugacgauguuagggcuuucucaguucuuaaaggacuuccuucgguuugaaugucuagucaacggcaacuaauaacagacacugucuaaacuaaagcaggugcugaaucacaacauagauauaucuuuaagcgacgucuuuauauagcucuaaauacaggucuuccaguuagggucggcaaauggccaacaccauccuccagaaaaucuacagcugacaaggcuucuguauuaguuuuuggauuaagaacagcagucuccggucaagaggugacugcuuaaucaucuucuucaucuuuucuccuugucuaacuuugacaacaacgggaccaaccucucgucucaugugcuuccuacacagcucggucgaugcguguuacgaaaccgguucuagauguagcuaagguuguuguuacggcuuucuaagaacuuccuuuuaguuaccaugcuaagggcucaacacccugcaauaacgcuuuucgcgcuagguguagaccgaacgcaacgaaugcuugcuccgguuacgcugucucuugacuaucgacauacauugcuuuugagagauaaauucagacuucgagcaauaaaccaggcaucugcacugccucuuaauacccgacuccaaaacuugcucucguuaggaaugucugcagucaacuaucugguucaucacguuugucgaaauucacuuuggguucuggggcuucuauagagacaauggcaauuucguaaguacugucgacuaaaugguuuacucgaguaacuuaacaaccuuuucuaacauaaccuaucaagacacaagaggcucguaucuuuggaaguuuuaaacgaauaggauugucguuaguuucggcuacgauguucucaauaccugauguaguuggcgaaccuauugaugcuacggggacuauagcgcuuauaucgguaguuguugguagagauacuucuucgaaagcgauaaaaguucuuuaaacuacaguuguggagucgauaaguucauaacuagcuuguucaguuguuagaccuagcacgaauacuuaagcgucuugcaacguuacuuggccggcauaccucagucgaccgguuucgcguugacuugguuccgaaucaguuccuucguuagcuaagaauguaauuucgacuacuaggaagucgaauauuccugcagcaacucuggcgaagcuuuuuauuaucgacccuccugaaucacgccauaaacgucuaccguucuuucuuccggucucucucgauguagcuuagacuuaacuaaauaagcaugcgcuucuggccuucuaaccgacuaaaccuucuuaaguagucaccuggguugguacgacuauaggucuucuaaccacuauccacgaaacuacuguucuacauacuacgacgauucgaugagauguuguuacauagguugaagcgagcagagcgauaaugaaaucacguagauuuucuuaaggucccucgacaacugucacgauccuuccgauuaucauggucuuguaccuuccuucacacaaaacgaacgcagcuacggcuucuuaagucuaaccgagucuacacaccauacguguagcaccaugugcgacuacucaacguucuaaacuaauuaauaauaguucuaucuccuaugaaacuucuuaauuagccggauaaccuucgucguaacccgaaccuuucccguguguacccauacaaguggcuuaaucguuaaaacauaagguuuauauucgggcgguuuuacgcgcuuguagaccuugagaagaccagagcucacuuauagggguuucaagaaucccgucgacuuguucguguaaacacccgucucgaucacaaaaacauacuguuuauacuucuuauacuauugcgacacaaucgguacuaccgaguaggguggcuucgaaccgcgcuuccaguaaaguuccuauaauaauguuuucaacgguuauagcuugaaauaauaucucgauaaguuaaaaugaaccuaauguuuggcgacaacaauuuacuggaaaacaaccacaaccguggguccuaccuaguaugaucccgacaaagaaagaaauguuuuuguccugugaaugucaaccaauuuaggauagaggccagacacguuuuaaacuuguuguuucgauaguugcuccgggaguugagagaugaauagcuucuucuucugaaggucccagacucuugcagguagcugcggaagcuauugaagcuguuguagccgaaccgagucuuuaaccucuucgugcuugacugccucaagucugcguagcggcggaugaacauguuuccguuguuggccaccuucgucucgcaucuugacacguuuuuccuaucugauaaaucucugcgauaccucaugugaagacuuagaucuuuaguucuuaaccggcuucucaacgaccguaccaagaaccuauccuuccggauacuaacaaaaagccguacaaacauagugacgaugcugaacaaugccgggcugcaauaggaacuugaucguaccuuuguguuguaauaccugaagcguuacggaaaggaauaaguucauugaucucuugacugcuguuuucaucuuuucgaucuuguuagucuacggguugcuguuucgcuccgacgacuucuuugcuuguucgguuacuacuauggucuugggguugaauacgauugccgaccgggaccguacccauaaggugggguugucauacauggagggguuccgaugcgcgucgguccgaugcggggcguuuaccgaauggucccuauggguccguacauu

SEQ ID NO: 376 - protein, 1684 aa, Diabrotica virgifera
MTQQLLPIKFQEHLQLTNVGIHATNITFANLTMESDKYICVREKVGETSQVVIIDMADTANPIRRPITAESAIMNPASKVIALKGKAGVETQKTLQIFNIEMKSKMKAHTMSEDVIFWKWISPNTLALVTETSVYHWSMEGDSIPQKMFDRHSSLNGCQIINYRTDPKQNWLLLVGISAQQSRVVGAMQLYSVERKCSQPIEGHAASFATFKMEGNPEPSTLFCFAVRTLQGGKLHIIEVGQSPAGNQSFPKKTVDVFFPPEAQNDFPVAMQVSAKYDVIYLITKYGYIHMYDIESGTCIYMNRISSDTIFVTAPHEATGGIIGVNRKGQVLSVSVDEESIIRYINTVLHNADLALRLATRNNLSGAEELFVSKFQMLFQNGQYAEAAKVAANAPKGILRTPATIQMFQQVPTQPGQNSPLLQYFGILLDQGQLNRYESLELCKPVLLQGRKQLLEKWLKEEKLECSEELGDLVKQADPTLALSVYLRANVPAKVIQSFAETGQFQKIVLYAKKVSYTPDYVFLLRQVMRTNPDQGAAFAGMLVADDEPLADINQIVDIFMEQNMVQQCTAFLLDALKNNRPTEGHLQTRLLEMNLMSAPQVADAILGNNMFTHYDRPHVAQLCEKAGLLQRALEHYTDLYDIKRAVVHTHLLPADWLVNFFGTLSVEDSLECLRAMLTANIRQNLQICVQIATKYHEQLTTKALIDLFEGFKSYEGLFYFLGSIVNFSQDQEVHFKYIQAACKTGQIKEVERICRESNCYNPERVKNFLKEAKLTDQLPLIIVCDRFDFVHDLVLYLYRNSLQKYIEIYVQKVNPSRLPVVVGGLLDVDCSEDIIKNLILVVRGQFSTDELVEEVEKRNRLKLLLPWLESRVHEGCVEPATHNALAKIYIDSNNNAERFLKENQWYDSRVVGRYCEKRDPHLACVAYERGQCDRELIAVCNENSLFKSEARYLVRRRDGELWAEVLNESNPYRRQLIDQVVQTALSETQDPEDISVTVKAFMTADLPNELIELLEKIVLDSSVFSEHRNLQNLLILTAIKADATRVMDYINRLDNYDAPDIANIAINNHLYEEAFAIFKKFDVNTSAIQVLIEQVNNLDRAYEFAERCNEPAVWSQLAKAQLNQGLVKEAIDSYIKADDPSAYKDVVETASKNNSWEDLVRYLQMARKKARESYIESELIYSYAKTGRLADLEEFISGPNHADIQKIGDRCFDDKMYDAAKLLYNNVSNFARLAITLVHLKEFQGAVDSARKANSTRTWKEVCFACVDAEEFRLAQMCGMHIVVHADELQDLINYYQDRGYFEELIGLLEAALGLERAHMGMFTELAILYSKYKPAKMREHLELFWSRVNIPKVLRAAEQAHLWAELVFLYDKYEEYDNAVLAMMAHPTEAWREGHFKDIITKVANIELYYRAIQFYLDYKPLLLNDLLLVLAPRMDHTRAVSFFTKTGHLQLVKSYLRSVQNLNNKAINEALNSLLIEEEDFQGLRTSIDAFDNFDNIGLAQKLEKHELTEFRRIAAYLYKGNNRWKQSVELCKKDRLFRDAMEYTSESRNQELAEELLAWFLDRKAYDCFSACLYHCYDLLRPDVILELAWKHNIMDFAMPFLIQVTRELTTKVEKLEQSDAQRQSEAAEETNKPMMIPEPQLMLTAGPGMGIPPQQYVPPQGYAQPGYAPQMAYQGYPGM

SEQ ID NO: 377 - DNA, 2975 bp, Diabrotica barberi
atgcaagtgtccgctaagtacgacgtcatttacctgatcaccaaatacggctatattcatatgtatgacatcgagagcggtacctgtatctacatattcgtaaccgcaccccacgaagctacaggaggaatcattggtgttaatagaaaaggtcaagtcctatccgtctccgtagacgaggagagcatcattcgatacatcaacaccgtcttacacaatgctgacttagcgctgcgtctagctacgagaaacaatctttcaggagcagaagaactgtttgttagtaaattccagatgttgttccagaatggacagtatgccgaagctgccaaagtggctgccaacgctccaaaaggaattttaagaaccccagctacaattcaaatgtttcaacaagtcccgacccaacctggacaaaacagtcctcttttgcaatatttcggtatacttctagaccaagggcaattgaacagatatgaatctttggaactgtgtaaaccagttttgttgcaaggtcgcaaacaacttctagaaaaatggttaaaagaggaaaaattagaatgttccgaagaattaggagacctagtcaaacaggcggatcctactctggctttatctgtgtatcttagagctaatgtacctgcaaaagttatccaaagctttgccgaaacaggccaattccaaaagatagtcctctacgccaaaaaagtgtcttatactcccgactatgtattcctgcttcgccaagtcatgcgcaccaatcccgaccaaggcgccgcattcgcagggatgttggtagcagacgacgaacctttggcagacatcaaccaaatcgtggacattttcatggaacaaaacatggtgcaacagtgtactgcgttcctgttggacgccttaaagaataacaggcctactgaggggcatctacaaactagattattagaaatgaacctgatgtctgcaccgcaagtggctgacgccatcctcggcaacaacatgttcactcactacgaccggccccacgtagcccagctctgcgagaaagctggtcttttacagagagctctagaacactacactgacttgtatgacatcaaacgtgctgtggtacacactcacttgcttccagccgattggttggttaacttcttcggaactctgagcgtggaagatagtttggagtgcttgagggccatgttgacggcgaatattcggcagaatttacagatttgtgtgcagatcgctactaagtaccacgaacaactcaccactaaggctttgatcgatttgtttgaaggatttaagagctatgagggtttgttctatttcctcggctccatcgtcaacttctcccaagaccaagaagtgcacttcaagtacatccaagccgcatgcaaaactggccagatcaaagaagtcgagcgtatttgtagggagtcgaactgctacaatcccgaaagagtcaagaatttcctgaaggaagccaaacttacagatcagttgccgttgattattgtctgtgacagatttgatttcgtccacgacttggtgttgtatctatatagaaattcgctgcagaaatatatcgagatttatgtccagaaggtcaatcctagccgtttaccggttgtagtaggaggtcttttggatgtcgactgttccgaagacataatcaaaaaccttattctagtcgtcagaggccagttctccactgacgaattagtagaagaagtagaaaagagaaacagattgaaacttttgttgccctggttggagagcagagtacacgaaggatgtgtcgaaccagccacgcacaatgctttggccaagatctacatcgattccaacaacaatgccgaaagattcttgaaggaaaatcaatggtacgattcccgagttgttggacgttattgcgaaaagcgcgatccacatctggcttgcgttgcttacgaacgaggccaatgcgacagagaactgatagctgtatgtaacgaaaactctctattcaagtcagaagcacgttatttggtccgtagacgtgacggagaattatgggctgaggttttgaacgagagcaatccttacagacgtcagttgatagaccaagtagtgcaaacagctttaagtgaaacccaagaccccgaagatatatccgttaccgttaaagcattcatgacagctgatttaccaaatgaactcattgaattgctggaaaagattgtgctggatagttctgtattctccgagcatagaaaccttcaaaacttgcttatcctaacagcaatcaaagccgatgctacaagagttatggactacatcaaccgcttggataactacgatgctcctgatatcgccaatatagccatcaacaaccatctctatgaagaagctttcgctattttcaagaaatttgatgtcaacacttctgctattcaagtattaatcgaacaagtcaacaacctggatcgtgcttacgaattcgcagaacgttgcaatgaaccagccgtatggagccagctggccaaagcccaactaaaccaaggcttagttaaagaagcaatcgattcttacattaaagctgatgatccttcagcatacaaggacgtcgttgagaccgcttctaaaaataatagttgggaggacttggtccggtatttgcagatggcaagaaagaaggctagagagagctacatcgaatctgaattgatttattcgtatgcaaagaccggaagattagctgatttggaagaattcatcagtggacccaaccatgctgatatccagaagattggtgataggtgctttgacgacaagatgtatgatgctgccaagctactctacaacaatgtatccaacttcgctcgtctcgctattactttagtgcatctaaaagaattccagggagctgttgacagtgctaggaaggctaatagtaccagaacatggaaggaagtgtgttttgcttgcgtcgatgc

SEQ ID NO: 378 - RNA, 2975 nt, Diabrotica barberi
augcaaguguccgcuaaguacgacgucauuuaccugaucaccaaauacggcuauauucauauguaugacaucgagagcgguaccuguaucuacauauucguaaccgcaccccacgaagcuacaggaggaaucauugguguuaauagaaaaggucaaguccuauccgucuccguagacgaggagagcaucauucgauacaucaacaccgucuuacacaaugcugacuuagcgcugcgucuagcuacgagaaacaaucuuucaggagcagaagaacuguuuguuaguaaauuccagauguuguuccagaauggacaguaugccgaagcugccaaaguggcugccaacgcuccaaaaggaauuuuaagaaccccagcuacaauucaaauguuucaacaagucccgacccaaccuggacaaaacaguccucuuuugcaauauuucgguauacuucuagaccaagggcaauugaacagauaugaaucuuuggaacuguguaaaccaguuuuguugcaaggucgcaaacaacuucuagaaaaaugguuaaaagaggaaaaauuagaauguuccgaagaauuaggagaccuagucaaacaggcggauccuacucuggcuuuaucuguguaucuuagagcuaauguaccugcaaaaguuauccaaagcuuugccgaaacaggccaauuccaaaagauaguccucuacgccaaaaaagugucuuauacucccgacuauguauuccugcuucgccaagucaugcgcaccaaucccgaccaaggcgccgcauucgcagggauguugguagcagacgacgaaccuuuggcagacaucaaccaaaucguggacauuuucauggaacaaaacauggugcaacaguguacugcguuccuguuggacgccuuaaagaauaacaggccuacugaggggcaucuacaaacuagauuauuagaaaugaaccugaugucugcaccgcaaguggcugacgccauccucggcaacaacauguucacucacuacgaccggccccacguagcccagcucugcgagaaagcuggucuuuuacagagagcucuagaacacuacacugacuuguaugacaucaaacgugcugugguacacacucacuugcuuccagccgauugguugguuaacuucuucggaacucugagcguggaagauaguuuggagugcuugagggccauguugacggcgaauauucggcagaauuuacagauuugugugcagaucgcuacuaaguaccacgaacaacucaccacuaaggcuuugaucgauuuguuugaaggauuuaagagcuaugaggguuuguucuauuuccucggcuccaucgucaacuucucccaagaccaagaagugcacuucaaguacauccaagccgcaugcaaaacuggccagaucaaagaagucgagcguauuuguagggagucgaacugcuacaaucccgaaagagucaagaauuuccugaaggaagccaaacuuacagaucaguugccguugauuauugucugugacagauuugauuucguccacgacuugguguuguaucuauauagaaauucgcugcagaaauauaucgagauuuauguccagaaggucaauccuagccguuuaccgguuguaguaggaggucuuuuggaugucgacuguuccgaagacauaaucaaaaaccuuauucuagucgucagaggccaguucuccacugacgaauuaguagaagaaguagaaaagagaaacagauugaaacuuuuguugcccugguuggagagcagaguacacgaaggaugugucgaaccagccacgcacaaugcuuuggccaagaucuacaucgauuccaacaacaaugccgaaagauucuugaaggaaaaucaaugguacgauucccgaguuguuggacguuauugcgaaaagcgcgauccacaucuggcuugcguugcuuacgaacgaggccaaugcgacagagaacugauagcuguauguaacgaaaacucucuauucaagucagaagcacguuauuugguccguagacgugacggagaauuaugggcugagguuuugaacgagagcaauccuuacagacgucaguugauagaccaaguagugcaaacagcuuuaagugaaacccaagaccccgaagauauauccguuaccguuaaagcauucaugacagcugauuuaccaaaugaacucauugaauugcuggaaaagauugugcuggauaguucuguauucuccgagcauagaaaccuucaaaacuugcuuauccuaacagcaaucaaagccgaugcuacaagaguuauggacuacaucaaccgcuuggauaacuacgaugcuccugauaucgccaauauagccaucaacaaccaucucuaugaagaagcuuucgcuauuuucaagaaauuugaugucaacacuucugcuauucaaguauuaaucgaacaagucaacaaccuggaucgugcuuacgaauucgcagaacguugcaaugaaccagccguauggagccagcuggccaaagcccaacuaaaccaaggcuuaguuaaagaagcaaucgauucuuacauuaaagcugaugauccuucagcauacaaggacgucguugagaccgcuucuaaaaauaauaguugggaggacuugguccgguauuugcagauggcaagaaagaaggcuagagagagcuacaucgaaucugaauugauuuauucguaugcaaagaccggaagauuagcugauuuggaagaauucaucaguggacccaaccaugcugauauccagaagauuggugauaggugcuuugacgacaagauguaugaugcugccaagcuacucuacaacaauguauccaacuucgcucgucucgcuauuacuuuagugcaucuaaaagaauuccagggagcuguugacagugcuaggaaggcuaauaguaccagaacauggaaggaaguguguuuugcuugcgucgaugc

SEQ ID NO: 379 - DNA, 5055 bp, Diabrotica undecimpunctata
atgacgcagcaactgttacctatcaagttccaagaacatttgcagcttaccaatgttggtatccatgctaccaacatcacgttcgccaatctcaccatggagagtgacaagtacatctgcgtgagagaaaaagtcggagagacgtcccaagtagtcatcatagatatggccgacacggccaatcccatcagacgaccaatcaccgccgaaagtgctattatgaatccagcatccaaagtcattgctcttaaaggtaaagccggcgtagaaacacaaaaaacacttcaaatatttaacatagaaatgaagtcaaaaatgaaagcccacaccatgtccgaagacgtaattttctggaaatggataagccccaatacgttagctctagtcaccgagacttcagtgtatcattggtccatggaaggtgattccactccacagaaaatgttcgacagacactcttctcttaacggctgccaaatcatcaactaccgtacagatcccaaacaaaactggctgctacttgtcggtatcagcgctcaacagtcccgcgtcgttggtgctatgcaactctattcagtagaaagaaaatgctcccagccgatcgaaggacacgccgcttcttttgccaccttcaaaatggaaggaaatcctgaaccatcgacgctcttctgtttcgcagtgagaactttacagggaggaaaattgcatattatcgaggttggccaaagtccagcaggcaatcaatcgttccccaaaaagacagtggacgttttcttcccgcccgaggcccaaaacgattttcctgtagccatgcaagtatcagctaagtacgacgtcatttacctgatcaccaaatacggctacattcatatgtatgatattgagaccggcacttgtatctatatgaacagaatatccagtgaaaccatattcgtaaccgcaccccacgaagctactggaggaataattggtgtaaatagaaaaggtcaagtactatccgtctccgtagacgaggagagcatcattcggtacatcaacaccgtcttgcacaatgcagacttagcgctgcgtctagctacgagaaacaatctctcaggagccgaagaactgtttgttagtaaatttcagatgttgttccagaatggacagtacgccgaagctgccaaagtggctgccaacgctccaaaaggaattttaagaaccccagctacaattcaaatgtttcaacaagtcccgactcaacctggacaaaacagtcctctcttacaatatttcggtatacttttagaccaaggacaactaaacagatacgaatctttggaactatgtaaaccagttttgttgcaaggtcgcaaacagctgctagaaaaatggttaaaagaagaaaaattagaatgttccgaggaattaggagacctagtcaaacaggcagaccctactctggctttatctgtgtatcttagagctaatgtacctgcaaaagttatccaaagctttgctgaaacaggccaattccaaaagatagtcctctacgccaaaaaagtgtcctatacgcccgactatatattcctgcttcgccaagtcatgcgcaccaatcccgaccaaggcgccgcgttcgccgggatgttggtagcagacgaagaacctttggccgacatcaaccaaatcgtggacattttcatggaacaaaacatggtgcagcagtgtactgcgtttttgttggacgccttaaagaataacaggcctactgaggggcatctacaaaccagactgttagaaatgaacctgatgtctgcaccgcaagtggcagacgccattctcggcaacaacatgttcactcactacgaccggcctcacgtagcccagctctgcgaaaaagctggtcttttacaaagagctctggaacactatactgatttgtacgatatcaaacgtgctgtcgtacacacccacttgcttccagctgattggttggttaacttcttcggaactctcagcgtggaagacagtttggagtgcttgagggccatgctgacggcgaatattcggcagaatttacagatttgcgtgcagatcgctactaagtaccacgaacaactcaccactaaggctttgatcgatttgtttgaagggttcaagagctatgagggtttgttctatttcctcggctccatcgtcaacttctcccaagaccaagaagtgcacttcaagtacattcaagccgcatgcaaaactggccagatcaaggaagtggagcgtatttgtagggaatcaaactgctacaattccgaaagagtcaagaatttcctgaaagaagccaaacttacagatcaattgccgttgattattgtctgtgacagatttgatttcgtccacgacttagtgttgtatttatacagaaactcgctgcagaaatatatcgagatttatgtgcagaaagtcaatcccagccgtttaccggttgtagtaggaggtcttttagatgtcgactgttccgaagacataatcaaaaacctaattctcgtagtcagaggccaattctccactgacgaattagtagaagaagtagaaaagaggaacagattaaaactgttgttgccctggttagaaagcagagtacacgaaggttgtgtcgaaccagccacacacaatgctttggctaagatctacatcgattccaacaacaatgccgaaagatttttgaaggaaaatcaatggtacgattcccgagttgtcggacgttattgcgaaaagcgcgatccacatctggcttgtgttgcttacgaacgaggccaatgcgacagagaattgatagctgtatgcaacgaaaattctctatttaagtctgaagcgcgttacctagtccgtagacgtgacggagaattatgggctgaagttttgaacgagagcaatcctttcagacgccagttgatagatcaagtagtgcaaacagctttaagtgaaacccaagaccctgaagatatttccgtcaccgttaaagcattcatgacagctgatttaccaaatgagctcattgaattgctggaaaagattgtgttggataattctgtattctccgagcatagaaaccttcaaaacttgcttatccttacagcaatcaaagccgatgctacaagagttatggactacatcaaccgcttggacaactacgatgcccctgatatcgcgaatatagccatcaacaaccatctctacgaagaagctttcgctattttcaagaagtttgatgtcaacacctcagctattcaagtattgatcgaacaagtcaacaatctggatcgtgcttacgaattcgcagaacgttgcaatgaaccagccgtatggagtcagctggccaaagctcaactgaaccaaggcttagtcaaagaagcaatcgattcttacattaaagctgacgatccttcggcttacaaggatgtcgtggaaaccgcttcgaaaaataatagctgggaggacttggtgcggtatttgcaaatggcaagaaagaaggccagagagagctacatcgaatccgaattgatttattcgtacgccaagaccggaagattggctgatttggaagaattcatcagcgggcccaaccatgccgatatccagaagattggtgataggtgctttgatgacaagatgtatgatgctgctaagctactgtacaacaatgtatccaatttcgctcgtctcgctattactttagttcatctaaaagaattccagggtgctgttgacagtgctagaaaggctaacagtacaagaacatggaaggaagtgtgttttgcttgtgtcgacgccgaagaattcagattggctcagatgtgtggtatgcacatcgtcgtgcacgctgatgagttgcaagacttgattaattattaccaggatagaggatactttgaagaattaatcggcctattggaagcagcattgggcttggaaagggcacacatgggtatgttcaccgaattagcaatactgtattccaaatacaagcccgccaaaatgcgcgaacatctagaactcttctggtctcgagtgaatatccccaaagttcttagggcagctgaacaagcacatttgtgggctgagctagtgttcttgtacgacaaatacgaagaatacgataatgcagtattggctatgatggcccatcctaccgaggcctggcgcgaaggtcatttcaaagatattattacaaaagtggccaatatcgaactttattatagagctattcaattttatctggactacaaacccctgttgttaaatgaccttttgttggttttggcacccagaatggatcatactagggctgtttctttcttcaccaaaacaggacacttacagttggttaaatcctatctccgttctgtgcaaaatttgaacaacaaagctatcaacgaggcccttaactctctacttattgacgaagaagacttccagggtctgagaacgtccatcgatgccttcgataacttcgacaatatcggtttggcgcagaaattagagaaacacgaactgaccgaatttagacgcatcgccgcctacttgtacaaaggaaacaaccggtggaagcagagcgtagaactgtgcaaaaaggatagattgtttagagacgcaatggagtacacttctgaatctagaaatcaagaattggccgaggagttgctagcctggttcttggataggcaggcctatgattgtttttcggcatgtttgtatcactgctacgacttgttacgacctgacgttatccttgaactagcatggaaacacaacattatggactttgcgatgcctttccttattcaagtaactagagaactgacgacaaaagtagaaaagctagaacaatccgacgcccaacgacaaagtgaggctgctgaagaaacgaacaagccaatgatgataccagaaccccaacttatgctaacggctggccctggcatgggtattccaccccaacagtatgtacctccccaagcttacgcgcagccaggctacgcaccgcaaatggcttaccagggatacccaggcatgtaa

SEQ ID NO: 380 - RNA, 5055 nt, Diabrotica undecimpunctata
augacgcagcaacuguuaccuaucaaguuccaagaacauuugcagcuuaccaauguugguauccaugcuaccaacaucacguucgccaaucucaccauggagagugacaaguacaucugcgugagagaaaaagucggagagacgucccaaguagucaucauagauauggccgacacggccaaucccaucagacgaccaaucaccgccgaaagugcuauuaugaauccagcauccaaagucauugcucuuaaagguaaagccggcguagaaacacaaaaaacacuucaaauauuuaacauagaaaugaagucaaaaaugaaagcccacaccauguccgaagacguaauuuucuggaaauggauaagccccaauacguuagcucuagucaccgagacuucaguguaucauugguccauggaaggugauuccacuccacagaaaauguucgacagacacucuucucuuaacggcugccaaaucaucaacuaccguacagaucccaaacaaaacuggcugcuacuugucgguaucagcgcucaacagucccgcgucguuggugcuaugcaacucuauucaguagaaagaaaaugcucccagccgaucgaaggacacgccgcuucuuuugccaccuucaaaauggaaggaaauccugaaccaucgacgcucuucuguuucgcagugagaacuuuacagggaggaaaauugcauauuaucgagguuggccaaaguccagcaggcaaucaaucguuccccaaaaagacaguggacguuuucuucccgcccgaggcccaaaacgauuuuccuguagccaugcaaguaucagcuaaguacgacgucauuuaccugaucaccaaauacggcuacauucauauguaugauauugagaccggcacuuguaucuauaugaacagaauauccagugaaaccauauucguaaccgcaccccacgaagcuacuggaggaauaauugguguaaauagaaaaggucaaguacuauccgucuccguagacgaggagagcaucauucgguacaucaacaccgucuugcacaaugcagacuuagcgcugcgucuagcuacgagaaacaaucucucaggagccgaagaacuguuuguuaguaaauuucagauguuguuccagaauggacaguacgccgaagcugccaaaguggcugccaacgcuccaaaaggaauuuuaagaaccccagcuacaauucaaauguuucaacaagucccgacucaaccuggacaaaacaguccucucuuacaauauuucgguauacuuuuagaccaaggacaacuaaacagauacgaaucuuuggaacuauguaaaccaguuuuguugcaaggucgcaaacagcugcuagaaaaaugguuaaaagaagaaaaauuagaauguuccgaggaauuaggagaccuagucaaacaggcagacccuacucuggcuuuaucuguguaucuuagagcuaauguaccugcaaaaguuauccaaagcuuugcugaaacaggccaauuccaaaagauaguccucuacgccaaaaaaguguccuauacgcccgacuauauauuccugcuucgccaagucaugcgcaccaaucccgaccaaggcgccgcguucgccgggauguugguagcagacgaagaaccuuuggccgacaucaaccaaaucguggacauuuucauggaacaaaacauggugcagcaguguacugcguuuuuguuggacgccuuaaagaauaacaggccuacugaggggcaucuacaaaccagacuguuagaaaugaaccugaugucugcaccgcaaguggcagacgccauucucggcaacaacauguucacucacuacgaccggccucacguagcccagcucugcgaaaaagcuggucuuuuacaaagagcucuggaacacuauacugauuuguacgauaucaaacgugcugucguacacacccacuugcuuccagcugauugguugguuaacuucuucggaacucucagcguggaagacaguuuggagugcuugagggccaugcugacggcgaauauucggcagaauuuacagauuugcgugcagaucgcuacuaaguaccacgaacaacucaccacuaaggcuuugaucgauuuguuugaaggguucaagagcuaugaggguuuguucuauuuccucggcuccaucgucaacuucucccaagaccaagaagugcacuucaaguacauucaagccgcaugcaaaacuggccagaucaaggaaguggagcguauuuguagggaaucaaacugcuacaauuccgaaagagucaagaauuuccugaaagaagccaaacuuacagaucaauugccguugauuauugucugugacagauuugauuucguccacgacuuaguguuguauuuauacagaaacucgcugcagaaauauaucgagauuuaugugcagaaagucaaucccagccguuuaccgguuguaguaggaggucuuuuagaugucgacuguuccgaagacauaaucaaaaaccuaauucucguagucagaggccaauucuccacugacgaauuaguagaagaaguagaaaagaggaacagauuaaaacuguuguugcccugguuagaaagcagaguacacgaagguugugucgaaccagccacacacaaugcuuuggcuaagaucuacaucgauuccaacaacaaugccgaaagauuuuugaaggaaaaucaaugguacgauucccgaguugucggacguuauugcgaaaagcgcgauccacaucuggcuuguguugcuuacgaacgaggccaaugcgacagagaauugauagcuguaugcaacgaaaauucucuauuuaagucugaagcgcguuaccuaguccguagacgugacggagaauuaugggcugaaguuuugaacgagagcaauccuuucagacgccaguugauagaucaaguagugcaaacagcuuuaagugaaacccaagacccugaagauauuuccgucaccguuaaagcauucaugacagcugauuuaccaaaugagcucauugaauugcuggaaaagauuguguuggauaauucuguauucuccgagcauagaaaccuucaaaacuugcuuauccuuacagcaaucaaagccgaugcuacaagaguuauggacuacaucaaccgcuuggacaacuacgaugccccugauaucgcgaauauagccaucaacaaccaucucuacgaagaagcuuucgcuauuuucaagaaguuugaugucaacaccucagcuauucaaguauugaucgaacaagucaacaaucuggaucgugcuuacgaauucgcagaacguugcaaugaaccagccguauggagucagcuggccaaagcucaacugaaccaaggcuuagucaaagaagcaaucgauucuuacauuaaagcugacgauccuucggcuuacaaggaugucguggaaaccgcuucgaaaaauaauagcugggaggacuuggugcgguauuugcaaauggcaagaaagaaggccagagagagcuacaucgaauccgaauugauuuauucguacgccaagaccggaagauuggcugauuuggaagaauucaucagcgggcccaaccaugccgauauccagaagauuggugauaggugcuuugaugacaagauguaugaugcugcuaagcuacuguacaacaauguauccaauuucgcucgucucgcuauuacuuuaguucaucuaaaagaauuccagggugcuguugacagugcuagaaaggcuaacaguacaagaacauggaaggaaguguguuuugcuugugucgacgccgaagaauucagauuggcucagaugugugguaugcacaucgucgugcacgcugaugaguugcaagacuugauuaauuauuaccaggauagaggauacuuugaagaauuaaucggccuauuggaagcagcauugggcuuggaaagggcacacauggguauguucaccgaauuagcaauacuguauuccaaauacaagcccgccaaaaugcgcgaacaucuagaacucuucuggucucgagugaauauccccaaaguucuuagggcagcugaacaagcacauuugugggcugagcuaguguucuuguacgacaaauacgaagaauacgauaaugcaguauuggcuaugauggcccauccuaccgaggccuggcgcgaaggucauuucaaagauauuauuacaaaaguggccaauaucgaacuuuauuauagagcuauucaauuuuaucuggacuacaaaccccuguuguuaaaugaccuuuuguugguuuuggcacccagaauggaucauacuagggcuguuucuuucuucaccaaaacaggacacuuacaguugguuaaauccuaucuccguucugugcaaaauuugaacaacaaagcuaucaacgaggcccuuaacucucuacuuauugacgaagaagacuuccagggucugagaacguccaucgaugccuucgauaacuucgacaauaucgguuuggcgcagaaauuagagaaacacgaacugaccgaauuuagacgcaucgccgccuacuuguacaaaggaaacaaccgguggaagcagagcguagaacugugcaaaaaggauagauuguuuagagacgcaauggaguacacuucugaaucuagaaaucaagaauuggccgaggaguugcuagccugguucuuggauaggcaggccuaugauuguuuuucggcauguuuguaucacugcuacgacuuguuacgaccugacguuauccuugaacuagcauggaaacacaacauuauggacuuugcgaugccuuuccuuauucaaguaacuagagaacugacgacaaaaguagaaaagcuagaacaauccgacgcccaacgacaaagugaggcugcugaagaaacgaacaagccaaugaugauaccagaaccccaacuuaugcuaacggcuggcccuggcauggguauuccaccccaacaguauguaccuccccaagcuuacgcgcagccaggcuacgcaccgcaaauggcuuaccagggauacccaggcauguaa

SEQ ID NO: 381 - DNA, 687 bp, Diabrotica virgifera
atgacgcagcaactgttacctatcaagttccaagaacatttgcagcttaccaatgttggtatccatgctaccaacatcacgttcgccaatctcaccatggagagcgacaagtacatctgcgtgagagaaaaagttggagagacgtcccaagtagtcatcatagatatggccgatacggccaatcccatcagacgaccaatcaccgccgaaagtgctattatgaatccagcatccaaagtcatcgctcttaaaggtaaagcaggcgtagaaacacaaaaaacccttcaaatattcaacatagaaatgaagtcaaaaatgaaagcccacaccatgtctgaagacgtaattttctggaaatggatcagccccaatacgttagcgctagtcactgaaacttcagtgtatcattggtccatggaaggtgattcaattccacagaaaatgtttgacaggcattcttctcttaacggctgccaaatcatcaactaccgaacagatcccaaacaaaactggctgctactggtcggtattagcgctcagcaatctcgcgtcgttggtgctatgcaactgtactcagtagaaagaaaatgctcgcagccaatcgaaggtcacgccgcttctttcgcgaccttcaaaatggaaggaaaccctgaaccatcgactctcttctgttttgcagtgaggact

SEQ ID NO: 382 - DNA, 693 bp, Diabrotica virgifera
tcgactctcttctgttttgcagtgaggactttacaaggaggaaagttacatattatcgaggttggtcaaagtccagcaggcaaccaatcgtttcctaaaaagacagtggatgttttcttcccacccgaggcccaaaatgattttcctgtagctatgcaagtgtccgctaaatacgacgtcatttacctgattaccaaatacggctatattcatatgtatgacatcgagagcggcacctgtatctacatgaacagaatatctagtgacacaatattcgtaaccgcaccccacgaagctacgggaggaatcattggtgttaatagaaagggtcaagtcctatctgtctcggtagatgaggagagcattattcgatacatcaacaccgtcttacacaatgctgacttagcgctgcgtctagctacgagaaacaatctttcaggagccgaagaactgtttgttagtaaattccagatgttgttccagaacggacagtacgccgaagctgctaaagtggctgccaacgctccaaaaggaattttaagaaccccagctacaattcaaatgtttcaacaagtcccgactcaacctggacaaaacagtccccttttgcaatatttcggtatacttctagaccaagggcaactaaacagatacgaatctttggaattgtgtaaaccagttttgttgcaaggt

SEQ ID NO: 383 - DNA, 700 bp, Diabrotica virgifera
gaattgtgtaaaccagttttgttgcaaggtcgcaaacagcttctagaaaaatggttaaaagaggaaaaattagaatgttccgaagaattaggagacctagtcaaacaggcagatcctactctggctttatctgtgtatcttagagctaatgtacctgcaaaagttatccaaagctttgccgaaactggccaattccaaaagatagtcctctacgccaaaaaagtgtcttatactcccgactatgtattcctgcttcgccaagtcatgcgcaccaatcccgaccaaggcgcagcatttgcagggatgttggtagcggacgacgaacctttggccgatatcaaccaaatcgtggacattttcatggagcaaaacatggtgcagcagtgtactgcgttcttgttggacgccttaaagaataacaggcctactgaggggcatctacaaactagactattagaaatgaacctgatgtccgcaccgcaagtagcagacgccattctcggcaacaacatgttcactcactacgaccggccccacgtagcccagctctgcgaaaaagctggtcttttacaaagagctctagaacactacactgatttgtatgacatcaaacgtgctgtggtacacacccacttgcttccagctgattggttggttaacttcttcggaactctcagcgtggaagacagtttggagtgct

SEQ ID NO: 384 - DNA, 549 bp, Diabrotica virgifera
tcagcgtggaagacagtttggagtgcttgagggccatgctgaccgcgaatattcgacagaatttgcagatttgcgtgcagatcgctaccaagtaccacgaacaactcaccactaaggctttgatcgatttgtttgaaggatttaagagctatgagggtttgttctatttcctcggctccatcgtcaacttctcccaagaccaagaagtgcacttcaagtacatccaagccgcatgcaagactggccaaatcaaagaagtcgagcgtatctgtagggaatcaaactgctacaatcccgaaagagtcaagaatttcctgaaggaagccaaacttacagatcagttgccgttgattattgtctgtgacagatttgatttcgtccacgacttagtgttgtatctatatagaaattcgctgcagaaatatatcgagatttatgtccagaaggtcaatcccagccgtttaccggttgtggtaggaggtcttttagatgtcgactgttccgaagacataatcaaaaacctaattcttgtcgtcagaggccagttct

SEQ ID NO: 385 - DNA, 677 bp, Diabrotica virgifera
taatcaaaaacctaattcttgtcgtcagaggccagttctccactgacgaattagtagaagaagtagaaaagaggaacagattgaaactgttgttgccctggttggagagcagagtacacgaaggatgtgtcgagccagctacgcacaatgctttggccaagatctacatcgattccaacaacaatgccgaaagattcttgaaggaaaatcaatggtacgattcccgagttgtgggacgttattgcgaaaagcgcgatccacatctggcttgcgttgcttacgaacgaggccaatgcgacagagaactgatagctgtatgtaacgaaaactctctatttaagtctgaagctcgttatttggtccgtagacgtgacggagaattatgggctgaggttttgaacgagagcaatccttacagacgtcagttgatagaccaagtagtgcaaacagctttaagtgaaacccaagaccccgaagatatctctgttaccgttaaagcattcatgacagctgatttaccaaatgagctcattgaattgttggaaaagattgtattggatagttctgtgttctccgagcatagaaaccttcaaaatttgcttatcctaacagcaatcaaagccgatgctacaagagttatggactacatcaaccgcttggataactacgatgcccct

SEQ ID NO: 386 - DNA, 706 bp, Diabrotica virgifera
aaccgcttggataactacgatgcccctgatatcgcgaatatagccatcaacaaccatctctatgaagaagctttcgctattttcaagaaatttgatgtcaacacctcagctattcaagtattgatcgaacaagtcaacaatctggatcgtgcttatgaattcgcagaacgttgcaatgaaccggccgtatggagtcagctggccaaagcgcaactgaaccaaggcttagtcaaggaagcaatcgattcttacattaaagctgatgatccttcagcttataaggacgtcgttgagaccgcttcgaaaaataatagctgggaggacttagtgcggtatttgcagatggcaagaaagaaggccagagagagctacatcgaatctgaattgatttattcgtacgcgaagaccggaagattggctgatttggaagaattcatcagtggacccaaccatgctgatatccagaagattggtgataggtgctttgatgacaagatgtatgatgctgctaagctactctacaacaatgtatccaacttcgctcgtctcgctattactttagtgcatctaaaagaattccagggagctgttgacagtgctaggaaggctaatagtaccagaacatggaaggaagtgtgttttgcttgcgtcgatgccgaagaattcagattggctcagatgtgtggtatgcacatcgtggtacacg

SEQ ID NO: 387 - DNA, 686 bp, Diabrotica virgifera
gcacatcgtggtacacgctgatgagttgcaagatttgattaattattatcaagatagaggatactttgaagaattaatcggcctattggaagcagcattgggcttggaaagggcacacatgggtatgttcaccgaattagcaattttgtattccaaatataagcccgccaaaatgcgcgaacatctggaactcttctggtctcgagtgaatatccccaaagttcttagggcagctgaacaagcacatttgtgggcagagctagtgtttttgtatgacaaatatgaagaatatgataacgctgtgttagccatgatggctcatcccaccgaagcttggcgcgaaggtcatttcaaggatattattacaaaagttgccaatatcgaactttattatagagctattcaattttacttggattacaaaccgctgttgttaaatgaccttttgttggtgttggcacccaggatggatcatactagggctgtttctttctttacaaaaacaggacacttacagttggttaaatcctatctccggtctgtgcaaaatttgaacaacaaagctatcaacgaggccctcaactctctacttatcgaagaagaagacttccagggtctgagaacgtccatcgacgccttcgataacttcgacaacatcggcttggctcagaaattggagaagcacg

SEQ ID NO: 388 - DNA, 565 bp, Diabrotica virgifera
cgacaacatcggcttggctcagaaattggagaagcacgaactgacggagttcagacgcatcgccgcctacttgtacaaaggcaacaaccggtggaagcagagcgtagaactgtgcaaaaaggatagactatttagagacgctatggagtacacttctgaatctagaaatcaagaattggccgaagagttgctggcatggttcttggataggaaggcctatgattgtttttcggcatgtttgtatcactgctacgacttgttacggcccgacgttatccttgaactagcatggaaacacaacattatggacttcgcaatgcctttccttattcaagtaactagagaactgacgacaaaagtagaaaagctagaacaatcagatgcccaacgacaaagcgaggctgctgaagaaacgaacaagccaatgatgataccagaaccccaacttatgctaacggctggccctggcatgggtattccaccccaacagtatgtacctccccaaggctacgcgcagccaggctacgccccgcaaatggcttaccagggatacccaggcatgtaa

SEQ ID NO: 389 - RNA, 687 nt, Diabrotica virgifera
augacgcagcaacuguuaccuaucaaguuccaagaacauuugcagcuuaccaauguugguauccaugcuaccaacaucacguucgccaaucucaccauggagagcgacaaguacaucugcgugagagaaaaaguuggagagacgucccaaguagucaucauagauauggccgauacggccaaucccaucagacgaccaaucaccgccgaaagugcuauuaugaauccagcauccaaagucaucgcucuuaaagguaaagcaggcguagaaacacaaaaaacccuucaaauauucaacauagaaaugaagucaaaaaugaaagcccacaccaugucugaagacguaauuuucuggaaauggaucagccccaauacguuagcgcuagucacugaaacuucaguguaucauugguccauggaaggugauucaauuccacagaaaauguuugacaggcauucuucucuuaacggcugccaaaucaucaacuaccgaacagaucccaaacaaaacuggcugcuacuggucgguauuagcgcucagcaaucucgcgucguuggugcuaugcaacuguacucaguagaaagaaaaugcucgcagccaaucgaaggucacgccgcuucuuucgcgaccuucaaaauggaaggaaacccugaaccaucgacucucuucuguuuugcagugaggacu

SEQ ID NO: 390 - RNA, 693 nt, Diabrotica virgifera
ucgacucucuucuguuuugcagugaggacuuuacaaggaggaaaguuacauauuaucgagguuggucaaaguccagcaggcaaccaaucguuuccuaaaaagacaguggauguuuucuucccacccgaggcccaaaaugauuuuccuguagcuaugcaaguguccgcuaaauacgacgucauuuaccugauuaccaaauacggcuauauucauauguaugacaucgagagcggcaccuguaucuacaugaacagaauaucuagugacacaauauucguaaccgcaccccacgaagcuacgggaggaaucauugguguuaauagaaagggucaaguccuaucugucucgguagaugaggagagcauuauucgauacaucaacaccgucuuacacaaugcugacuuagcgcugcgucuagcuacgagaaacaaucuuucaggagccgaagaacuguuuguuaguaaauuccagauguuguuccagaacggacaguacgccgaagcugcuaaaguggcugccaacgcuccaaaaggaauuuuaagaaccccagcuacaauucaaauguuucaacaagucccgacucaaccuggacaaaacaguccccuuuugcaauauuucgguauacuucuagaccaagggcaacuaaacagauacgaaucuuuggaauuguguaaaccaguuuuguugcaaggu

SEQ ID NO: 391 - RNA, 700 nt, Diabrotica virgifera
gaauuguguaaaccaguuuuguugcaaggucgcaaacagcuucuagaaaaaugguuaaaagaggaaaaauuagaauguuccgaagaauuaggagaccuagucaaacaggcagauccuacucuggcuuuaucuguguaucuuagagcuaauguaccugcaaaaguuauccaaagcuuugccgaaacuggccaauuccaaaagauaguccucuacgccaaaaaagugucuuauacucccgacuauguauuccugcuucgccaagucaugcgcaccaaucccgaccaaggcgcagcauuugcagggauguugguagcggacgacgaaccuuuggccgauaucaaccaaaucguggacauuuucauggagcaaaacauggugcagcaguguacugcguucuuguuggacgccuuaaagaauaacaggccuacugaggggcaucuacaaacuagacuauuagaaaugaaccugauguccgcaccgcaaguagcagacgccauucucggcaacaacauguucacucacuacgaccggccccacguagcccagcucugcgaaaaagcuggucuuuuacaaagagcucuagaacacuacacugauuuguaugacaucaaacgugcugugguacacacccacuugcuuccagcugauugguugguuaacuucuucggaacucucagcguggaagacaguuuggagugcu

SEQ ID NO: 392 - RNA, 549 nt, Diabrotica virgifera
ucagcguggaagacaguuuggagugcuugagggccaugcugaccgcgaauauucgacagaauuugcagauuugcgugcagaucgcuaccaaguaccacgaacaacucaccacuaaggcuuugaucgauuuguuugaaggauuuaagagcuaugaggguuuguucuauuuccucggcuccaucgucaacuucucccaagaccaagaagugcacuucaaguacauccaagccgcaugcaagacuggccaaaucaaagaagucgagcguaucuguagggaaucaaacugcuacaaucccgaaagagucaagaauuuccugaaggaagccaaacuuacagaucaguugccguugauuauugucugugacagauuugauuucguccacgacuuaguguuguaucuauauagaaauucgcugcagaaauauaucgagauuuauguccagaaggucaaucccagccguuuaccgguugugguaggaggucuuuuagaugucgacuguuccgaagacauaaucaaaaaccuaauucuugucgucagaggccaguucu

SEQ ID NO: 393 - RNA, 677 nt, Diabrotica virgifera
uaaucaaaaaccuaauucuugucgucagaggccaguucuccacugacgaauuaguagaagaaguagaaaagaggaacagauugaaacuguuguugcccugguuggagagcagaguacacgaaggaugugucgagccagcuacgcacaaugcuuuggccaagaucuacaucgauuccaacaacaaugccgaaagauucuugaaggaaaaucaaugguacgauucccgaguugugggacguuauugcgaaaagcgcgauccacaucuggcuugcguugcuuacgaacgaggccaaugcgacagagaacugauagcuguauguaacgaaaacucucuauuuaagucugaagcucguuauuugguccguagacgugacggagaauuaugggcugagguuuugaacgagagcaauccuuacagacgucaguugauagaccaaguagugcaaacagcuuuaagugaaacccaagaccccgaagauaucucuguuaccguuaaagcauucaugacagcugauuuaccaaaugagcucauugaauuguuggaaaagauuguauuggauaguucuguguucuccgagcauagaaaccuucaaaauuugcuuauccuaacagcaaucaaagccgaugcuacaagaguuauggacuacaucaaccgcuuggauaacuacgaugccccu

SEQ ID NO: 394 - RNA, 706 nt, Diabrotica virgifera
aaccgcuuggauaacuacgaugccccugauaucgcgaauauagccaucaacaaccaucucuaugaagaagcuuucgcuauuuucaagaaauuugaugucaacaccucagcuauucaaguauugaucgaacaagucaacaaucuggaucgugcuuaugaauucgcagaacguugcaaugaaccggccguauggagucagcuggccaaagcgcaacugaaccaaggcuuagucaaggaagcaaucgauucuuacauuaaagcugaugauccuucagcuuauaaggacgucguugagaccgcuucgaaaaauaauagcugggaggacuuagugcgguauuugcagauggcaagaaagaaggccagagagagcuacaucgaaucugaauugauuuauucguacgcgaagaccggaagauuggcugauuuggaagaauucaucaguggacccaaccaugcugauauccagaagauuggugauaggugcuuugaugacaagauguaugaugcugcuaagcuacucuacaacaauguauccaacuucgcucgucucgcuauuacuuuagugcaucuaaaagaauuccagggagcuguugacagugcuaggaaggcuaauaguaccagaacauggaaggaaguguguuuugcuugcgucgaugccgaagaauucagauuggcucagaugugugguaugcacaucgugguacacg

SEQ ID NO: 395 - RNA, 686 nt, Diabrotica virgifera
gcacaucgugguacacgcugaugaguugcaagauuugauuaauuauuaucaagauagaggauacuuugaagaauuaaucggccuauuggaagcagcauugggcuuggaaagggcacacauggguauguucaccgaauuagcaauuuuguauuccaaauauaagcccgccaaaaugcgcgaacaucuggaacucuucuggucucgagugaauauccccaaaguucuuagggcagcugaacaagcacauuugugggcagagcuaguguuuuuguaugacaaauaugaagaauaugauaacgcuguguuagccaugauggcucaucccaccgaagcuuggcgcgaaggucauuucaaggauauuauuacaaaaguugccaauaucgaacuuuauuauagagcuauucaauuuuacuuggauuacaaaccgcuguuguuaaaugaccuuuuguugguguuggcacccaggauggaucauacuagggcuguuucuuucuuuacaaaaacaggacacuuacaguugguuaaauccuaucuccggucugugcaaaauuugaacaacaaagcuaucaacgaggcccucaacucucuacuuaucgaagaagaagacuuccagggucugagaacguccaucgacgccuucgauaacuucgacaacaucggcuuggcucagaaauuggagaagcacg

SEQ ID NO: 396 - RNA, 565 nt, Diabrotica virgifera
cgacaacaucggcuuggcucagaaauuggagaagcacgaacugacggaguucagacgcaucgccgccuacuuguacaaaggcaacaaccgguggaagcagagcguagaacugugcaaaaaggauagacuauuuagagacgcuauggaguacacuucugaaucuagaaaucaagaauuggccgaagaguugcuggcaugguucuuggauaggaaggccuaugauuguuuuucggcauguuuguaucacugcuacgacuuguuacggcccgacguuauccuugaacuagcauggaaacacaacauuauggacuucgcaaugccuuuccuuauucaaguaacuagagaacugacgacaaaaguagaaaagcuagaacaaucagaugcccaacgacaaagcgaggcugcugaagaaacgaacaagccaaugaugauaccagaaccccaacuuaugcuaacggcuggcccuggcauggguauuccaccccaacaguauguaccuccccaaggcuacgcgcagccaggcuacgccccgcaaauggcuuaccagggauacccaggcauguaa

SEQ ID NO: 397 - DNA, 20 bp, Diabrotica virgifera
aagaaaaagcaacatgacgc

SEQ ID NO: 398 - DNA, 20 bp, Diabrotica virgifera
ggggccttatattacatgcc

SEQ ID NO: 399 - DNA, 130 bp, Diabrotica virgifera
gatatcacagacgtattgtagacctagaaaataagaaatttgacctcgaaaaagaagtggaattcagagattttcagatctccgaattgaacagccaagtaaacgaccttagaggcaaattcgtcaaacc

SEQ ID NO: 400 - DNA, 119 bp, Diabrotica virgifera
gtaaccaactcaaagttgtcaagaagaaagaattcaccttagaagaagaagacaaagaaaagaaaccagactggtcaaagaagggagacgaaaagaaggtacaagaggctgaagcatga

SEQ ID NO: 401 - RNA, 130 nt, Diabrotica virgifera
gauaucacagacguauuguagaccuagaaaauaagaaauuugaccucgaaaaagaaguggaauucagagauuuucagaucuccgaauugaacagccaaguaaacgaccuuagaggcaaauucgucaaacc

SEQ ID NO: 402 - RNA, 119 nt, Diabrotica virgifera
guaaccaacucaaaguugucaagaagaaagaauucaccuuagaagaagaagacaaagaaaagaaaccagacuggucaaagaagggagacgaaaagaagguacaagaggcugaagcauga

SEQ ID NO: 403 - DNA, 692 bp, Artificial Sequence
  Diabrotica virgifera, Arabidopsis thaliana
gaccttagaggcaaattcgtcaaaccaaccttgaagaaggtatccaaatacgaaaacaaattcgccaaacttcaaaagaaggcagctgaatttaacttccgtaaccaactcaaagttgtcaagaagaaagaatggtaccaagctgcgaatcttcgtttttttaaggaattctcgatctttatggtgtataggctctgggttttctgttttttgtatctcttaggattttgtaaattccagatctttctatggccacttagtagtatatttcaaaaattctccaatcgagttcttcattcgcattttcagtcattttctcttcgacgttgtttttaagcctgggtattactcctatttagttgaactctgcagcaatcttagaaaattagggttttgaggtttcgatttctctaggtaaccgatctattgcattcatctgaatttctgcatatatgtcttagatttctgataagcttacgatacgttaggtgtaattgaagtttatttttcaagagtgttattttttgtttctgaatttttcagtcactccatggcctagattctttcttcttgacaactttgagttggttacggaagttaaattcagctgccttcttttgaagtttggcgaatttgttttcgtatttggataccttcttcaaggttggtttgacgaatttgcctctaaggtc